European Patent Application EP 4 491 717 A1, published January 15, 2025. Title: Producer cell, method for producing producer cell, and method for producing adeno-associated virus. Applicant: FUJIFILM Corporation. The sequence listing filed with the application follows.

SEQUENCE LISTING (42 sequences)

SEQ ID NO: 1 - DNA, 11635 bp, synthetic construct
  misc_feature 1..11635: note = plasmid
  source 1..11635: mol_type = other DNA
ggtacccaactccatgcttaacagtccccaggtacagcccaccctgcgtcgcaaccaggaacagctctacagcttcctggagcgccactcgccctacttccgcagccacagtgcgcagattaggagcgccacttctttttgtcacttgaaaaacatgtaaaaataatgtactaggagacactttcaataaaggcaaatgtttttatttgtacactctcgggtgattatttaccccccacccttgccgtctgcgccgtttaaaaatcaaaggggttctgccgcgcatcgctatgcgccactggcagggacacgttgcgatactggtgtttagtgctccacttaaactcaggcacaaccatccgcggcagctcggtgaagttttcactccacaggctgcgcaccatcaccaacgcgtttagcaggtcgggcgccgatatcttgaagtcgcagttggggcctccgccctgcgcgcgcgagttgcgatacacagggttgcagcactggaacactatcagcgccgggtggtgcacgctggccagcacgctcttgtcggagatcagatccgcgtccaggtcctccgcgttgctcagggcgaacggagtcaactttggtagctgccttcccaaaaagggtgcatgcccaggctttgagttgcactcgcaccgtagtggcatcagaaggtgaccgtgcccggtctgggcgttaggatacagcgcctgcatgaaagccttgatctgcttaaaagccacctgagcctttgcgccttcagagaagaacatgccgcaagacttgccggaaaactgattggccggacaggccgcgtcatgcacgcagcaccttgcgtcggtgttggagatctgcaccacatttcggccccaccggttcttcacgatcttggccttgctagactgctccttcagcgcgcgctgcccgttttcgctcgtcacatccatttcaatcacgtgctccttatttatcataatgctcccgtgtagacacttaagctcgccttcgatctcagcgcagcggtgcagccacaacgcgcagcccgtgggctcgtggtgcttgtaggttacctctgcaaacgactgcaggtacgcctgcaggaatcgccccatcatcgtcacaaaggtcttgttgctggtgaaggtcagctgcaacccgcggtgctcctcgtttagccaggtcttgcatacggccgccagagcttccacttggtcaggcagtagcttgaagtttgcctttagatcgttatccacgtggtacttgtccatcaacgcgcgcgcagcctccatgcccttctcccacgcagacacgatcggcaggctcagcgggtttatcaccgtgctttcactttccgcttcactggactcttccttttcctcttgcgtccgcataccccgcgccactgggtcgtcttcattcagccgccgcaccgtgcgcttacctcccttgccgtgcttgattagcaccggtgggttgctgaaacccaccatttgtagcgccacatcttctctttcttcctcgctgtccacgatcacctctggggatggcgggcgctcgggcttgggagaggggcgcttctttttctttttggacgcaatggccaaatccgccgtcgaggtcgatggccgcgggctgggtgtgcgcggcaccagcgcatcttgtgacgagtcttcttcgtcctcggactcgagacgccgcctcagccgcttttttgggggcgcgcggggaggcggcggcgacggcgacggggacgacacgtcctccatggttggtggacgtcgcgccgcaccgcgtccgcgctcgggggtggtttcgcgctgctcctcttcccgactggccatttccttctcctataggcagaaaaagatcatggagtcagtcgagaaggaggacagcctaaccgccccctttgagttcgccaccaccgcctccaccgatgccgccaacgcgcctaccaccttccccgtcgaggcacccccgcttgaggaggaggaagtgattatcgagcaggacccaggttttgtaagcgaagacgacgaggatcgctcagtaccaacagaggataaaaagcaagaccaggacgacgcagaggcaaacgaggaacaagtcgggcggggggaccaaaggcatggcgactacctagatgtgggagacgacgtgctgttgaagcatctgcagcgccagtgcgccattatctgcgacgcgttgcaagagcgcagcgatgtgcccctcgccatagcggatgtcagccttgcctacgaacgccacctgttctcaccgcgcgtaccccccaaacgccaagaaaacggcacatgcgagcccaacccgcgcctcaacttctaccccgtatttgccgtgccagaggtgcttgccacctatcacatctttttccaaaactgcaagatacccctatcctgccgtgccaaccgcagccgagcggacaagcagctggccttgcggcagggcgctgtcatacctgatatcgcctcgctcgacgaagtgccaaaaatctttgagggtcttggacgcgacgagaaacgcgcggcaaacgctctgcaacaagaaaacagcgaaaatgaaagtcactgtggagtgctggtggaacttgagggtgacaacgcgcgcctagccgtgctgaaacgcagcatcgaggtcacccactttgcctacccggcacttaacctaccccccaaggttatgagcacagtcatgagcgagctgatcgtgcgccgtgcacgacccctggagagggatgcaaacttgcaagaacaaaccgaggagggcctacccgcagttggcgatgagcagctggcgcgctggcttgagacgcgcgagcctgccgacttggaggagcgacgcaagctaatgatggccgcagtgcttgttaccgtggagcttgagtgcatgcagcggttctttgctgacccggagatgcagcgcaagctagaggaaacgttgcactacacctttcgccagggctacgtgcgccaggcctgcaaaatttccaacgtggagctctgcaacctggtctcctaccttggaattttgcacgaaaaccgcctcgggcaaaacgtgcttcattccacgctcaagggcgaggcgcgccgcgactacgtccgcgactgcgtttacttatttctgtgctacacctggcaaacggccatgggcgtgtggcagcaatgcctggaggagcgcaacctaaaggagctgcagaagctgctaaagcaaaacttgaaggacctatggacggccttcaacgagcgctccgtggccgcgcacctggcggacattatcttccccgaacgcctgcttaaaaccctgcaacagggtctgccagacttcaccagtcaaagcatgttgcaaaactttaggaactttatcctagagcgttcaggaattctgcccgccacctgctgtgcgcttcctagcgactttgtgcccattaagtaccgtgaatgccctccgccgctttggggtcactgctaccttctgcagctagccaactaccttgcctaccactccgacatcatggaagacgtgagcggtgacggcctactggagtgtcactgtcgctgcaacctatgcaccccgcaccgctccctggtctgcaattcgcaactgcttagcgaaagtcaaattatcggtacctttgagctgcagggtccctcgcctgacgaaaagtccgcggctccggggttgaaactcactccggggctgtggacgtcggcttaccttcgcaaatttgtacctgaggactaccacgcccacgagattaggttctacgaagaccaatcccgcccgccaaatgcggagcttaccgcctgcgtcattacccagggccacatccttggccaattgcaagccatcaacaaagcccgccaagagtttctgctacgaaagggacggggggtttacctggacccccagtccggcgaggagctcaacccaatccccccgccgccgcagccctatcagcagccgcgggcccttgcttcccaggatggcacccaaaaagaagctgcagctgccgccgccgccacccacggacgaggaggaatactgggacagtcaggcagaggaggttttggacgaggaggaggagatgatggaagactgggacagcctagacgaagcttccgaggccgaagaggtgtcagacgaaacaccgtcaccctcggtcgcattcccctcgccggcgccccagaaattggcaaccgttcccagcatcgctacaacctccgctcctcaggcgccgccggcactgcctgttcgccgacccaaccgtagatgggacaccactggaaccagggccggtaagtctaagcagccgccgccgttagcccaagagcaacaacagcgccaaggctaccgctcgtggcgcgggcacaagaacgccatagttgcttgcttgcaagactgtgggggcaacatctccttcgcccgccgctttcttctctaccatcacggcgtggccttcccccgtaacatcctgcattactaccgtcatctctacagcccctactgcaccggcggcagcggcagcggcagcaacagcagcggtcacacagaagcaaaggcgaccggatagcaagactctgacaaagcccaagaaatccacagcggcggcagcagcaggaggaggagcgctgcgtctggcgcccaacgaacccgtatcgacccgcgagcttagaaataggatttttcccactctgtatgctatatttcaacaaagcaggggccaagaacaagagctgaaaataaaaaacaggtctctgcgctccctcacccgcagctgcctgtatcacaaaagcgaagatcagcttcggcgcacgctggaagacgcggaggctctcttcagcaaatactgcgcgctgactcttaaggactagtttcgcgccctttctcaaatttaagcgcgaaaactacgtcatctccagcggccacacccggcgccagcacctgtcgtcagcgccattatgagcaaggaaattcccacgccctacatgtggagttaccagccacaaatgggacttgcggctggagctgcccaagactactcaacccgaataaactacatgagcgcgggaccccacatgatatcccgggtcaacggaatccgcgcccaccgaaaccgaattctcctcgaacaggcggctattaccaccacacctcgtaataaccttaatccccgtagttggcccgctgccctggtgtaccaggaaagtcccgctcccaccactgtggtacttcccagagacgcccaggccgaagttcagatgactaactcaggggcgcagcttgcgggcggctttcgtcacagggtgcggtcgcccgggcgttttagggcggagtaacttgcatgtattgggaattgtagtttttttaaaatgggaagtgacgtatcgtgggaaaacggaagtgaagatttgaggaagttgtgggttttttggctttcgtttctgggcgtaggttcgcgtgcggttttctgggtgttttttgtggactttaaccgttacgtcattttttagtcctatatatactcgctctgtacttggccctttttacactgtgactgattgagctggtgccgtgtcgagtggtgttttttaataggtttttttactggtaaggctgactgttatggctgccgctgtggaagcgctgtatgttgttctggagcgggagggtgctattttgcctaggcaggagggtttttcaggtgtttatgtgtttttctctcctattaattttgttatacctcctatgggggctgtaatgttgtctctacgcctgcgggtatgtattcccccgggctatttcggtcgctttttagcactgaccgatgttaaccaacctgatgtgtttaccgagtcttacattatgactccggacatgaccgaggaactgtcggtggtgctttttaatcacggtgaccagtttttttacggtcacgccggcatggccgtagtccgtcttatgcttataagggttgtttttcctgttgtaagacaggcttctaatgtttaaatgtttttttttttgttattttattttgtgtttaatgcaggaacccgcagacatgtttgagagaaaaatggtgtctttttctgtggtggttccggaacttacctgcctttatctgcatgagcatgactacgatgtgcttgcttttttgcgcgaggctttgcctgattttttgagcagcaccttgcattttatatcgccgcccatgcaacaagcttacataggggctacgctggttagcatagctccgagtatgcgtgtcataatcagtgtgggttcttttgtcatggttcctggcggggaagtggccgcgctggtccgtgcagacctgcacgattatgttcagctggccctgcgaagggacctacgggatcgcggtatttttgttaatgttccgcttttgaatcttatacaggtctgtgaggaacctgaatttttgcaatcatgattcgctgcttgaggctgaaggtggagggcgctctggagcagatttttacaatggccggacttaatattcgggatttgcttagagacatattgataaggtggcgagatgaaaattatttgggcatggttgaaggtgctggaatgtttatagaggagattcaccctgaagggtttagcctttacgtccacttggacgtgagggcagtttgccttttggaagccattgtgcaacatcttacaaatgccattatctgttctttggctgtagagtttgaccacgccaccggaggggagcgcgttcacttaatagatcttcattttgaggttttggataatcttttggaataaaaaaaaaaaaacatggttcttccagctcttcccgctcctcccgtgtgtgactcgcagaacgaatgtgtaggttggctgggtgtggcttattctgcggtggtggatgttatcagggcagcggcgcatgaaggagtttacatagaacccgaagccagggggcgcctggatgctttgagagagtggatatactacaactactacacagagcgagctaagcgacgagaccggagacgcagatctgtttgtcacgcccgcacctggttttgcttcaggaaatatgactacgtccggcgttccatttggcatgacactacgaccaacacgatctcggttgtctcggcgcactccgtacagtagggatcgcctacctccttttgagacagagacccgcgctaccatactggaggatcatccgctgctgcccgaatgtaacactttgacaatgcacaacgtgagttacgtgcgaggtcttccctgcagtgtgggatttacgctgattcaggaatgggttgttccctgggatatggttctgacgcgggaggagcttgtaatcctgaggaagtgtatgcacgtgtgcctgtgttgtgccaacattgatatcatgacgagcatgatgatccatggttacgagtcctgggctctccactgtcattgttccagtcccggttccctgcagtgcatagccggcgggcaggttttggccagctggtttaggatggtggtggatggcgccatgtttaatcagaggtttatatggtaccgggaggtggtgaattacaacatgccaaaagaggtaatgtttatgtccagcgtgtttatgaggggtcgccacttaatctacctgcgcttgtggtatgatggccacgtgggttctgtggtccccgccatgagctttggatacagcgccttgcactgtgggattttgaacaatattgtggtgctgtgctgcagttactgtgctgatttaagtgagatcagggtgcgctgctgtgcccggaggacaaggcgtctcatgctgcgggcggtgcgaatcatcgctgaggagaccactgccatgttgtattcctgcaggacggagcggcggcggcagcagtttattcgcgcgctgctgcagcaccaccgccctatcctgatgcacgattatgactctacccccatgtaggcgtggacttccccttcgccgcccgttgagcaaccgcaagttggacagcagcctgtggctcagcagctggacagcgacatgaacttaagcgagctgcccggggagtttattaatatcactgatgagcgtttggctcgacaggaaaccgtgtggaatataacacctaagaatatgtctgttacccatgatatgatgctttttaaggccagccggggagaaaggactgtgtactctgtgtgttgggagggaggtggcaggttgaatactagggttctgtgagtttgattaaggtacggtgatcaatataagctatgtggtggtggggctatactactgaatgaaaaatgacttgaaattttctgcaattgaaaaataaacacgttgaaacataacatgcaacaggttcacgattctttattcctgggcaatgtaggagaaggtgtaagagttggtagcaaaagtttcagtggtgtattttccactttcccaggaccatgtaaaagacatagagtaagtgcttacctcgctagtttctgtggattcactagaatcgatgtaggatgttgcccctcctgacgcggtaggagaaggggagggtgccctgcatgtctgccgctgctcttgctcttgccgctgctgaggaggggggcgcatctgccgcagcaccggatgcatctgggaaaagcaaaaaaggggctcgtccctgtttccggaggaatttgcaagcggggtcttgcatgacggggaggcaaacccccgttcgccgcagtccggccggcccgagactcgaaccgggggtcctgcgactcaacccttggaaaataaccctccggctacagggagcgagccacttaatgctttcgctttccagcctaaccgcttacgccgcgcgcggccagtggccaaaaaagctagcgcagcagccgccgcgcctggaaggaagccaaaaggagcgctcccccgttgtctgacgtcgcacacctgggttcgacacgcgggcggtaaccgcatggatcacggcggacggccggatccggggttcgaaccccggtcgtccgccatgatacccttgcgaatttatccaccagaccacggaagagtgcccgcttacaggctctccttttgcacggtctagagcgtcaacgactgcgcacgcctcaccggccagagcgtcccgaccatggagcactttttgccgctgcgcaacatctggaaccgcgtccgcgactttccgcgcgcctccaccaccgccgccggcatcacctggatgtccaggtacatctacggattacgtcgacgtttaaaccatatgatcagctcactcaaaggcggtaatacggttatccacagaatcaggggataacgcaggaaagaacatgtgagcaaaaggccagcaaaaggccaggaaccgtaaaaaggccgcgttgctggcgtttttccataggctccgcccccctgacgagcatcacaaaaatcgacgctcaagtcagaggtggcgaaacccgacaggactataaagataccaggcgtttccccctggaagctccctcgtgcgctctcctgttccgaccctgccgcttaccggatacctgtccgcctttctcccttcgggaagcgtggcgctttctcatagctcacgctgtaggtatctcagttcggtgtaggtcgttcgctccaagctgggctgtgtgcacgaaccccccgttcagcccgaccgctgcgccttatccggtaactatcgtcttgagtccaacccggtaagacacgacttatcgccactggcagcagccactggtaacaggattagcagagcgaggtatgtaggcggtgctacagagttcttgaagtggtggcctaactacggctacactagaagaacagtatttggtatctgcgctctgctgaagccagttaccttcggaaaaagagttggtagctcttgatccggcaaacaaaccaccgctggtagcggtggtttttttgtttgcaagcagcagattacgcgcagaaaaaaaggatctcaagaagatcctttgatcttttctacggggtctgacgctcagtggaacgaaaactcacgttaagggattttggtcatgagattatcaaaaaggatcttcacctagatccttttaaattaaaaatgaagttttaaatcaatctaaagtatatatgagtaaacttggtctgacagttaccaatgcttaatcagtgaggcacctatctcagcgatctgtctatttcgttcatccatagttgcctgactccccgtcgtgtagataactacgatacgggagggcttaccatctggccccagtgctgcaatgataccgcgagacccacgctcaccggctccagatttatcagcaataaaccagccagccggaagggccgagcgcagaagtggtcctgcaactttatccgcctccatccagtctattaattgttgccgggaagctagagtaagtagttcgccagttaatagtttgcgcaacgttgttgccattgctacaggcatcgtggtgtcacgctcgtcgtttggtatggcttcattcagctccggttcccaacgatcaaggcgagttacatgatcccccatgttgtgcaaaaaagcggttagctccttcggtcctccgatcgttgtcagaagtaagttggccgcagtgttatcactcatggttatggcagcactgcataattctcttactgtcatgccatccgtaagatgcttttctgtgactggtgagtactcaaccaagtcattctgagaatagtgtatgcggcgaccgagttgctcttgcccggcgtcaatacgggataataccgcgccacatagcagaactttaaaagtgctcatcattggaaaacgttcttcggggcgaaaactctcaaggatcttaccgctgttgagatccagttcgatgtaacccactcgtgcacccaactgatcttcagcatcttttactttcaccagcgtttctgggtgagcaaaaacaggaaggcaaaatgccgcaaaaaagggaataagggcgacacggaaatgttgaatactcatactcttcctttttcaatattattgaagcatttatcagggttattgtctcatgagcggatacatatttgaatgtatttagaaaaataaacaaataggggttccgcgcacatttccccgaaaagtgccacctaaattgtaagcgttaatattttgttaaaattcgcgttaaatttttgttaaatcagctcattttttaaccaataggccgaaatcggcaaaatcccttataaatcaaaagaatagaccgagatagggttgagtgttgttccagtttggaacaagagtccactattaaagaacgtggactccaacgtcaaagggcgaaaaaccgtctatcagggcgatggcccactacgtgaaccatcaccctaatcaagttttttggggtcgaggtgccgtaaagcactaaatcggaaccctaaagggagcccccgatttagagcttgacggggaaagccggcgaacgtggcgagaaaggaagggaagaaagcgaaaggagcgggcgctagggcgctggcaagtgtagcggtcacgctgcgcgtaaccaccacacccgccgcgcttaatgcgccgctacagggcgcgatggatcc

SEQ ID NO: 2 - DNA, 7294 bp, synthetic construct
  misc_feature 1..7294: note = plasmid
  source 1..7294: mol_type = other DNA
gcgcgccgatatcgttaacgccccgcgccggccgctctagaactagtggatcccccggaagatcagaagttcctattccgaagttcctattctctagaaagtataggaacttctgatctgcgcagccgccatgccggggttttacgagattgtgattaaggtccccagcgaccttgacgagcatctgcccggcatttctgacagctttgtgaactgggtggccgagaaggaatgggagttgccgccagattctgacatggatctgaatctgattgagcaggcacccctgaccgtggccgagaagctgcagcgcgactttctgacggaatggcgccgtgtgagtaaggccccggaggcccttttctttgtgcaatttgagaagggagagagctacttccacatgcacgtgctcgtggaaaccaccggggtgaaatccatggttttgggacgtttcctgagtcagattcgcgaaaaactgattcagagaatttaccgcgggatcgagccgactttgccaaactggttcgcggtcacaaagaccagaaatggcgccggaggcgggaacaaggtggtggatgagtgctacatccccaattacttgctccccaaaacccagcctgagctccagtgggcgtggactaatatggaacagtatttaagcgcctgtttgaatctcacggagcgtaaacggttggtggcgcagcatctgacgcacgtgtcgcagacgcaggagcagaacaaagagaatcagaatcccaattctgatgcgccggtgatcagatcaaaaacttcagccaggtacatggagctggtcgggtggctcgtggacaaggggattacctcggagaagcagtggatccaggaggaccaggcctcatacatctccttcaatgcggcctccaactcgcggtcccaaatcaaggctgccttggacaatgcgggaaagattatgagcctgactaaaaccgcccccgactacctggtgggccagcagcccgtggaggacatttccagcaatcggatttataaaattttggaactaaacgggtacgatccccaatatgcggcttccgtctttctgggatgggccacgaaaaagttcggcaagaggaacaccatctggctgtttgggcctgcaactaccgggaagaccaacatcgcggaggccatagcccacactgtgcccttctacgggtgcgtaaactggaccaatgagaactttcccttcaacgactgtgtcgacaagatggtgatctggtgggaggaggggaagatgaccgccaaggtcgtggagtcggccaaagccattctcggaggaagcaaggtgcgcgtggaccagaaatgcaagtcctcggcccagatagacccgactcccgtgatcgtcacctccaacaccaacatgtgcgccgtgattgacgggaactcaacgaccttcgaacaccagcagccgttgcaagaccggatgttcaaatttgaactcacccgccgtctggatcatgactttgggaaggtcaccaagcaggaagtcaaagactttttccggtgggcaaaggatcacgtggttgaggtggagcatgaattctacgtcaaaaagggtggagccaagaaaagacccgcccccagtgacgcagatataagtgagcccaaacgggtgcgcgagtcagttgcgcagccatcgacgtcagacgcggaagcttcgatcaactacgcagacaggtaccaaaacaaatgttctcgtcacgtgggcatgaatctgatgctgtttccctgcagacaatgcgagagaatgaatcagaattcaaatatctgcttcactcacggacagaaagactgtttagagtgctttcccgtgtcagaatctcaacccgtttctgtcgtcaaaaaggcgtatcagaaactgtgctacattcatcatatcatgggaaaggtgccagacgcttgcactgcctgcgatctggtcaatgtggatttggatgactgcatctttgaacaataaatgatttaaatcaggtatgtcttttgttgatcaccctccagattggttggaagaagttggtgaaggtcttcgcgagtttttgggccttgaagcgggcccaccgaaaccaaaacccaatcagcagcatcaagatcaagcccgtggtcttgtgctgcctggttataactatctcggacccggaaacggtctcgatcgaggagagcctgtcaacagggcagacgaggtcgcgcgagagcacgacatctcgtacaacgagcagcttgaggcgggagacaacccctacctcaagtacaaccacgcggacgccgagtttcaggagaagctcgccgacgacacatccttcgggggaaacctcggaaaggcagtctttcaggccaagaaaagggttctcgaaccttttggcctggttgaagagggtgctaagacggcccctaccggaaagcggatagacgaccactttccaaaaagaaagaaggctcggaccgaagaggactccaagccttccacctcgtcagacgccgaagctggacccagcggatcccagcagctgcaaatcccagcccaaccagcctcaagtttgggagctgatacaatgtctgcgggaggtggcggcccattgggcgacaataaccaaggtgccgatggagtgggcaatgcctcgggagattggcattgcgattccacgtggatgggggacagagtcgtcaccaagtccacccgaacctgggtgctgcccagctacaacaaccaccagtaccgagagatcaaaagcggctccgtcgacggaagcaacgccaacgcctactttggatacagcaccccctgggggtactttgactttaaccgcttccacagccactggagcccccgagactggcaaagactcatcaacaactactggggcttcagaccccggtccctcagagtcaaaatcttcaacattcaagtcaaagaggtcacggtgcaggactccaccaccaccatcgccaacaacctcacctccaccgtccaagtgtttacggacgacgactaccagctgccctacgtcgtcggcaacgggaccgagggatgcctgccggccttccctccgcaggtctttacgctgccgcagtacggttacgcgacgctgaaccgcgacaacacagaaaatcccaccgagaggagcagcttcttctgcctagagtactttcccagcaagatgctgagaacgggcaacaactttgagtttacctacaactttgaggaggtgcccttccactccagcttcgctcccagtcagaacctgttcaagctggccaacccgctggtggaccagtacttgtaccgcttcgtgagcacaaataacactggcggagtccagttcaacaagaacctggccgggagatacgccaacacctacaaaaactggttcccggggcccatgggccgaacccagggctggaacctgggctccggggtcaaccgcgccagtgtcagcgccttcgccacgaccaataggatggagctcgagggcgcgagttaccaggtgcccccgcagccgaacggcatgaccaacaacctccagggcagcaacacctatgccctggagaacactatgatcttcaacagccagccggcgaacccgggcaccaccgccacgtacctcgagggcaacatgctcatcaccagcgagagcgagacgcagccggtgaaccgcgtggcgtacaacgtcggcgggcagatggccaccaacaaccagagctccaccactgcccccgcgaccggcacgtacaacctccaggaaatcgtgcccggcagcgtgtggatggagagggacgtgtacctccaaggacccatctgggccaagatcccagagacgggggcgcactttcacccctctccggccatgggcggattcggactcaaacacccaccgcccatgatgctcatcaagaacacgcctgtgcccggaaatatcaccagcttctcggacgtgcccgtcagcagcttcatcacccagtacagcaccgggcaggtcaccgtggagatggagtgggagctcaagaaggaaaactccaagaggtggaacccagagatccagtacacaaacaactacaacgacccccagtttgtggactttgccccggacagcaccggggaatacagaaccaccagacctatcggaacccgataccttacccgacccctttaattgcttgttaatcaataaaccgtttaattcgtttcagttgaactttggtctctgcgtatttctttcttatctagtttccatggctacgtagataagtagcatggcgggttaatcattaactacagcccgggcgtttaaacagcgggcggaggggtggagtcgtgacgtgaattacgtcatagggttagggaggtcctgtattagaggtcacgtgagtgttttgcgacattttgcgacaccatgtggtctcgctgggggggggggcccgagtgagcacgcagggtctccattttgaagcgggaggtttgaacgagcgctggcgcgctcactggccgtcgttttacaacgtcgtgactgggaaaaccctggcgttacccaacttaatcgccttgcagcacatccccctttcgccagctggcgtaatagcgaagaggcccgcaccgatcgcccttcccaacagttgcgcagcctgaatggcgaatggaaattgtaagcgttaatattttgttaaaattcgcgttaaatttttgttaaatcagctcatttttttaaccaataggccgaaatcggcaaaatcccttataaatcaaaagaatagaccgagatagggttgagtgttgttccagtttggaacaagagtccactattaagaacgtggactccaacgtcaaagggcgaaaaaccgtctatcagggcgatggcccactacgtgaaccatcaccctaatcaagttttttggggtcgaggtgccgtaaagcactaaatcggaaccctaaagggagcccccgatttagagcttgacggggaaagccggcgaacgtggcgagaaaggaagggaagaaagcgaaaggagcgggcgctagggcgctggcaagtgtagcggtcacgctgcgcgtaaccaccacacccgccgcgcttaatgcgccgctacagggcgcgtcaggtggcacttttcggggaaatgtgcgcggaacccctatttgtttatttttctaaatacattcaaatatgtatccgctcatgagacaataaccctgataaatgcttcaataatattgaaaaaggaagagtatgagtattcaacatttccgtgtcgcccttattcccttttttgcggcattttgccttcctgtttttgctcacccagaaacgctggtgaaagtaaaagatgctgaagatcagttgggtgcacgagtgggttacatcgaactggatctcaacagcggtaagatccttgagagttttcgccccgaagaacgttttccaatgatgagcacttttaaagttctgctatgtggcgcggtattatcccgtattgacgccgggcaagagcaactcggtcgccgcatacactattctcagaatgacttggttgagtactcaccagtcacagaaaagcatcttacggatggcatgacagtaagagaattatgcagtgctgccataaccatgagtgataacactgcggccaacttacttctgacaacgatcggaggaccgaaggagctaaccgcttttttgcacaacatgggggatcatgtaactcgccttgatcgttgggaaccggagctgaatgaagccataccaaacgacgagcgtgacaccacgatgcctgtagcaatggcaacaacgttgcgcaaactattaactggcgaactacttactctagcttcccggcaacaattaatagactggatggaggcggataaagttgcaggaccacttctgcgctcggcccttccggctggctggtttattgctgataaatctggagccggtgagcgtgggtctcgcggtatcattgcagcactggggccagatggtaagccctcccgtatcgtagttatctacacgacggggagtcaggcaactatggatgaacgaaatagacagatcgctgagataggtgcctcactgattaagcattggtaactgtcagaccaagtttactcatatatactttagattgatttaaaacttcatttttaatttaaaaggatctaggtgaagatcctttttgataatctcatgaccaaaatcccttaacgtgagttttcgttccactgagcgtcagaccccgtagaaaagatcaaaggatcttcttgagatcctttttttctgcgcgtaatctgctgcttgcaaacaaaaaaaccaccgctaccagcggtggtttgtttgccggatcaagagctaccaactctttttccgaaggtaactggcttcagcagagcgcagataccaaatactgttcttctagtgtagccgtagttaggccaccacttcaagaactctgtagcaccgcctacatacctcgctctgctaatcctgttaccagtggctgctgccagtggcgataagtcgtgtcttaccgggttggactcaagacgatagttaccggataaggcgcagcggtcgggctgaacggggggttcgtgcacacagcccagcttggagcgaacgacctacaccgaactgagatacctacagcgtgagctatgagaaagcgccacgcttcccgaagggagaaaggcggacaggtatccggtaagcggcagggtcggaacaggagagcgcacgagggagcttccagggggaaacgcctggtatctttatagtcctgtcgggtttcgccacctctgacttgagcgtcgatttttgtgatgctcgtcaggggggcggagcctatggaaaaacgccagcaacgcggcctttttacggttcctggccttttgctggccttttgctcacatgttctttcctgcgttatcccctgattctgtggataaccgtattaccgcctttgagtgagctgataccgctcgccgcagccgaacgaccgagcgcagcgagtcagtgagcgaggaagcggaagagcgcccaatacgcaaaccgcctctccccgcgcgttggccgattcattaatgcagctggcacgacaggtttcccgactggaaagcgggcagtgagcgcaacgcaattaatgtgagttagctcactcattaggcaccccaggctttacactttatgcttccggctcgtatgttgtgtggaattgtgagcggataacaatttcacacaggaaacagctatgaccatgattacgccaa

SEQ ID NO: 3 - DNA, 7622 bp, synthetic construct
  misc_feature 1..7622: note = plasmid
  source 1..7622: mol_type = other DNA
agcgcccaatacgcaaaccgcctctccccgcgcgttggccgattcattaatgcagctggcacgacaggtttcccgactggaaagcgggcagtgagcgcaacgcaattaatgtgagttagctcactcattaggcaccccaggctttacactttatgcttccggctcgtatgttgtgtggaattgtgagcggataacaatttcacacaggaaacagctatgaccatgattacgaattgcctgcaggcagctgcgcgctcgctcgctcactgaggccgcccgggcaaagcccgggcgtcgggcgacctttggtcgcccggcctcagtgagcgagcgagcgcgcagagagggagtggccaactccatcactaggggttcctatcgatatcaagctttaatagtaatcaattacggggtcattagttcatagcccatatatggagttccgcgttacataacttacggtaaatggcccgcctggctgaccgcccaacgacccccgcccattgacgtcaataatgacgtatgttcccatagtaacgccaatagggactttccattgacgtcaatgggtggagtatttacggtaaactgcccacttggcagtacatcaagtgtatcatatgccaagtacgccccctattgacgtcaatgacggtaaatggcccgcctggcattatgcccagtacatgaccttatgggactttcctacttggcagtacatctacgtattagtcatcgctattaccatggtgatgcggttttggcagtacatcaatgggcgtggatagcggtttgactcacggggatttccaagtctccaccccattgacgtcaatgggagtttgttttggcaccaaaatcaacgggactttccaaaatgtcgtaacaactccgccccattgacgcaaatgggcggtaggcgtgtacggtgggaggtctatataagcagagctggtttagtggatatccttaagggcccagccggcctcgcgagaattctctagaacgccgccatgaccatgattacggattcactggccgtcgttttacaacgtcgtgactgggaaaaccctggcgttacccaacttaatcgccttgcagcacatccccctttcgccagctggcgtaatagcgaagaggcccgcaccgatcgcccttcccaacagttgcgcagcctgaatggcgaatggcgctttgcctggtttccggcaccagaagcggtgccggaaagctggctggagtgcgatcttcctgaggccgatactgtcgtcgtcccctcaaactggcagatgcacggttacgatgcgcccatctacaccaacgtgacctatcccattacggtcaatccgccgtttgttcccacggagaatccgacgggttgttactcgctcacatttaatgttgatgaaagctggctacaggaaggccagacgcgaattatttttgatggcgttaactcggcgtttcatctgtggtgcaacgggcgctgggtcggttacggccaggacagtcgtttgccgtctgaatttgacctgagcgcatttttacgcgccggagaaaaccgcctcgcggtgatggtgctgcgctggagtgacggcagttatctggaagatcaggatatgtggcggatgagcggcattttccgtgacgtctcgttgctgcataaaccgactacacaaatcagcgatttccatgttgccactcgctttaatgatgatttcagccgcgctgtactggaggctgaagttcagatgtgcggcgagttgcgtgactacctacgggtaacagtttctttatggcagggtgaaacgcaggtcgccagcggcaccgcgcctttcggcggtgaaattatcgatgagcgtggtggttatgccgatcgcgtcacactacgtctgaacgtcgaaaacccgaaactgtggagcgccgaaatcccgaatctctatcgtgcggtggttgaactgcacaccgccgacggcacgctgattgaagcagaagcctgcgatgtcggtttccgcgaggtgcggattgaaaatggtctgctgctgctgaacggcaagccgttgctgattcgaggcgttaaccgtcacgagcatcatcctctgcatggtcaggtcatggatgagcagacgatggtgcaggatatcctgctgatgaagcagaacaactttaacgccgtgcgctgttcgcattatccgaaccatccgctgtggtacacgctgtgcgaccgctacggcctgtatgtggtggatgaagccaatattgaaacccacggcatggtgccaatgaatcgtctgaccgatgatccgcgctggctaccggcgatgagcgaacgcgtaacgcgaatggtgcagcgcgatcgtaatcacccgagtgtgatcatctggtcgctggggaatgaatcaggccacggcgctaatcacgacgcgctgtatcgctggatcaaatctgtcgatccttcccgcccggtgcagtatgaaggcggcggagccgacaccacggccaccgatattatttgcccgatgtacgcgcgcgtggatgaagaccagcccttcccggctgtgccgaaatggtccatcaaaaaatggctttcgctacctggagagacgcgcccgctgatcctttgcgaatacgcccacgcgatgggtaacagtcttggcggtttcgctaaatactggcaggcgtttcgtcagtatccccgtttacagggcggcttcgtctgggactgggtggatcagtcgctgattaaatatgatgaaaacggcaacccgtggtcggcttacggcggtgattttggcgatacgccgaacgatcgccagttctgtatgaacggtctggtctttgccgaccgcacgccgcatccagcgctgacggaagcaaaacaccagcagcagtttttccagttccgtttatccgggcaaaccatcgaagtgaccagcgaatacctgttccgtcatagcgataacgagctcctgcactggatggtggcgctggatggtaagccgctggcaagcggtgaagtgcctctggatgtcgctccacaaggtaaacagttgattgaactgcctgaactaccgcagccggagagcgccgggcaactctggctcacagtacgcgtagtgcaaccgaacgcgaccgcatggtcagaagccgggcacatcagcgcctggcagcagtggcgtctggcggaaaacctcagtgtgacgctccccgccgcgtcccacgccatcccgcatctgaccaccagcgaaatggatttttgcatcgagctgggtaataagcgttggcaatttaaccgccagtcaggctttctttcacagatgtggattggcgataaaaaacaactgctgacgccgctgcgcgatcagttcacccgtgcaccgctggataacgacattggcgtaagtgaagcgacccgcattgaccctaacgcctgggtcgaacgctggaaggcggcgggccattaccaggccgaagcagcgttgttgcagtgcacggcagatacacttgctgatgcggtgctgattacgaccgctcacgcgtggcagcatcaggggaaaaccttatttatcagccggaaaacctaccggattgatggtagtggtcaaatggcgattaccgttgatgttgaagtggcgagcgatacaccgcatccggcgcggattggcctgaactgccagctggcgcaggtagcagagcgggtaaactggctcggattagggccgcaagaaaactatcccgaccgccttactgccgcctgttttgaccgctgggatctgccattgtcagacatgtataccccgtacgtcttcccgagcgaaaacggtctgcgctgcgggacgcgcgaattgaattatggcccacaccagtggcgcggcgacttccagttcaacatcagccgctacagtcaacagcaactgatggaaaccagccatcgccatctgctgcacgcggaagaaggcacatggctgaatatcgacggtttccatatggggattggtggcgacgactcctggagcccgtcagtatcggcggaattccagctgagcgccggtcgctaccattaccagttggtctggtgtcaaaaataaagctgacactagtgcggatccacgggtggcatccctgtgacccctccccagtgcctctcctggccctggaagttgccactccagtgcccaccagccttgtcctaataaaattaagttgcatcattttgtctgactaggtgtccttctataatattatggggtggaggggggtggtatggagcaaggggcaagttgggaagacaacctgtagggcctgcggggtctattgggaaccaagctggagtgcagtggcacaatcttggctcactgcaatctccgcctcctgggttcaagcgattctcctgcctcagcctcccgagttgttgggattccaggcatgcatgaccaggctcagctaatttttgtttttttggtagagacggggtttcaccatattggccaggctggtctccaactcctaatctcaggtgatctacccaccttggcctcccaaattgctgggattacaggcgtgaaccactgctcccttccctgtccttatcgatagatctaggaacccctagtgatggagttggccactccctctctgcgcgctcgctcgctcactgaggccgggcgaccaaaggtcgcccgacgcccgggctttgcccgggcggcctcagtgagcgagcgagcgcgcagctgcctgcaggcagcttggcactggccgtcgttttacaacgtcgtgactgggaaaaccctggcgttacccaacttaatcgccttgcagcacatccccctttcgccagctggcgtaatagcgaagaggcccgcaccgatcgcccttcccaacagttgcgcagcctgaatggcgaatggcgcctgatgcggtattttctccttacgcatctgtgcggtatttcacaccgcatacgtcaaagcaaccatagtacgcgccctgtagcggcgcattaagcgcggcgggtgtggtggttacgcgcagcgtgaccgctacacttgccagcgccctagcgcccgctcctttcgctttcttcccttcctttctcgccacgttcgccggctttccccgtcaagctctaaatcgggggctccctttagggttccgatttagtgctttacggcacctcgaccccaaaaaacttgatttgggtgatggttcacgtagtgggccatcgccctgatagacggtttttcgccctttgacgttggagtccacgttctttaatagtggactcttgttccaaactggaacaacactcaaccctatctcgggctattcttttgatttataagggattttgccgatttcggcctattggttaaaaaatgagctgatttaacaaaaatttaacgcgaattttaacaaaatattaacgtttacaattttatggtgcactctcagtacaatctgctctgatgccgcatagttaagccagccccgacacccgccaacacccgctgacgcgccctgacgggcttgtctgctcccggcatccgcttacagacaagctgtgaccgtctccgggagctgcatgtgtcagaggttttcaccgtcatcaccgaaacgcgcgagacgaaagggcctcgtgatacgcctatttttataggttaatgtcatgataataatggtttcttagacgtcaggtggcacttttcggggaaatgtgcgcggaacccctatttgtttatttttctaaatacattcaaatatgtatccgctcatgagacaataaccctgataaatgcttcaataatattgaaaaaggaagagtatgagtattcaacatttccgtgtcgcccttattcccttttttgcggcattttgccttcctgtttttgctcacccagaaacgctggtgaaagtaaaagatgctgaagatcagttgggtgcacgagtgggttacatcgaactggatctcaacagcggtaagatccttgagagttttcgccccgaagaacgttttccaatgatgagcacttttaaagttctgctatgtggcgcggtattatcccgtattgacgccgggcaagagcaactcggtcgccgcatacactattctcagaatgacttggttgagtactcaccagtcacagaaaagcatcttacggatggcatgacagtaagagaattatgcagtgctgccataaccatgagtgataacactgcggccaacttacttctgacaacgatcggaggaccgaaggagctaaccgcttttttgcacaacatgggggatcatgtaactcgccttgatcgttgggaaccggagctgaatgaagccataccaaacgacgagcgtgacaccacgatgcctgtagcaatggcaacaacgttgcgcaaactattaactggcgaactacttactctagcttcccggcaacaattaatagactggatggaggcggataaagttgcaggaccacttctgcgctcggcccttccggctggctggtttattgctgataaatctggagccggtgagcgtgggtctcgcggtatcattgcagcactggggccagatggtaagccctcccgtatcgtagttatctacacgacggggagtcaggcaactatggatgaacgaaatagacagatcgctgagataggtgcctcactgattaagcattggtaactgtcagaccaagtttactcatatatactttagattgatttaaaacttcatttttaatttaaaaggatctaggtgaagatcctttttgataatctcatgaccaaaatcccttaacgtgagttttcgttccactgagcgtcagaccccgtagaaaagatcaaaggatcttcttgagatcctttttttctgcgcgtaatctgctgcttgcaaacaaaaaaaccaccgctaccagcggtggtttgtttgccggatcaagagctaccaactctttttccgaaggtaactggcttcagcagagcgcagataccaaatactgttcttctagtgtagccgtagttaggccaccacttcaagaactctgtagcaccgcctacatacctcgctctgctaatcctgttaccagtggctgctgccagtggcgataagtcgtgtcttaccgggttggactcaagacgatagttaccggataaggcgcagcggtcgggctgaacggggggttcgtgcacacagcccagcttggagcgaacgacctacaccgaactgagatacctacagcgtgagctatgagaaagcgccacgcttcccgaagggagaaaggcggacaggtatccggtaagcggcagggtcggaacaggagagcgcacgagggagcttccagggggaaacgcctggtatctttatagtcctgtcgggtttcgccacctctgacttgagcgtcgatttttgtgatgctcgtcaggggggcggagcctatggaaaaacgccagcaacgcggcctttttacggttcctggccttttgctggccttttgctcacatgttctttcctgcgttatcccctgattctgtggataaccgtattaccgcctttgagtgagctgataccgctcgccgcagccgaacgaccgagcgcagcgagtcagtgagcgaggaagcggaag

SEQ ID NO: 4 - DNA, 5909 bp, synthetic construct
  misc_feature 1..5909: note = plasmid
  source 1..5909: mol_type = other DNA
agcgcccaatacgcaaaccgcctctccccgcgcgttggccgattcattaatgcagctggcacgacaggtttcccgactggaaagcgggcagtgagcgcaacgcaattaatgtgagttagctcactcattaggcaccccaggctttacactttatgcttccggctcgtatgttgtgtggaattgtgagcggataacaatttcacacaggaaacagctatgaccatgattacgaattgcctgcaggcagctgcgcgctcgctcgctcactgaggccgcccgggcaaagcccgggcgtcgggcgacctttggtcgcccggcctcagtgagcgagcgagcgcgcagagagggagtggccaactccatcactaggggttcctgcggccgcacgcgtggagctagttattaatagtaatcaattacggggtcattagttcatagcccatatatggagttccgcgttacataacttacggtaaatggcccgcctggctgaccgcccaacgacccccgcccattgacgtcaataatgacgtatgttcccatagtaacgtcaatagggactttccattgacgtcaatgggtggagtatttacggtaaactgcccacttggcagtacatcaagtgtatcatatgccaagtacgccccctattgacgtcaatgacggtaaatggcccgcctggcattatgcccagtacatgaccttatgggactttcctacttggcagtacatctacgtattagtcatcgctattaccatggtgatgcggttttggcagtacatcaatgggcgtggatagcggtttgactcacggggatttccaagtctccaccccattgacgtcaatgggagtttgttttgcaccaaaatcaacgggactttccaaaatgtcgtaacaactccgccccattgacgcaaatgggcggtaggcgtgtacggtgggaggtctatataagcagagctcgtttagtgaaccgtcagatcgcctggagacgccatccacgctgttttgacctccatagaagacaccgggaccgatccagcctccgcggattcgaatcccggccgggaacggtgcattggaacgcggattccccgtgccaagagtgacgtaagtaccgcctatagagtctataggcccacaaaaaatgctttcttcttttaatatacttttttgtttatcttatttctaatactttccctaatctctttctttcagggcaataatgatacaatgtatcatgcctctttgcaccattctaaagaataacagtgataatttctgggttaaggcaatagcaatatttctgcatataaatatttctgcatataaattgtaactgatgtaagaggtttcatattgctaatagcagctacaatccagctaccattctgcttttattttatggttgggataaggctggattattctgagtccaagctaggcccttttgctaatcatgttcatacctcttatcttcctcccacagctcctgggcaacgtgctggtctgtgtgctggcccatcactttggcaaagaattgggattcgaacatcgattgaattctgaatggtgagcaagggcgaggagctgttcaccggggtggtgcccatcctggtcgagctggacggcgacgtaaacggccacaagttcagcgtgtccggcgagggcgagggcgatgccacctacggcaagctgaccctgaagttcatctgcaccaccggcaagctgcccgtgccctggcccaccctcgtgaccaccctgacctacggcgtgcagtgcttcagccgctaccccgaccacatgaagcagcacgacttcttcaagtccgccatgcccgaaggctacgtccaggagcgcaccatcttcttcaaggacgacggcaactacaagacccgcgccgaggtgaagttcgagggcgacaccctggtgaaccgcatcgagctgaagggcatcgacttcaaggaggacggcaacatcctggggcacaagctggagtacaactacaacagccacaacgtctatatcatggccgacaagcagaagaacggcatcaaggtgaacttcaagatccgccacaacatcgaggacggcagcgtgcagctcgccgaccactaccagcagaacacccccatcggcgacggccccgtgctgctgcccgacaaccactacctgagcacccagtccgccctgagcaaagaccccaacgagaagcgcgatcacatggtcctgctggagttcgtgaccgccgccgggatcactctcggcatggacgagctgtacaagtactcagatctcgagctcaagtagggatcctctagagtcgacctgcagaagcttgcctcgagcagcgctgctcgagagatctacgggtggcatccctgtgacccctccccagtgcctctcctggccctggaagttgccactccagtgcccaccagccttgtcctaataaaattaagttgcatcattttgtctgactaggtgtccttctataatattatggggtggaggggggtggtatggagcaaggggcaagttgggaagacaacctgtagggcctgcggggtctattgggaaccaagctggagtgcagtggcacaatcttggctcactgcaatctccgcctcctgggttcaagcgattctcctgcctcagcctcccgagttgttgggattccaggcatgcatgaccaggctcagctaatttttgtttttttggtagagacggggtttcaccatattggccaggctggtctccaactcctaatctcaggtgatctacccaccttggcctcccaaattgctgggattacaggcgtgaaccactgctcccttccctgtccttctgattttgtaggtaaccacgtgcggaccgagcggccgcaggaacccctagtgatggagttggccactccctctctgcgcgctcgctcgctcactgaggccgggcgaccaaaggtcgcccgacgcccgggctttgcccgggcggcctcagtgagcgagcgagcgcgcagctgcctgcaggcagcttggcactggccgtcgttttacaacgtcgtgactgggaaaaccctggcgttacccaacttaatcgccttgcagcacatccccctttcgccagctggcgtaatagcgaagaggcccgcaccgatcgcccttcccaacagttgcgcagcctgaatggcgaatggcgcctgatgcggtattttctccttacgcatctgtgcggtatttcacaccgcatacgtcaaagcaaccatagtacgcgccctgtagcggcgcattaagcgcggcgggtgtggtggttacgcgcagcgtgaccgctacacttgccagcgccctagcgcccgctcctttcgctttcttcccttcctttctcgccacgttcgccggctttccccgtcaagctctaaatcgggggctccctttagggttccgatttagtgctttacggcacctcgaccccaaaaaacttgatttgggtgatggttcacgtagtgggccatcgccctgatagacggtttttcgccctttgacgttggagtccacgttctttaatagtggactcttgttccaaactggaacaacactcaaccctatctcgggctattcttttgatttataagggattttgccgatttcggcctattggttaaaaaatgagctgatttaacaaaaatttaacgcgaattttaacaaaatattaacgtttacaattttatggtgcactctcagtacaatctgctctgatgccgcatagttaagccagccccgacacccgccaacacccgctgacgcgccctgacgggcttgtctgctcccggcatccgcttacagacaagctgtgaccgtctccgggagctgcatgtgtcagaggttttcaccgtcatcaccgaaacgcgcgagacgaaagggcctcgtgatacgcctatttttataggttaatgtcatgataataatggtttcttagacgtcaggtggcacttttcggggaaatgtgcgcggaacccctatttgtttatttttctaaatacattcaaatatgtatccgctcatgagacaataaccctgataaatgcttcaataatattgaaaaaggaagagtatgagtattcaacatttccgtgtcgcccttattcccttttttgcggcattttgccttcctgtttttgctcacccagaaacgctggtgaaagtaaaagatgctgaagatcagttgggtgcacgagtgggttacatcgaactggatctcaacagcggtaagatccttgagagttttcgccccgaagaacgttttccaatgatgagcacttttaaagttctgctatgtggcgcggtattatcccgtattgacgccgggcaagagcaactcggtcgccgcatacactattctcagaatgacttggttgagtactcaccagtcacagaaaagcatcttacggatggcatgacagtaagagaattatgcagtgctgccataaccatgagtgataacactgcggccaacttacttctgacaacgatcggaggaccgaaggagctaaccgcttttttgcacaacatgggggatcatgtaactcgccttgatcgttgggaaccggagctgaatgaagccataccaaacgacgagcgtgacaccacgatgcctgtagcaatggcaacaacgttgcgcaaactattaactggcgaactacttactctagcttcccggcaacaattaatagactggatggaggcggataaagttgcaggaccacttctgcgctcggcccttccggctggctggtttattgctgataaatctggagccggtgagcgtgggtctcgcggtatcattgcagcactggggccagatggtaagccctcccgtatcgtagttatctacacgacggggagtcaggcaactatggatgaacgaaatagacagatcgctgagataggtgcctcactgattaagcattggtaactgtcagaccaagtttactcatatatactttagattgatttaaaacttcatttttaatttaaaaggatctaggtgaagatcctttttgataatctcatgaccaaaatcccttaacgtgagttttcgttccactgagcgtcagaccccgtagaaaagatcaaaggatcttcttgagatcctttttttctgcgcgtaatctgctgcttgcaaacaaaaaaaccaccgctaccagcggtggtttgtttgccggatcaagagctaccaactctttttccgaaggtaactggcttcagcagagcgcagataccaaatactgttcttctagtgtagccgtagttaggccaccacttcaagaactctgtagcaccgcctacatacctcgctctgctaatcctgttaccagtggctgctgccagtggcgataagtcgtgtcttaccgggttggactcaagacgatagttaccggataaggcgcagcggtcgggctgaacggggggttcgtgcacacagcccagcttggagcgaacgacctacaccgaactgagatacctacagcgtgagctatgagaaagcgccacgcttcccgaagggagaaaggcggacaggtatccggtaagcggcagggtcggaacaggagagcgcacgagggagcttccagggggaaacgcctggtatctttatagtcctgtcgggtttcgccacctctgacttgagcgtcgatttttgtgatgctcgtcaggggggcggagcctatggaaaaacgccagcaacgcggcctttttacggttcctggccttttgctggccttttgctcacatgttctttcctgcgttatcccctgattctgtggataaccgtattaccgcctttgagtgagctgataccgctcgccgcagccgaacgaccgagcgcagcgagtcagtgagcgaggaagcggaag

SEQ ID NO: 5 - DNA, 8451 bp, synthetic construct
  misc_feature 1..8451: note = plasmid
  source 1..8451: mol_type = other DNA
ggtacccaactccatgcttaacagtccccaggtacagcccaccctgcgtcgcaaccaggaacagctctacagcttcctggagcgccactcgccctacttccgcagccacagtgcgcagattaggagcgccacttctttttgtcacttgaaaaacatgtaaaaataatgtactaggagacactttcaataaaggcaaatgtttttatttgtacactctcgggtgattatttaccccccacccttgccgtctgcgccgtttaaaaatcaaaggggttctgccgcgcatcgctatgcgccactggcagggacacgttgcgatactggtgtttagtgctccacttaaactcaggcacaaccatccgcggcagctcggtgaagttttcactccacaggctgcgcaccatcaccaacgcgtttagcaggtcgggcgccgatatcttgaagtcgcagttggggcctccgccctgcgcgcgcgagttgcgatacacagggttgcagcactggaacactatcagcgccgggtggtgcacgctggccagcacgctcttgtcggagatcagatccgcgtccaggtcctccgcgttgctcagggcgaacggagtcaactttggtagctgccttcccaaaaagggtgcatgcccaggctttgagttgcactcgcaccgtagtggcatcagaaggtgaccgtgcccggtctgggcgttaggatacagcgcctgcatgaaagccttgatctgcttaaaagccacctgagcctttgcgccttcagagaagaacatgccgcaagacttgccggaaaactgattggccggacaggccgcgtcatgcacgcagcaccttgcgtcggtgttggagatctgcaccacatttcggccccaccggttcttcacgatcttggccttgctagactgctccttcagcgcgcgctgcccgttttcgctcgtcacatccatttcaatcacgtgctccttatttatcataatgctcccgtgtagacacttaagctcgccttcgatctcagcgcagcggtgcagccacaacgcgcagcccgtgggctcgtggtgcttgtaggttacctctgcaaacgactgcaggtacgcctgcaggaatcgccccatcatcgtcacaaaggtcttgttgctggtgaaggtcagctgcaacccgcggtgctcctcgtttagccaggtcttgcatacggccgccagagcttccacttggtcaggcagtagcttgaagtttgcctttagatcgttatccacgtggtacttgtccatcaacgcgcgcgcagcctccatgcccttctcccacgcagacacgatcggcaggctcagcgggtttatcaccgtgctttcactttccgcttcactggactcttccttttcctcttgcgtccgcataccccgcgccactgggtcgtcttcattcagccgccgcaccgtgcgcttacctcccttgccgtgcttgattagcaccggtgggttgctgaaacccaccatttgtagcgccacatcttctctttcttcctcgctgtccacgatcacctctggggatggcgggcgctcgggcttgggagaggggcgcttctttttctttttggacgcaatggccaaatccgccgtcgaggtcgatggccgcgggctgggtgtgcgcggcaccagcgcatcttgtgacgagtcttcttcgtcctcggactcgagacgccgcctcagccgcttttttgggggcgcgcggggaggcggcggcgacggcgacggggacgacacgtcctccatggttggtggacgtcgcgccgcaccgcgtccgcgctcgggggtggtttcgcgctgctcctcttcccgactggccatttccttctcctataggcagaaaaagatcatggagtcagtcgagaaggaggacagcctaaccgccccctttgagttcgccaccaccgcctccaccgatgccgccaacgcgcctaccaccttccccgtcgaggcacccccgcttgaggaggaggaagtgattatcgagcaggacccaggttttgtaagcgaagacgacgaggatcgctcagtaccaacagaggataaaaagcaagaccaggacgacgcagaggcaaacgaggaacaagtcgggcggggggaccaaaggcatggcgactacctagatgtgggagacgacgtgctgttgaagcatctgcagcgccagtgcgccattatctgcgacgcgttgcaagagcgcagcgatgtgcccctcgccatagcggatgtcagccttgcctacgaacgccacctgttctcaccgcgcgtaccccccaaacgccaagaaaacggcacatgcgagcccaacccgcgcctcaacttctaccccgtatttgccgtgccagaggtgcttgccacctatcacatctttttccaaaactgcaagatacccctatcctgccgtgccaaccgcagccgagcggacaagcagctggccttgcggcagggcgctgtcatacctgatatcgcctcgctcgacgaagtgccaaaaatctttgagggtcttggacgcgacgagaaacgcgcggcaaacgctctgcaacaagaaaacagcgaaaatgaaagtcactgtggagtgctggtggaacttgagggtgacaacgcgcgcctagccgtgctgaaacgcagcatcgaggtcacccactttgcctacccggcacttaacctaccccccaaggttatgagcacagtcatgagcgagctgatcgtgcgccgtgcacgacccctggagagggatgcaaacttgcaagaacaaaccgaggagggcctacccgcagttggcgatgagcagctggcgcgctggcttgagacgcgcgagcctgccgacttggaggagcgacgcaagctaatgatggccgcagtgcttgttaccgtggagcttgagtgcatgcagcggttctttgctgacccggagatgcagcgcaagctagaggaaacgttgcactacacctttcgccagggctacgtgcgccaggcctgcaaaatttccaacgtggagctctgcaacctggtctcctaccttggaattttgcacgaaaaccgcctcgggcaaaacgtgcttcattccacgctcaagggcgaggcgcgccgcgactacgtccgcgactgcgtttacttatttctgtgctacacctggcaaacggccatgggcgtgtggcagcaatgcctggaggagcgcaacctaaaggagctgcagaagctgctaaagcaaaacttgaaggacctatggacggccttcaacgagcgctccgtggccgcgcacctggcggacattatcttccccgaacgcctgcttaaaaccctgcaacagggtctgccagacttcaccagtcaaagcatgttgcaaaactttaggaactttatcctagagcgttcaggaattctgcccgccacctgctgtgcgcttcctagcgactttgtgcccattaagtaccgtgaatgccctccgccgctttggggtcactgctaccttctgcagctagccaactaccttgcctaccactccgacatcatggaagacgtgagcggtgacggcctactggagtgtcactgtcgctgcaacctatgcaccccgcaccgctccctggtctgcaattcgcaactgcttagcgaaagtcaaattatcggtacctttgagctgcagggtccctcgcctgacgaaaagtccgcggctccggggttgaaactcactccggggctgtggacgtcggcttaccttcgcaaatttgtacctgaggactaccacgcccacgagattaggttctacgaagaccaatcccgcccgccaaatgcggagcttaccgcctgcgtcattacccagggccacatccttggccaattgcaagccatcaacaaagcccgccaagagtttctgctacgaaagggacggggggtttacctggacccccagtccggcgaggagctcaacccaatccccccgccgccgcagccctatcagcagccgcgggcccttgcttcccaggatggcacccaaaaagaagctgcagctgccgccgccgccacccacggacgaggaggaatactgggacagtcaggcagaggaggttttggacgaggaggaggagatgatggaagactgggacagcctagacgaagcttccgaggccgaagaggtgtcagacgaaacaccgtcaccctcggtcgcattcccctcgccggcgccccagaaattggcaaccgttcccagcatcgctacaacctccgctcctcaggcgccgccggcactgcctgttcgccgacccaaccgtagatgggacaccactggaaccagggccggtaagtctaagcagccgccgccgttagcccaagagcaacaacagcgccaaggctaccgctcgtggcgcgggcacaagaacgccatagttgcttgcttgcaagactgtgggggcaacatctccttcgcccgccgctttcttctctaccatcacggcgtggccttcccccgtaacatcctgcattactaccgtcatctctacagcccctactgcaccggcggcagcggcagcggcagcaacagcagcggtcacacagaagcaaaggcgaccggatagcaagactctgacaaagcccaagaaatccacagcggcggcagcagcaggaggaggagcgctgcgtctggcgcccaacgaacccgtatcgacccgcgagcttagaaataggatttttcccactctgtatgctatatttcaacaaagcaggggccaagaacaagagctgaaaataaaaaacaggtctctgcgctccctcacccgcagctgcctgtatcacaaaagcgaagatcagcttcggcgcacgctggaagacgcggaggctctcttcagcaaatactgcgcgctgactcttaaggactagtttcgcgccctttctcaaatttaagcgcgaaaactacgtcatctccagcggccacacccggcgccagcacctgtcgtcagcgccattatgagcaaggaaattcccacgccctacatgtggagttaccagccacaaatgggacttgcggctggagctgcccaagactactcaacccgaataaactacatgagcgcgggaccccacatgatatcccgggtcaacggaatccgcgcccaccgaaaccgaattctcctcgaacaggcggctattaccaccacacctcgtaataaccttaatccccgtagttggcccgctgccctggtgtaccaggaaagtcccgctcccaccactgtggtacttcccagagacgcccaggccgaagttcagatgactaactcaggggcgcagcttgcgggcggctttcgtcacagggtgcggtcgcccgggcgcggccgcaatcgatgtaggatgttgcccctcctgacgcggtaggagaaggggagggtgccctgcatgtctgccgctgctcttgctcttgccgctgctgaggaggggggcgcatctgccgcagcaccggatgcatctgggaaaagcaaaaaaggggctcgtccctgtttccggaggaatttgcaagcggggtcttgcatgacggggaggcaaacccccgttcgccgcagtccggccggcccgagactcgaaccgggggtcctgcgactcaacccttggaaaataaccctccggctacagggagcgagccacttaatgctttcgctttccagcctaaccgcttacgccgcgcgcggccagtggccaaaaaagctagcgcagcagccgccgcgcctggaaggaagccaaaaggagcgctcccccgttgtctgacgtcgcacacctgggttcgacacgcgggcggtaaccgcatggatcacggcggacggccggatccggggttcgaaccccggtcgtccgccatgatacccttgcgaatttatccaccagaccacggaagagtgcccgcttacaggctctccttttgcacggtctagagcgtcaacgactgcgcacgcctcaccggccagagcgtcccgaccatggagcactttttgccgctgcgcaacatctggaaccgcgtccgcgactttccgcgcgcctccaccaccgccgccggcatcacctggatgtccaggtacatctacggattacgtcgacgtttaaaccatatgatcagctcactcaaaggcggtaatacggttatccacagaatcaggggataacgcaggaaagaacatgtgagcaaaaggccagcaaaaggccaggaaccgtaaaaaggccgcgttgctggcgtttttccataggctccgcccccctgacgagcatcacaaaaatcgacgctcaagtcagaggtggcgaaacccgacaggactataaagataccaggcgtttccccctggaagctccctcgtgcgctctcctgttccgaccctgccgcttaccggatacctgtccgcctttctcccttcgggaagcgtggcgctttctcatagctcacgctgtaggtatctcagttcggtgtaggtcgttcgctccaagctgggctgtgtgcacgaaccccccgttcagcccgaccgctgcgccttatccggtaactatcgtcttgagtccaacccggtaagacacgacttatcgccactggcagcagccactggtaacaggattagcagagcgaggtatgtaggcggtgctacagagttcttgaagtggtggcctaactacggctacactagaagaacagtatttggtatctgcgctctgctgaagccagttaccttcggaaaaagagttggtagctcttgatccggcaaacaaaccaccgctggtagcggtggtttttttgtttgcaagcagcagattacgcgcagaaaaaaaggatctcaagaagatcctttgatcttttctacggggtctgacgctcagtggaacgaaaactcacgttaagggattttggtcatgagattatcaaaaaggatcttcacctagatccttttaaattaaaaatgaagttttaaatcaatctaaagtatatatgagtaaacttggtctgacagttaccaatgcttaatcagtgaggcacctatctcagcgatctgtctatttcgttcatccatagttgcctgactccccgtcgtgtagataactacgatacgggagggcttaccatctggccccagtgctgcaatgataccgcgagacccacgctcaccggctccagatttatcagcaataaaccagccagccggaagggccgagcgcagaagtggtcctgcaactttatccgcctccatccagtctattaattgttgccgggaagctagagtaagtagttcgccagttaatagtttgcgcaacgttgttgccattgctacaggcatcgtggtgtcacgctcgtcgtttggtatggcttcattcagctccggttcccaacgatcaaggcgagttacatgatcccccatgttgtgcaaaaaagcggttagctccttcggtcctccgatcgttgtcagaagtaagttggccgcagtgttatcactcatggttatggcagcactgcataattctcttactgtcatgccatccgtaagatgcttttctgtgactggtgagtactcaaccaagtcattctgagaatagtgtatgcggcgaccgagttgctcttgcccggcgtcaatacgggataataccgcgccacatagcagaactttaaaagtgctcatcattggaaaacgttcttcggggcgaaaactctcaaggatcttaccgctgttgagatccagttcgatgtaacccactcgtgcacccaactgatcttcagcatcttttactttcaccagcgtttctgggtgagcaaaaacaggaaggcaaaatgccgcaaaaaagggaataagggcgacacggaaatgttgaatactcatactcttcctttttcaatattattgaagcatttatcagggttattgtctcatgagcggatacatatttgaatgtatttagaaaaataaacaaataggggttccgcgcacatttccccgaaaagtgccacctaaattgtaagcgttaatattttgttaaaattcgcgttaaatttttgttaaatcagctcattttttaaccaataggccgaaatcggcaaaatcccttataaatcaaaagaatagaccgagatagggttgagtgttgttccagtttggaacaagagtccactattaaagaacgtggactccaacgtcaaagggcgaaaaaccgtctatcagggcgatggcccactacgtgaaccatcaccctaatcaagttttttggggtcgaggtgccgtaaagcactaaatcggaaccctaaagggagcccccgatttagagcttgacggggaaagccggcgaacgtggcgagaaaggaagggaagaaagcgaaaggagcgggcgctagggcgctggcaagtgtagcggtcacgctgcgcgtaaccaccacacccgccgcgcttaatgcgccgctacagggcgcgatggatcc

SEQ ID NO: 6 - DNA, 10912 bp, synthetic construct
  misc_feature 1..10912: note = plasmid
  source 1..10912: mol_type = other DNA
ggtacccaactccatgcttaacagtccccaggtacagcccaccctgcgtcgcaaccaggaacagctctacagcttcctggagcgccactcgccctacttccgcagccacagtgcgcagattaggagcgccacttctttttgtcacttgaaaaacatgtaaaaataatgtactaggagacactttcaataaaggcaaatgtttttatttgtacactctcgggtgattatttaccccccacccttgccgtctgcgccgtttaaaaatcaaaggggttctgccgcgcatcgctatgcgccactggcagggacacgttgcgatactggtgtttagtgctccacttaaactcaggcacaaccatccgcggcagctcggtgaagttttcactccacaggctgcgcaccatcaccaacgcgtttagcaggtcgggcgccgatatcttgaagtcgcagttggggcctccgccctgcgcgcgcgagttgcgatacacagggttgcagcactggaacactatcagcgccgggtggtgcacgctggccagcacgctcttgtcggagatcagatccgcgtccaggtcctccgcgttgctcagggcgaacggagtcaactttggtagctgccttcccaaaaagggtgcatgcccaggctttgagttgcactcgcaccgtagtggcatcagaaggtgaccgtgcccggtctgggcgttaggatacagcgcctgcatgaaagccttgatctgcttaaaagccacctgagcctttgcgccttcagagaagaacatgccgcaagacttgccggaaaactgattggccggacaggccgcgtcatgcacgcagcaccttgcgtcggtgttggagatctgcaccacatttcggccccaccggttcttcacgatcttggccttgctagactgctccttcagcgcgcgctgcccgttttcgctcgtcacatccatttcaatcacgtgctccttatttatcataatgctcccgtgtagacacttaagctcgccttcgatctcagcgcagcggtgcagccacaacgcgcagcccgtgggctcgtggtgcttgtaggttacctctgcaaacgactgcaggtacgcctgcaggaatcgccccatcatcgtcacaaaggtcttgttgctggtgaaggtcagctgcaacccgcggtgctcctcgtttagccaggtcttgcatacggccgccagagcttccacttggtcaggcagtagcttgaagtttgcctttagatcgttatccacgtggtacttgtccatcaacgcgcgcgcagcctccatgcccttctcccacgcagacacgatcggcaggctcagcgggtttatcaccgtgctttcactttccgcttcactggactcttccttttcctcttgcgtccgcataccccgcgccactgggtcgtcttcattcagccgccgcaccgtgcgcttacctcccttgccgtgcttgattagcaccggtgggttgctgaaacccaccatttgtagcgccacatcttctctttcttcctcgctgtccacgatcacctctggggatggcgggcgctcgggcttgggagaggggcgcttctttttctttttggacgcaatggccaaatccgccgtcgaggtcgatggccgcgggctgggtgtgcgcggcaccagcgcatcttgtgacgagtcttcttcgtcctcggactcgagacgccgcctcagccgcttttttgggggcgcgcggggaggcggcggcgacggcgacggggacgacacgtcctccatggttggtggacgtcgcgccgcaccgcgtccgcgctcgggggtggtttcgcgctgctcctcttcccgactggccatttccttctcctataggcagaaaaagatcatggagtcagtcgagaaggaggacagcctaaccgccccctttgagttcgccaccaccgcctccaccgatgccgccaacgcgcctaccaccttccccgtcgaggcacccccgcttgaggaggaggaagtgattatcgagcaggacccaggttttgtaagcgaagacgacgaggatcgctcagtaccaacagaggataaaaagcaagaccaggacgacgcagaggcaaacgaggaacaagtcgggcggggggaccaaaggcatggcgactacctagatgtgggagacgacgtgctgttgaagcatctgcagcgccagtgcgccattatctgcgacgcgttgcaagagcgcagcgatgtgcccctcgccatagcggatgtcagccttgcctacgaacgccacctgttctcaccgcgcgtaccccccaaacgccaagaaaacggcacatgcgagcccaacccgcgcctcaacttctaccccgtatttgccgtgccagaggtgcttgccacctatcacatctttttccaaaactgcaagatacccctatcctgccgtgccaaccgcagccgagcggacaagcagctggccttgcggcagggcgctgtcatacctgatatcgcctcgctcgacgaagtgccaaaaatctttgagggtcttggacgcgacgagaaacgcgcggcaaacgctctgcaacaagaaaacagcgaaaatgaaagtcactgtggagtgctggtggaacttgagggtgacaacgcgcgcctagccgtgctgaaacgcagcatcgaggtcacccactttgcctacccggcacttaacctaccccccaaggttatgagcacagtcatgagcgagctgatcgtgcgccgtgcacgacccctggagagggatgcaaacttgcaagaacaaaccgaggagggcctacccgcagttggcgatgagcagctggcgcgctggcttgagacgcgcgagcctgccgacttggaggagcgacgcaagctaatgatggccgcagtgcttgttaccgtggagcttgagtgcatgcagcggttctttgctgacccggagatgcagcgcaagctagaggaaacgttgcactacacctttcgccagggctacgtgcgccaggcctgcaaaatttccaacgtggagctctgcaacctggtctcctaccttggaattttgcacgaaaaccgcctcgggcaaaacgtgcttcattccacgctcaagggcgaggcgcgccgcgactacgtccgcgactgcgtttacttatttctgtgctacacctggcaaacggccatgggcgtgtggcagcaatgcctggaggagcgcaacctaaaggagctgcagaagctgctaaagcaaaacttgaaggacctatggacggccttcaacgagcgctccgtggccgcgcacctggcggacattatcttccccgaacgcctgcttaaaaccctgcaacagggtctgccagacttcaccagtcaaagcatgttgcaaaactttaggaactttatcctagagcgttcaggaattctgcccgccacctgctgtgcgcttcctagcgactttgtgcccattaagtaccgtgaatgccctccgccgctttggggtcactgctaccttctgcagctagccaactaccttgcctaccactccgacatcatggaagacgtgagcggtgacggcctactggagtgtcactgtcgctgcaacctatgcaccccgcaccgctccctggtctgcaattcgcaactgcttagcgaaagtcaaattatcggtacctttgagctgcagggtccctcgcctgacgaaaagtccgcggctccggggttgaaactcactccggggctgtggacgtcggcttaccttcgcaaatttgtacctgaggactaccacgcccacgagattaggttctacgaagaccaatcccgcccgccaaatgcggagcttaccgcctgcgtcattacccagggccacatccttggccaattgcaagccatcaacaaagcccgccaagagtttctgctacgaaagggacggggggtttacctggacccccagtccggcgaggagctcaacccaatccccccgccgccgcagccctatcagcagccgcgggcccttgcttcccaggatggcacccaaaaagaagctgcagctgccgccgccgccacccacggacgaggaggaatactgggacagtcaggcagaggaggttttggacgaggaggaggagatgatggaagactgggacagcctagacgaagcttccgaggccgaagaggtgtcagacgaaacaccgtcaccctcggtcgcattcccctcgccggcgccccagaaattggcaaccgttcccagcatcgctacaacctccgctcctcaggcgccgccggcactgcctgttcgccgacccaaccgtagatgggacaccactggaaccagggccggtaagtctaagcagccgccgccgttagcccaagagcaacaacagcgccaaggctaccgctcgtggcgcgggcacaagaacgccatagttgcttgcttgcaagactgtgggggcaacatctccttcgcccgccgctttcttctctaccatcacggcgtggccttcccccgtaacatcctgcattactaccgtcatctctacagcccctactgcaccggcggcagcggcagcggcagcaacagcagcggtcacacagaagcaaaggcgaccggatagcaagactctgacaaagcccaagaaatccacagcggcggcagcagcaggaggaggagcgctgcgtctggcgcccaacgaacccgtatcgacccgcgagcttagaaataggatttttcccactctgtatgctatatttcaacaaagcaggggccaagaacaagagctgaaaataaaaaacaggtctctgcgctccctcacccgcagctgcctgtatcacaaaagcgaagatcagcttcggcgcacgctggaagacgcggaggctctcttcagcaaatactgcgcgctgactcttaaggactagtttcgcgccctttctcaaatttaagcgcgaaaactacgtcatctccagcggccacacccggcgccagcacctgtcgtcagcgccattatgagcaaggaaattcccacgccctacatgtggagttaccagccacaaatgggacttgcggctggagctgcccaagactactcaacccgaataaactacatgagcgcgggaccccacatgatatcccgggtcaacggaatccgcgcccaccgaaaccgaattctcctcgaacaggcggctattaccaccacacctcgtaataaccttaatccccgtagttggcccgctgccctggtgtaccaggaaagtcccgctcccaccactgtggtacttcccagagacgcccaggccgaagttcagatgactaactcaggggcgcagcttgcgggcggctttcgtcacagggtgcggtcgcccgggcgttttagggcggagtaacttgcatgtattgggaattgtagtttttttaaaatgggaagtgacgtatcgtgggaaaacggaagtgaagatttgaggaagttgtgggttttttggctttcgtttctgggcgtaggttcgcgtgcggttttctgggtgttttttgtggactttaaccgttacgtcattttttagtcctatatatactcgctctgtacttggccctttttacactgtgactgattgagctggtgccgtgtcgagtggtgttttttaataggtttttttactggtaaggctgactgttatggctgccgctgtggaagcgctgtatgttgttctggagcgggagggtgctattttgcctaggcaggagggtttttcaggtgtttatgtgtttttctctcctattaattttgttatacctcctatgggggctgtaatgttgtctctacgcctgcgggtatgtattcccccgggctatttcggtcgctttttagcactgaccgatgttaaccaacctgatgtgtttaccgagtcttacattatgactccggacatgaccgaggaactgtcggtggtgctttttaatcacggtgaccagtttttttacggtcacgccggcatggccgtagtccgtcttatgcttataagggttgtttttcctgttgtaagacaggcttctaatgtttaaatgtttttttttttgttattttattttgtgtttaatgcaggaacccgcagacatgtttgagagaaaaatggtgtctttttctgtggtggttccggaacttacctgcctttatctgcatgagcatgactacgatgtgcttgcttttttgcgcgaggctttgcctgattttttgagcagcaccttgcattttatatcgccgcccatgcaacaagcttacataggggctacgctggttagcatagctccgagtatgcgtgtcataatcagtgtgggttcttttgtcatggttcctggcggggaagtggccgcgctggtccgtgcagacctgcacgattatgttcagctggccctgcgaagggacctacgggatcgcggtatttttgttaatgttccgcttttgaatcttatacaggtctgtgaggaacctgaatttttgcaatcatgattcgctgcttgaggctgaaggtggagggcgctctggagcagatttttacaatggccggacttaatattcgggatttgcttagagacatattgataaggtggcgagatgaaaattatttgggcatggttgaaggtgctggaatgtttatagaggagattcaccctgaagggtttagcctttacgtccacttggacgtgagggcagtttgccttttggaagccattgtgcaacatcttacaaatgccattatctgttctttggctgtagagtttgaccacgccaccggaggggagcgcgttcacttaatagatcttcattttgaggttttggataatcttttggaataaaaaaaaaaaaacatggttcttccagctcttcccgctcctcccgtgtgtgactcgcagaacgaatgtgtaggttggctgggtgtggcttattctgcggtggtggatgttatcagggcagcggcgcatgaaggagtttacatagaacccgaagccagggggcgcctggatgctttgagagagtggatatactacaactactacacagagcgagctaagcgacgagaccggagacgcagatctgtttgtcacgcccgcacctggttttgcttcaggaaatatgactacgtccggcgttccatttggcatgacactacgaccaacacgatctcggttgtctcggcgcactccgtacagtagggatcgcctacctccttttgagacagagacccgcgctaccatactggaggatcatccgctgctgcccgaatgtaacactttgacaatgcacaacgtgagttacgtgcgaggtcttccctgcagtgtgggatttacgctgattcaggaatgggttgttccctgggatatggttctgacgcgggaggagcttgtaatcctgaggaagtgtatgcacgtgtgcctgtgttgtgccaacattgatatcatgacgagcatgatgatccatggttacgagtcctgggctctccactgtcattgttccagtcccggttccctgcagtgcatagccggcgggcaggttttggccagctggtttaggatggtggtggatggcgccatgtttaatcagaggtttatatggtaccgggaggtggtgaattacaacatgccaaaagaggtaatgtttatgtccagcgtgtttatgaggggtcgccacttaatctacctgcgcttgtggtatgatggccacgtgggttctgtggtccccgccatgagctttggatacagcgccttgcactgtgggattttgaacaatattgtggtgctgtgctgcagttactgtgctgatttaagtgagatcagggtgcgctgctgtgcccggaggacaaggcgtctcatgctgcgggcggtgcgaatcatcgctgaggagaccactgccatgttgtattcctgcaggacggagcggcggcggcagcagtttattcgcgcgctgctgcagcaccaccgccctatcctgatgcacgattatgactctacccccatgtaggcgtggacttccccttcgccgcccgttgagcaaccgcaagttggacagcagcctgtggctcagcagctggacagcgacatgaacttaagcgagctgcccggggagtttattaatatcactgatgagcgtttggctcgacaggaaaccgtgtggaatataacacctaagaatatgtctgttacccatgatatgatgctttttaaggccagccggggagaaaggactgtgtactctgtgtgttgggagggaggtggcaggttgaatactagggttctgtgagtttgattaaggtacggtgatcaatataagctatgtggtggtggggctatactactgaatgaaaaatgacttgaaattttctgcaattgaaaaataaacacgttgaaacataacatgcaacaggttcacgattctttattcctgggcaatgtaggagaaggtgtaagagttggtagcaaaagtttcagtggtgtattttccactttcccaggaccatgtaaaagacatagagtaagtgcttacctcgctagtttctgtggattcactagaatcgatgtagcggccgctacgtcgacgtttaaaccatatgatcagctcactcaaaggcggtaatacggttatccacagaatcaggggataacgcaggaaagaacatgtgagcaaaaggccagcaaaaggccaggaaccgtaaaaaggccgcgttgctggcgtttttccataggctccgcccccctgacgagcatcacaaaaatcgacgctcaagtcagaggtggcgaaacccgacaggactataaagataccaggcgtttccccctggaagctccctcgtgcgctctcctgttccgaccctgccgcttaccggatacctgtccgcctttctcccttcgggaagcgtggcgctttctcatagctcacgctgtaggtatctcagttcggtgtaggtcgttcgctccaagctgggctgtgtgcacgaaccccccgttcagcccgaccgctgcgccttatccggtaactatcgtcttgagtccaacccggtaagacacgacttatcgccactggcagcagccactggtaacaggattagcagagcgaggtatgtaggcggtgctacagagttcttgaagtggtggcctaactacggctacactagaagaacagtatttggtatctgcgctctgctgaagccagttaccttcggaaaaagagttggtagctcttgatccggcaaacaaaccaccgctggtagcggtggtttttttgtttgcaagcagcagattacgcgcagaaaaaaaggatctcaagaagatcctttgatcttttctacggggtctgacgctcagtggaacgaaaactcacgttaagggattttggtcatgagattatcaaaaaggatcttcacctagatccttttaaattaaaaatgaagttttaaatcaatctaaagtatatatgagtaaacttggtctgacagttaccaatgcttaatcagtgaggcacctatctcagcgatctgtctatttcgttcatccatagttgcctgactccccgtcgtgtagataactacgatacgggagggcttaccatctggccccagtgctgcaatgataccgcgagacccacgctcaccggctccagatttatcagcaataaaccagccagccggaagggccgagcgcagaagtggtcctgcaactttatccgcctccatccagtctattaattgttgccgggaagctagagtaagtagttcgccagttaatagtttgcgcaacgttgttgccattgctacaggcatcgtggtgtcacgctcgtcgtttggtatggcttcattcagctccggttcccaacgatcaaggcgagttacatgatcccccatgttgtgcaaaaaagcggttagctccttcggtcctccgatcgttgtcagaagtaagttggccgcagtgttatcactcatggttatggcagcactgcataattctcttactgtcatgccatccgtaagatgcttttctgtgactggtgagtactcaaccaagtcattctgagaatagtgtatgcggcgaccgagttgctcttgcccggcgtcaatacgggataataccgcgccacatagcagaactttaaaagtgctcatcattggaaaacgttcttcggggcgaaaactctcaaggatcttaccgctgttgagatccagttcgatgtaacccactcgtgcacccaactgatcttcagcatcttttactttcaccagcgtttctgggtgagcaaaaacaggaaggcaaaatgccgcaaaaaagggaataagggcgacacggaaatgttgaatactcatactcttcctttttcaatattattgaagcatttatcagggttattgtctcatgagcggatacatatttgaatgtatttagaaaaataaacaaataggggttccgcgcacatttccccgaaaagtgccacctaaattgtaagcgttaatattttgttaaaattcgcgttaaatttttgttaaatcagctcattttttaaccaataggccgaaatcggcaaaatcccttataaatcaaaagaatagaccgagatagggttgagtgttgttccagtttggaacaagagtccactattaaagaacgtggactccaacgtcaaagggcgaaaaaccgtctatcagggcgatggcccactacgtgaaccatcaccctaatcaagttttttggggtcgaggtgccgtaaagcactaaatcggaaccctaaagggagcccccgatttagagcttgacggggaaagccggcgaacgtggcgagaaaggaagggaagaaagcgaaaggagcgggcgctagggcgctggcaagtgtagcggtcacgctgcgcgtaaccaccacacccgccgcgcttaatgcgccgctacagggcgcgatggatcc

SEQ ID NO: 7 - DNA, 10975 bp, synthetic construct
  misc_feature 1..10975: note = plasmid
  source 1..10975: mol_type = other DNA
tcgcgcgtttcggtgatgacggtgaaaacctctgacacatgcagctcccggagactgtcacagcttgtctgtaagcggatgccgggagcagacaagcccgtcagggcgcgtcagcgggtgttggcgggtgtcggggctggcttaactatgcggcatcagagcagattgtactgagagtgcaccatatgcggtgtgaaataccgcacagatgcgtaaggagaaaataccgcatcaggcgccattcgccattcaggctgcgcaactgttgggaagggcgatcggtgcgggcctcttcgctattacgccagctggcgaaagggggatgtgctgcaaggcgattaagttgggtaacgccagggttttcccagtcacgacgttgtaaaacgacggccagtgaattgacgcgtattgacattgattattgactagttattaatagtaatcaattacggggtcattagttcatagcccatatatggagttccgcgttacataacttacggtaaatggcccgcctggctgaccgcccaacgacccccgcccattgacgtcaataatgacgtatgttcccatagtaacgccaatagggactttccattgacgtcaatgggtggagtatttacggtaaactgcccacttggcagtacatcaagtgtatcatatgccaagtacgccccctattgacgtcaatgacggtaaatggcccgcctggcattatgcccagtacatgaccttatgggactttcctacttggcagtacatctacgtattagtcatcgctattaccatggtgatgcggttttggcagtacatcaatgggcgtggatagcggtttgactcacggggatttccaagtctccaccccattgacgtcaatgggagtttgttttggcaccaaaatcaacgggactttccaaaatgtcgtaacaactccgccccattgacgcaaatgggcggtaggcgtgtacggtgggaggtctatataagcagagctggtttagtgaaccgtcagatcagatctttgtcgatcctaccatccactcgacacacccgccagcggccgatgtcttttgttgatcaccctccagattggttggaagaagttggtgaaggtcttcgcgagtttttgggccttgaagcgggcccaccgaaaccaaaacccaatcagcagcatcaagatcaagcccgtggtcttgtgctgcctggttataactatctcggacccggaaacggtctcgatcgaggagagcctgtcaacagggcagacgaggtcgcgcgagagcacgacatctcgtacaacgagcagcttgaggcgggagacaacccctacctcaagtacaaccacgcggacgccgagtttcaggagaagctcgccgacgacacatccttcgggggaaacctcggaaaggcagtctttcaggccaagaaaagggttctcgaaccttttggcctggttgaagagggtgctaagacggcccctaccggaaagcggatagacgaccactttccaaaaagaaagaaggctcggaccgaagaggactccaagccttccacctcgtcagacgccgaagctggacccagcggatcccagcagctgcaaatcccagcccaaccagcctcaagtttgggagctgatacaatgtctgcgggaggtggcggcccattgggcgacaataaccaaggtgccgatggagtgggcaatgcctcgggagattggcattgcgattccacgtggatgggggacagagtcgtcaccaagtccacccgaacctgggtgctgcccagctacaacaaccaccagtaccgagagatcaaaagcggctccgtcgacggaagcaacgccaacgcctactttggatacagcaccccctgggggtactttgactttaaccgcttccacagccactggagcccccgagactggcaaagactcatcaacaactactggggcttcagaccccggtccctcagagtcaaaatcttcaacattcaagtcaaagaggtcacggtgcaggactccaccaccaccatcgccaacaacctcacctccaccgtccaagtgtttacggacgacgactaccagctgccctacgtcgtcggcaacgggaccgagggatgcctgccggccttccctccgcaggtctttacgctgccgcagtacggttacgcgacgctgaaccgcgacaacacagaaaatcccaccgagaggagcagcttcttctgcctagagtactttcccagcaagatgctgagaacgggcaacaactttgagtttacctacaactttgaggaggtgcccttccactccagcttcgctcccagtcagaacctgttcaagctggccaacccgctggtggaccagtacttgtaccgcttcgtgagcacaaataacactggcggagtccagttcaacaagaacctggccgggagatacgccaacacctacaaaaactggttcccggggcccatgggccgaacccagggctggaacctgggctccggggtcaaccgcgccagtgtcagcgccttcgccacgaccaataggatggagctcgagggcgcgagttaccaggtgcccccgcagccgaacggcatgaccaacaacctccagggcagcaacacctatgccctggagaacactatgatcttcaacagccagccggcgaacccgggcaccaccgccacgtacctcgagggcaacatgctcatcaccagcgagagcgagacgcagccggtgaaccgcgtggcgtacaacgtcggcgggcagatggccaccaacaaccagagctccaccactgcccccgcgaccggcacgtacaacctccaggaaatcgtgcccggcagcgtgtggatggagagggacgtgtacctccaaggacccatctgggccaagatcccagagacgggggcgcactttcacccctctccggccatgggcggattcggactcaaacacccaccgcccatgatgctcatcaagaacacgcctgtgcccggaaatatcaccagcttctcggacgtgcccgtcagcagcttcatcacccagtacagcaccgggcaggtcaccgtggagatggagtgggagctcaagaaggaaaactccaagaggtggaacccagagatccagtacacaaacaactacaacgacccccagtttgtggactttgccccggacagcaccggggaatacagaaccaccagacctatcggaacccgataccttacccgacccctttaacccgggagttctagggatctggcggccgctcgagtctagagggcccgtttaaacccgctgatcagcctcgactgtgccttctagttgccagccatctgttgtttgcccctcccccgtgccttccttgaccctggaaggtgccactcccactgtcctttcctaataaaatgaggaaattgcatcgcattgtctgagtaggtgtcattctattctggggggtggggtggggcaggacagcaagggggaggattgggaagacaatagcaggcatgctggggatgcggtgggctctatggtgaattccactttggccgcggctcgagggggacagcccccccccaaagcccccagggatgtaattacgtccctcccccgctagggggcagcagcgagccgcccggggctccgctccggtccggcgctccccccgcatccccgagccggcagcgtgcggggacagcccgggcacggggaaggtggcacgggatcgctttcctctgaacgcttctcgctgctctttgagcctgcagacacctggggggatacggggaaaaagctttaggctgagtgcacggggacagcccccccccaaagcccccagggatgtaattacgtccctcccccgctagggggcagcagcgagccgcccggggctccgctccggtccggcgctccccccgcatccccgagccggcagcgtgcggggacagcccgggcacggggaaggtggcacgggatcgctttcctctgaacgcttctcgctgctctttgagcctgcagacacctggggggatacggggaaaaagctttaggctgaaacttgtttattgcagcttataatggttacaaataaagcaatagcatcacaaatttcacaaataaagcatttttttcactgcattctagttgtggtttgtccaaactcatcaatgtatcttatcatgtctggatccccgcggccgcggtacccacgtgggcgcgccatttaaatgataactcagagagagtgtcctcgagccaatctggaagataaccatcggcagccatacctgatttaaatcatttattgttcaaagatgcagtcatccaaatccacattgaccagatcgcaggcagtgcaagcgtctggcacctttcccatgatatgatgaatgtagcacagtttctgatacgcctttttgacgacagaaacgggttgagattctgacacgggaaagcactctaaacagtctttctgtccgtgagtgaagcagatatttgaattctgattcattctctcgcattgtctgcagggaaacagcatcagattcatgcccacgtgacgagaacatttgttttggtacctgtctgcgtagttgatcgaagcttccgcgtctgacgtcgatggctgcgcaactgactcgcgcacccgtttgggctcacttatatctgcgtcactgggggcgggtcttttcttggctccaccctttttgacgtagaattcatgctccacctcaaccacgtgatcctttgcccaccggaaaaagtctttgacttcctgcttggtgaccttcccaaagtcatgatccagacggcgggtgagttcaaatttgaacatccggtcttgcaacggctgctggtgttcgaaggtcgttgagttcccgtcaatcacggcgcacatgttggtgttggaggtgacgatcacgggagtcgggtctatctgggccgaggacttgcatttctggtccacgcgcaccttgcttcctccgagaatggctttggccgactccacgaccttggcggtcatcttcccctcctcccaccagatcaccatcttgtcgacacagtcgttgaagggaaagttctcattggtccagtttacgcacccgtagaagggcacagtgtgggctatggcctccgcgatgttggtcttcccggtagttgcaggcccaaacagccagatggtgttcctcttgccgaactttttcgtggcccatcccagaaagacggaagccgcatattggggatcgtacccgtttagttccaaaattttataaatccgattgctggaaatgtcctccacgggctgctggcccaccaggtagtcgggggcggttttagtcaggctcataatctttcccgcattgtccaaggcagccttgatttgggaccgcgagttggaggccgcattgaaggagatgtatgaggcctggtcctcctggatccactgcttctccgaggtaatccccttgtccacgagccacccgaccagctccatgtacctggctgaagtttttgatctgatcaccggcgcatcagaattgggattctgattctctttgttctgctcctgcgtctgcgacacgtgcgtcagatgctgcgccaccaaccgtttacgctccgtgagattcaaacaggcgcttaaatactgttccatattagtccacgcccactggagctcaggctgggttttggggagcaagtaattggggatgtagcactcatccaccaccttgttcccgcctccggcgccatttctggtctttgtgaccgcgaaccagtttggcaaagtcggctcgatcccgcggtaaattctctgaatcagtttttcgcgaatctgactcaggaaacgtcccaaaaccatggatttcaccccggtggtttccacgagcacgtgcatgtggaagtagctctctcccttctcaaattgcacaaagaaaagggcctccggggccttactcacacggcgccattccgtcagaaagtcgcgctgcagcttctcggccacggtcaggggtgcctgctcaatcagattcagatccatgtcagaatctggcggcaactcccattccttctcggccacccagttcacaaagctgtcagaaatgccgggcagatgctcgtcaaggtcgctggggaccttaatcacaatctcgtaaaaccccggcatggcggcgataactattatcatcgtgtttttcaaaggaaaaccacgtccccgtggttcggggggcctagacgtttttttaacctcgactaaacacatgtaaagcatgtgcaccgaggccccagatcagatcccatacaatggggtaccttctgggcatccttcagccccttgttgaatacgcttgaggagagccatttgactctttccacaactatccaactcacaacgtggcactggggttgtgccgcctttgcaggtgtatcttatacacgtggcttttggccgcagaggcacctgtcgccaggtggggggttccgctgcctgcaaagggtcgctacagacgttgtttgtcttcaagaagcttccagaggaactgcttccttcacgacattcaacagaccttgcattcctttggcgagaggggaaagacccctaggaatgctcgtcaagaagacagggccaggtttccgggccctcacattgccaaaagacggcaatatggtggaaaataacatatagacaaacgcacaccggccttattccaagcggcttcggccagtaacgttagggggggggggcggaattctatccctcagttatctcagagagagtgtcctcgagccaatctggaagataaccatcggcagccatacctgatttaaatcatttattgttcaaagatgcagtcatccaaatccacattgaccagatcgcaggcagtgcaagcgtctggcacctttcccatgatatgatgaatgtagcacagtttctgatacgcctttttgacgacagaaacgggttgagattctgacacgggaaagcactctaaacagtctttctgtccgtgagtgaagcagatatttgaattctgattcattctctcgcattgtctgcagggaaacagcatcagattcatgcccacgtgacgagaacatttgttttggtacctgtctgcgtagttgatcgaagcttccgcgtctgacgtcgatggctgcgcaactgactcgcgcacccgtttgggctcacttatatctgcgtcactgggggcgggtcttttcttggctccaccctttttgacgtagaattcatgctccacctcaaccacgtgatcctttgcccaccggaaaaagtctttgacttcctgcttggtgaccttcccaaagtcatgatccagacggcgggtgagttcaaatttgaacatccggtcttgcaacggctgctggtgttcgaaggtcgttgagttcccgtcaatcacggcgcacatgttggtgttggaggtgacgatcacgggagtcgggtctatctgggccgaggacttgcatttctggtccacgcgcaccttgcttcctccgagaatggctttggccgactccacgaccttggcggtcatcttcccctcctcccaccagatcaccatcttgtcgacacagtcgttgaagggaaagttctcattggtccagtttacgcacccgtagaagggcacagtgtgggctatggcctccgcgatgttggtcttcccggtagttgcaggcccaaacagccagatggtgttcctcttgccgaactttttcgtggcccatcccagaaagacggaagccgcatattggggatcgtacccgtttagttccaaaattttataaatccgattgctggaaatgtcctccacgggctgctggcccaccaggtagtcgggggcggttttagtcaggctcataatctttcccgcattgtccaaggcagccttgatttgggaccgcgagttggaggccgcattgaaggagatgtatgaggcctggtcctcctggatccactgcttctccgaggtaatccccttgtccacgagccacccgaccagctccatggtggcgttatccggccgatcgatagatctgggccccggtgtcgactttacgagggtaggaagtggtacggaaagttggtataagacaaaagtgttgtggaattgctggaggcgatctgacggttcactaaacgagctctgcttttataggcgcccaccgtacacgcctaaagcttatacgtagctctgcttatatagacctcccaccgtacacgcctaccgcccatttgcgtcaatggggcggagttgttacgacattttggaaagtcccgttgattttggtgccaaaacaaactcccattgacgtcaatggggtggagacttggaaatccccgtgagtcaaaccgctatccacgcccattgatgtactgccaaaaccgcatcaccatggtaatagcgatgactaatacgtagatgtactgccaagtaggaaagtcccataaggtcatgtactgggcataatgccaggcgggccatttaccgtcattgacgtcaatagggggcgtacttggcatatgatacacttgatgtactgccaagtgggcagtttaccgtaaatactccacccattgacgtcaatggaaagtccctattggcgttactatgggaacatacgtcattattgacgtcaatgggcgggggtcgttgggcggtcagccaggcgggccatttaccgtaagttatgtaacgcggaactccatatatgggctatgaactaatgaccccgtaattgattactattaataactagtcaataatcaatgtcttccacacaacatacgagccggaagcataaagtgtaaagcctggggtgcctaatgagtgagctaactcacattaattgcgttgcgctcactgcccgctttccagtcgggaaacctgtcgtgccagctgcattaatgaatcggccaacgcgcggggagaggcggtttgcgtattgggcgctgttccgcttcctcgctcactgactcgctgcgctcggtcgttcggctgcggcgagcggtatcagctcactcaaaggcggtaatacggttatccacagaatcaggggataacgcaggaaagaacatgtgagcaaaaggccagcaaaaggccaggaaccgtaaaaaggccgcgttgctggcgtttttccataggctccgcccccctgacgagcatcacaaaaatcgacgctcaagtcagaggtggcgaaacccgacaggactataaagataccaggcgtttccccctggaagctccctcgtgcgctctcctgttccgaccctgccgcttaccggatacctgtccgcctttctcccttcgggaagcgtggcgctttctcatagctcacgctgtaggtatctcagttcggtgtaggtcgttcgctccaagctgggctgtgtgcacgaaccccccgttcagcccgaccgctgcgccttatccggtaactatcgtcttgagtccaacccggtaagacacgacttatcgccactggcagcagccactggtaacaggattagcagagcgaggtatgtaggcggtgctacagagttcttgaagtggtggcctaactacggctacactagaagaacagtatttggtatctgcgctctgctgaagccagttaccttcggaaaaagagttggtagctcttgatccggcaaacaaaccaccgctggtagcggtggtttttttgtttgcaagcagcagattacgcgcagaaaaaaaggatctcaagaagatcctttgatcttttctacggggtctgacgctcagtggaacgaaaactcacgttaagggattttggtcatgagattatcaaaaaggatcttcacctagatccttttaaattaaaaatgaagttttaaatcaatctaaagtatatatgagtaaacttggtctgacagttaccaatgcttaatcagtgaggcacctatctcagcgatctgtctatttcgttcatccatagttgcctgactccccgtcgtgtagataactacgatacgggagggcttaccatctggccccagtgctgcaatgataccgcgagaaccacgctcaccggctccagatttatcagcaataaaccagccagccggaagggccgagcgcagaagtggtcctgcaactttatccgcctccatccagtctattaattgttgccgggaagctagagtaagtagttcgccagttaatagtttgcgcaacgttgttgccattgctacaggcatcgtggtgtcacgctcgtcgtttggtatggcttcattcagctccggttcccaacgatcaaggcgagttacatgatcccccatgttgtgcaaaaaagcggttagctccttcggtcctccgatcgttgtcagaagtaagttggccgcagtgttatcactcatggttatggcagcactgcataattctcttactgtcatgccatccgtaagatgcttttctgtgactggtgagtactcaaccaagtcattctgagaatagtgtatgcggcgaccgagttgctcttgcccggcgtcaatacgggataataccgcgccacatagcagaactttaaaagtgctcatcattggaaaacgttcttcggggcgaaaactctcaaggatcttaccgctgttgagatccagttcgatgtaacccactcgtgcacccaactgatcttcagcatcttttactttcaccagcgtttctgggtgagcaaaaacaggaaggcaaaatgccgcaaaaaagggaataagggcgacacggaaatgttgaatactcatactcttcctttttcaatattattgaagcatttatcagggttattgtctcatgagcggatacatatttgaatgtatttagaaaaataaacaaataggggttccgcgcacatttccccgaaaagtgccacctgacgtctaagaaaccattattatcatgacattaacctataaaaataggcgtatcacgaggcccttttgtc

SEQ ID NO: 8 - DNA, 5144 bp, synthetic construct
  misc_feature 1..5144: note = plasmid
  source 1..5144: mol_type = other DNA
tcgcgcgtttcggtgatgacggtgaaaacctctgacacatgcagctcccggagactgtcacagcttgtctgtaagcggatgccgggagcagacaagcccgtcagggcgcgtcagcgggtgttggcgggtgtcggggctggcttaactatgcggcatcagagcagattgtactgagagtgcaccatatgcggtgtgaaataccgcacagatgcgtaaggagaaaataccgcatcaggcgccattcgccattcaggctgcgcaactgttgggaagggcgatcggtgcgggcctcttcgctattacgccagctggcgaaagggggatgtgctgcaaggcgattaagttgggtaacgccagggttttcccagtcacgacgttgtaaaacgacggccagtgaattgacgcgtattgggatactagtcccgggccgcggcgttacataacttacggtaaatggcccgcctggctgaccgcccaacgacccccgcccattgacgtcaataatgacgtatgttcccatagtaacgccaatagggactttccattgacgtcaatgggtggagtatttacggtaaactgcccacttggcagtacatcaagtgtatcatatgccaagtacgccccctattgacgtcaatgacggtaaatggcccgcctggcattatgcccagtacatgaccttatgggactttcctacttggcagtacatctacgtattagtcatcgctattaccatggtgatgcggttttggcagtacatcaatgggcgtggatagcggtttgactcacggggatttccaagtctccaccccattgacgtcaatgggagtttgttttggcaccaaaatcaacgggactttccaaaatgtcgtaacaactccgccccattgacgcaaatgggcggtaggcgtgtacggtgggaggtctatataagcagagctggtttagtgaaccgtcagatccgctagcgctaccggactcagatctcgagctcaagcttcgaattctgcagtcgacggtaccgccacccgccaccatggccagtcgggaagaggagcagcgcgaaaccacccccgagcgcggacgcggtgcggcgcgacgtcccccaaccatggaggacgtgtcgtccccgtccccgtcgccgccgcctccccgggcgcccccaaaaaagcggatgaggcggcgtatcgagtccgaggacgaggaagactcatcacaagacgcgctggtgccgcgcacacccagcccgcggccatcgacctcggcggcggatttggccattgcgcccaagaagaaaaagaagcgcccttctcccaagcccgagcgcccgccatcaccagaggtaatcgtggacagcgaggaagaaagagaagatgtggcgctacaaatggtgggtttcagcaacccaccggtgctaatcaagcatggcaaaggaggtaagcgcacagtgcggcggctgaatgaagacgacccagtggcgcgtggtatgcggacgcaagaggaagaggaagagcccagcgaagcggaaagtgaaattacggtgatgaacccgctgagtgtgccgatcgtgtctgcgtgggagaagggcatggaggctgcgcgcgcgctgatggacaagtaccacgtggataacgatctaaaggcgaacttcaaactactgcctgaccaagtggaagctctggcggccgtatgcaagacctggctgaacgaggagcaccgcgggttgcagctgaccttcaccagcaacaagacctttgtgacgatgatggggcgattcctgcaggcgtacctgcagtcgtttgcagaggtgacctacaagcatcacgagcccacgggctgcgcgttgtggctgcaccgctgcgctgagatcgaaggcgagcttaagtgtctacacggaagcattatgataaataaggagcacgtgattgaaatggatgtgacgagcgaaaacgggcagcgcgcgctgaaggagcagtctagcaaggccaagatcgtgaagaaccggtggggccgaaatgtggtgcagatctccaacaccgacgcaaggtgctgcgtgcacgacgcggcctgtccggccaatcagttttccggcaagtcttgcggcatgttcttctctgaaggcgcaaaggctcaggtggcttttaagcagatcaaggcttttatgcaggcgctgtatcctaacgcccagaccgggcacggtcaccttttgatgccactacggtgcgagtgcaactcaaagcctgggcacgcgccctttttgggaaggcagctaccaaagttgactccgttcgccctgagcaacgcggaggacctggacgcggatctgatctccgacaagagcgtgctggccagcgtgcaccacccggcgctgatagtgttccagtgctgcaaccctgtgtatcgcaactcgcgcgcgcagggcggaggccccaactgcgacttcaagatatcggcgcccgacctgctaaacgcgttggtgatggtgcgcagcctgtggagtgaaaacttcaccgagctgccgcggatggttgtgcctgagtttaagtggagcactaaacaccagtatcgcaacgtgtccctgccagtggcgcatagcgatgcgcggcagaacccctttgattttttcgaatttaaatcggatccctgtgccttctagttgccagccatctgttgtttgcccctcccccgtgccttccttgaccctggaaggtgccactcccactgtcctttcctaataaaatgaggaaattgcatcgcattgtctgagtaggtgtcattctattctggggggtggggtggggcaggacagcaagggggaggattgggaagacaatagcaggcatgctggggatgcggtgggctctatggggcgcgcctctagaatcgatatcccaatggcgcgccgagcttggcgtaatcatggtcatagctgtttcctgtgtgaaattgttatccgctcacaattccacacaacatacgagccggaagcataaagtgtaaagcctggggtgcctaatgagtgagctaactcacattaattgcgttgcgctcactgcccgctttccagtcgggaaacctgtcgtgccagctgcattaatgaatcggccaacgcgcggggagaggcggtttgcgtattgggcgctgttccgcttcctcgctcactgactcgctgcgctcggtcgttcggctgcggcgagcggtatcagctcactcaaaggcggtaatacggttatccacagaatcaggggataacgcaggaaagaacatgtgagcaaaaggccagcaaaaggccaggaaccgtaaaaaggccgcgttgctggcgtttttccataggctccgcccccctgacgagcatcacaaaaatcgacgctcaagtcagaggtggcgaaacccgacaggactataaagataccaggcgtttccccctggaagctccctcgtgcgctctcctgttccgaccctgccgcttaccggatacctgtccgcctttctcccttcgggaagcgtggcgctttctcatagctcacgctgtaggtatctcagttcggtgtaggtcgttcgctccaagctgggctgtgtgcacgaaccccccgttcagcccgaccgctgcgccttatccggtaactatcgtcttgagtccaacccggtaagacacgacttatcgccactggcagcagccactggtaacaggattagcagagcgaggtatgtaggcggtgctacagagttcttgaagtggtggcctaactacggctacactagaagaacagtatttggtatctgcgctctgctgaagccagttaccttcggaaaaagagttggtagctcttgatccggcaaacaaaccaccgctggtagcggtggtttttttgtttgcaagcagcagattacgcgcagaaaaaaaggatctcaagaagatcctttgatcttttctacggggtctgacgctcagtggaacgaaaactcacgttaagggattttggtcatgagattatcaaaaaggatcttcacctagatccttttaaattaaaaatgaagttttaaatcaatctaaagtatatatgagtaaacttggtctgacagttaccaatgcttaatcagtgaggcacctatctcagcgatctgtctatttcgttcatccatagttgcctgactccccgtcgtgtagataactacgatacgggagggcttaccatctggccccagtgctgcaatgataccgcgagaaccacgctcaccggctccagatttatcagcaataaaccagccagccggaagggccgagcgcagaagtggtcctgcaactttatccgcctccatccagtctattaattgttgccgggaagctagagtaagtagttcgccagttaatagtttgcgcaacgttgttgccattgctacaggcatcgtggtgtcacgctcgtcgtttggtatggcttcattcagctccggttcccaacgatcaaggcgagttacatgatcccccatgttgtgcaaaaaagcggttagctccttcggtcctccgatcgttgtcagaagtaagttggccgcagtgttatcactcatggttatggcagcactgcataattctcttactgtcatgccatccgtaagatgcttttctgtgactggtgagtactcaaccaagtcattctgagaatagtgtatgcggcgaccgagttgctcttgcccggcgtcaatacgggataataccgcgccacatagcagaactttaaaagtgctcatcattggaaaacgttcttcggggcgaaaactctcaaggatcttaccgctgttgagatccagttcgatgtaacccactcgtgcacccaactgatcttcagcatcttttactttcaccagcgtttctgggtgagcaaaaacaggaaggcaaaatgccgcaaaaaagggaataagggcgacacggaaatgttgaatactcatactcttcctttttcaatattattgaagcatttatcagggttattgtctcatgagcggatacatatttgaatgtatttagaaaaataaacaaataggggttccgcgcacatttccccgaaaagtgccacctgacgtctaagaaaccattattatcatgacattaacctataaaaataggcgtatcacgaggcccttttgtc

SEQ ID NO: 9 - DNA, 12673 bp, synthetic construct
  misc_feature 1..12673: note = plasmid
  source 1..12673: mol_type = other DNA
tcgcgcgtttcggtgatgacggtgaaaacctctgacacatgcagctcccggagactgtcacagcttgtctgtaagcggatgccgggagcagacaagcccgtcagggcgcgtcagcgggtgttggcgggtgtcggggctggcttaactatgcggcatcagagcagattgtactgagagtgcaccatatgcggtgtgaaataccgcacagatgcgtaaggagaaaataccgcatcaggcgccattcgccattcaggctgcgcaactgttgggaagggcgatcggtgcgggcctcttcgctattacgccagctggcgaaagggggatgtgctgcaaggcgattaagttgggtaacgccagggttttcccagtcacgacgttgtaaaacgacggccagtgaattgacgcgtattgggattttactccctatcagtgatagagaacgtatgaagagtttactccctatcagtgatagagaacgtatgcagactttactccctatcagtgatagagaacgtataaggagtttactccctatcagtgatagagaacgtatgaccagtttactccctatcagtgatagagaacgtatctacagtttactccctatcagtgatagagaacgtatatccagtttactccctatcagtgatagagaacgtatgtcgaggtaggcgtgtacggtgggcgcctataaaagcagagctcgtttagtgaaccgtcagatcgcctggagcaattccacaacacttttgtcttatacttggtttagtgaaccgtcagatcagatctttgtcgatcctaccatccactcgacacacccgccagcggccgatgtcttttgttgatcaccctccagattggttggaagaagttggtgaaggtcttcgcgagtttttgggccttgaagcgggcccaccgaaaccaaaacccaatcagcagcatcaagatcaagcccgtggtcttgtgctgcctggttataactatctcggacccggaaacggtctcgatcgaggagagcctgtcaacagggcagacgaggtcgcgcgagagcacgacatctcgtacaacgagcagcttgaggcgggagacaacccctacctcaagtacaaccacgcggacgccgagtttcaggagaagctcgccgacgacacatccttcgggggaaacctcggaaaggcagtctttcaggccaagaaaagggttctcgaaccttttggcctggttgaagagggtgctaagacggcccctaccggaaagcggatagacgaccactttccaaaaagaaagaaggctcggaccgaagaggactccaagccttccacctcgtcagacgccgaagctggacccagcggatcccagcagctgcaaatcccagcccaaccagcctcaagtttgggagctgatacaatgtctgcgggaggtggcggcccattgggcgacaataaccaaggtgccgatggagtgggcaatgcctcgggagattggcattgcgattccacgtggatgggggacagagtcgtcaccaagtccacccgaacctgggtgctgcccagctacaacaaccaccagtaccgagagatcaaaagcggctccgtcgacggaagcaacgccaacgcctactttggatacagcaccccctgggggtactttgactttaaccgcttccacagccactggagcccccgagactggcaaagactcatcaacaactactggggcttcagaccccggtccctcagagtcaaaatcttcaacattcaagtcaaagaggtcacggtgcaggactccaccaccaccatcgccaacaacctcacctccaccgtccaagtgtttacggacgacgactaccagctgccctacgtcgtcggcaacgggaccgagggatgcctgccggccttccctccgcaggtctttacgctgccgcagtacggttacgcgacgctgaaccgcgacaacacagaaaatcccaccgagaggagcagcttcttctgcctagagtactttcccagcaagatgctgagaacgggcaacaactttgagtttacctacaactttgaggaggtgcccttccactccagcttcgctcccagtcagaacctgttcaagctggccaacccgctggtggaccagtacttgtaccgcttcgtgagcacaaataacactggcggagtccagttcaacaagaacctggccgggagatacgccaacacctacaaaaactggttcccggggcccatgggccgaacccagggctggaacctgggctccggggtcaaccgcgccagtgtcagcgccttcgccacgaccaataggatggagctcgagggcgcgagttaccaggtgcccccgcagccgaacggcatgaccaacaacctccagggcagcaacacctatgccctggagaacactatgatcttcaacagccagccggcgaacccgggcaccaccgccacgtacctcgagggcaacatgctcatcaccagcgagagcgagacgcagccggtgaaccgcgtggcgtacaacgtcggcgggcagatggccaccaacaaccagagctccaccactgcccccgcgaccggcacgtacaacctccaggaaatcgtgcccggcagcgtgtggatggagagggacgtgtacctccaaggacccatctgggccaagatcccagagacgggggcgcactttcacccctctccggccatgggcggattcggactcaaacacccaccgcccatgatgctcatcaagaacacgcctgtgcccggaaatatcaccagcttctcggacgtgcccgtcagcagcttcatcacccagtacagcaccgggcaggtcaccgtggagatggagtgggagctcaagaaggaaaactccaagaggtggaacccagagatccagtacacaaacaactacaacgacccccagtttgtggactttgccccggacagcaccggggaatacagaaccaccagacctatcggaacccgataccttacccgacccctttaacccgggagttctagggatctgcccctctccctcccccccccctaacgttactggccgaagccgcttggaataaggccggtgtgcgtttgtctatatgttattttccaccatattgccgtcttttggcaatgtgagggcccggaaacctggccctgtcttcttgacgagcattcctaggggtctttcccctctcgccaaaggaatgcaaggtctgttgaatgtcgtgaaggaagcagttcctctggaagcttcttgaagacaaacaacgtctgtagcgaccctttgcaggcagcggaaccccccacctggcgacaggtgcctctgcggccaaaagccacgtgtataagatacacctgcaaaggcggcacaaccccagtgccacgttgtgagttggatagttgtggaaagagtcaaatggctctcctcaagcgtattcaacaaggggctgaaggatgcccagaaggtaccccattgtatgggatctgatctggggcctcggtgcacatgctttacatgtgtttagtcgaggttaaaaaaacgtctaggccccccgaaccacggggacgtggttttcctttgaaaaacacgatgataaggatccaccggaggccaccatggccagtcgggaagaggagcagcgcgaaaccacccccgagcgcggacgcggtgcggcgcgacgtcccccaaccatggaggacgtgtcgtccccgtccccgtcgccgccgcctccccgggcgcccccaaaaaagcggatgaggcggcgtatcgagtccgaggacgaggaagactcatcacaagacgcgctggtgccgcgcacacccagcccgcggccatcgacctcggcggcggatttggccattgcgcccaagaagaaaaagaagcgcccttctcccaagcccgagcgcccgccatcaccagaggtaatcgtggacagcgaggaagaaagagaagatgtggcgctacaaatggtgggtttcagcaacccaccggtgctaatcaagcatggcaaaggaggtaagcgcacagtgcggcggctgaatgaagacgacccagtggcgcgtggtatgcggacgcaagaggaagaggaagagcccagcgaagcggaaagtgaaattacggtgatgaacccgctgagtgtgccgatcgtgtctgcgtgggagaagggcatggaggctgcgcgcgcgctgatggacaagtaccacgtggataacgatctaaaggcgaacttcaaactactgcctgaccaagtggaagctctggcggccgtatgcaagacctggctgaacgaggagcaccgcgggttgcagctgaccttcaccagcaacaagacctttgtgacgatgatggggcgattcctgcaggcgtacctgcagtcgtttgcagaggtgacctacaagcatcacgagcccacgggctgcgcgttgtggctgcaccgctgcgctgagatcgaaggcgagcttaagtgtctacacggaagcattatgataaataaggagcacgtgattgaaatggatgtgacgagcgaaaacgggcagcgcgcgctgaaggagcagtctagcaaggccaagatcgtgaagaaccggtggggccgaaatgtggtgcagatctccaacaccgacgcaaggtgctgcgtgcacgacgcggcctgtccggccaatcagttttccggcaagtcttgcggcatgttcttctctgaaggcgcaaaggctcaggtggcttttaagcagatcaaggcttttatgcaggcgctgtatcctaacgcccagaccgggcacggtcaccttttgatgccactacggtgcgagtgcaactcaaagcctgggcacgcgccctttttgggaaggcagctaccaaagttgactccgttcgccctgagcaacgcggaggacctggacgcggatctgatctccgacaagagcgtgctggccagcgtgcaccacccggcgctgatagtgttccagtgctgcaaccctgtgtatcgcaactcgcgcgcgcagggcggaggccccaactgcgacttcaagatatcggcgcccgacctgctaaacgcgttggtgatggtgcgcagcctgtggagtgaaaacttcaccgagctgccgcggatggttgtgcctgagtttaagtggagcactaaacaccagtatcgcaacgtgtccctgccagtggcgcatagcgatgcgcggcagaacccctttgatttttaacccgggagttctagggatctggcggccgctcgagtctagagggcccgtttaaacccgctgatcagcctcgactgtgccttctagttgccagccatctgttgtttgcccctcccccgtgccttccttgaccctggaaggtgccactcccactgtcctttcctaataaaatgaggaaattgcatcgcattgtctgagtaggtgtcattctattctggggggtggggtggggcaggacagcaagggggaggattgggaagacaatagcaggcatgctggggatgcggtgggctctatggtgaattccactttggccgcggctcgagggggacagcccccccccaaagcccccagggatgtaattacgtccctcccccgctagggggcagcagcgagccgcccggggctccgctccggtccggcgctccccccgcatccccgagccggcagcgtgcggggacagcccgggcacggggaaggtggcacgggatcgctttcctctgaacgcttctcgctgctctttgagcctgcagacacctggggggatacggggaaaaagctttaggctgagtgcacggggacagcccccccccaaagcccccagggatgtaattacgtccctcccccgctagggggcagcagcgagccgcccggggctccgctccggtccggcgctccccccgcatccccgagccggcagcgtgcggggacagcccgggcacggggaaggtggcacgggatcgctttcctctgaacgcttctcgctgctctttgagcctgcagacacctggggggatacggggaaaaagctttaggctgaaacttgtttattgcagcttataatggttacaaataaagcaatagcatcacaaatttcacaaataaagcatttttttcactgcattctagttgtggtttgtccaaactcatcaatgtatcttatcatgtctggatccccgcggccgcggtacccacgtgggcgcgccatttaaatgataactcagagagagtgtcctcgagccaatctggaagataaccatcggcagccatacctgatttaaatcatttattgttcaaagatgcagtcatccaaatccacattgaccagatcgcaggcagtgcaagcgtctggcacctttcccatgatatgatgaatgtagcacagtttctgatacgcctttttgacgacagaaacgggttgagattctgacacgggaaagcactctaaacagtctttctgtccgtgagtgaagcagatatttgaattctgattcattctctcgcattgtctgcagggaaacagcatcagattcatgcccacgtgacgagaacatttgttttggtacctgtctgcgtagttgatcgaagcttccgcgtctgacgtcgatggctgcgcaactgactcgcgcacccgtttgggctcacttatatctgcgtcactgggggcgggtcttttcttggctccaccctttttgacgtagaattcatgctccacctcaaccacgtgatcctttgcccaccggaaaaagtctttgacttcctgcttggtgaccttcccaaagtcatgatccagacggcgggtgagttcaaatttgaacatccggtcttgcaacggctgctggtgttcgaaggtcgttgagttcccgtcaatcacggcgcacatgttggtgttggaggtgacgatcacgggagtcgggtctatctgggccgaggacttgcatttctggtccacgcgcaccttgcttcctccgagaatggctttggccgactccacgaccttggcggtcatcttcccctcctcccaccagatcaccatcttgtcgacacagtcgttgaagggaaagttctcattggtccagtttacgcacccgtagaagggcacagtgtgggctatggcctccgcgatgttggtcttcccggtagttgcaggcccaaacagccagatggtgttcctcttgccgaactttttcgtggcccatcccagaaagacggaagccgcatattggggatcgtacccgtttagttccaaaattttataaatccgattgctggaaatgtcctccacgggctgctggcccaccaggtagtcgggggcggttttagtcaggctcataatctttcccgcattgtccaaggcagccttgatttgggaccgcgagttggaggccgcattgaaggagatgtatgaggcctggtcctcctggatccactgcttctccgaggtaatccccttgtccacgagccacccgaccagctccatgtacctggctgaagtttttgatctgatcaccggcgcatcagaattgggattctgattctctttgttctgctcctgcgtctgcgacacgtgcgtcagatgctgcgccaccaaccgtttacgctccgtgagattcaaacaggcgcttaaatactgttccatattagtccacgcccactggagctcaggctgggttttggggagcaagtaattggggatgtagcactcatccaccaccttgttcccgcctccggcgccatttctggtctttgtgaccgcgaaccagtttggcaaagtcggctcgatcccgcggtaaattctctgaatcagtttttcgcgaatctgactcaggaaacgtcccaaaaccatggatttcaccccggtggtttccacgagcacgtgcatgtggaagtagctctctcccttctcaaattgcacaaagaaaagggcctccggggccttactcacacggcgccattccgtcagaaagtcgcgctgcagcttctcggccacggtcaggggtgcctgctcaatcagattcagatccatgtcagaatctggcggcaactcccattccttctcggccacccagttcacaaagctgtcagaaatgccgggcagatgctcgtcaaggtcgctggggaccttaatcacaatctcgtaaaaccccggcatggcggcgataactattatcatcgtgtttttcaaaggaaaaccacgtccccgtggttcggggggcctagacgtttttttaacctcgactaaacacatgtaaagcatgtgcaccgaggccccagatcagatcccatacaatggggtaccttctgggcatccttcagccccttgttgaatacgcttgaggagagccatttgactctttccacaactatccaactcacaacgtggcactggggttgtgccgcctttgcaggtgtatcttatacacgtggcttttggccgcagaggcacctgtcgccaggtggggggttccgctgcctgcaaagggtcgctacagacgttgtttgtcttcaagaagcttccagaggaactgcttccttcacgacattcaacagaccttgcattcctttggcgagaggggaaagacccctaggaatgctcgtcaagaagacagggccaggtttccgggccctcacattgccaaaagacggcaatatggtggaaaataacatatagacaaacgcacaccggccttattccaagcggcttcggccagtaacgttagggggggggggcggaattctatccctcagttatctcagagagagtgtcctcgagccaatctggaagataaccatcggcagccatacctgatttaaatcatttattgttcaaagatgcagtcatccaaatccacattgaccagatcgcaggcagtgcaagcgtctggcacctttcccatgatatgatgaatgtagcacagtttctgatacgcctttttgacgacagaaacgggttgagattctgacacgggaaagcactctaaacagtctttctgtccgtgagtgaagcagatatttgaattctgattcattctctcgcattgtctgcagggaaacagcatcagattcatgcccacgtgacgagaacatttgttttggtacctgtctgcgtagttgatcgaagcttccgcgtctgacgtcgatggctgcgcaactgactcgcgcacccgtttgggctcacttatatctgcgtcactgggggcgggtcttttcttggctccaccctttttgacgtagaattcatgctccacctcaaccacgtgatcctttgcccaccggaaaaagtctttgacttcctgcttggtgaccttcccaaagtcatgatccagacggcgggtgagttcaaatttgaacatccggtcttgcaacggctgctggtgttcgaaggtcgttgagttcccgtcaatcacggcgcacatgttggtgttggaggtgacgatcacgggagtcgggtctatctgggccgaggacttgcatttctggtccacgcgcaccttgcttcctccgagaatggctttggccgactccacgaccttggcggtcatcttcccctcctcccaccagatcaccatcttgtcgacacagtcgttgaagggaaagttctcattggtccagtttacgcacccgtagaagggcacagtgtgggctatggcctccgcgatgttggtcttcccggtagttgcaggcccaaacagccagatggtgttcctcttgccgaactttttcgtggcccatcccagaaagacggaagccgcatattggggatcgtacccgtttagttccaaaattttataaatccgattgctggaaatgtcctccacgggctgctggcccaccaggtagtcgggggcggttttagtcaggctcataatctttcccgcattgtccaaggcagccttgatttgggaccgcgagttggaggccgcattgaaggagatgtatgaggcctggtcctcctggatccactgcttctccgaggtaatccccttgtccacgagccacccgaccagctccatggtggcgttatccggccgatcgatagatctgggccccggtgtcgactttacgagggtaggaagtggtacggaaagttggtataagacaaaagtgttgtggaattgctggaggcgatctgacggttcactaaacgagctctgcttttataggcgcccaccgtacacgcctaaagcttatacgttctctatcactgatagggagtaaactggatatacgttctctatcactgatagggagtaaactgtagatacgttctctatcactgatagggagtaaactggtcatacgttctctatcactgatagggagtaaactccttatacgttctctatcactgatagggagtaaagtctgcatacgttctctatcactgatagggagtaaactcttcatacgttctctatcactgatagggaatcccaatggcgcgccgagcttggcgtaatcatggtcatagctgtttcctgtgtgaaattgttatccgctcacaattccacacaacatacgagccggaagcataaagtgtaaagcctggggtgcctaatgagtgagctaactcacattaattgcgttgcgctcactgcccgctttccagtcgggaaacctgtcgtgccagctgcattaatgaatcggccaacgcgcggggagaggcggtttgcgtattgggcgctgttccgcttcctcgctcactgactcgctgcgctcggtcgttcggctgcggcgagcggtatcagctcactcaaaggcggtaatacggttatccacagaatcaggggataacgcaggaaagaacatgtgagcaaaaggccagcaaaaggccaggaaccgtaaaaaggccgcgttgctggcgtttttccataggctccgcccccctgacgagcatcacaaaaatcgacgctcaagtcagaggtggcgaaacccgacaggactataaagataccaggcgtttccccctggaagctccctcgtgcgctctcctgttccgaccctgccgcttaccggatacctgtccgcctttctcccttcgggaagcgtggcgctttctcatagctcacgctgtaggtatctcagttcggtgtaggtcgttcgctccaagctgggctgtgtgcacgaaccccccgttcagcccgaccgctgcgccttatccggtaactatcgtcttgagtccaacccggtaagacacgacttatcgccactggcagcagccactggtaacaggattagcagagcgaggtatgtaggcggtgctacagagttcttgaagtggtggcctaactacggctacactagaagaacagtatttggtatctgcgctctgctgaagccagttaccttcggaaaaagagttggtagctcttgatccggcaaacaaaccaccgctggtagcggtggtttttttgtttgcaagcagcagattacgcgcagaaaaaaaggatctcaagaagatcctttgatcttttctacggggtctgacgctcagtggaacgaaaactcacgttaagggattttggtcatgagattatcaaaaaggatcttcacctagatccttttaaattaaaaatgaagttttaaatcaatctaaagtatatatgagtaaacttggtctgacagttaccaatgcttaatcagtgaggcacctatctcagcgatctgtctatttcgttcatccatagttgcctgactccccgtcgtgtagataactacgatacgggagggcttaccatctggccccagtgctgcaatgataccgcgagaaccacgctcaccggctccagatttatcagcaataaaccagccagccggaagggccgagcgcagaagtggtcctgcaactttatccgcctccatccagtctattaattgttgccgggaagctagagtaagtagttcgccagttaatagtttgcgcaacgttgttgccattgctacaggcatcgtggtgtcacgctcgtcgtttggtatggcttcattcagctccggttcccaacgatcaaggcgagttacatgatcccccatgttgtgcaaaaaagcggttagctccttcggtcctccgatcgttgtcagaagtaagttggccgcagtgttatcactcatggttatggcagcactgcataattctcttactgtcatgccatccgtaagatgcttttctgtgactggtgagtactcaaccaagtcattctgagaatagtgtatgcggcgaccgagttgctcttgcccggcgtcaatacgggataataccgcgccacatagcagaactttaaaagtgctcatcattggaaaacgttcttcggggcgaaaactctcaaggatcttaccgctgttgagatccagttcgatgtaacccactcgtgcacccaactgatcttcagcatcttttactttcaccagcgtttctgggtgagcaaaaacaggaaggcaaaatgccgcaaaaaagggaataagggcgacacggaaatgttgaatactcatactcttcctttttcaatattattgaagcatttatcagggttattgtctcatgagcggatacatatttgaatgtatttagaaaaataaacaaataggggttccgcgcacatttccccgaaaagtgccacctgacgtctaagaaaccattattatcatgacattaacctataaaaataggcgtatcacgaggcccttttgtc

SEQ ID NO: 10 - DNA, 5754 bp, synthetic construct
  misc_feature 1..5754: note = plasmid
  source 1..5754: mol_type = other DNA
tggaagggctaattcactcccaaagaagacaagatatccttgatctgtggatctaccacacacaaggctacttccctgattagcagaactacacaccagggccaggggtcagatatccactgacctttggatggtgctacaagctagtaccagttgagccagataaggtagaagaggccaataaaggagagaacaccagcttgttacaccctgtgagcctgcatgggatggatgacccggagagagaagtgttagagtggaggtttgacagccgcctagcatttcatcacgtggcccgagagctgcatccggagtacttcaagaactgctgatatcgagcttgctacaagggactttccgctggggactttccagggaggcgtggcctgggcgggactggggagtggcgagccctcagatcctgcatataagcagctgctttttgcctgtactgggtctctctggttagaccagatctgagcctgggagctctctggctaactagggaacccactgcttaagcctcaataaagcttgccttgagtgcttcaagtagtgtgtgcccgtctgttgtgtgactctggtaactagagatccctcagacccttttagtcagtgtggaaaatctctagcagtggcgcccgagaggctccggtgcccgtcagtgggcagagcgcacatcgcccacagtccccgagaagttggggggaggggtcggcaattgaaccggtgcctagagaaggtggcgcggggtaaactgggaaagtgatgtcgtgtactggctccgcctttttcccgagggtgggggagaaccgtatataagtgcagtagtcgccgtgaacgttctttttcgcaacgggtttgccgccagaacacaggtaagtgccgtgtgtggttcccgcgggcctggcctctttacgggttatggcccttgcgtgccttgaattacttccacgcccctggctgcagtacgtgattcttgatcccgagcttcgggttggaagtgggtgggagagttcgaggccttgcgcttaaggagccccttcgcctcgtgcttgagttgaggcctggcttgggcgctggggccgccgcgtgcgaatctggtggcaccttcgcgcctgtctcgctgctttcgataagtctctagccatttaaaatttttgatgacctgctgcgacgctttttttctggcaagatagtcttgtaaatgcgggccaagatctgcacactggtatttcggtttttggggccgcgggcggcgacggggcccgtgcgtcccagcgcacatgttcggcgaggcggggcctgcgagcgcggccaccgagaatcggacgggggtagtctcaagctggccggcctgctctggtgcctggcctcgcgccgccgtgtatcgccccgccctgggcggcaaggctggcccggtcggcaccagttgcgtgagcggaaagatggccgcttcccggccctgctgcagggagctcaaaatggaggacgcggcgctcgggagagcgggcgggtgagtcacccacacaaaggaaaagggcctttccgtcctcagccgtcgcttcatgtgactccacggagtaccgggcgccgtccaggcacctcgattagttctcgagcttttggagtacgtcgtctttaggttggggggaggggttttatgcgatggagtttccccacactgagtgggtggagactgaagttaggccagcttggcacttgatgtaattctccttggaatttgccctttttgagtttggatcttggttcattctcaagcctcagacagtggttcaaagtttttttcttccatttcaggtgtcgtgaacctgcaggatttaaattctagttcaccatgtctagactggacaagagcaaagtcataaactctgctctggaattactcaatggagtcggtatcgaaggcctgacgacaaggaaactcgctcaaaagctgggagttgagcagcctaccctgtactggcacgtgaagaacaagcgggccctgctcgatgccctgccaatcgagatgctggacaggcatcatacccactcctgccccctggaaggcgagtcatggcaagactttctgcggaacaacgccaagtcataccgctgtgctctcctctcacatcgcgacggggctaaagtgcatctcggcacccgcccaacagagaaacagtacgaaaccctggaaaatcagctcgcgttcctgtgtcagcaaggcttctccctggagaacgcactgtacgctctgtccgccgtgggccactttacactgggctgcgtattggaggaacaggagcatcaagtagcaaaagaggaaagagagacacctaccaccgattctatgcccccacttctgaaacaagcaattgagctgttcgaccggcagggagccgaacctgccttccttttcggcctggaactaatcatatgtggcctggagaaacagctaaagtgcgaaagcggcgggccgaccgacgcccttgacgattttgacttagacatgctcccagccgatgcccttgacgactttgaccttgatatgctgcctgctgacgctcttgacgattttgaccttgacatgctccccgggtaactagatccaattctacccgagggcaaaggaatagacgcgtctggaacaatcaacctctggattacaaaatttgtgaaagattgactggtattcttaactatgttgctccttttacgctatgtggatacgctgctttaatgcctttgtatcatgctattgcttcccgtatggctttcattttctcctccttgtataaatcctggttgctgtctctttatgaggagttgtggcccgttgtcaggcaacgtggcgtggtgtgcactgtgtttgctgacgcaacccccactggttggggcattgccaccacctgtcagctcctttccgggactttcgctttccccctccctattgccacggcggaactcatcgccgcctgccttgcccgctgctggacaggggctcggctgttgggcactgacaattccgtggtgttgtcggggaagctgacgtcctttccatggctgctcgcctgtgttgccacctggattctgcgcgggacgtccttctgctacgtcccttcggccctcaatccagcggaccttccttcccgcggcctgctgccggctctgcggcctcttccgcgtcttcgccttcgccctcagacgagtcggatctccctttgggccgcctccccgcctggaattaattctggctagagcttggcgtaatcatggtcatagctgtttcctgtgtgaaattgttatccgctcacaattccacacaacatacgagccggaagcataaagtgtaaagcctggggtgcctaatgagtgagctaactcacattaattgcgttgcgctcactgcccgctttccagtcgggaaacctgtcgtgccagctgcattaatgaatcggccaacgcgcggggagaggcggtttgcgtattgggcgctcttccgcttcctcgctcactgactcgctgcgctcggtcgttcggctgcggcgagcggtatcagctcactcaaaggcggtaatacggttatccacagaatcaggggataacgcaggaaagaacatgtgagcaaaaggccagcaaaaggccaggaaccgtaaaaaggccgcgttgctggcgtttttccataggctccgcccccctgacgagcatcacaaaaatcgacgctcaagtcagaggtggcgaaacccgacaggactataaagataccaggcgtttccccctggaagctccctcgtgcgctctcctgttccgaccctgccgcttaccggatacctgtccgcctttctcccttcgggaagcgtggcgctttctcatagctcacgctgtaggtatctcagttcggtgtaggtcgttcgctccaagctgggctgtgtgcacgaaccccccgttcagcccgaccgctgcgccttatccggtaactatcgtcttgagtccaacccggtaagacacgacttatcgccactggcagcagccactggtaacaggattagcagagcgaggtatgtaggcggtgctacagagttcttgaagtggtggcctaactacggctacactagaagaacagtatttggtatctgcgctctgctgaagccagttaccttcggaaaaagagttggtagctcttgatccggcaaacaaaccaccgctggtagcggtggtttttttgtttgcaagcagcagattacgcgcagaaaaaaaggatctcaagaagatcctttgatcttttctacggggtctgacgctcagtggaacgaaaactcacgttaagggattttggtcatgagattatcaaaaaggatcttcacctagatccttttaaattaaaaatgaagttttaaatcaatctaaagtatatatgagtaaacttggtctgacagttaccaatgcttaatcagtgaggcacctatctcagcgatctgtctatttcgttcatccatagttgcctgactccccgtcgtgtagataactacgatacgggagggcttaccatctggccccagtgctgcaatgataccgcgagacccacgctcaccggctccagatttatcagcaataaaccagccagccggaagggccgagcgcagaagtggtcctgcaactttatccgcctccatccagtctattaattgttgccgggaagctagagtaagtagttcgccagttaatagtttgcgcaacgttgttgccattgctacaggcatcgtggtgtcacgctcgtcgtttggtatggcttcattcagctccggttcccaacgatcaaggcgagttacatgatcccccatgttgtgcaaaaaagcggttagctccttcggtcctccgatcgttgtcagaagtaagttggccgcagtgttatcactcatggttatggcagcactgcataattctcttactgtcatgccatccgtaagatgcttttctgtgactggtgagtactcaaccaagtcattctgagaatagtgtatgcggcgaccgagttgctcttgcccggcgtcaatacgggataataccgcgccacatagcagaactttaaaagtgctcatcattggaaaacgttcttcggggcgaaaactctcaaggatcttaccgctgttgagatccagttcgatgtaacccactcgtgcacccaactgatcttcagcatcttttactttcaccagcgtttctgggtgagcaaaaacaggaaggcaaaatgccgcaaaaaagggaataagggcgacacggaaatgttgaatactcatactcttcctttttcaatattattgaagcatttatcagggttattgtctcatgagcggatacatatttgaatgtatttagaaaaataaacaaataggggttccgcgcacatttccccgaaaagtgccacctgacgtcgacggatcgggagatcaacttgtttattgcagcttataatggttacaaataaagcaatagcatcacaaatttcacaaataaagcatttttttcactgcattctagttgtggtttgtccaaactcatcaatgtatcttatcatgtctggatcaactggataactcaagctaaccaaaatcatcccaaacttcccaccccataccctattaccactgccaattacctgtggtttcatttactctaaacctgtgattcctctgaattattttcattttaaagaaattgtatttgttaaatatgtactacaaacttagtagt

SEQ ID NO: 11 - DNA, 8777 bp, synthetic construct
  misc_feature 1..8777: note = plasmid
  source 1..8777: mol_type = other DNA
acgcgtgtagtcttatgcaatactcttgtagtcttgcaacatggtaacgatgagttagcaacatgccttacaaggagagaaaaagcaccgtgcatgccgattggtggaagtaaggtggtacgatcgtgccttattaggaaggcaacagacgggtctgacatggattggacgaaccactgaattgccgcattgcagagatattgtatttaagtgcctagctcgatacaataaacgggtctctctggttagaccagatctgagcctgggagctctctggctaactagggaacccactgcttaagcctcaataaagcttgccttgagtgcttcaagtagtgtgtgcccgtctgttgtgtgactctggtaactagagatccctcagacccttttagtcagtgtggaaaatctctagcagtggcgcccgaacagggacctgaaagcgaaagggaaaccagagctctctcgacgcaggactcggcttgctgaagcgcgcacggcaagaggcgaggggcggcgactggtgagtacgccaaaaattttgactagcggaggctagaaggagagagatgggtgcgagagcgtcagtattaagcgggggagaattagatcgcgatgggaaaaaattcggttaaggccagggggaaagaaaaaatataaattaaaacatatagtatgggcaagcagggagctagaacgattcgcagttaatcctggcctgttagaaacatcagaaggctgtagacaaatactgggacagctacaaccatcccttcagacaggatcagaagaacttagatcattatataatacagtagcaaccctctattgtgtgcatcaaaggatagagataaaagacaccaaggaagctttagacaagatagaggaagagcaaaacaaaagtaagaccaccgcacagcaagcggccactgatcttcagacctggaggaggagatatgagggacaattggagaagtgaattatataaatataaagtagtaaaaattgaaccattaggagtagcacccaccaaggcaaagagaagagtggtgcagagagaaaaaagagcagtgggaataggagctttgttccttgggttcttgggagcagcaggaagcactatgggcgcagcctcaatgacgctgacggtacaggccagacaattattgtctggtatagtgcagcagcagaacaatttgctgagggctattgaggcgcaacagcatctgttgcaactcacagtctggggcatcaagcagctccaggcaagaatcctggctgtggaaagatacctaaaggatcaacagctcctggggatttggggttgctctggaaaactcatttgcaccactgctgtgccttggaatgctagttggagtaataaatctctggaacagattggaatcacacgacctggatggagtgggacagagaaattaacaattacacaagcttaatacactccttaattgaagaatcgcaaaaccagcaagaaaagaatgaacaagaattattggaattagataaatgggcaagtttgtggaattggtttaacataacaaattggctgtggtatataaaattattcataatgatagtaggaggcttggtaggtttaagaatagtttttgctgtactttctatagtgaatagagttaggcagggatattcaccattatcgtttcagacccacctcccaaccccgaggggacccgacaggcccgaaggaatagaagaagaaggtggagagagagacagagacagatccattcgattagtgaacggatctcgacggttaacttttaaaagaaaaggggggattggggggtacagtgcaggggaaagaatagtagacataatagcaacagacatacaaactaaagaattacaaaaacaaattacaaaaattcaaaattttatcgatactagagcccaaggatcgagagatatgcaggcagctgcgcgctcgctcgctcactgaggccgcccgggcaaagcccgggcgtcgggcgacctttggtcgcccggcctcagtgagcgagcgagcgcgcagagagggagtggccaactccatcactaggggttcctagagatcgcctgcagatccagaaatcgattgtatcagtcagtcagtgcaggaggagacaacttctacttgtacagctcgtccatgccgagagtgatcccggcggcggtcacgaactccagcaggaccatgtgatcgcgcttctcgttggggtctttgctcagggcggactgggtgctcaggtagtggttgtcgggcagcagcacggggccgtcgccgatgggggtgttctgctggtagtggtcggcgagttgcacgctgccgtcctcgatgttgtggcggatcttgaagttcaccttgatgccgttcttctgcttgtcggccatgatatagacgttgtggctgttgtagttgtactccagcttgtgccccaggatgttgccgtcctccttgaagtcgatgcccttcagctcgatgcggttcaccagggtgtcgccctcgaacttcacctcggcgcgggtcttgtagttgccgtcgtccttgaagaagatggtgcgctcctggacgtagccttcgggcatggcggacttgaagaagtcgtgctgcttcatgtggtcggggtagcggctgaagcattgcacgccgtaggtcagggtggtcacgagggtgggccagggcacgggcagcttgccggtggtacagatgaacttcagggtcagcttgccgtaggtggcatcgccctcgccctcgccggacacgctgaacttgtggccgtttacgtcgccgtccagctcgaccaggatgggcaccaccccggtgaacagttcctcgcccttgctgaccatggtgggtacctcctttgaattcgagagctcggaagcttggcagcggccgctggcgggtgtgtcgagtggatggtaggatcgacaaagatctgatctgacggttcactaaaccagctctgcttatatagacctcccaccgtacacgcctaccgcccatttgcgtcaatggggcggagttgttacgacattttggaaagtcccgttgattttggtgccaaaacaaactcccattgacgtcaatggggtggagacttggaaatccccgtgagtcaaaccgctatccacgcccattgatgtactgccaaaaccgcatcagcatggtaatagcgatgactaatacgtagatgtactgccaagtaggaaagtcccataaggtcatgtactgggcataatgccaggcgggccatttaccgtcattgacgtcaatagggggcgtacttggcatatgatacacttgatgtactgccaagtgggcagtttaccgtaaatactccacccattgacgtcaatggaaagtccctattggcgttactatgggaacatacgtcattattgacgtcaatgggcgggggtcgttgggcggtcagccaggcgggccatttaccgtaagttatgtaacgcggaactccatatatgggctatgaactaatgaccccgtaattgattactagatctgatatcaggaacccctagtgatggagttggccactccctctctgcgcgctcgctcgctcactgaggccgggcgaccaaaggtcgcccgacgcccgggctttgcccgggcggcctcagtgagcgagcgagcgcgcagctgcctgcatgcgtcaattttacgcagacggccgcaaggatctgcgatcgctccggtgcccgtcagtgggcagagcgcacatcgcccacagtccccgagaagttggggggaggggtcggcaattgaacgggtgcctagagaaggtggcgcggggtaaactgggaaagtgatgtcgtgtactggctccgcctttttcccgagggtgggggagaaccgtatataagtgcagtagtcgccgtgaacgttctttttcgcaacgggtttgccgccagaacacagctgaagcttcgaggggctcgcatctctccttcacgcgcccgccgccctacctgaggccgccatccacgccggttgagtcgcgttctgccgcctcccgcctgtggtgcctcctgaactgcgtccgccgtctaggtaagtttaaagctcaggtcgagaccgggcctttgtccggcgctcccttggagcctacctagactcagccggctctccacgctttgcctgaccctgcttgctcaactctacgtctttgtttcgttttctgttctgcgccgttacagatccaagctgtgaccggcgcctacgctagatgaccgagtacaagcccacggtgcgcctcgccacccgcgacgacgtccccagggccgtacgcaccctcgccgccgcgttcgccgactaccccgccacgcgccacaccgtcgatccggaccgccacatcgagcgggtcaccgagctgcaagaactcttcctcacgcgcgtcgggctcgacatcggcaaggtgtgggtcgcggacgacggcgccgcggtggcggtctggaccacgccggagagcgtcgaagcgggggcggtgttcgccgagatcggcccgcgcatggccgagttgagcggttcccggctggccgcgcagcaacagatggaaggcctcctggcgccgcaccggcccaaggagcccgcgtggttcctggccaccgtcggcgtctcgcccgaccaccagggcaagggtctgggcagcgccgtcgtgctccccggagtggaggcggccgagcgcgccggggtgcccgccttcctggagacctccgcgccccgcaacctccccttctacgagcggctcggcttcaccgtcaccgccgacgtcgaggtgcccgaaggaccgcgcacctggtgcatgacccgcaagcccggtgcctgagtcgacaatcaacctctggattacaaaatttgtgaaagattgactggtattcttaactatgttgctccttttacgctatgtggatacgctgctttaatgcctttgtatcatgctattgcttcccgtatggctttcattttctcctccttgtataaatcctggttgctgtctctttatgaggagttgtggcccgttgtcaggcaacgtggcgtggtgtgcactgtgtttgctgacgcaacccccactggttggggcattgccaccacctgtcagctcctttccgggactttcgctttccccctccctattgccacggcggaactcatcgccgcctgccttgcccgctgctggacaggggctcggctgttgggcactgacaattccgtggtgttgtcggggaaatcatcgtcctttccttggctgctcgcctgtgttgccacctggattctgcgcgggacgtccttctgctacgtcccttcggccctcaatccagcggaccttccttcccgcggcctgctgccggctctgcggcctcttccgcgtcttcgccttcgccctcagacgagtcggatctccctttgggccgcctccccgcctggtacctttaagaccaatgacttacaaggcagctgtagatcttagccactttttaaaagaaaaggggggactggaagggctaattcactcccaacgaaaataagatctgctttttgcttgtactgggtctctctggttagaccagatctgagcctgggagctctctggctaactagggaacccactgcttaagcctcaataaagcttgccttgagtgcttcaagtagtgtgtgcccgtctgttgtgtgactctggtaactagagatccctcagacccttttagtcagtgtggaaaatctctagcagtagtagttcatgtcatcttattattcagtatttataacttgcaaagaaatgaatatcagagagtgagaggaacttgtttattgcagcttataatggttacaaataaagcaatagcatcacaaatttcacaaataaagcatttttttcactgcattctagttgtggtttgtccaaactcatcaatgtatcttatcatgtctggctctagctatcccgcccctaactccgcccagttccgcccattctccgccccatggctgactaattttttttatttatgcagaggccgaggccgcctcggcctctgagctattccagaagtagtgaggaggcttttttggaggcctagacttttgcagagacggcccaaattcgtaatcatggtcatagctgtttcctgtgtgaaattgttatccgctcacaattccacacaacatacgagccggaagcataaagtgtaaagcctggggtgcctaatgagtgagctaactcacattaattgcgttgcgctcactgcccgctttccagtcgggaaacctgtcgtgccagctgcattaatgaatcggccaacgcgcggggagaggcggtttgcgtattgggcgctcttccgcttcctcgctcactgactcgctgcgctcggtcgttcggctgcggcgagcggtatcagctcactcaaaggcggtaatacggttatccacagaatcaggggataacgcaggaaagaacatgtgagcaaaaggccagcaaaaggccaggaaccgtaaaaaggccgcgttgctggcgtttttccataggctccgcccccctgacgagcatcacaaaaatcgacgctcaagtcagaggtggcgaaacccgacaggactataaagataccaggcgtttccccctggaagctccctcgtgcgctctcctgttccgaccctgccgcttaccggatacctgtccgcctttctcccttcgggaagcgtggcgctttctcatagctcacgctgtaggtatctcagttcggtgtaggtcgttcgctccaagctgggctgtgtgcacgaaccccccgttcagcccgaccgctgcgccttatccggtaactatcgtcttgagtccaacccggtaagacacgacttatcgccactggcagcagccactggtaacaggattagcagagcgaggtatgtaggcggtgctacagagttcttgaagtggtggcctaactacggctacactagaaggacagtatttggtatctgcgctctgctgaagccagttaccttcggaaaaagagttggtagctcttgatccggcaaacaaaccaccgctggtagcggtggtttttttgtttgcaagcagcagattacgcgcagaaaaaaaggatctcaagaagatcctttgatcttttctacggggtctgacgctcagtggaacgaaaactcacgttaagggattttggtcatgagattatcaaaaaggatcttcacctagatccttttaaattaaaaatgaagttttaaatcaatctaaagtatatatgagtaaacttggtctgacagttaccaatgcttaatcagtgaggcacctatctcagcgatctgtctatttcgttcatccatagttgcctgactccccgtcgtgtagataactacgatacgggagggcttaccatctggccccagtgctgcaatgataccgcgagacccacgctcaccggctccagatttatcagcaataaaccagccagccggaagggccgagcgcagaagtggtcctgcaactttatccgcctccatccagtctattaattgttgccgggaagctagagtaagtagttcgccagttaatagtttgcgcaacgttgttgccattgctacaggcatcgtggtgtcacgctcgtcgtttggtatggcttcattcagctccggttcccaacgatcaaggcgagttacatgatcccccatgttgtgcaaaaaagcggttagctccttcggtcctccgatcgttgtcagaagtaagttggccgcagtgttatcactcatggttatggcagcactgcataattctcttactgtcatgccatccgtaagatgcttttctgtgactggtgagtactcaaccaagtcattctgagaatagtgtatgcggcgaccgagttgctcttgcccggcgtcaatacgggataataccgcgccacatagcagaactttaaaagtgctcatcattggaaaacgttcttcggggcgaaaactctcaaggatcttaccgctgttgagatccagttcgatgtaacccactcgtgcacccaactgatcttcagcatcttttactttcaccagcgtttctgggtgagcaaaaacaggaaggcaaaatgccgcaaaaaagggaataagggcgacacggaaatgttgaatactcatactcttcctttttcaatattattgaagcatttatcagggttattgtctcatgagcggatacatatttgaatgtatttagaaaaataaacaaataggggttccgcgcacatttccccgaaaagtgccacctgacgtctaagaaaccattattatcatgacattaacctataaaaataggcgtatcacgaggccctttcgtctcgcgcgtttcggtgatgacggtgaaaacctctgacacatgcagctcccggagacggtcacagcttgtctgtaagcggatgccgggagcagacaagcccgtcagggcgcgtcagcgggtgttggcgggtgtcggggctggcttaactatgcggcatcagagcagattgtactgagagtgcaccatatgcggtgtgaaataccgcacagatgcgtaaggagaaaataccgcatcaggcgccattcgccattcaggctgcgcaactgttgggaagggcgatcggtgcgggcctcttcgctattacgccagctggcgaaagggggatgtgctgcaaggcgattaagttgggtaacgccagggttttcccagtcacgacgttgtaaaacgacggccagtgccaagctg

SEQ ID NO: 12 - DNA, 10239 bp, synthetic construct
  misc_feature 1..10239: note = plasmid
  source 1..10239: mol_type = other DNA
tggaagggctaattcactcccaaagaagacaagatatccttgatctgtggatctaccacacacaaggctacttccctgattagcagaactacacaccagggccaggggtcagatatccactgacctttggatggtgctacaagctagtaccagttgagccagataaggtagaagaggccaataaaggagagaacaccagcttgttacaccctgtgagcctgcatgggatggatgacccggagagagaagtgttagagtggaggtttgacagccgcctagcatttcatcacgtggcccgagagctgcatccggagtacttcaagaactgctgatatcgagcttgctacaagggactttccgctggggactttccagggaggcgtggcctgggcgggactggggagtggcgagccctcagatcctgcatataagcagctgctttttgcctgtactgggtctctctggttagaccagatctgagcctgggagctctctggctaactagggaacccactgcttaagcctcaataaagcttgccttgagtgcttcaagtagtgtgtgcccgtctgttgtgtgactctggtaactagagatccctcagacccttttagtcagtgtggaaaatctctagcagtggcgcccgaacagggacttgaaagcgaaagggaaaccagaggagctctctcgacgcaggactcggcttgctgaagcgcgcacggcaagaggcgaggggcggcgactggtgagtacgccaaaaattttgactagcggaggctagaaggagagagatgggtgcgagagcgtcagtattaagcgggggagaattagatcgcgatgggaaaaaattcggttaaggccagggggaaagaaaaaatataaattaaaacatatagtatgggcaagcagggagctagaacgattcgcagttaatcctggcctgttagaaacatcagaaggctgtagacaaatactgggacagctacaaccatcccttcagacaggatcagaagaacttagatcattatataatacagtagcaaccctctattgtgtgcatcaaaggatagagataaaagacaccaaggaagctttagacaagatagaggaagagcaaaacaaaagtaagaccaccgcacagcaagcggccggccgctgatcttcagacctggaggaggagatatgagggacaattggagaagtgaattatataaatataaagtagtaaaaattgaaccattaggagtagcacccaccaaggcaaagagaagagtggtgcagagagaaaaaagagcagtgggaataggagctttgttccttgggttcttgggagcagcaggaagcactatgggcgcagcgtcaatgacgctgacggtacaggccagacaattattgtctggtatagtgcagcagcagaacaatttgctgagggctattgaggcgcaacagcatctgttgcaactcacagtctggggcatcaagcagctccaggcaagaatcctggctgtggaaagatacctaaaggatcaacagctcctggggatttggggttgctctggaaaactcatttgcaccactgctgtgccttggaatgctagttggagtaataaatctctggaacagatttggaatcacacgacctggatggagtgggacagagaaattaacaattacacaagcttaatacactccttaattgaagaatcgcaaaaccagcaagaaaagaatgaacaagaattattggaattagataaatgggcaagtttgtggaattggtttaacataacaaattggctgtggtatataaaattattcataatgatagtaggaggcttggtaggtttaagaatagtttttgctgtactttctatagtgaatagagttaggcagggatattcaccattatcgtttcagacccacctcccaaccccgaggggacccgacaggcccgaaggaatagaagaagaaggtggagagagagacagagacagatccattcgattagtgaacggatctcgacggtatcgcctttaaaagaaaaggggggattggggggtacagtgcaggggaaagaatagtagacataatagcaacagacatacaaactaaagaattacaaaaacaaattacaaaaattcaaaattttcgggtttattacagggacagcagagatccagtttatcgatatcgaattcgtgaggctccggtgcccgtcagtgggcagagcgcacatcgcccacagtccccgagaagttggggggaggggtcggcaattgaaccggtgcctagagaaggtggcgcggggtaaactgggaaagtgatgtcgtgtactggctccgcctttttcccgagggtgggggagaaccgtatataagtgcagtagtcgccgtgaacgttctttttcgcaacgggtttgccgccagaacacaggtaagtgccgtgtgtggttcccgcgggcctggcctctttacgggttatggcccttgcgtgccttgaattacttccacgcccctggctgcagtacgtgattcttgatcccgagcttcgggttggaagtgggtgggagagttcgaggccttgcgcttaaggagccccttcgcctcgtgcttgagttgaggcctggcttgggcgctggggccgccgcgtgcgaatctggtggcaccttcgcgcctgtctcgctgctttcgataagtctctagccatttaaaatttttgatgacctgctgcgacgctttttttctggcaagatagtcttgtaaatgcgggccaagatctgcacactggtatttcggtttttggggccgcgggcggcgacggggcccgtgcgtcccagcgcacatgttcggcgaggcggggcctgcgagcgcggccaccgagaatcggacgggggtagtctcaagctggccggcctgctctggtgcctggcctcgcgccgccgtgtatcgccccgccctgggcggcaaggctggcccggtcggcaccagttgcgtgagcggaaagatggccgcttcccggccctgctgcagggagctcaaaatggaggacgcggcgctcgggagagcgggcgggtgagtcacccacacaaaggaaaagggcctttccgtcctcagccgtcgcttcatgtgactccacggagtaccgggcgccgtccaggcacctcgattagttctcgagcttttggagtacgtcgtctttaggttggggggaggggttttatgcgatggagtttccccacactgagtgggtggagactgaagttaggccagcttggcacttgatgtaattctccttggaatttgccctttttgagtttggatcttggttcattctcaagcctcagacagtggttcaaagtttttttcttccatttcaggtgtcgtgaacctgcaggatttaaattctagatgccaccatggccagtcgggaagaggagcagcgcgaaaccacccccgagcgcggacgcggtgcggcgcgacgtcccccaaccatggaggacgtgtcgtccccgtccccgtcgccgccgcctccccgggcgcccccaaaaaagcggatgaggcggcgtatcgagtccgaggacgaggaagactcatcacaagacgcgctggtgccgcgcacacccagcccgcggccatcgacctcggcggcggatttggccattgcgcccaagaagaaaaagaagcgcccttctcccaagcccgagcgcccgccatcaccagaggtaatcgtggacagcgaggaagaaagagaagatgtggcgctacaaatggtgggtttcagcaacccaccggtgctaatcaagcatggcaaaggaggtaagcgcacagtgcggcggctgaatgaagacgacccagtggcgcgtggtatgcggacgcaagaggaagaggaagagcccagcgaagcggaaagtgaaattacggtgatgaacccgctgagtgtgccgatcgtgtctgcgtgggagaagggcatggaggctgcgcgcgcgctgatggacaagtaccacgtggataacgatctaaaggcgaacttcaaactactgcctgaccaagtggaagctctggcggccgtatgcaagacctggctgaacgaggagcaccgcgggttgcagctgaccttcaccagcaacaagacctttgtgacgatgatggggcgattcctgcaggcgtacctgcagtcgtttgcagaggtgacctacaagcatcacgagcccacgggctgcgcgttgtggctgcaccgctgcgctgagatcgaaggcgagcttaagtgtctacacggaagcattatgataaataaggagcacgtgattgaaatggatgtgacgagcgaaaacgggcagcgcgcgctgaaggagcagtctagcaaggccaagatcgtgaagaaccggtggggccgaaatgtggtgcagatctccaacaccgacgcaaggtgctgcgtgcacgacgcggcctgtccggccaatcagttttccggcaagtcttgcggcatgttcttctctgaaggcgcaaaggctcaggtggcttttaagcagatcaaggcttttatgcaggcgctgtatcctaacgcccagaccgggcacggtcaccttttgatgccactacggtgcgagtgcaactcaaagcctgggcacgcgccctttttgggaaggcagctaccaaagttgactccgttcgccctgagcaacgcggaggacctggacgcggatctgatctccgacaagagcgtgctggccagcgtgcaccacccggcgctgatagtgttccagtgctgcaaccctgtgtatcgcaactcgcgcgcgcagggcggaggccccaactgcgacttcaagatatcggcgcccgacctgctaaacgcgttggtgatggtgcgcagcctgtggagtgaaaacttcaccgagctgccgcggatggttgtgcctgagtttaagtggagcactaaacaccagtatcgcaacgtgtccctgccagtggcgcatagcgatgcgcggcagaacccctttgattttgattacaaggacgacgatgacaagtaaggatccaattctaccgggtaggggaggcgcttttcccaaggcagtctggagcatgcgctttagcagccccgctgggcacttggcgctacacaagtggcctctggcctcgcacacattccacatccaccggtaggcgccaaccggctccgttctttggtggccccttcgcgccaccttctactcctcccctagtcaggaagttcccccccgccccgcagctcgcgtcgtgcaggacgtgacaaatggaagtagcacgtctcactagtctcgtgcagatggacagcaccgctgagcaatggaagcgggtaggcctttggggcagcggccaatagcagctttgctccttcgctttctgggctcagaggctgggaaggggtgggtccgggggcgggctcaggggcgggctcaggggcggggcgggcgcccgaaggtcctccggaggcccggcattctgcacgcttcaaaagcgcacgtctgccgcgctgttctcctcttcctcatctccgggcctttcgacctgcagttaacgccgccatggatagatccggaaagcctgaactcaccgcgacgtctgtcgagaagtttctgatcgaaaagttcgacagcgtctccgacctgatgcagctctcggagggcgaagaatctcgtgctttcagcttcgatgtaggagggcgtggatatgtcctgcgggtaaatagctgcgccgatggtttctacaaagatcgttatgtttatcggcactttgcatcggccgcgctcccgattccggaagtgcttgacattggggaattcagcgagagcctgacctattgcatctcccgccgtgcacagggtgtcacgttgcaagacctgcctgaaaccgaactgcccgctgttctgcagccggtcgcggaggccatggatgcgatcgctgcggccgatcttagccagacgagcgggttcggcccattcggaccgcaaggaatcggtcaatacactacatggcgtgatttcatatgcgcgattgctgatccccatgtgtatcactggcaaactgtgatggacgacaccgtcagtgcgtccgtcgcgcaggctctcgatgagctgatgctttgggccgaggactgccccgaagtccggcacctcgtgcacgcggatttcggctccaacaatgtcctgacggacaatggccgcataacagcggtcattgactggagcgaggcgatgttcggggattcccaatacgaggtcgccaacatcttcttctggaggccgtggttggcttgtatggagcagcagacgcgctacttcgagcggaggcatccggagcttgcaggatcgccgcggctccgggcgtatatgctccgcattggtcttgaccaactctatcagagcttggttgacggcaatttcgatgatgcagcttgggcgcagggtcgatgcgacgcaatcgtccgatccggagccgggactgtcgggcgtacacaaatcgcccgcagaagcgcggccgtctggaccgatggctgtgtagaagtactcgccgatagtggaaaccgacgccccagcactcgtccgagggcaaaggaatagacgcgtctggaacaatcaacctctggattacaaaatttgtgaaagattgactggtattcttaactatgttgctccttttacgctatgtggatacgctgctttaatgcctttgtatcatgctattgcttcccgtatggctttcattttctcctccttgtataaatcctggttgctgtctctttatgaggagttgtggcccgttgtcaggcaacgtggcgtggtgtgcactgtgtttgctgacgcaacccccactggttggggcattgccaccacctgtcagctcctttccgggactttcgctttccccctccctattgccacggcggaactcatcgccgcctgccttgcccgctgctggacaggggctcggctgttgggcactgacaattccgtggtgttgtcggggaagctgacgtcctttccatggctgctcgcctgtgttgccacctggattctgcgcgggacgtccttctgctacgtcccttcggccctcaatccagcggaccttccttcccgcggcctgctgccggctctgcggcctcttccgcgtcttcgccttcgccctcagacgagtcggatctccctttgggccgcctccccgcctggaattaattctgcagtcgagacctagaaaaacatggagcaatcacaagtagcaatacagcagctaccaatgctgattgtgcctggctagaagcacaagaggaggaggaggtgggttttccagtcacacctcaggtacctttaagaccaatgacttacaaggcagctgtagatcttagccactttttaaaagaaaagaggggactggaagggctaattcactcccaacgaagacaagatctgctttttgcttgtactgggtctctctggttagaccagatctgagcctgggagctctctggctaactagggaacccactgcttaagcctcaataaagcttgccttgagtgcttcaagtagtgtgtgcccgtctgttgtgtgactctggtaactagagatccctcagacccttttagtcagtgtggaaaatctctagcagtagtagttcatgtcatcttattattcagtatttataacttgcaaagaaatgaatatcagagagtgagaggccttgacattgctagcgttttaccgtcgacctctagctagagcttggcgtaatcatggtcatagctgtttcctgtgtgaaattgttatccgctcacaattccacacaacatacgagccggaagcataaagtgtaaagcctggggtgcctaatgagtgagctaactcacattaattgcgttgcgctcactgcccgctttccagtcgggaaacctgtcgtgccagctgcattaatgaatcggccaacgcgcggggagaggcggtttgcgtattgggcgctcttccgcttcctcgctcactgactcgctgcgctcggtcgttcggctgcggcgagcggtatcagctcactcaaaggcggtaatacggttatccacagaatcaggggataacgcaggaaagaacatgtgagcaaaaggccagcaaaaggccaggaaccgtaaaaaggccgcgttgctggcgtttttccataggctccgcccccctgacgagcatcacaaaaatcgacgctcaagtcagaggtggcgaaacccgacaggactataaagataccaggcgtttccccctggaagctccctcgtgcgctctcctgttccgaccctgccgcttaccggatacctgtccgcctttctcccttcgggaagcgtggcgctttctcatagctcacgctgtaggtatctcagttcggtgtaggtcgttcgctccaagctgggctgtgtgcacgaaccccccgttcagcccgaccgctgcgccttatccggtaactatcgtcttgagtccaacccggtaagacacgacttatcgccactggcagcagccactggtaacaggattagcagagcgaggtatgtaggcggtgctacagagttcttgaagtggtggcctaactacggctacactagaagaacagtatttggtatctgcgctctgctgaagccagttaccttcggaaaaagagttggtagctcttgatccggcaaacaaaccaccgctggtagcggtggtttttttgtttgcaagcagcagattacgcgcagaaaaaaaggatctcaagaagatcctttgatcttttctacggggtctgacgctcagtggaacgaaaactcacgttaagggattttggtcatgagattatcaaaaaggatcttcacctagatccttttaaattaaaaatgaagttttaaatcaatctaaagtatatatgagtaaacttggtctgacagttaccaatgcttaatcagtgaggcacctatctcagcgatctgtctatttcgttcatccatagttgcctgactccccgtcgtgtagataactacgatacgggagggcttaccatctggccccagtgctgcaatgataccgcgagacccacgctcaccggctccagatttatcagcaataaaccagccagccggaagggccgagcgcagaagtggtcctgcaactttatccgcctccatccagtctattaattgttgccgggaagctagagtaagtagttcgccagttaatagtttgcgcaacgttgttgccattgctacaggcatcgtggtgtcacgctcgtcgtttggtatggcttcattcagctccggttcccaacgatcaaggcgagttacatgatcccccatgttgtgcaaaaaagcggttagctccttcggtcctccgatcgttgtcagaagtaagttggccgcagtgttatcactcatggttatggcagcactgcataattctcttactgtcatgccatccgtaagatgcttttctgtgactggtgagtactcaaccaagtcattctgagaatagtgtatgcggcgaccgagttgctcttgcccggcgtcaatacgggataataccgcgccacatagcagaactttaaaagtgctcatcattggaaaacgttcttcggggcgaaaactctcaaggatcttaccgctgttgagatccagttcgatgtaacccactcgtgcacccaactgatcttcagcatcttttactttcaccagcgtttctgggtgagcaaaaacaggaaggcaaaatgccgcaaaaaagggaataagggcgacacggaaatgttgaatactcatactcttcctttttcaatattattgaagcatttatcagggttattgtctcatgagcggatacatatttgaatgtatttagaaaaataaacaaataggggttccgcgcacatttccccgaaaagtgccacctgacgtcgacggatcgggagatcaacttgtttattgcagcttataatggttacaaataaagcaatagcatcacaaatttcacaaataaagcatttttttcactgcattctagttgtggtttgtccaaactcatcaatgtatcttatcatgtctggatcaactggataactcaagctaaccaaaatcatcccaaacttcccaccccataccctattaccactgccaattacctgtggtttcatttactctaaacctgtgattcctctgaattattttcattttaaagaaattgtatttgttaaatatgtactacaaacttagtagt

SEQ ID NO: 13 - DNA, 16199 bp, synthetic construct
  misc_feature 1..16199: note = plasmid
  source 1..16199: mol_type = other DNA
tcgcgcgtttcggtgatgacggtgaaaacctctgacacatgcagctcccggagactgtcacagcttgtctgtaagcggatgccgggagcagacaagcccgtcagggcgcgtcagcgggtgttggcgggtgtcggggctggcttaactatgcggcatcagagcagattgtactgagagtgcaccatatgcggtgtgaaataccgcacagatgcgtaaggagaaaataccgcatcaggcgccattcgccattcaggctgcgcaactgttgggaagggcgatcggtgcgggcctcttcgctattacgccagctggcgaaagggggatgtgctgcaaggcgattaagttgggtaacgccagggttttcccagtcacgacgttgtaaaacgacggccagtgaattgacgcgtattgggattttactccctatcagtgatagagaacgtatgaagagtttactccctatcagtgatagagaacgtatgcagactttactccctatcagtgatagagaacgtataaggagtttactccctatcagtgatagagaacgtatgaccagtttactccctatcagtgatagagaacgtatctacagtttactccctatcagtgatagagaacgtatatccagtttactccctatcagtgatagagaacgtatgtcgaggtaggcgtgtacggtgggcgcctataaaagcagagctcgtttagtgaaccgtcagatcgcctggagcaattccacaacacttttgtcttatacttggtttagtgaaccgtcagatcagatctttgtcgatcctaccatccactcgacacacccgccagcggccgatgtcttttgttgatcaccctccagattggttggaagaagttggtgaaggtcttcgcgagtttttgggccttgaagcgggcccaccgaaaccaaaacccaatcagcagcatcaagatcaagcccgtggtcttgtgctgcctggttataactatctcggacccggaaacggtctcgatcgaggagagcctgtcaacagggcagacgaggtcgcgcgagagcacgacatctcgtacaacgagcagcttgaggcgggagacaacccctacctcaagtacaaccacgcggacgccgagtttcaggagaagctcgccgacgacacatccttcgggggaaacctcggaaaggcagtctttcaggccaagaaaagggttctcgaaccttttggcctggttgaagagggtgctaagacggcccctaccggaaagcggatagacgaccactttccaaaaagaaagaaggctcggaccgaagaggactccaagccttccacctcgtcagacgccgaagctggacccagcggatcccagcagctgcaaatcccagcccaaccagcctcaagtttgggagctgatacaatgtctgcgggaggtggcggcccattgggcgacaataaccaaggtgccgatggagtgggcaatgcctcgggagattggcattgcgattccacgtggatgggggacagagtcgtcaccaagtccacccgaacctgggtgctgcccagctacaacaaccaccagtaccgagagatcaaaagcggctccgtcgacggaagcaacgccaacgcctactttggatacagcaccccctgggggtactttgactttaaccgcttccacagccactggagcccccgagactggcaaagactcatcaacaactactggggcttcagaccccggtccctcagagtcaaaatcttcaacattcaagtcaaagaggtcacggtgcaggactccaccaccaccatcgccaacaacctcacctccaccgtccaagtgtttacggacgacgactaccagctgccctacgtcgtcggcaacgggaccgagggatgcctgccggccttccctccgcaggtctttacgctgccgcagtacggttacgcgacgctgaaccgcgacaacacagaaaatcccaccgagaggagcagcttcttctgcctagagtactttcccagcaagatgctgagaacgggcaacaactttgagtttacctacaactttgaggaggtgcccttccactccagcttcgctcccagtcagaacctgttcaagctggccaacccgctggtggaccagtacttgtaccgcttcgtgagcacaaataacactggcggagtccagttcaacaagaacctggccgggagatacgccaacacctacaaaaactggttcccggggcccatgggccgaacccagggctggaacctgggctccggggtcaaccgcgccagtgtcagcgccttcgccacgaccaataggatggagctcgagggcgcgagttaccaggtgcccccgcagccgaacggcatgaccaacaacctccagggcagcaacacctatgccctggagaacactatgatcttcaacagccagccggcgaacccgggcaccaccgccacgtacctcgagggcaacatgctcatcaccagcgagagcgagacgcagccggtgaaccgcgtggcgtacaacgtcggcgggcagatggccaccaacaaccagagctccaccactgcccccgcgaccggcacgtacaacctccaggaaatcgtgcccggcagcgtgtggatggagagggacgtgtacctccaaggacccatctgggccaagatcccagagacgggggcgcactttcacccctctccggccatgggcggattcggactcaaacacccaccgcccatgatgctcatcaagaacacgcctgtgcccggaaatatcaccagcttctcggacgtgcccgtcagcagcttcatcacccagtacagcaccgggcaggtcaccgtggagatggagtgggagctcaagaaggaaaactccaagaggtggaacccagagatccagtacacaaacaactacaacgacccccagtttgtggactttgccccggacagcaccggggaatacagaaccaccagacctatcggaacccgataccttacccgacccctttaacccgggagttctagggatctgcccctctccctcccccccccctaacgttactggccgaagccgcttggaataaggccggtgtgcgtttgtctatatgttattttccaccatattgccgtcttttggcaatgtgagggcccggaaacctggccctgtcttcttgacgagcattcctaggggtctttcccctctcgccaaaggaatgcaaggtctgttgaatgtcgtgaaggaagcagttcctctggaagcttcttgaagacaaacaacgtctgtagcgaccctttgcaggcagcggaaccccccacctggcgacaggtgcctctgcggccaaaagccacgtgtataagatacacctgcaaaggcggcacaaccccagtgccacgttgtgagttggatagttgtggaaagagtcaaatggctctcctcaagcgtattcaacaaggggctgaaggatgcccagaaggtaccccattgtatgggatctgatctggggcctcggtgcacatgctttacatgtgtttagtcgaggttaaaaaaacgtctaggccccccgaaccacggggacgtggttttcctttgaaaaacacgatgataaggatccaccggaggccaccatggccagtcgggaagaggagcagcgcgaaaccacccccgagcgcggacgcggtgcggcgcgacgtcccccaaccatggaggacgtgtcgtccccgtccccgtcgccgccgcctccccgggcgcccccaaaaaagcggatgaggcggcgtatcgagtccgaggacgaggaagactcatcacaagacgcgctggtgccgcgcacacccagcccgcggccatcgacctcggcggcggatttggccattgcgcccaagaagaaaaagaagcgcccttctcccaagcccgagcgcccgccatcaccagaggtaatcgtggacagcgaggaagaaagagaagatgtggcgctacaaatggtgggtttcagcaacccaccggtgctaatcaagcatggcaaaggaggtaagcgcacagtgcggcggctgaatgaagacgacccagtggcgcgtggtatgcggacgcaagaggaagaggaagagcccagcgaagcggaaagtgaaattacggtgatgaacccgctgagtgtgccgatcgtgtctgcgtgggagaagggcatggaggctgcgcgcgcgctgatggacaagtaccacgtggataacgatctaaaggcgaacttcaaactactgcctgaccaagtggaagctctggcggccgtatgcaagacctggctgaacgaggagcaccgcgggttgcagctgaccttcaccagcaacaagacctttgtgacgatgatggggcgattcctgcaggcgtacctgcagtcgtttgcagaggtgacctacaagcatcacgagcccacgggctgcgcgttgtggctgcaccgctgcgctgagatcgaaggcgagcttaagtgtctacacggaagcattatgataaataaggagcacgtgattgaaatggatgtgacgagcgaaaacgggcagcgcgcgctgaaggagcagtctagcaaggccaagatcgtgaagaaccggtggggccgaaatgtggtgcagatctccaacaccgacgcaaggtgctgcgtgcacgacgcggcctgtccggccaatcagttttccggcaagtcttgcggcatgttcttctctgaaggcgcaaaggctcaggtggcttttaagcagatcaaggcttttatgcaggcgctgtatcctaacgcccagaccgggcacggtcaccttttgatgccactacggtgcgagtgcaactcaaagcctgggcacgcgccctttttgggaaggcagctaccaaagttgactccgttcgccctgagcaacgcggaggacctggacgcggatctgatctccgacaagagcgtgctggccagcgtgcaccacccggcgctgatagtgttccagtgctgcaaccctgtgtatcgcaactcgcgcgcgcagggcggaggccccaactgcgacttcaagatatcggcgcccgacctgctaaacgcgttggtgatggtgcgcagcctgtggagtgaaaacttcaccgagctgccgcggatggttgtgcctgagtttaagtggagcactaaacaccagtatcgcaacgtgtccctgccagtggcgcatagcgatgcgcggcagaacccctttgatttttaacccgggagttctagggatctggcggccgctcgagtctagagggcccgtttaaacccgctgatcagcctcgactgtgccttctagttgccagccatctgttgtttgcccctcccccgtgccttccttgaccctggaaggtgccactcccactgtcctttcctaataaaatgaggaaattgcatcgcattgtctgagtaggtgtcattctattctggggggtggggtggggcaggacagcaagggggaggattgggaagacaatagcaggcatgctggggatgcggtgggctctatggtgaattccactttggccgcggctcgagggggacagcccccccccaaagcccccagggatgtaattacgtccctcccccgctagggggcagcagcgagccgcccggggctccgctccggtccggcgctccccccgcatccccgagccggcagcgtgcggggacagcccgggcacggggaaggtggcacgggatcgctttcctctgaacgcttctcgctgctctttgagcctgcagacacctggggggatacggggaaaaagctttaggctgagtgcacggggacagcccccccccaaagcccccagggatgtaattacgtccctcccccgctagggggcagcagcgagccgcccggggctccgctccggtccggcgctccccccgcatccccgagccggcagcgtgcggggacagcccgggcacggggaaggtggcacgggatcgctttcctctgaacgcttctcgctgctctttgagcctgcagacacctggggggatacggggaaaaagctttaggctgaaacttgtttattgcagcttataatggttacaaataaagcaatagcatcacaaatttcacaaataaagcatttttttcactgcattctagttgtggtttgtccaaactcatcaatgtatcttatcatgtctggatccccgcggccgcggtacccacgtgggcgcgccatttaaatgataactcagagagagtgtcctcgagccaatctggaagataaccatcggcagccatacctgatttaaatcatttattgttcaaagatgcagtcatccaaatccacattgaccagatcgcaggcagtgcaagcgtctggcacctttcccatgatatgatgaatgtagcacagtttctgatacgcctttttgacgacagaaacgggttgagattctgacacgggaaagcactctaaacagtctttctgtccgtgagtgaagcagatatttgaattctgattcattctctcgcattgtctgcagggaaacagcatcagattcatgcccacgtgacgagaacatttgttttggtacctgtctgcgtagttgatcgaagcttccgcgtctgacgtcgatggctgcgcaactgactcgcgcacccgtttgggctcacttatatctgcgtcactgggggcgggtcttttcttggctccaccctttttgacgtagaattcatgctccacctcaaccacgtgatcctttgcccaccggaaaaagtctttgacttcctgcttggtgaccttcccaaagtcatgatccagacggcgggtgagttcaaatttgaacatccggtcttgcaacggctgctggtgttcgaaggtcgttgagttcccgtcaatcacggcgcacatgttggtgttggaggtgacgatcacgggagtcgggtctatctgggccgaggacttgcatttctggtccacgcgcaccttgcttcctccgagaatggctttggccgactccacgaccttggcggtcatcttcccctcctcccaccagatcaccatcttgtcgacacagtcgttgaagggaaagttctcattggtccagtttacgcacccgtagaagggcacagtgtgggctatggcctccgcgatgttggtcttcccggtagttgcaggcccaaacagccagatggtgttcctcttgccgaactttttcgtggcccatcccagaaagacggaagccgcatattggggatcgtacccgtttagttccaaaattttataaatccgattgctggaaatgtcctccacgggctgctggcccaccaggtagtcgggggcggttttagtcaggctcataatctttcccgcattgtccaaggcagccttgatttgggaccgcgagttggaggccgcattgaaggagatgtatgaggcctggtcctcctggatccactgcttctccgaggtaatccccttgtccacgagccacccgaccagctccatgtacctggctgaagtttttgatctgatcaccggcgcatcagaattgggattctgattctctttgttctgctcctgcgtctgcgacacgtgcgtcagatgctgcgccaccaaccgtttacgctccgtgagattcaaacaggcgcttaaatactgttccatattagtccacgcccactggagctcaggctgggttttggggagcaagtaattggggatgtagcactcatccaccaccttgttcccgcctccggcgccatttctggtctttgtgaccgcgaaccagtttggcaaagtcggctcgatcccgcggtaaattctctgaatcagtttttcgcgaatctgactcaggaaacgtcccaaaaccatggatttcaccccggtggtttccacgagcacgtgcatgtggaagtagctctctcccttctcaaattgcacaaagaaaagggcctccggggccttactcacacggcgccattccgtcagaaagtcgcgctgcagcttctcggccacggtcaggggtgcctgctcaatcagattcagatccatgtcagaatctggcggcaactcccattccttctcggccacccagttcacaaagctgtcagaaatgccgggcagatgctcgtcaaggtcgctggggaccttaatcacaatctcgtaaaaccccggcatggcggcgataactattatcatcgtgtttttcaaaggaaaaccacgtccccgtggttcggggggcctagacgtttttttaacctcgactaaacacatgtaaagcatgtgcaccgaggccccagatcagatcccatacaatggggtaccttctgggcatccttcagccccttgttgaatacgcttgaggagagccatttgactctttccacaactatccaactcacaacgtggcactggggttgtgccgcctttgcaggtgtatcttatacacgtggcttttggccgcagaggcacctgtcgccaggtggggggttccgctgcctgcaaagggtcgctacagacgttgtttgtcttcaagaagcttccagaggaactgcttccttcacgacattcaacagaccttgcattcctttggcgagaggggaaagacccctaggaatgctcgtcaagaagacagggccaggtttccgggccctcacattgccaaaagacggcaatatggtggaaaataacatatagacaaacgcacaccggccttattccaagcggcttcggccagtaacgttagggggggggggcggaattctatccctcagttatctcagagagagtgtcctcgagccaatctggaagataaccatcggcagccatacctgatttaaatcatttattgttcaaagatgcagtcatccaaatccacattgaccagatcgcaggcagtgcaagcgtctggcacctttcccatgatatgatgaatgtagcacagtttctgatacgcctttttgacgacagaaacgggttgagattctgacacgggaaagcactctaaacagtctttctgtccgtgagtgaagcagatatttgaattctgattcattctctcgcattgtctgcagggaaacagcatcagattcatgcccacgtgacgagaacatttgttttggtacctgtctgcgtagttgatcgaagcttccgcgtctgacgtcgatggctgcgcaactgactcgcgcacccgtttgggctcacttatatctgcgtcactgggggcgggtcttttcttggctccaccctttttgacgtagaattcatgctccacctcaaccacgtgatcctttgcccaccggaaaaagtctttgacttcctgcttggtgaccttcccaaagtcatgatccagacggcgggtgagttcaaatttgaacatccggtcttgcaacggctgctggtgttcgaaggtcgttgagttcccgtcaatcacggcgcacatgttggtgttggaggtgacgatcacgggagtcgggtctatctgggccgaggacttgcatttctggtccacgcgcaccttgcttcctccgagaatggctttggccgactccacgaccttggcggtcatcttcccctcctcccaccagatcaccatcttgtcgacacagtcgttgaagggaaagttctcattggtccagtttacgcacccgtagaagggcacagtgtgggctatggcctccgcgatgttggtcttcccggtagttgcaggcccaaacagccagatggtgttcctcttgccgaactttttcgtggcccatcccagaaagacggaagccgcatattggggatcgtacccgtttagttccaaaattttataaatccgattgctggaaatgtcctccacgggctgctggcccaccaggtagtcgggggcggttttagtcaggctcataatctttcccgcattgtccaaggcagccttgatttgggaccgcgagttggaggccgcattgaaggagatgtatgaggcctggtcctcctggatccactgcttctccgaggtaatccccttgtccacgagccacccgaccagctccatggtggcgttatccggccgatcgatagatctgggccccggtgtcgactttacgagggtaggaagtggtacggaaagttggtataagacaaaagtgttgtggaattgctggaggcgatctgacggttcactaaacgagctctgcttttataggcgcccaccgtacacgcctaaagcttatacgttctctatcactgatagggagtaaactggatatacgttctctatcactgatagggagtaaactgtagatacgttctctatcactgatagggagtaaactggtcatacgttctctatcactgatagggagtaaactccttatacgttctctatcactgatagggagtaaagtctgcatacgttctctatcactgatagggagtaaactcttcatacgttctctatcactgatagggaatcccaatggcgcgccgagcttggcgtaatcatggtcatagctgtttcctggacattgattattgactagttattaatagtaatcaattacggggtcattagttcatagcccatatatggagttccgcgttacataacttacggtaaatggcccgcctggctgaccgcccaacgacccccgcccattgacgtcaataatgacgtatgttcccatagtaacgccaatagggactttccattgacgtcaatgggtggagtatttacggtaaactgcccacttggcagtacatcaagtgtatcatatgccaagtacgccccctattgacgtcaatgacggtaaatggcccgcctggcattatgcccagtacatgaccttatgggactttcctacttggcagtacatctacgtattagtcatcgctattaccatggtgatgcggttttggcagtacatcaatgggcgtggatagcggtttgactcacggggatttccaagtctccaccccattgacgtcaatgggagtttgttttggcaccaaaatcaacgggactttccaaaatgtcgtaacaactccgccccattgacgcaaatgggcggtaggcgtgtacggtgggaggtctatataagcagagctcgtttagtgaaccgtcagatcgcctggagacgccatccacgctgttttgacctccatagaagacaccgggaccgatccagcctccgcggccccgaattcaccatgtctagactggacaagagcaaagtcataaactctgctctggaattactcaatggagtcggtatcgaaggcctgacgacaaggaaactcgctcaaaagctgggagttgagcagcctaccctgtactggcacgtgaagaacaagcgggccctgctcgatgccctgccaatcgagatgctggacaggcatcatacccactcctgccccctggaaggcgagtcatggcaagactttctgcggaacaacgccaagtcataccgctgtgctctcctctcacatcgcgacggggctaaagtgcatctcggcacccgcccaacagagaaacagtacgaaaccctggaaaatcagctcgcgttcctgtgtcagcaaggcttctccctggagaacgcactgtacgctctgtccgccgtgggccactttacactgggctgcgtattggaggaacaggagcatcaagtagcaaaagaggaaagagagacacctaccaccgattctatgcccccacttctgaaacaagcaattgagctgttcgaccggcagggagccgaacctgccttccttttcggcctggaactaatcatatgtggcctggagaaacagctaaagtgcgaaagcggcgggccgaccgacgcccttgacgattttgacttagacatgctcccagccgatgcccttgacgactttgaccttgatatgctgcctgctgacgctcttgacgattttgaccttgacatgctccccgggtaaatcgatctgagaacttcagggtgagtttggggacccttgattgttctttctttttcgctattgtaaaattcatgttatatggagggggcaaagttttcagggtgttgtttagaatgggaagatgtcccttgtatcaccatggaccctcatgataattttgtttctttcactttctactctgttgacaaccattgtctcctcttattttcttttcattttctgtaactttttcgttaaactttagcttgcatttgtaacgaatttttaaattcacttttgtttatttgtcagattgtaagtactttctctaatcacttttttttcaaggcaatcagggtatattatattgtacttcagcacagttttagagaacaattgttataattaaatgataaggtagaatatttctgcatataaattctggctggcgtggaaatattcttattggtagaaacaactacaccctggtcatcatcctgcctttctctttatggttacaatgatatacactgtttgagatgaggataaaatactctgagtccaaaccgggcccctctgctaaccatgttcatgccttcttctctttcctacagctcctgggcaacgtgctggttgttgtgctgtctcatcattttggcaaagaattcactcctcaggtgcaggctgcctatcagaaggtggtggctggtgtggccaatgccctggctcacaaataccactgagatctttttccctctgccaaaaattatggggacatcatgaagccccttgagcatctgacttctggctaataaaggaaatttattttcattgcaatagtgtgttggaattttttgtgtctctcactctagagcggccgcggatccaattctaccgtgatgcggttttggcagtacatcaatgggcgtggatagcggtttgactcacggggatttccaagtctccaccccattgacgtcaatgggagtttgttttggcaccaaaatcaacgggactttccaaaatgtcgtaacaactccgccccattgacgcaaatgggcggtaggcgtgtacggtgggaggtctatataagcagagctcgtttagtgaaccgtcagatcgcctggagacgccatccacgctgttttgacctccatagaagattctagaatggcccttagtaagcacggcctgactaaggacatgaccatgaagtaccatatggagggctcggtggacgggcacaagttcgtgattacgggccacgggaacggcaacccattcgaggggaaacagacaatgaacctgtgtgtggtggaaggcggacccctgcccttctcggaggacatcctgtccgcaacctttgactacggcaatcgcgtgttcacagagtatccacagggtatggtggatttctttaagaacagctgtcccgcaggatacacctggcaccgcagcctgctcttcgaggacggggcggtgtgtaccacctccgctgatatcaccgtgtccgtcgaggagaactgcttctaccacaacagcaaattccacggcgtgaactttcctgccgacgggcctgtgatgaagaaaatgactacgaattgggagcccagctgcgagaaaatcatcccggtccctcgtcagggaatcttgaagggcgacatcgcaatgtacctcctgctcaaggacgggggaagataccgatgccagttcgataccatctacaaggcaaagtccgatcccaaggagatgccagagtggcacttcatccagcacaaactcacccgcgaggaccgctcagatgccaagaaccagaagtggcaactggtcgagcacgccgtggcatcccgtagcgccctgccagggtaattcgaatttaaatcggatccctgtgccttctagttgccagccatctgttgtttgcccctcccccgtgccttccttgaccctggaaggtgccactcccactgtcctttcctaataaaatgaggaaattgcatcgcattgtctgagtaggtgtcattctattctggggggtggggtggggcaggacagcaagggggaggattgggaagacaatagcaggcatgctggggatgcggtgggctctatggtgtgaaattgttatccgctcacaattccacacaacatacgagccggaagcataaagtgtaaagcctggggtgcctaatgagtgagctaactcacattaattgcgttgcgctcactgcccgctttccagtcgggaaacctgtcgtgccagctgcattaatgaatcggccaacgcgcggggagaggcggtttgcgtattgggcgctgttccgcttcctcgctcactgactcgctgcgctcggtcgttcggctgcggcgagcggtatcagctcactcaaaggcggtaatacggttatccacagaatcaggggataacgcaggaaagaacatgtgagcaaaaggccagcaaaaggccaggaaccgtaaaaaggccgcgttgctggcgtttttccataggctccgcccccctgacgagcatcacaaaaatcgacgctcaagtcagaggtggcgaaacccgacaggactataaagataccaggcgtttccccctggaagctccctcgtgcgctctcctgttccgaccctgccgcttaccggatacctgtccgcctttctcccttcgggaagcgtggcgctttctcatagctcacgctgtaggtatctcagttcggtgtaggtcgttcgctccaagctgggctgtgtgcacgaaccccccgttcagcccgaccgctgcgccttatccggtaactatcgtcttgagtccaacccggtaagacacgacttatcgccactggcagcagccactggtaacaggattagcagagcgaggtatgtaggcggtgctacagagttcttgaagtggtggcctaactacggctacactagaagaacagtatttggtatctgcgctctgctgaagccagttaccttcggaaaaagagttggtagctcttgatccggcaaacaaaccaccgctggtagcggtggtttttttgtttgcaagcagcagattacgcgcagaaaaaaaggatctcaagaagatcctttgatcttttctacggggtctgacgctcagtggaacgaaaactcacgttaagggattttggtcatgagattatcaaaaaggatcttcacctagatccttttaaattaaaaatgaagttttaaatcaatctaaagtatatatgagtaaacttggtctgacagttaccaatgcttaatcagtgaggcacctatctcagcgatctgtctatttcgttcatccatagttgcctgactccccgtcgtgtagataactacgatacgggagggcttaccatctggccccagtgctgcaatgataccgcgagaaccacgctcaccggctccagatttatcagcaataaaccagccagccggaagggccgagcgcagaagtggtcctgcaactttatccgcctccatccagtctattaattgttgccgggaagctagagtaagtagttcgccagttaatagtttgcgcaacgttgttgccattgctacaggcatcgtggtgtcacgctcgtcgtttggtatggcttcattcagctccggttcccaacgatcaaggcgagttacatgatcccccatgttgtgcaaaaaagcggttagctccttcggtcctccgatcgttgtcagaagtaagttggccgcagtgttatcactcatggttatggcagcactgcataattctcttactgtcatgccatccgtaagatgcttttctgtgactggtgagtactcaaccaagtcattctgagaatagtgtatgcggcgaccgagttgctcttgcccggcgtcaatacgggataataccgcgccacatagcagaactttaaaagtgctcatcattggaaaacgttcttcggggcgaaaactctcaaggatcttaccgctgttgagatccagttcgatgtaacccactcgtgcacccaactgatcttcagcatcttttactttcaccagcgtttctgggtgagcaaaaacaggaaggcaaaatgccgcaaaaaagggaataagggcgacacggaaatgttgaatactcatactcttcctttttcaatattattgaagcatttatcagggttattgtctcatgagcggatacatatttgaatgtatttagaaaaataaacaaataggggttccgcgcacatttccccgaaaagtgccacctgacgtctaagaaaccattattatcatgacattaacctataaaaataggcgtatcacgaggcccttttgtc

SEQ ID NO: 14 - DNA, 16897 bp, synthetic construct
  misc_feature 1..16897: note = plasmid
  source 1..16897: mol_type = other DNA
tcgcgcgtttcggtgatgacggtgaaaacctctgacacatgcagctcccggagactgtcacagcttgtctgtaagcggatgccgggagcagacaagcccgtcagggcgcgtcagcgggtgttggcgggtgtcggggctggcttaactatgcggcatcagagcagattgtactgagagtgcaccatatgcggtgtgaaataccgcacagatgcgtaaggagaaaataccgcatcaggcgccattcgccattcaggctgcgcaactgttgggaagggcgatcggtgcgggcctcttcgctattacgccagctggcgaaagggggatgtgctgcaaggcgattaagttgggtaacgccagggttttcccagtcacgacgttgtaaaacgacggccagtgaattgacgcgtattgggattttactccctatcagtgatagagaacgtatgaagagtttactccctatcagtgatagagaacgtatgcagactttactccctatcagtgatagagaacgtataaggagtttactccctatcagtgatagagaacgtatgaccagtttactccctatcagtgatagagaacgtatctacagtttactccctatcagtgatagagaacgtatatccagtttactccctatcagtgatagagaacgtatgtcgaggtaggcgtgtacggtgggcgcctataaaagcagagctcgtttagtgaaccgtcagatcgcctggagcaattccacaacacttttgtcttatacttggtttagtgaaccgtcagatcagatctttgtcgatcctaccatccactcgacacacccgccagcggccgatgtcttttgttgatcaccctccagattggttggaagaagttggtgaaggtcttcgcgagtttttgggccttgaagcgggcccaccgaaaccaaaacccaatcagcagcatcaagatcaagcccgtggtcttgtgctgcctggttataactatctcggacccggaaacggtctcgatcgaggagagcctgtcaacagggcagacgaggtcgcgcgagagcacgacatctcgtacaacgagcagcttgaggcgggagacaacccctacctcaagtacaaccacgcggacgccgagtttcaggagaagctcgccgacgacacatccttcgggggaaacctcggaaaggcagtctttcaggccaagaaaagggttctcgaaccttttggcctggttgaagagggtgctaagacggcccctaccggaaagcggatagacgaccactttccaaaaagaaagaaggctcggaccgaagaggactccaagccttccacctcgtcagacgccgaagctggacccagcggatcccagcagctgcaaatcccagcccaaccagcctcaagtttgggagctgatacaatgtctgcgggaggtggcggcccattgggcgacaataaccaaggtgccgatggagtgggcaatgcctcgggagattggcattgcgattccacgtggatgggggacagagtcgtcaccaagtccacccgaacctgggtgctgcccagctacaacaaccaccagtaccgagagatcaaaagcggctccgtcgacggaagcaacgccaacgcctactttggatacagcaccccctgggggtactttgactttaaccgcttccacagccactggagcccccgagactggcaaagactcatcaacaactactggggcttcagaccccggtccctcagagtcaaaatcttcaacattcaagtcaaagaggtcacggtgcaggactccaccaccaccatcgccaacaacctcacctccaccgtccaagtgtttacggacgacgactaccagctgccctacgtcgtcggcaacgggaccgagggatgcctgccggccttccctccgcaggtctttacgctgccgcagtacggttacgcgacgctgaaccgcgacaacacagaaaatcccaccgagaggagcagcttcttctgcctagagtactttcccagcaagatgctgagaacgggcaacaactttgagtttacctacaactttgaggaggtgcccttccactccagcttcgctcccagtcagaacctgttcaagctggccaacccgctggtggaccagtacttgtaccgcttcgtgagcacaaataacactggcggagtccagttcaacaagaacctggccgggagatacgccaacacctacaaaaactggttcccggggcccatgggccgaacccagggctggaacctgggctccggggtcaaccgcgccagtgtcagcgccttcgccacgaccaataggatggagctcgagggcgcgagttaccaggtgcccccgcagccgaacggcatgaccaacaacctccagggcagcaacacctatgccctggagaacactatgatcttcaacagccagccggcgaacccgggcaccaccgccacgtacctcgagggcaacatgctcatcaccagcgagagcgagacgcagccggtgaaccgcgtggcgtacaacgtcggcgggcagatggccaccaacaaccagagctccaccactgcccccgcgaccggcacgtacaacctccaggaaatcgtgcccggcagcgtgtggatggagagggacgtgtacctccaaggacccatctgggccaagatcccagagacgggggcgcactttcacccctctccggccatgggcggattcggactcaaacacccaccgcccatgatgctcatcaagaacacgcctgtgcccggaaatatcaccagcttctcggacgtgcccgtcagcagcttcatcacccagtacagcaccgggcaggtcaccgtggagatggagtgggagctcaagaaggaaaactccaagaggtggaacccagagatccagtacacaaacaactacaacgacccccagtttgtggactttgccccggacagcaccggggaatacagaaccaccagacctatcggaacccgataccttacccgacccctttaacccgggagttctagggatctgcccctctccctcccccccccctaacgttactggccgaagccgcttggaataaggccggtgtgcgtttgtctatatgttattttccaccatattgccgtcttttggcaatgtgagggcccggaaacctggccctgtcttcttgacgagcattcctaggggtctttcccctctcgccaaaggaatgcaaggtctgttgaatgtcgtgaaggaagcagttcctctggaagcttcttgaagacaaacaacgtctgtagcgaccctttgcaggcagcggaaccccccacctggcgacaggtgcctctgcggccaaaagccacgtgtataagatacacctgcaaaggcggcacaaccccagtgccacgttgtgagttggatagttgtggaaagagtcaaatggctctcctcaagcgtattcaacaaggggctgaaggatgcccagaaggtaccccattgtatgggatctgatctggggcctcggtgcacatgctttacatgtgtttagtcgaggttaaaaaaacgtctaggccccccgaaccacggggacgtggttttcctttgaaaaacacgatgataaggatccaccggaggccaccatggccagtcgggaagaggagcagcgcgaaaccacccccgagcgcggacgcggtgcggcgcgacgtcccccaaccatggaggacgtgtcgtccccgtccccgtcgccgccgcctccccgggcgcccccaaaaaagcggatgaggcggcgtatcgagtccgaggacgaggaagactcatcacaagacgcgctggtgccgcgcacacccagcccgcggccatcgacctcggcggcggatttggccattgcgcccaagaagaaaaagaagcgcccttctcccaagcccgagcgcccgccatcaccagaggtaatcgtggacagcgaggaagaaagagaagatgtggcgctacaaatggtgggtttcagcaacccaccggtgctaatcaagcatggcaaaggaggtaagcgcacagtgcggcggctgaatgaagacgacccagtggcgcgtggtatgcggacgcaagaggaagaggaagagcccagcgaagcggaaagtgaaattacggtgatgaacccgctgagtgtgccgatcgtgtctgcgtgggagaagggcatggaggctgcgcgcgcgctgatggacaagtaccacgtggataacgatctaaaggcgaacttcaaactactgcctgaccaagtggaagctctggcggccgtatgcaagacctggctgaacgaggagcaccgcgggttgcagctgaccttcaccagcaacaagacctttgtgacgatgatggggcgattcctgcaggcgtacctgcagtcgtttgcagaggtgacctacaagcatcacgagcccacgggctgcgcgttgtggctgcaccgctgcgctgagatcgaaggcgagcttaagtgtctacacggaagcattatgataaataaggagcacgtgattgaaatggatgtgacgagcgaaaacgggcagcgcgcgctgaaggagcagtctagcaaggccaagatcgtgaagaaccggtggggccgaaatgtggtgcagatctccaacaccgacgcaaggtgctgcgtgcacgacgcggcctgtccggccaatcagttttccggcaagtcttgcggcatgttcttctctgaaggcgcaaaggctcaggtggcttttaagcagatcaaggcttttatgcaggcgctgtatcctaacgcccagaccgggcacggtcaccttttgatgccactacggtgcgagtgcaactcaaagcctgggcacgcgccctttttgggaaggcagctaccaaagttgactccgttcgccctgagcaacgcggaggacctggacgcggatctgatctccgacaagagcgtgctggccagcgtgcaccacccggcgctgatagtgttccagtgctgcaaccctgtgtatcgcaactcgcgcgcgcagggcggaggccccaactgcgacttcaagatatcggcgcccgacctgctaaacgcgttggtgatggtgcgcagcctgtggagtgaaaacttcaccgagctgccgcggatggttgtgcctgagtttaagtggagcactaaacaccagtatcgcaacgtgtccctgccagtggcgcatagcgatgcgcggcagaacccctttgatttttaacccgggagttctagggatctggcggccgctcgagtctagagggcccgtttaaacccgctgatcagcctcgactgtgccttctagttgccagccatctgttgtttgcccctcccccgtgccttccttgaccctggaaggtgccactcccactgtcctttcctaataaaatgaggaaattgcatcgcattgtctgagtaggtgtcattctattctggggggtggggtggggcaggacagcaagggggaggattgggaagacaatagcaggcatgctggggatgcggtgggctctatggtgaattccactttggccgcggctcgagggggacagcccccccccaaagcccccagggatgtaattacgtccctcccccgctagggggcagcagcgagccgcccggggctccgctccggtccggcgctccccccgcatccccgagccggcagcgtgcggggacagcccgggcacggggaaggtggcacgggatcgctttcctctgaacgcttctcgctgctctttgagcctgcagacacctggggggatacggggaaaaagctttaggctgagtgcacggggacagcccccccccaaagcccccagggatgtaattacgtccctcccccgctagggggcagcagcgagccgcccggggctccgctccggtccggcgctccccccgcatccccgagccggcagcgtgcggggacagcccgggcacggggaaggtggcacgggatcgctttcctctgaacgcttctcgctgctctttgagcctgcagacacctggggggatacggggaaaaagctttaggctgaaacttgtttattgcagcttataatggttacaaataaagcaatagcatcacaaatttcacaaataaagcatttttttcactgcattctagttgtggtttgtccaaactcatcaatgtatcttatcatgtctggatccccgcggccgcggtacccacgtgggcgcgccatttaaatgataactcagagagagtgtcctcgagccaatctggaagataaccatcggcagccatacctgatttaaatcatttattgttcaaagatgcagtcatccaaatccacattgaccagatcgcaggcagtgcaagcgtctggcacctttcccatgatatgatgaatgtagcacagtttctgatacgcctttttgacgacagaaacgggttgagattctgacacgggaaagcactctaaacagtctttctgtccgtgagtgaagcagatatttgaattctgattcattctctcgcattgtctgcagggaaacagcatcagattcatgcccacgtgacgagaacatttgttttggtacctgtctgcgtagttgatcgaagcttccgcgtctgacgtcgatggctgcgcaactgactcgcgcacccgtttgggctcacttatatctgcgtcactgggggcgggtcttttcttggctccaccctttttgacgtagaattcatgctccacctcaaccacgtgatcctttgcccaccggaaaaagtctttgacttcctgcttggtgaccttcccaaagtcatgatccagacggcgggtgagttcaaatttgaacatccggtcttgcaacggctgctggtgttcgaaggtcgttgagttcccgtcaatcacggcgcacatgttggtgttggaggtgacgatcacgggagtcgggtctatctgggccgaggacttgcatttctggtccacgcgcaccttgcttcctccgagaatggctttggccgactccacgaccttggcggtcatcttcccctcctcccaccagatcaccatcttgtcgacacagtcgttgaagggaaagttctcattggtccagtttacgcacccgtagaagggcacagtgtgggctatggcctccgcgatgttggtcttcccggtagttgcaggcccaaacagccagatggtgttcctcttgccgaactttttcgtggcccatcccagaaagacggaagccgcatattggggatcgtacccgtttagttccaaaattttataaatccgattgctggaaatgtcctccacgggctgctggcccaccaggtagtcgggggcggttttagtcaggctcataatctttcccgcattgtccaaggcagccttgatttgggaccgcgagttggaggccgcattgaaggagatgtatgaggcctggtcctcctggatccactgcttctccgaggtaatccccttgtccacgagccacccgaccagctccatgtacctggctgaagtttttgatctgatcaccggcgcatcagaattgggattctgattctctttgttctgctcctgcgtctgcgacacgtgcgtcagatgctgcgccaccaaccgtttacgctccgtgagattcaaacaggcgcttaaatactgttccatattagtccacgcccactggagctcaggctgggttttggggagcaagtaattggggatgtagcactcatccaccaccttgttcccgcctccggcgccatttctggtctttgtgaccgcgaaccagtttggcaaagtcggctcgatcccgcggtaaattctctgaatcagtttttcgcgaatctgactcaggaaacgtcccaaaaccatggatttcaccccggtggtttccacgagcacgtgcatgtggaagtagctctctcccttctcaaattgcacaaagaaaagggcctccggggccttactcacacggcgccattccgtcagaaagtcgcgctgcagcttctcggccacggtcaggggtgcctgctcaatcagattcagatccatgtcagaatctggcggcaactcccattccttctcggccacccagttcacaaagctgtcagaaatgccgggcagatgctcgtcaaggtcgctggggaccttaatcacaatctcgtaaaaccccggcatggcggcgataactattatcatcgtgtttttcaaaggaaaaccacgtccccgtggttcggggggcctagacgtttttttaacctcgactaaacacatgtaaagcatgtgcaccgaggccccagatcagatcccatacaatggggtaccttctgggcatccttcagccccttgttgaatacgcttgaggagagccatttgactctttccacaactatccaactcacaacgtggcactggggttgtgccgcctttgcaggtgtatcttatacacgtggcttttggccgcagaggcacctgtcgccaggtggggggttccgctgcctgcaaagggtcgctacagacgttgtttgtcttcaagaagcttccagaggaactgcttccttcacgacattcaacagaccttgcattcctttggcgagaggggaaagacccctaggaatgctcgtcaagaagacagggccaggtttccgggccctcacattgccaaaagacggcaatatggtggaaaataacatatagacaaacgcacaccggccttattccaagcggcttcggccagtaacgttagggggggggggcggaattctatccctcagttatctcagagagagtgtcctcgagccaatctggaagataaccatcggcagccatacctgatttaaatcatttattgttcaaagatgcagtcatccaaatccacattgaccagatcgcaggcagtgcaagcgtctggcacctttcccatgatatgatgaatgtagcacagtttctgatacgcctttttgacgacagaaacgggttgagattctgacacgggaaagcactctaaacagtctttctgtccgtgagtgaagcagatatttgaattctgattcattctctcgcattgtctgcagggaaacagcatcagattcatgcccacgtgacgagaacatttgttttggtacctgtctgcgtagttgatcgaagcttccgcgtctgacgtcgatggctgcgcaactgactcgcgcacccgtttgggctcacttatatctgcgtcactgggggcgggtcttttcttggctccaccctttttgacgtagaattcatgctccacctcaaccacgtgatcctttgcccaccggaaaaagtctttgacttcctgcttggtgaccttcccaaagtcatgatccagacggcgggtgagttcaaatttgaacatccggtcttgcaacggctgctggtgttcgaaggtcgttgagttcccgtcaatcacggcgcacatgttggtgttggaggtgacgatcacgggagtcgggtctatctgggccgaggacttgcatttctggtccacgcgcaccttgcttcctccgagaatggctttggccgactccacgaccttggcggtcatcttcccctcctcccaccagatcaccatcttgtcgacacagtcgttgaagggaaagttctcattggtccagtttacgcacccgtagaagggcacagtgtgggctatggcctccgcgatgttggtcttcccggtagttgcaggcccaaacagccagatggtgttcctcttgccgaactttttcgtggcccatcccagaaagacggaagccgcatattggggatcgtacccgtttagttccaaaattttataaatccgattgctggaaatgtcctccacgggctgctggcccaccaggtagtcgggggcggttttagtcaggctcataatctttcccgcattgtccaaggcagccttgatttgggaccgcgagttggaggccgcattgaaggagatgtatgaggcctggtcctcctggatccactgcttctccgaggtaatccccttgtccacgagccacccgaccagctccatggtggcgttatccggccgatcgatagatctgggccccggtgtcgactttacgagggtaggaagtggtacggaaagttggtataagacaaaagtgttgtggaattgctggaggcgatctgacggttcactaaacgagctctgcttttataggcgcccaccgtacacgcctaaagcttatacgttctctatcactgatagggagtaaactggatatacgttctctatcactgatagggagtaaactgtagatacgttctctatcactgatagggagtaaactggtcatacgttctctatcactgatagggagtaaactccttatacgttctctatcactgatagggagtaaagtctgcatacgttctctatcactgatagggagtaaactcttcatacgttctctatcactgatagggaatcccaatggcgcgccgagcttggcgtaatcatggtcatagctgtttcctggacattgattattgactagttattaatagtaatcaattacggggtcattagttcatagcccatatatggagttccgcgttacataacttacggtaaatggcccgcctggctgaccgcccaacgacccccgcccattgacgtcaataatgacgtatgttcccatagtaacgccaatagggactttccattgacgtcaatgggtggagtatttacggtaaactgcccacttggcagtacatcaagtgtatcatatgccaagtacgccccctattgacgtcaatgacggtaaatggcccgcctggcattatgcccagtacatgaccttatgggactttcctacttggcagtacatctacgtattagtcatcgctattaccatggtgatgcggttttggcagtacatcaatgggcgtggatagcggtttgactcacggggatttccaagtctccaccccattgacgtcaatgggagtttgttttggcaccaaaatcaacgggactttccaaaatgtcgtaacaactccgccccattgacgcaaatgggcggtaggcgtgtacggtgggaggtctatataagcagagctcgtttagtgaaccgtcagatcgcctggagacgccatccacgctgttttgacctccatagaagacaccgggaccgatccagcctccgcggccccgaattcaccatgtctagactggacaagagcaaagtcataaactctgctctggaattactcaatggagtcggtatcgaaggcctgacgacaaggaaactcgctcaaaagctgggagttgagcagcctaccctgtactggcacgtgaagaacaagcgggccctgctcgatgccctgccaatcgagatgctggacaggcatcatacccactcctgccccctggaaggcgagtcatggcaagactttctgcggaacaacgccaagtcataccgctgtgctctcctctcacatcgcgacggggctaaagtgcatctcggcacccgcccaacagagaaacagtacgaaaccctggaaaatcagctcgcgttcctgtgtcagcaaggcttctccctggagaacgcactgtacgctctgtccgccgtgggccactttacactgggctgcgtattggaggaacaggagcatcaagtagcaaaagaggaaagagagacacctaccaccgattctatgcccccacttctgaaacaagcaattgagctgttcgaccggcagggagccgaacctgccttccttttcggcctggaactaatcatatgtggcctggagaaacagctaaagtgcgaaagcggcgggccgaccgacgcccttgacgattttgacttagacatgctcccagccgatgcccttgacgactttgaccttgatatgctgcctgctgacgctcttgacgattttgaccttgacatgctccccgggtaaatcgatctgagaacttcagggtgagtttggggacccttgattgttctttctttttcgctattgtaaaattcatgttatatggagggggcaaagttttcagggtgttgtttagaatgggaagatgtcccttgtatcaccatggaccctcatgataattttgtttctttcactttctactctgttgacaaccattgtctcctcttattttcttttcattttctgtaactttttcgttaaactttagcttgcatttgtaacgaatttttaaattcacttttgtttatttgtcagattgtaagtactttctctaatcacttttttttcaaggcaatcagggtatattatattgtacttcagcacagttttagagaacaattgttataattaaatgataaggtagaatatttctgcatataaattctggctggcgtggaaatattcttattggtagaaacaactacaccctggtcatcatcctgcctttctctttatggttacaatgatatacactgtttgagatgaggataaaatactctgagtccaaaccgggcccctctgctaaccatgttcatgccttcttctctttcctacagctcctgggcaacgtgctggttgttgtgctgtctcatcattttggcaaagaattcactcctcaggtgcaggctgcctatcagaaggtggtggctggtgtggccaatgccctggctcacaaataccactgagatctttttccctctgccaaaaattatggggacatcatgaagccccttgagcatctgacttctggctaataaaggaaatttattttcattgcaatagtgtgttggaattttttgtgtctctcactctagagcggccgcggatccaattctaccgggtaggggaggcgcttttcccaaggcagtctggagcatgcgctttagcagccccgctgggcacttggcgctacacaagtggcctctggcctcgcacacattccacatccaccggtaggcgccaaccggctccgttctttggtggccccttcgcgccaccttctactcctcccctagtcaggaagttcccccccgccccgcagctcgcgtcgtgcaggacgtgacaaatggaagtagcacgtctcactagtctcgtgcagatggacagcaccgctgagcaatggaagcgggtaggcctttggggcagcggccaatagcagctttgctccttcgctttctgggctcagaggctgggaaggggtgggtccgggggcgggctcaggggcgggctcaggggcggggcgggcgcccgaaggtcctccggaggcccggcattctgcacgcttcaaaagcgcacgtctgccgcgctgttctcctcttcctcatctccgggcctttcgacctgcagttaacgccgccatggctgaacaagatggattgcacgcaggttctccggccgcttgggtggagaggctattcggctatgactgggcacaacagacaatcggctgctctgatgccgccgtgttccggctgtcagcgcaggggcgcccggttctttttgtcaagaccgacctgtccggtgccctgaatgaactgcaggacgaggcagcgcggctatcgtggctggccacgacgggcgttccttgcgcagctgtgctcgacgttgtcactgaagcgggaagggactggctgctattgggcgaagtgccggggcaggatctcctgtcatctcaccttgctcctgccgagaaagtatccatcatggctgatgcaatgcggcggctgcatacgcttgatccggctacctgcccattcgaccaccaagcgaaacatcgcatcgagcgagcacgtactcggatggaagccggtcttgtcgatcaggatgatctggacgaagagcatcaggggctcgcgccagccgaactgttcgccaggctcaaggcgcgcatgcccgacggcgaggatctcgtcgtgacccatggcgatgcctgcttgccgaatatcatggtggaaaatggccgcttttctggattcatcgactgtggccggctgggtgtggcggaccgctatcaggacatagcgttggctacccgtgatattgctgaagagcttggcggcgaatgggctgaccgcttcctcgtgctttacggtatcgccgctcccgattcgcagcgcatcgccttctatcgccttcttgacgagttcttctgaacgcgtctggaacaatcaacctctggattacaaaatttgtgaaagattgactggtattcttaactatgttgctccttttacgctatgtggatacgctgctttaatgcctttgtatcatgctattgcttcccgtatggctttcattttctcctccttgtataaatcctggttgctgtctctttatgaggagttgtggcccgttgtcaggcaacgtggcgtggtgtgcactgtgtttgctgacgcaacccccactggttggggcattgccaccacctgtcagctcctttccgggactttcgctttccccctccctattgccacggcggaactcatcgccgcctgccttgcccgctgctggacaggggctcggctgttgggcactgacaattccgtggtgttgtcggggaagctgacgtcctttccatggctgctcgcctgtgttgccacctggattctgcgcgggacgtccttctgctacgtcccttcggccctcaatccagcggaccttccttcccgcggcctgctgccggctctgcggcctcttccgcgtcttcgccttcgccctcagacgagtcggatctccctttgggccgcctccccgctgtgaaattgttatccgctcacaattccacacaacatacgagccggaagcataaagtgtaaagcctggggtgcctaatgagtgagctaactcacattaattgcgttgcgctcactgcccgctttccagtcgggaaacctgtcgtgccagctgcattaatgaatcggccaacgcgcggggagaggcggtttgcgtattgggcgctgttccgcttcctcgctcactgactcgctgcgctcggtcgttcggctgcggcgagcggtatcagctcactcaaaggcggtaatacggttatccacagaatcaggggataacgcaggaaagaacatgtgagcaaaaggccagcaaaaggccaggaaccgtaaaaaggccgcgttgctggcgtttttccataggctccgcccccctgacgagcatcacaaaaatcgacgctcaagtcagaggtggcgaaacccgacaggactataaagataccaggcgtttccccctggaagctccctcgtgcgctctcctgttccgaccctgccgcttaccggatacctgtccgcctttctcccttcgggaagcgtggcgctttctcatagctcacgctgtaggtatctcagttcggtgtaggtcgttcgctccaagctgggctgtgtgcacgaaccccccgttcagcccgaccgctgcgccttatccggtaactatcgtcttgagtccaacccggtaagacacgacttatcgccactggcagcagccactggtaacaggattagcagagcgaggtatgtaggcggtgctacagagttcttgaagtggtggcctaactacggctacactagaagaacagtatttggtatctgcgctctgctgaagccagttaccttcggaaaaagagttggtagctcttgatccggcaaacaaaccaccgctggtagcggtggtttttttgtttgcaagcagcagattacgcgcagaaaaaaaggatctcaagaagatcctttgatcttttctacggggtctgacgctcagtggaacgaaaactcacgttaagggattttggtcatgagattatcaaaaaggatcttcacctagatccttttaaattaaaaatgaagttttaaatcaatctaaagtatatatgagtaaacttggtctgacagttaccaatgcttaatcagtgaggcacctatctcagcgatctgtctatttcgttcatccatagttgcctgactccccgtcgtgtagataactacgatacgggagggcttaccatctggccccagtgctgcaatgataccgcgagaaccacgctcaccggctccagatttatcagcaataaaccagccagccggaagggccgagcgcagaagtggtcctgcaactttatccgcctccatccagtctattaattgttgccgggaagctagagtaagtagttcgccagttaatagtttgcgcaacgttgttgccattgctacaggcatcgtggtgtcacgctcgtcgtttggtatggcttcattcagctccggttcccaacgatcaaggcgagttacatgatcccccatgttgtgcaaaaaagcggttagctccttcggtcctccgatcgttgtcagaagtaagttggccgcagtgttatcactcatggttatggcagcactgcataattctcttactgtcatgccatccgtaagatgcttttctgtgactggtgagtactcaaccaagtcattctgagaatagtgtatgcggcgaccgagttgctcttgcccggcgtcaatacgggataataccgcgccacatagcagaactttaaaagtgctcatcattggaaaacgttcttcggggcgaaaactctcaaggatcttaccgctgttgagatccagttcgatgtaacccactcgtgcacccaactgatcttcagcatcttttactttcaccagcgtttctgggtgagcaaaaacaggaaggcaaaatgccgcaaaaaagggaataagggcgacacggaaatgttgaatactcatactcttcctttttcaatattattgaagcatttatcagggttattgtctcatgagcggatacatatttgaatgtatttagaaaaataaacaaataggggttccgcgcacatttccccgaaaagtgccacctgacgtctaagaaaccattattatcatgacattaacctataaaaataggcgtatcacgaggcccttttgtc

SEQ ID NO: 15 - DNA, 21 bp, synthetic construct
  misc_feature 1..21: note = primer
  source 1..21: mol_type = other DNA
ggaacccctagtgatggagtt

SEQ ID NO: 16 - DNA, 16 bp, synthetic construct
  misc_feature 1..16: note = primer
  source 1..16: mol_type = other DNA
cggcctcagtgagcga

SEQ ID NO: 17 - DNA, 21 bp, synthetic construct
  misc_feature 1..21: note = probe
  source 1..21: mol_type = other DNA
cactccctctctgcgcgctcg

SEQ ID NO: 18 - DNA, 22048 bp, synthetic construct
  misc_feature 1..22048: note = plasmid
  source 1..22048: mol_type = other DNA
atgactctcttaaggtagccaaatttccataggctccgcccccctgacgagcatcacaaaaatcgacgctcaagtcagaggtggcgaaacccgacaggactataaagataccaggcgtttccccctggaagctccctcgtgcgctctcctgttccgaccctgccgcttaccggatacctgtccgcctttctcccttcgggaagcgtggcgctttctcatagctcacgctgtaggtatctcagttcggtgtaggtcgttcgctccaagctgggctgtgtgcacgaaccccccgttcagcccgaccgctgcgccttatccggtaactatcgtcttgagtccaacccggtaagacacgacttatcgccactggcagcagccactggtaacaggattagcagagcgaggtatgtaggcggtgctacagagttcttgaagtggtggcctaactacggctacactagaaggacagtatttggtatctgcgctctgctgaagccagttaccttcggaaaaagagttggtagctcttgatccggcaaacaaaccaccgctggtagcggtggtttttttgtttgcaagcagcagattacgcgcagaaaaaaaggatctcaagaagatcctttgatcttttctacggggtctgacgctcagtggaacgaaaactcacgttaagggattttggtcatgagattatcaaaaaggatcttcacctagatccttttaaattaaaaatgaagttttaaatcaatctaaagtatatatgagtaaacttggtctgacagttaccaatgcttaatcagtgaggcacctatctcagcgatctgtctatttcgttcatccatagttgcctgactccccgtcgtgtagataactacgatacgggagggcttaccatctggccccagtgctgcaatgataccgcgagacccacgctcaccggctccagatttatcagcaataaaccagccagccggaagggccgagcgcagaagtggtcctgcaactttatccgcctccatccagtctattaattgttgccgggaagctagagtaagtagttcgccagttaatagtttgcgcaacgttgttgccattgctacaggcatcgtggtgtcacgctcgtcgtttggtatggcttcattcagctccggttcccaacgatcaaggcgagttacatgatcccccatgttgtgcaaaaaagcggttagctccttcggtcctccgatcgttgtcagaagtaagttggccgcagtgttatcactcatggttatggcagcactgcataattctcttactgtcatgccatccgtaagatgcttttctgtgactggtgagtactcaaccaagtcattctgagaatagtgtatgcggcgaccgagttgctcttgcccggcgtcaatacgggataataccgcgccacatagcagaactttaaaagtgctcatcattggaaaacgttcttcggggcgaaaactctcaaggatcttaccgctgttgagatccagttcgatgtaacccactcgtgcacccaactgatcttcagcatcttttactttcaccagcgtttctgggtgagcaaaaacaggaaggcaaaatgccgcaaaaaagggaataagggcgacacggaaatgttgaatactcatactcttcctttttcaatattattgaagcatttatcagggttattgtctcatgagcggatacatatttgaatgtatttagaaaaataaacaaataggggttccgcgcacatttccccgaaaagtgccacctaaattgtaagcgttaatattttgttaaaattcgcgttaaatttttgttaaatcagctcattttttaaccaataggccgaaatcggcaaaatcccttataaatcaaaagaatagaccgagatagggttgagtgttgttccagtttggaacaagagtccactattaaagaacgtggactccaacgtcaaagggcgaaaaaccgtctatcagggcgatggcccactacgtgaaccatcaccctaatcaagttttttggggtcgaggtgccgtaaagcactaaatcggaaccctaaagggagcccccgatttagagcttgacggggaaagccggcgaacgtggcgagaaaggaagggaagaaagcgaaaggagcgggcgctagggcgctggcaagtgtagcggtcacgctgcgcgtaaccaccacacccgccgcgcttaatgcgccgctacagggcgcgtcccattcgccattcaggctgcgcaactgttgggaagggcgatcggtgcgggcctcttcgctattacgccagctggcgaaagggggatgtgctgcaaggcgattaagttgggtaacgccagggttttcccagtcacgacgttaccccacagtggggccactagggtcaatttctgagaactgtcattctcggaaattgagtaaaacgacggccagtgagcgcgcctcgttcattcacgtttttgaacccgtggaggacgggcagactcgcggtgcaaatgtgttttacagcgtgatggagcagatgaagatgctcgacacgctgcagaacacgcagctagattaaccctagaaagataatcatattgtgacgtacgttaaagataatcatgcgtaaaattgacgcatgtgttttatcggtctgtatatcgaggtttatttattaatttgaatagatattaagttttattatatttacacttacatactaataataaattcaacaaacaatttatttatgtttatttatttattaaaaaaaaacaaaaactcaaaatttcttctataaagtaacaaaacttttatcgaattcctgcagcccgggggatccactagttctagagggacagcccccccccaaagcccccagggatgtaattacgtccctcccccgctagggggcagcagcgagccgcccggggctccgctccggtccggcgctccccccgcatccccgagccggcagcgtgcggggacagcccgggcacggggaaggtggcacgggatcgctttcctctgaacgcttctcgctgctctttgagcctgcagacacctggggggatacggggaaaaggcctccaaggccagcttcccacaataagttgggtgaattttggctcattcctcctttctataggattgaggtcagagctttgtgatgggaattctgtggaatgtgtgtcagttagggtgtggaaagtccctttactccctatcagtgatagagaacgtatgaagagtttactccctatcagtgatagagaacgtatgcagactttactccctatcagtgatagagaacgtataaggagtttactccctatcagtgatagagaacgtatgaccagtttactccctatcagtgatagagaacgtatctacagtttactccctatcagtgatagagaacgtatatccagtttactccctatcagtgatagagaacgtataagctttaggcgtgtacggtgggcgcctataaaagcagagctcgtttagtgaaccgtcagatcgcctccagcaattccacaacacttttgtcttataccaactttccgtaccacttcctaccctcgtaaagtcgacaccggggcccagatctatcgatcggccggataacgccaccatggagctggtcgggtggctcgtggacaaggggattacctcggagaagcagtggatccaggaggaccaggcctcatacatctccttcaatgcggcctccaactcgcggtcccaaatcaaggctgccttggacaatgcgggaaagattatgagcctgactaaaaccgcccccgactacctggtgggccagcagcccgtggaggacatttccagcaatcggatttataaaattttggaactaaacgggtacgatccccaatatgcggcttccgtctttctgggatgggccacgaaaaagttcggcaagaggaacaccatctggctgtttgggcctgcaactaccgggaagaccaacatcgcggaggccatagcccacactgtgcccttctacgggtgcgtaaactggaccaatgagaactttcccttcaacgactgtgtcgacaagatggtgatctggtgggaggaggggaagatgaccgccaaggtcgtggagtcggccaaagccattctcggaggaagcaaggtgcgcgtggaccagaaatgcaagtcctcggcccagatagacccgactcccgtgatcgtcacctccaacaccaacatgtgcgccgtgattgacgggaactcaacgaccttcgaacaccagcagccgttgcaagaccggatgttcaaatttgaactcacccgccgtctggatcatgactttgggaaggtcaccaagcaggaagtcaaagactttttccggtgggcaaaggatcacgtggttgaggtggagcatgaattctacgtcaaaaagggtggagccaagaaaagacccgcccccagtgacgcagatataagtgagcccaaacgggtgcgcgagtcagttgcgcagccatcgacgtcagacgcggaagcttcgatcaactacgcagacaggtaccaaaacaaatgttctcgtcacgtgggcatgaatctgatgctgtttccctgcagacaatgcgagagaatgaatcagaattcaaatatctgcttcactcacggacagaaagactgtttagagtgctttcccgtgtcagaatctcaacccgtttctgtcgtcaaaaaggcgtatcagaaactgtgctacattcatcatatcatgggaaaggtgccagacgcttgcactgcctgcgatctggtcaatgtggatttggatgactgcatctttgaacaataaatgatttaaatcaggtatggctgccgatggttatcttccagattggctcgaggacactctctctgagataactgagggatagaattccgccccccccccctaacgttactggccgaagccgcttggaataaggccggtgtgcgtttgtctatatgttattttccaccatattgccgtcttttggcaatgtgagggcccggaaacctggccctgtcttcttgacgagcattcctaggggtctttcccctctcgccaaaggaatgcaaggtctgttgaatgtcgtgaaggaagcagttcctctggaagcttcttgaagacaaacaacgtctgtagcgaccctttgcaggcagcggaaccccccacctggcgacaggtgcctctgcggccaaaagccacgtgtataagatacacctgcaaaggcggcacaaccccagtgccacgttgtgagttggatagttgtggaaagagtcaaatggctctcctcaagcgtattcaacaaggggctgaaggatgcccagaaggtaccccattgtatgggatctgatctggggcctcggtgcacatgctttacatgtgtttagtcgaggttaaaaaaacgtctaggccccccgaaccacggggacgtggttttcctttgaaaaacacgatgataatagttatcgccgccatggccagtcgggaagaggagcagcgcgaaaccacccccgagcgcggacgcggtgcggcgcgacgtcccccaaccatggaggacgtgtcgtccccgtccccgtcgccgccgcctccccgggcgcccccaaaaaagcggatgaggcggcgtatcgagtccgaggacgaggaagactcatcacaagacgcgctggtgccgcgcacacccagcccgcggccatcgacctcggcggcggatttggccattgcgcccaagaagaaaaagaagcgcccttctcccaagcccgagcgcccgccatcaccagaggtaatcgtggacagcgaggaagaaagagaagatgtggcgctacaaatggtgggtttcagcaacccaccggtgctaatcaagcatggcaaaggaggtaagcgcacagtgcggcggctgaatgaagacgacccagtggcgcgtggtatgcggacgcaagaggaagaggaagagcccagcgaagcggaaagtgaaattacggtgatgaacccgctgagtgtgccgatcgtgtctgcgtgggagaagggcatggaggctgcgcgcgcgctgatggacaagtaccacgtggataacgatctaaaggcgaacttcaaactactgcctgaccaagtggaagctctggcggccgtatgcaagacctggctgaacgaggagcaccgcgggttgcagctgaccttcaccagcaacaagacctttgtgacgatgatggggcgattcctgcaggcgtacctgcagtcgtttgcagaggtgacctacaagcatcacgagcccacgggctgcgcgttgtggctgcaccgctgcgctgagatcgaaggcgagcttaagtgtctacacggaagcattatgataaataaggagcacgtgattgaaatggatgtgacgagcgaaaacgggcagcgcgcgctgaaggagcagtctagcaaggccaagatcgtgaagaaccggtggggccgaaatgtggtgcagatctccaacaccgacgcaaggtgctgcgtgcacgacgcggcctgtccggccaatcagttttccggcaagtcttgcggcatgttcttctctgaaggcgcaaaggctcaggtggcttttaagcagatcaaggcttttatgcaggcgctgtatcctaacgcccagaccgggcacggtcaccttttgatgccactacggtgcgagtgcaactcaaagcctgggcacgcgccctttttgggaaggcagctaccaaagttgactccgttcgccctgagcaacgcggaggacctggacgcggatctgatctccgacaagagcgtgctggccagcgtgcaccacccggcgctgatagtgttccagtgctgcaaccctgtgtatcgcaactcgcgcgcgcagggcggaggccccaactgcgacttcaagatatcggcgcccgacctgctaaacgcgttggtgatggtgcgcagcctgtggagtgaaaacttcaccgagctgccgcggatggttgtgcctgagtttaagtggagcactaaacaccagtatcgcaacgtgtccctgccagtggcgcatagcgatgcgcggcagaacccctttgatttttaacccgggagttctagggatctggcggccgctcgagtctagagggcccgtttaaacccgctgatcagcctcgactgtgccttctagttgccagccatctgttgtttgcccctcccccgtgccttccttgaccctggaaggtgccactcccactgtcctttcctaataaaatgaggaaattgcatcgcattgtctgagtaggtgtcattctattctggggggtggggtggggcaggacagcaagggggaggattgggaagacaatagcaggcatgctggggatgcggtgggctctatgggcgatcgctagcgtttaaacttaagcttggtaccgagctcggatccactagtccagtgtggtggaattcctgcttcgcgatgtacgggccagatatacgcgttgtttacgctccggtgcccgtcagtgggcagagcgcacatcgcccacagtccccgagaagttggggggaggggtcggcaattgaaccggtgcctagagaaggtggcgcggggtaaactgggaaagtgatgtcgtgtactggctccgcctttttcccgagggtgggggagaaccgtatataagtgcagtagtcgccgtgaacgttctttttcgcaacgggtttgccgccagaacacaggtaagtgccgtgtgtggttcccgcgggcctggcctctttacgggttatggcccttgcgtgccttgaattacttccacgcccctggctgcagtacgtgattcttgatcccgagcttcgggttggaagtgggtgggagagttcgaggccttgcgcttaaggagccccttcgcctcgtgcttgagttgaggcctggcttgggcgctggggccgccgcgtgcgaatctggtggcaccttcgcgcctgtctcgctgctttcgataagtctctagccatttaaaatttttgatgacctgctgcgacgctttttttctggcaagatagtcttgtaaatgcgggccaagatctgcacactggtatttcggtttttggggccgcgggcggcgacggggcccgtgcgtcccagcgcacatgttcggcgaggcggggcctgcgagcgcggccaccgagaatcggacgggggtagtctcaagctggccggcctgctctggtgcctggcctcgcgccgccgtgtatcgccccgccctgggcggcaaggctggcccggtcggcaccagttgcgtgagcggaaagatggccgcttcccggccctgctgcagggagctcaaaatggaggacgcggcgctcgggagagcgggcgggtgagtcacccacacaaaggaaaagggcctttccgtcctcagccgtcgcttcatgtgactccacggagtaccgggcgccgtccaggcacctcgattagttctcgagcttttggagtacgtcgtctttaggttggggggaggggttttatgcgatggagtttccccacactgagtgggtggagactgaagttaggccagcttggcacttgatgtaattctccttggaatttgccctttttgagtttggatcttggttcattctcaagcctcagacagtggttcaaagtttttttcttccatttcaggtgtcgtgaacctgcaggatttaaattctagttcaccatgtctagactggacaagagcaaagtcataaactctgctctggaattactcaatggagtcggtatcgaaggcctgacgacaaggaaactcgctcaaaagctgggagttgagcagcctaccctgtactggcacgtgaagaacaagcgggccctgctcgatgccctgccaatcgagatgctggacaggcatcatacccactcctgccccctggaaggcgagtcatggcaagactttctgcggaacaacgccaagtcataccgctgtgctctcctctcacatcgcgacggggctaaagtgcatctcggcacccgcccaacagagaaacagtacgaaaccctggaaaatcagctcgcgttcctgtgtcagcaaggcttctccctggagaacgcactgtacgctctgtccgccgtgggccactttacactgggctgcgtattggaggaacaggagcatcaagtagcaaaagaggaaagagagacacctaccaccgattctatgcccccacttctgaaacaagcaattgagctgttcgaccggcagggagccgaacctgccttccttttcggcctggaactaatcatatgtggcctggagaaacagctaaagtgcgaaagcggcgggccgaccgacgcccttgacgattttgacttagacatgctcccagccgatgcccttgacgactttgaccttgatatgctgcctgctgacgctcttgacgattttgaccttgacatgctccccgggtaagcgtacagcggctcccgggagttctagggatctgcccctctccctcccccccccctaacgttactggccgaagccgcttggaataaggccggtgtgcgtttgtctatatgttattttccaccatattgccgtcttttggcaatgtgagggcccggaaacctggccctgtcttcttgacgagcattcctaggggtctttcccctctcgccaaaggaatgcaaggtctgttgaatgtcgtgaaggaagcagttcctctggaagcttcttgaagacaaacaacgtctgtagcgaccctttgcaggcagcggaaccccccacctggcgacaggtgcctctgcggccaaaagccacgtgtataagatacacctgcaaaggcggcacaaccccagtgccacgttgtgagttggatagttgtggaaagagtcaaatggctctcctcaagcgtattcaacaaggggctgaaggatgcccagaaggtaccccattgtatgggatctgatctggggcctcggtgcacatgctttacatgtgtttagtcgaggttaaaaaaacgtctaggccccccgaaccacggggacgtggttttcctttgaaaaacacgatgataaggatccaccggaggccaccatgaccgagtacaagcccacggtgcgcctcgccacccgcgacgacgtccccagggccgtacgcaccctcgccgccgcgttcgccgactaccccgccacgcgccacaccgtcgatccggaccgccacatcgagcgggtcaccgagctgcaagaactcttcctcacgcgcgtcgggctcgacatcggcaaggtgtgggtcgcggacgacggcgccgcggtggcggtctggaccacgccggagagcgtcgaagcgggggcggtgttcgccgagatcggcccgcgcatggccgagttgagcggttcccggctggccgcgcagcaacagatggaaggcctcctggcgccgcaccggcccaaggagcccgcgtggttcctggccaccgtcggcgtctcgcccgaccaccagggcaagggtctgggcagcgccgtcgtgctccccggagtggaggcggccgagcgcgccggggtgcccgccttcctggagacctccgcgccccgcaacctccccttctacgagcggctcggcttcaccgtcaccgccgacgtcgaggtgcccgaaggaccgcgcacctggtgcatgacccgcaagcccggtgcctgaccgcgtctggaacaatcaacctctggattacaaaatttgtgaaagattgactggtattcttaactatgttgctccttttacgctatgtggatacgctgctttaatgcctttgtatcatgctattgcttcccgtatggctttcattttctcctccttgtataaatcctggttgctgtctctttatgaggagttgtggcccgttgtcaggcaacgtggcgtggtgtgcactgtgtttgctgacgcaacccccactggttggggcattgccaccacctgtcagctcctttccgggactttcgctttccccctccctattgccacggcggaactcatcgccgcctgccttgcccgctgctggacaggggctcggctgttgggcactgacaattccgtggtgttgtcggggaagctgacgtcctttccatggctgctcgcctgtgttgccacctggattctgcgcgggacgtccttctgctacgtcccttcggccctcaatccagcggaccttccttcccgcggcctgctgccggctctgcggcctcttccgcgtcttcgccttcgccctcagacgagtcggatctccctttgggccgcctccccgcaaaatgaccgaccaagcgacgcccaacctgccatcacgagatttcgattccaccgccgccttctatgatcatgtctggtcatgtctgggggtgggcgaagaactccagcatgagatccccgcgctggaggatcatccagccggcgtcccggaaaacgattccgaagcccaacctttgcctgcaggtcgactctagaggatccgaaaaaacctcccacacctccccctgaacctgaaacataaaatgaatgcaattgttgttgttaacttgtttattgcagcttataatggttacaaataaagcaatagcatcacaaatttcacaaataaagcatttttttcactgcattctagttgtggtttgtccaaactcatcaatgtatcttatcatgtctggatccccgcggccgcggtacccacgtgggcgcgccatttaaatgataactcagagagagtgtcctcgagccaatctggaagataaccatcggcagccatacctgatttaaatcatttcagagagagtgtcctcgagccaatctggaagataaccatcggcagccatacctgatttaaatcatttattgttcaaagatgcagtcatccaaatccacattgaccagatcgcaggcagtgcaagcgtctggcacctttcccatgatatgatgaatgtagcacagtttctgatacgcctttttgacgacagaaacgggttgagattctgacacgggaaagcactctaaacagtctttctgtccgtgagtgaagcagatatttgaattctgattcattctctcgcattgtctgcagggaaacagcatcagattcatgcccacgtgacgagaacatttgttttggtacctgtctgcgtagttgatcgaagcttccgcgtctgacgtcgatggctgcgcaactgactcgcgcacccgtttgggctcacttatatctgcgtcactgggggcgggtcttttcttggctccaccctttttgacgtagaattcatgctccacctcaaccacgtgatcctttgcccaccggaaaaagtctttgacttcctgcttggtgaccttcccaaagtcatgatccagacggcgggtgagttcaaatttgaacatccggtcttgcaacggctgctggtgttcgaaggtcgttgagttcccgtcaatcacggcgcacatgttggtgttggaggtgacgatcacgggagtcgggtctatctgggccgaggacttgcatttctggtccacgcgcaccttgcttcctccgagaatggctttggccgactccacgaccttggcggtcatcttcccctcctcccaccagatcaccatcttgtcgacacagtcgttgaagggaaagttctcattggtccagtttacgcacccgtagaagggcacagtgtgggctatggcctccgcgatgttggtcttcccggtagttgcaggcccaaacagccagatggtgttcctcttgccgaactttttcgtggcccatcccagaaagacggaagccgcatattggggatcgtacccgtttagttccaaaattttataaatccgattgctggaaatgtcctccacgggctgctggcccaccaggtagtcgggggcggttttagtcaggctcataatctttcccgcattgtccaaggcagccttgatttgggaccgcgagttggaggccgcattgaaggagatgtatgaggcctggtcctcctggatccactgcttctccgaggtaatccccttgtccacgagccacccgaccagctccatgtacctggctgaagtttttgatctgatcaccggcgcatcagaattgggattctgattctctttgttctgctcctgcgtctgcgacacgtgcgtcagatgctgcgccaccaaccgtttacgctccgtgagattcaaacaggcgcttaaatactgttccatattagtccacgcccactggagctcaggctgggttttggggagcaagtaattggggatgtagcactcatccaccaccttgttcccgcctccggcgccatttctggtctttgtgaccgcgaaccagtttggcaaagtcggctcgatcccgcggtaaattctctgaatcagtttttcgcgaatctgactcaggaaacgtcccaaaaccatggatttcaccccggtggtttccacgagcacgtgcatgtggaagtagctctctcccttctcaaattgcacaaagaaaagggcctccggggccttactcacacggcgccattccgtcagaaagtcgcgctgcagcttctcggccacggtcaggggtgcctgctcaatcagattcagatccatgtcagaatctggcggcaactcccattccttctcggccacccagttcacaaagctgtcagaaatgccgggcagatgctcgtcaaggtcgctggggaccttaatcacaatctcgtaaaaccccggcatggtattatcatcgtgtttttcaaagaaaaccacgtccccgtggttcggggggcctagacgttttttaacctcgactaaacacatgtaaagcatgtgcaccgaggccccagatcagatcccatacaatggggtaccttctgggcatccttcagccccttgttgaatacgcttgaggggagccatttgactctttccacaactatccaactcacaacgtggcactggggttgtgccgcctttgcaggtgtatcttatacacgtggcttttggccgcagaggcacctgtcgccaggtggggggttccgctgcctgcaaagggtcgctacagacgttgtttgtcttcaagaagcttccagaggaactgcttccttcacgacattcaacagaccttgcattcctttggcgagaggggaaagacccctaggaatgctcgtcaagaagacagggccaggtttccgggccctcacattgccaaaagacggcaatatggtggaaaataacatatagacaaacgcacaccggccttattccaagcggcttcggccagtaacgattaaaggggtcgggtaaggtatcgggttccgataggtctggtggttctgtattccccggtgctgtccggggcaaagtccacaaactgggggtcgttgtagttgtttgtgtactggatctctgggttccacctcttggagttttccttcttgagctcccactccatctccacggtgacctgcccggtgctgtactgggtgatgaagctgctgacgggcacgtccgagaagctggtgatatttccgggcacaggcgtgttcttgatgagcatcatgggcggtgggtgtttgagtccgaatccgcccatggccggagaggggtgaaagtgcgcccccgtctctgggatcttggcccagatgggtccttggaggtacacgtccctctccatccacacgctgccgggcacgatttcctggaggttgtacgtgccggtcgcgggggcagtggtggagctctggttgttggtggccatctgcccgccgacgttgtacgccacgcggttcaccggctgcgtctcgctctcgctggtgatgagcatgttgccctcgaggtacgtggcggtggtgcccgggttcgccggctggctgttgaagatcatagtgttctccagggcataggtgttgctgccctggaggttgttggtcatgccgttcggctgcgggggcacctggtaactcgcgccctcgagctccatcctattggtcgtggcgaaggcgctgacactggcgcggttgaccccggagcccaggttccagccctgggttcggcccatgggccccgggaaccagtttttgtaggtgttggcgtatctcccggccaggttcttgttgaactggactccgccagtgttatttgtgctcacgaagcggtacaagtactggtccaccagcgggttggccagcttgaacaggttctgactgggagcgaagctggagtggaagggcacctcctcaaagttgtaggtaaactcaaagttgttgcccgttctcagcatcttgctgggaaagtactctaggcagaagaagctgctcctctcggtgggattttctgtgttgtcgcggttcagcgtcgcgtaaccgtactgcggcagcgtaaagacctgcggagggaaggccggcaggcatccctcggtcccgttgccgacgacgtagggcagctggtagtcgtcgtccgtaaacacttggacggtggaggtgaggttgttggcgatggtggtggtggagtcctgcaccgtgacctctttgacttgaatgttgaagattttgactctgagggaccggggtctgaagccccagtagttgttgatgagtctttgccagtctcgggggctccagtggctgtggaagcggttaaagtcaaagtacccccagggggtgctgtatccaaagtaggcgttggcgttgcttccgtcgacggagccgcttttgatctctcggtactggtggttgttgtagctgggcagcacccaggttcgggtggacttggtgacgactctgtcccccatccacgtggaatcgcaatgccaatctcccgaggcattgcccactccatcggcaccttggttattgtcgcccaatgggccgccacctcccgcagacattgtatcagctcccaaacttgaggctggttgggctgggatttgcagctgctgggatccgctgggtccagcttcggcgtctgacgaggtggaaggcttggagtcctcttcggtccgagccttctttctttttggaaagtggtcgtctatccgctttccggtaggggccgtcttagcaccctcttcaaccaggccaaaaggttcgagaacccttttcttggcctgaaagactgcctttccgaggtttcccccgaaggatgtgtcgtcggcgagcttctcctgaaactcggcgtccgcgtggttgtacttgaggtaggggttgtctcccgcctcaagctgctcgttgtacgagatgtcgtgctctcgcgcgacctcgtctgccctgttgacaggctctcctcgatcgagaccgtttccgggtccgagatagttataaccaggcagcacaagaccacgggcttgatcttgatgctgctgattgggttttggtttcggtgggcccgcttcaaggcccaaaaactcgcgaagaccttcaccaacttcttccaaccaatctggagggtgatcaacaaaagacatacctgatttaaatcatttattgttcaaagatgcagtcatccaaatccacattgaccagatcgcaggcagtgcaagcgtctggcacctttcccatgatatgatgaatgtagcacagtttctgatacgcctttttgacgacagaaacgggttgagattctgacacgggaaagcactctaaacagtctttctgtccgtgagtgaagcagatatttgaattctgattcattctctcgcattgtctgcagggaaacagcatcagattcatgcccacgtgacgagaacatttgttttggtacctgtctgcgtagttgatcgaagcttccgcgtctgacgtcgatggctgcgcaactgcggccgctggcgggtgtgtcgagtggatggtaggatcgacaaagatctgatctgacggttcactaaaccaagtataagacaaaagtgttgtggaattgctccaggcgatctgacggttcactaaacgagctctgcttttataggcgcccaccgtacacgcctacctcgacatacgttctctatcactgatagggagtaaactggatatacgttctctatcactgatagggagtaaactgtagatacgttctctatcactgatagggagtaaactggtcatacgttctctatcactgatagggagtaaactccttatacgttctctatcactgatagggagtaaagtctgcatacgttctctatcactgatagggagtaaactcttcatacgttctctatcactgatagggagtaaagaatggctaggatccggccggcctgcaggtgtcctcacaggaacgaagtccctaaagaaacagtggcagccaggtttagccccggaattgactggattccttttttagggcccattggtatggctttttccccgtatccccccaggtgtctgcaggctcaaagagcagcgagaagcgttcagaggaaagcgatcccgtgccaccttccccgtgcccgggctgtccccgcacgctgccggctcggggatgcggggggagcgccggaccggagcggagccccgggcggctcgctgctgccccctagcgggggagggacgtaattacatccctgggggctttgggggggggctgtccctctagagcggccgccaccgcggtggagctccagcttttgttccctttagtgagggttaattagatcttaatacgactcactatagggcgaattgggtaccgggccccccctcgaggtcgacggtatcgcctccaaggccagcttcccacaataagttgggtgaattttggctcattcctcctttctataggattgaggtcagagctttgtgatgggaattctgtggaatgtgtgtcagttagggtgtggaaagtcccgcgatcgctagcaaacgccagcaacgcggcctttttacggttcctggccttttgctggccttttgctcacatgtcctgcaggcagctgcgcgctcgctcgctcactgaggccgcccgggcaaagcccgggcgtcgggcgacctttggtcgcccggcctcagtgagcgagcgagcgcgcagagagggagtggccaactccatcactaggggttcctgcggccgcacgcgtggagctagttattaatagtaatcaattacggggtcattagttcatagcccatatatggagttccgcgttacataacttacggtaaatggcccgcctggctgaccgcccaacgacccccgcccattgacgtcaataatgacgtatgttcccatagtaacgtcaatagggactttccattgacgtcaatgggtggagtatttacggtaaactgcccacttggcagtacatcaagtgtatcatatgccaagtacgccccctattgacgtcaatgacggtaaatggcccgcctggcattatgcccagtacatgaccttatgggactttcctacttggcagtacatctacgtattagtcatcgctattaccatggtgatgcggttttggcagtacatcaatgggcgtggatagcggtttgactcacggggatttccaagtctccaccccattgacgtcaatgggagtttgttttgcaccaaaatcaacgggactttccaaaatgtcgtaacaactccgccccattgacgcaaatgggcggtaggcgtgtacggtgggaggtctatataagcagagctcgtttagtgaaccgtcagatcgcctggagacgccatccacgctgttttgacctccatagaagacaccgggaccgatccagcctccgcggattcgaatcccggccgggaacggtgcattggaacgcggattccccgtgccaagagtgacgtaagtaccgcctatagagtctataggcccacaaaaaatgctttcttcttttaatatacttttttgtttatcttatttctaatactttccctaatctctttctttcagggcaataatgatacaatgtatcatgcctctttgcaccattctaaagaataacagtgataatttctgggttaaggcaatagcaatatttctgcatataaatatttctgcatataaattgtaactgatgtaagaggtttcatattgctaatagcagctacaatccagctaccattctgcttttattttatggttgggataaggctggattattctgagtccaagctaggcccttttgctaatcatgttcatacctcttatcttcctcccacagctcctgggcaacgtgctggtctgtgtgctggcccatcactttggcaaagaattgggattcgaacatcgattgaattctgaatggtgagcaagggcgaggagctgttcaccggggtggtgcccatcctggtcgagctggacggcgacgtaaacggccacaagttcagcgtgtccggcgagggcgagggcgatgccacctacggcaagctgaccctgaagttcatctgcaccaccggcaagctgcccgtgccctggcccaccctcgtgaccaccctgacctacggcgtgcagtgcttcagccgctaccccgaccacatgaagcagcacgacttcttcaagtccgccatgcccgaaggctacgtccaggagcgcaccatcttcttcaaggacgacggcaactacaagacccgcgccgaggtgaagttcgagggcgacaccctggtgaaccgcatcgagctgaagggcatcgacttcaaggaggacggcaacatcctggggcacaagctggagtacaactacaacagccacaacgtctatatcatggccgacaagcagaagaacggcatcaaggtgaacttcaagatccgccacaacatcgaggacggcagcgtgcagctcgccgaccactaccagcagaacacccccatcggcgacggccccgtgctgctgcccgacaaccactacctgagcacccagtccgccctgagcaaagaccccaacgagaagcgcgatcacatggtcctgctggagttcgtgaccgccgccgggatcactctcggcatggacgagctgtacaagtactcagatctcgagctcaagtagggatcctctagagtcgacctgcagaagcttgcctcgagcagcgctgctcgagagatctacgggtggcatccctgtgacccctccccagtgcctctcctggccctggaagttgccactccagtgcccaccagccttgtcctaataaaattaagttgcatcattttgtctgactaggtgtccttctataatattatggggtggaggggggtggtatggagcaaggggcaagttgggaagacaacctgtagggcctgcggggtctattgggaaccaagctggagtgcagtggcacaatcttggctcactgcaatctccgcctcctgggttcaagcgattctcctgcctcagcctcccgagttgttgggattccaggcatgcatgaccaggctcagctaatttttgtttttttggtagagacggggtttcaccatattggccaggctggtctccaactcctaatctcaggtgatctacccaccttggcctcccaaattgctgggattacaggcgtgaaccactgctcccttccctgtccttctgattttgtaggtaaccacgtgcggaccgagcggccgcaggaacccctagtgatggagttggccactccctctctgcgcgctcgctcgctcactgaggccgggcgaccaaaggtcgcccgacgcccgggctttgcccgggcggcctcagtgagcgagcgagcgcgcagctgcctgcaggggcgcctgatgcggtattttctccttacgcatctgtgcggtatttcacaccgcatacgtcgtagctgatcaattggcgcgccgaattcgttaacaagctttaattaacgcgtacgataagcttgatatctataacaagaaaatatatatataataagttatcacgtaagtagaacatgaaataacaatataattatcgtatgagttaaatcttaaaagtcacgtaaaagataatcatgcgtcattttgactcacgcggtcgttatagttcaaaatcagtgacacttaccgcattgacaagcacgcctcacgggagctccaagcggcgactgagatgtcctaaatgcacagcgacggattcgcgctatttagaaagagagagcaatatttcaagaatgcatgcgtcaattttacgcagactatctttctagggttaatctagctgcatcaggatcatatcgtcgggtcttttttccggctcagtcatcgcccaagctggcgctatctgggcatcggggaggaagaagcccgtgccttttcccgcgaggttgaagcggcatggaaagagtttgccgaggatgactgctgctgcattgacgttgagcgaaaacgcacgtttaccatgatgattcgggaaggtgtggccatgcacgcctttaacggtgaactgttcgttcaggccacctgggataccagttcgtcgcggcttttccggacacagttccggatggtcagcccgaagcgcatcagcaacccgaacaataccggcgacagccggaactgccgtgccggtgtgcagattaatgacagcggtgcggcgctgggatattacgtcagcgaggacgggtatcctggctggatgccgcagaaatggacatggataccccgtgagttacccggcgggcgcgcttggcgtaatcatggtcatagctgtttcctgctcgtgtccgataactgtaattatcggacatgattgtgaaattgttatccgctcacaattccacacaacatacgagccggaagcataaagtgtaaagcctggggtgcctaatgagtgagctaactcacattaattgcgttgcgctcactgcccgctttccagtcgggaaacctgtcgtgccagctgcattaatgaatcggccaacgcgcggggagaggcggtttgcgtattgggcgctcttccgcttcctcgctcactgactcgctgcgctcggtcgttcggctgcggcgagcggtatcagctcactcaaaggcggtaatacggttatccacagaatcaggggataacgcaggaaagaacatgtgagcaaaaggccagcaaaaggccaggaaccgtaaaaaggccgcgttgctggcgtt

SEQ ID NO: 19 - DNA, 22033 bp, synthetic construct
  misc_feature 1..22033: note = plasmid
  source 1..22033: mol_type = other DNA
atgactctcttaaggtagccaaatttccataggctccgcccccctgacgagcatcacaaaaatcgacgctcaagtcagaggtggcgaaacccgacaggactataaagataccaggcgtttccccctggaagctccctcgtgcgctctcctgttccgaccctgccgcttaccggatacctgtccgcctttctcccttcgggaagcgtggcgctttctcatagctcacgctgtaggtatctcagttcggtgtaggtcgttcgctccaagctgggctgtgtgcacgaaccccccgttcagcccgaccgctgcgccttatccggtaactatcgtcttgagtccaacccggtaagacacgacttatcgccactggcagcagccactggtaacaggattagcagagcgaggtatgtaggcggtgctacagagttcttgaagtggtggcctaactacggctacactagaaggacagtatttggtatctgcgctctgctgaagccagttaccttcggaaaaagagttggtagctcttgatccggcaaacaaaccaccgctggtagcggtggtttttttgtttgcaagcagcagattacgcgcagaaaaaaaggatctcaagaagatcctttgatcttttctacggggtctgacgctcagtggaacgaaaactcacgttaagggattttggtcatgagattatcaaaaaggatcttcacctagatccttttaaattaaaaatgaagttttaaatcaatctaaagtatatatgagtaaacttggtctgacagttaccaatgcttaatcagtgaggcacctatctcagcgatctgtctatttcgttcatccatagttgcctgactccccgtcgtgtagataactacgatacgggagggcttaccatctggccccagtgctgcaatgataccgcgagacccacgctcaccggctccagatttatcagcaataaaccagccagccggaagggccgagcgcagaagtggtcctgcaactttatccgcctccatccagtctattaattgttgccgggaagctagagtaagtagttcgccagttaatagtttgcgcaacgttgttgccattgctacaggcatcgtggtgtcacgctcgtcgtttggtatggcttcattcagctccggttcccaacgatcaaggcgagttacatgatcccccatgttgtgcaaaaaagcggttagctccttcggtcctccgatcgttgtcagaagtaagttggccgcagtgttatcactcatggttatggcagcactgcataattctcttactgtcatgccatccgtaagatgcttttctgtgactggtgagtactcaaccaagtcattctgagaatagtgtatgcggcgaccgagttgctcttgcccggcgtcaatacgggataataccgcgccacatagcagaactttaaaagtgctcatcattggaaaacgttcttcggggcgaaaactctcaaggatcttaccgctgttgagatccagttcgatgtaacccactcgtgcacccaactgatcttcagcatcttttactttcaccagcgtttctgggtgagcaaaaacaggaaggcaaaatgccgcaaaaaagggaataagggcgacacggaaatgttgaatactcatactcttcctttttcaatattattgaagcatttatcagggttattgtctcatgagcggatacatatttgaatgtatttagaaaaataaacaaataggggttccgcgcacatttccccgaaaagtgccacctaaattgtaagcgttaatattttgttaaaattcgcgttaaatttttgttaaatcagctcattttttaaccaataggccgaaatcggcaaaatcccttataaatcaaaagaatagaccgagatagggttgagtgttgttccagtttggaacaagagtccactattaaagaacgtggactccaacgtcaaagggcgaaaaaccgtctatcagggcgatggcccactacgtgaaccatcaccctaatcaagttttttggggtcgaggtgccgtaaagcactaaatcggaaccctaaagggagcccccgatttagagcttgacggggaaagccggcgaacgtggcgagaaaggaagggaagaaagcgaaaggagcgggcgctagggcgctggcaagtgtagcggtcacgctgcgcgtaaccaccacacccgccgcgcttaatgcgccgctacagggcgcgtcccattcgccattcaggctgcgcaactgttgggaagggcgatcggtgcgggcctcttcgctattacgccagctggcgaaagggggatgtgctgcaaggcgattaagttgggtaacgccagggttttcccagtcacgacgttaccccacagtggggccactagggtcaatttctgagaactgtcattctcggaaattgagtaaaacgacggccagtgagcgcgcctcgttcattcacgtttttgaacccgtggaggacgggcagactcgcggtgcaaatgtgttttacagcgtgatggagcagatgaagatgctcgacacgctgcagaacacgcagctagattaaccctagaaagataatcatattgtgacgtacgttaaagataatcatgcgtaaaattgacgcatgtgttttatcggtctgtatatcgaggtttatttattaatttgaatagatattaagttttattatatttacacttacatactaataataaattcaacaaacaatttatttatgtttatttatttattaaaaaaaaacaaaaactcaaaatttcttctataaagtaacaaaacttttatcgaattcctgcagcccgggggatccactagttctagagggacagcccccccccaaagcccccagggatgtaattacgtccctcccccgctagggggcagcagcgagccgcccggggctccgctccggtccggcgctccccccgcatccccgagccggcagcgtgcggggacagcccgggcacggggaaggtggcacgggatcgctttcctctgaacgcttctcgctgctctttgagcctgcagacacctggggggatacggggaaaaggcctccaaggccagcttcccacaataagttgggtgaattttggctcattcctcctttctataggattgaggtcagagctttgtgatgggaattctgtggaatgtgtgtcagttagggtgtggaaagtccctttactccctatcagtgatagagaacgtatgaagagtttactccctatcagtgatagagaacgtatgcagactttactccctatcagtgatagagaacgtataaggagtttactccctatcagtgatagagaacgtatgaccagtttactccctatcagtgatagagaacgtatctacagtttactccctatcagtgatagagaacgtatatccagtttactccctatcagtgatagagaacgtatgtcgaggtaggcgtgtacggtgggcgcctataaaagcagagctcgtttagtgaaccgtcagatcgcctggagcaattccacaacacttttgtcttatacttggtttagtgaaccgtcagatcagatctttgtcgatcctaccatccactcgacacacccgccagcggccgcagttgcgcagccatcgacgtcagacgcggaagcttcgatcaactacgcagacaggtaccaaaacaaatgttctcgtcacgtgggcatgaatctgatgctgtttccctgcagacaatgcgagagaatgaatcagaattcaaatatctgcttcactcacggacagaaagactgtttagagtgctttcccgtgtcagaatctcaacccgtttctgtcgtcaaaaaggcgtatcagaaactgtgctacattcatcatatcatgggaaaggtgccagacgcttgcactgcctgcgatctggtcaatgtggatttggatgactgcatctttgaacaataaatgatttaaatcaggtatgtcttttgttgatcaccctccagattggttggaagaagttggtgaaggtcttcgcgagtttttgggccttgaagcgggcccaccgaaaccaaaacccaatcagcagcatcaagatcaagcccgtggtcttgtgctgcctggttataactatctcggacccggaaacggtctcgatcgaggagagcctgtcaacagggcagacgaggtcgcgcgagagcacgacatctcgtacaacgagcagcttgaggcgggagacaacccctacctcaagtacaaccacgcggacgccgagtttcaggagaagctcgccgacgacacatccttcgggggaaacctcggaaaggcagtctttcaggccaagaaaagggttctcgaaccttttggcctggttgaagagggtgctaagacggcccctaccggaaagcggatagacgaccactttccaaaaagaaagaaggctcggaccgaagaggactccaagccttccacctcgtcagacgccgaagctggacccagcggatcccagcagctgcaaatcccagcccaaccagcctcaagtttgggagctgatacaatgtctgcgggaggtggcggcccattgggcgacaataaccaaggtgccgatggagtgggcaatgcctcgggagattggcattgcgattccacgtggatgggggacagagtcgtcaccaagtccacccgaacctgggtgctgcccagctacaacaaccaccagtaccgagagatcaaaagcggctccgtcgacggaagcaacgccaacgcctactttggatacagcaccccctgggggtactttgactttaaccgcttccacagccactggagcccccgagactggcaaagactcatcaacaactactggggcttcagaccccggtccctcagagtcaaaatcttcaacattcaagtcaaagaggtcacggtgcaggactccaccaccaccatcgccaacaacctcacctccaccgtccaagtgtttacggacgacgactaccagctgccctacgtcgtcggcaacgggaccgagggatgcctgccggccttccctccgcaggtctttacgctgccgcagtacggttacgcgacgctgaaccgcgacaacacagaaaatcccaccgagaggagcagcttcttctgcctagagtactttcccagcaagatgctgagaacgggcaacaactttgagtttacctacaactttgaggaggtgcccttccactccagcttcgctcccagtcagaacctgttcaagctggccaacccgctggtggaccagtacttgtaccgcttcgtgagcacaaataacactggcggagtccagttcaacaagaacctggccgggagatacgccaacacctacaaaaactggttcccggggcccatgggccgaacccagggctggaacctgggctccggggtcaaccgcgccagtgtcagcgccttcgccacgaccaataggatggagctcgagggcgcgagttaccaggtgcccccgcagccgaacggcatgaccaacaacctccagggcagcaacacctatgccctggagaacactatgatcttcaacagccagccggcgaacccgggcaccaccgccacgtacctcgagggcaacatgctcatcaccagcgagagcgagacgcagccggtgaaccgcgtggcgtacaacgtcggcgggcagatggccaccaacaaccagagctccaccactgcccccgcgaccggcacgtacaacctccaggaaatcgtgcccggcagcgtgtggatggagagggacgtgtacctccaaggacccatctgggccaagatcccagagacgggggcgcactttcacccctctccggccatgggcggattcggactcaaacacccaccgcccatgatgctcatcaagaacacgcctgtgcccggaaatatcaccagcttctcggacgtgcccgtcagcagcttcatcacccagtacagcaccgggcaggtcaccgtggagatggagtgggagctcaagaaggaaaactccaagaggtggaacccagagatccagtacacaaacaactacaacgacccccagtttgtggactttgccccggacagcaccggggaatacagaaccaccagacctatcggaacccgataccttacccgacccctttaacccgggagttctagggatctgcccctctccctcccccccccctaacgttactggccgaagccgcttggaataaggccggtgtgcgtttgtctatatgttattttccaccatattgccgtcttttggcaatgtgagggcccggaaacctggccctgtcttcttgacgagcattcctaggggtctttcccctctcgccaaaggaatgcaaggtctgttgaatgtcgtgaaggaagcagttcctctggaagcttcttgaagacaaacaacgtctgtagcgaccctttgcaggcagcggaaccccccacctggcgacaggtgcctctgcggccaaaagccacgtgtataagatacacctgcaaaggcggcacaaccccagtgccacgttgtgagttggatagttgtggaaagagtcaaatggctctcctcaagcgtattcaacaaggggctgaaggatgcccagaaggtaccccattgtatgggatctgatctggggcctcggtgcacatgctttacatgtgtttagtcgaggttaaaaaaacgtctaggccccccgaaccacggggacgtggttttcctttgaaaaacacgatgataaggatccaccggaggccaccatggccagtcgggaagaggagcagcgcgaaaccacccccgagcgcggacgcggtgcggcgcgacgtcccccaaccatggaggacgtgtcgtccccgtccccgtcgccgccgcctccccgggcgcccccaaaaaagcggatgaggcggcgtatcgagtccgaggacgaggaagactcatcacaagacgcgctggtgccgcgcacacccagcccgcggccatcgacctcggcggcggatttggccattgcgcccaagaagaaaaagaagcgcccttctcccaagcccgagcgcccgccatcaccagaggtaatcgtggacagcgaggaagaaagagaagatgtggcgctacaaatggtgggtttcagcaacccaccggtgctaatcaagcatggcaaaggaggtaagcgcacagtgcggcggctgaatgaagacgacccagtggcgcgtggtatgcggacgcaagaggaagaggaagagcccagcgaagcggaaagtgaaattacggtgatgaacccgctgagtgtgccgatcgtgtctgcgtgggagaagggcatggaggctgcgcgcgcgctgatggacaagtaccacgtggataacgatctaaaggcgaacttcaaactactgcctgaccaagtggaagctctggcggccgtatgcaagacctggctgaacgaggagcaccgcgggttgcagctgaccttcaccagcaacaagacctttgtgacgatgatggggcgattcctgcaggcgtacctgcagtcgtttgcagaggtgacctacaagcatcacgagcccacgggctgcgcgttgtggctgcaccgctgcgctgagatcgaaggcgagcttaagtgtctacacggaagcattatgataaataaggagcacgtgattgaaatggatgtgacgagcgaaaacgggcagcgcgcgctgaaggagcagtctagcaaggccaagatcgtgaagaaccggtggggccgaaatgtggtgcagatctccaacaccgacgcaaggtgctgcgtgcacgacgcggcctgtccggccaatcagttttccggcaagtcttgcggcatgttcttctctgaaggcgcaaaggctcaggtggcttttaagcagatcaaggcttttatgcaggcgctgtatcctaacgcccagaccgggcacggtcaccttttgatgccactacggtgcgagtgcaactcaaagcctgggcacgcgccctttttgggaaggcagctaccaaagttgactccgttcgccctgagcaacgcggaggacctggacgcggatctgatctccgacaagagcgtgctggccagcgtgcaccacccggcgctgatagtgttccagtgctgcaaccctgtgtatcgcaactcgcgcgcgcagggcggaggccccaactgcgacttcaagatatcggcgcccgacctgctaaacgcgttggtgatggtgcgcagcctgtggagtgaaaacttcaccgagctgccgcggatggttgtgcctgagtttaagtggagcactaaacaccagtatcgcaacgtgtccctgccagtggcgcatagcgatgcgcggcagaacccctttgatttttaacccgggagttctagggatctggcggccgctcgagtctagagggcccgtttaaacccgctgatcagcctcgactgtgccttctagttgccagccatctgttgtttgcccctcccccgtgccttccttgaccctggaaggtgccactcccactgtcctttcctaataaaatgaggaaattgcatcgcattgtctgagtaggtgtcattctattctggggggtggggtggggcaggacagcaagggggaggattgggaagacaatagcaggcatgctggggatgcggtgggctctatgggcgatcgctagcgtttaaacttaagcttggtaccgagctcggatccactagtccagtgtggtggaattcctgcttcgcgatgtacgggccagatatacgcgttgtttacgctccggtgcccgtcagtgggcagagcgcacatcgcccacagtccccgagaagttggggggaggggtcggcaattgaaccggtgcctagagaaggtggcgcggggtaaactgggaaagtgatgtcgtgtactggctccgcctttttcccgagggtgggggagaaccgtatataagtgcagtagtcgccgtgaacgttctttttcgcaacgggtttgccgccagaacacaggtaagtgccgtgtgtggttcccgcgggcctggcctctttacgggttatggcccttgcgtgccttgaattacttccacgcccctggctgcagtacgtgattcttgatcccgagcttcgggttggaagtgggtgggagagttcgaggccttgcgcttaaggagccccttcgcctcgtgcttgagttgaggcctggcttgggcgctggggccgccgcgtgcgaatctggtggcaccttcgcgcctgtctcgctgctttcgataagtctctagccatttaaaatttttgatgacctgctgcgacgctttttttctggcaagatagtcttgtaaatgcgggccaagatctgcacactggtatttcggtttttggggccgcgggcggcgacggggcccgtgcgtcccagcgcacatgttcggcgaggcggggcctgcgagcgcggccaccgagaatcggacgggggtagtctcaagctggccggcctgctctggtgcctggcctcgcgccgccgtgtatcgccccgccctgggcggcaaggctggcccggtcggcaccagttgcgtgagcggaaagatggccgcttcccggccctgctgcagggagctcaaaatggaggacgcggcgctcgggagagcgggcgggtgagtcacccacacaaaggaaaagggcctttccgtcctcagccgtcgcttcatgtgactccacggagtaccgggcgccgtccaggcacctcgattagttctcgagcttttggagtacgtcgtctttaggttggggggaggggttttatgcgatggagtttccccacactgagtgggtggagactgaagttaggccagcttggcacttgatgtaattctccttggaatttgccctttttgagtttggatcttggttcattctcaagcctcagacagtggttcaaagtttttttcttccatttcaggtgtcgtgaacctgcaggatttaaattctagttcaccatgtctagactggacaagagcaaagtcataaactctgctctggaattactcaatggagtcggtatcgaaggcctgacgacaaggaaactcgctcaaaagctgggagttgagcagcctaccctgtactggcacgtgaagaacaagcgggccctgctcgatgccctgccaatcgagatgctggacaggcatcatacccactcctgccccctggaaggcgagtcatggcaagactttctgcggaacaacgccaagtcataccgctgtgctctcctctcacatcgcgacggggctaaagtgcatctcggcacccgcccaacagagaaacagtacgaaaccctggaaaatcagctcgcgttcctgtgtcagcaaggcttctccctggagaacgcactgtacgctctgtccgccgtgggccactttacactgggctgcgtattggaggaacaggagcatcaagtagcaaaagaggaaagagagacacctaccaccgattctatgcccccacttctgaaacaagcaattgagctgttcgaccggcagggagccgaacctgccttccttttcggcctggaactaatcatatgtggcctggagaaacagctaaagtgcgaaagcggcgggccgaccgacgcccttgacgattttgacttagacatgctcccagccgatgcccttgacgactttgaccttgatatgctgcctgctgacgctcttgacgattttgaccttgacatgctccccgggtaagcgtacagcggctcccgggagttctagggatctgcccctctccctcccccccccctaacgttactggccgaagccgcttggaataaggccggtgtgcgtttgtctatatgttattttccaccatattgccgtcttttggcaatgtgagggcccggaaacctggccctgtcttcttgacgagcattcctaggggtctttcccctctcgccaaaggaatgcaaggtctgttgaatgtcgtgaaggaagcagttcctctggaagcttcttgaagacaaacaacgtctgtagcgaccctttgcaggcagcggaaccccccacctggcgacaggtgcctctgcggccaaaagccacgtgtataagatacacctgcaaaggcggcacaaccccagtgccacgttgtgagttggatagttgtggaaagagtcaaatggctctcctcaagcgtattcaacaaggggctgaaggatgcccagaaggtaccccattgtatgggatctgatctggggcctcggtgcacatgctttacatgtgtttagtcgaggttaaaaaaacgtctaggccccccgaaccacggggacgtggttttcctttgaaaaacacgatgataaggatccaccggaggccaccatgaccgagtacaagcccacggtgcgcctcgccacccgcgacgacgtccccagggccgtacgcaccctcgccgccgcgttcgccgactaccccgccacgcgccacaccgtcgatccggaccgccacatcgagcgggtcaccgagctgcaagaactcttcctcacgcgcgtcgggctcgacatcggcaaggtgtgggtcgcggacgacggcgccgcggtggcggtctggaccacgccggagagcgtcgaagcgggggcggtgttcgccgagatcggcccgcgcatggccgagttgagcggttcccggctggccgcgcagcaacagatggaaggcctcctggcgccgcaccggcccaaggagcccgcgtggttcctggccaccgtcggcgtctcgcccgaccaccagggcaagggtctgggcagcgccgtcgtgctccccggagtggaggcggccgagcgcgccggggtgcccgccttcctggagacctccgcgccccgcaacctccccttctacgagcggctcggcttcaccgtcaccgccgacgtcgaggtgcccgaaggaccgcgcacctggtgcatgacccgcaagcccggtgcctgaccgcgtctggaacaatcaacctctggattacaaaatttgtgaaagattgactggtattcttaactatgttgctccttttacgctatgtggatacgctgctttaatgcctttgtatcatgctattgcttcccgtatggctttcattttctcctccttgtataaatcctggttgctgtctctttatgaggagttgtggcccgttgtcaggcaacgtggcgtggtgtgcactgtgtttgctgacgcaacccccactggttggggcattgccaccacctgtcagctcctttccgggactttcgctttccccctccctattgccacggcggaactcatcgccgcctgccttgcccgctgctggacaggggctcggctgttgggcactgacaattccgtggtgttgtcggggaagctgacgtcctttccatggctgctcgcctgtgttgccacctggattctgcgcgggacgtccttctgctacgtcccttcggccctcaatccagcggaccttccttcccgcggcctgctgccggctctgcggcctcttccgcgtcttcgccttcgccctcagacgagtcggatctccctttgggccgcctccccgcaaaatgaccgaccaagcgacgcccaacctgccatcacgagatttcgattccaccgccgccttctatgatcatgtctgggggtgggcgaagaactccagcatgagatccccgcgctggaggatcatccagccggcgtcccggaaaacgattccgaagcccaacctttgcctgcaggtcgactctagaggatccgaaaaaacctcccacacctccccctgaacctgaaacataaaatgaatgcaattgttgttgttaacttgtttattgcagcttataatggttacaaataaagcaatagcatcacaaatttcacaaataaagcatttttttcactgcattctagttgtggtttgtccaaactcatcaatgtatcttatcatgtctggatccccgcggccgcggtacccacgtgggcgcgccatttaaatgataactcagagagagtgtcctcgagccaatctggaagataaccatcggcagccatacctgatttaaatcatttattgttcaaagatgcagtcatccaaatccacattgaccagatcgcaggcagtgcaagcgtctggcacctttcccatgatatgatgaatgtagcacagtttctgatacgcctttttgacgacagaaacgggttgagattctgacacgggaaagcactctaaacagtctttctgtccgtgagtgaagcagatatttgaattctgattcattctctcgcattgtctgcagggaaacagcatcagattcatgcccacgtgacgagaacatttgttttggtacctgtctgcgtagttgatcgaagcttccgcgtctgacgtcgatggctgcgcaactgactcgcgcacccgtttgggctcacttatatctgcgtcactgggggcgggtcttttcttggctccaccctttttgacgtagaattcatgctccacctcaaccacgtgatcctttgcccaccggaaaaagtctttgacttcctgcttggtgaccttcccaaagtcatgatccagacggcgggtgagttcaaatttgaacatccggtcttgcaacggctgctggtgttcgaaggtcgttgagttcccgtcaatcacggcgcacatgttggtgttggaggtgacgatcacgggagtcgggtctatctgggccgaggacttgcatttctggtccacgcgcaccttgcttcctccgagaatggctttggccgactccacgaccttggcggtcatcttcccctcctcccaccagatcaccatcttgtcgacacagtcgttgaagggaaagttctcattggtccagtttacgcacccgtagaagggcacagtgtgggctatggcctccgcgatgttggtcttcccggtagttgcaggcccaaacagccagatggtgttcctcttgccgaactttttcgtggcccatcccagaaagacggaagccgcatattggggatcgtacccgtttagttccaaaattttataaatccgattgctggaaatgtcctccacgggctgctggcccaccaggtagtcgggggcggttttagtcaggctcataatctttcccgcattgtccaaggcagccttgatttgggaccgcgagttggaggccgcattgaaggagatgtatgaggcctggtcctcctggatccactgcttctccgaggtaatccccttgtccacgagccacccgaccagctccatgtacctggctgaagtttttgatctgatcaccggcgcatcagaattgggattctgattctctttgttctgctcctgcgtctgcgacacgtgcgtcagatgctgcgccaccaaccgtttacgctccgtgagattcaaacaggcgcttaaatactgttccatattagtccacgcccactggagctcaggctgggttttggggagcaagtaattggggatgtagcactcatccaccaccttgttcccgcctccggcgccatttctggtctttgtgaccgcgaaccagtttggcaaagtcggctcgatcccgcggtaaattctctgaatcagtttttcgcgaatctgactcaggaaacgtcccaaaaccatggatttcaccccggtggtttccacgagcacgtgcatgtggaagtagctctctcccttctcaaattgcacaaagaaaagggcctccggggccttactcacacggcgccattccgtcagaaagtcgcgctgcagcttctcggccacggtcaggggtgcctgctcaatcagattcagatccatgtcagaatctggcggcaactcccattccttctcggccacccagttcacaaagctgtcagaaatgccgggcagatgctcgtcaaggtcgctggggaccttaatcacaatctcgtaaaaccccggcatggcggcgataactattatcatcgtgtttttcaaaggaaaaccacgtccccgtggttcggggggcctagacgtttttttaacctcgactaaacacatgtaaagcatgtgcaccgaggccccagatcagatcccatacaatggggtaccttctgggcatccttcagccccttgttgaatacgcttgaggagagccatttgactctttccacaactatccaactcacaacgtggcactggggttgtgccgcctttgcaggtgtatcttatacacgtggcttttggccgcagaggcacctgtcgccaggtggggggttccgctgcctgcaaagggtcgctacagacgttgtttgtcttcaagaagcttccagaggaactgcttccttcacgacattcaacagaccttgcattcctttggcgagaggggaaagacccctaggaatgctcgtcaagaagacagggccaggtttccgggccctcacattgccaaaagacggcaatatggtggaaaataacatatagacaaacgcacaccggccttattccaagcggcttcggccagtaacgttagggggggggggcggaattctatccctcagttatctcagagagagtgtcctcgagccaatctggaagataaccatcggcagccatacctgatttaaatcatttattgttcaaagatgcagtcatccaaatccacattgaccagatcgcaggcagtgcaagcgtctggcacctttcccatgatatgatgaatgtagcacagtttctgatacgcctttttgacgacagaaacgggttgagattctgacacgggaaagcactctaaacagtctttctgtccgtgagtgaagcagatatttgaattctgattcattctctcgcattgtctgcagggaaacagcatcagattcatgcccacgtgacgagaacatttgttttggtacctgtctgcgtagttgatcgaagcttccgcgtctgacgtcgatggctgcgcaactgactcgcgcacccgtttgggctcacttatatctgcgtcactgggggcgggtcttttcttggctccaccctttttgacgtagaattcatgctccacctcaaccacgtgatcctttgcccaccggaaaaagtctttgacttcctgcttggtgaccttcccaaagtcatgatccagacggcgggtgagttcaaatttgaacatccggtcttgcaacggctgctggtgttcgaaggtcgttgagttcccgtcaatcacggcgcacatgttggtgttggaggtgacgatcacgggagtcgggtctatctgggccgaggacttgcatttctggtccacgcgcaccttgcttcctccgagaatggctttggccgactccacgaccttggcggtcatcttcccctcctcccaccagatcaccatcttgtcgacacagtcgttgaagggaaagttctcattggtccagtttacgcacccgtagaagggcacagtgtgggctatggcctccgcgatgttggtcttcccggtagttgcaggcccaaacagccagatggtgttcctcttgccgaactttttcgtggcccatcccagaaagacggaagccgcatattggggatcgtacccgtttagttccaaaattttataaatccgattgctggaaatgtcctccacgggctgctggcccaccaggtagtcgggggcggttttagtcaggctcataatctttcccgcattgtccaaggcagccttgatttgggaccgcgagttggaggccgcattgaaggagatgtatgaggcctggtcctcctggatccactgcttctccgaggtaatccccttgtccacgagccacccgaccagctccatggtggcgttatccggccgatcgatagatctgggccccggtgtcgactttacgagggtaggaagtggtacggaaagttggtataagacaaaagtgttgtggaattgctggaggcgatctgacggttcactaaacgagctctgcttttataggcgcccaccgtacacgcctaaagcttatacgttctctatcactgatagggagtaaactggatatacgttctctatcactgatagggagtaaactgtagatacgttctctatcactgatagggagtaaactggtcatacgttctctatcactgatagggagtaaactccttatacgttctctatcactgatagggagtaaagtctgcatacgttctctatcactgatagggagtaaactcttcatacgttctctatcactgatagggagtaaacgaatggctaggatccggccggcctgcaggtgtcctcacaggaacgaagtccctaaagaaacagtggcagccaggtttagccccggaattgactggattccttttttagggcccattggtatggctttttccccgtatccccccaggtgtctgcaggctcaaagagcagcgagaagcgttcagaggaaagcgatcccgtgccaccttccccgtgcccgggctgtccccgcacgctgccggctcggggatgcggggggagcgccggaccggagcggagccccgggcggctcgctgctgccccctagcgggggagggacgtaattacatccctgggggctttgggggggggctgtccctctagagcggccgccaccgcggtggagctccagcttttgttccctttagtgagggttaattagatcttaatacgactcactatagggcgaattgggtaccgggccccccctcgaggtcgacggtatcgcctccaaggccagcttcccacaataagttgggtgaattttggctcattcctcctttctataggattgaggtcagagctttgtgatgggaattctgtggaatgtgtgtcagttagggtgtggaaagtcccgcgatcgctagcaaacgccagcaacgcggcctttttacggttcctggccttttgctggccttttgctcacatgtcctgcaggcagctgcgcgctcgctcgctcactgaggccgcccgggcaaagcccgggcgtcgggcgacctttggtcgcccggcctcagtgagcgagcgagcgcgcagagagggagtggccaactccatcactaggggttcctgcggccgcacgcgtggagctagttattaatagtaatcaattacggggtcattagttcatagcccatatatggagttccgcgttacataacttacggtaaatggcccgcctggctgaccgcccaacgacccccgcccattgacgtcaataatgacgtatgttcccatagtaacgtcaatagggactttccattgacgtcaatgggtggagtatttacggtaaactgcccacttggcagtacatcaagtgtatcatatgccaagtacgccccctattgacgtcaatgacggtaaatggcccgcctggcattatgcccagtacatgaccttatgggactttcctacttggcagtacatctacgtattagtcatcgctattaccatggtgatgcggttttggcagtacatcaatgggcgtggatagcggtttgactcacggggatttccaagtctccaccccattgacgtcaatgggagtttgttttgcaccaaaatcaacgggactttccaaaatgtcgtaacaactccgccccattgacgcaaatgggcggtaggcgtgtacggtgggaggtctatataagcagagctcgtttagtgaaccgtcagatcgcctggagacgccatccacgctgttttgacctccatagaagacaccgggaccgatccagcctccgcggattcgaatcccggccgggaacggtgcattggaacgcggattccccgtgccaagagtgacgtaagtaccgcctatagagtctataggcccacaaaaaatgctttcttcttttaatatacttttttgtttatcttatttctaatactttccctaatctctttctttcagggcaataatgatacaatgtatcatgcctctttgcaccattctaaagaataacagtgataatttctgggttaaggcaatagcaatatttctgcatataaatatttctgcatataaattgtaactgatgtaagaggtttcatattgctaatagcagctacaatccagctaccattctgcttttattttatggttgggataaggctggattattctgagtccaagctaggcccttttgctaatcatgttcatacctcttatcttcctcccacagctcctgggcaacgtgctggtctgtgtgctggcccatcactttggcaaagaattgggattcgaacatcgattgaattctgaatggtgagcaagggcgaggagctgttcaccggggtggtgcccatcctggtcgagctggacggcgacgtaaacggccacaagttcagcgtgtccggcgagggcgagggcgatgccacctacggcaagctgaccctgaagttcatctgcaccaccggcaagctgcccgtgccctggcccaccctcgtgaccaccctgacctacggcgtgcagtgcttcagccgctaccccgaccacatgaagcagcacgacttcttcaagtccgccatgcccgaaggctacgtccaggagcgcaccatcttcttcaaggacgacggcaactacaagacccgcgccgaggtgaagttcgagggcgacaccctggtgaaccgcatcgagctgaagggcatcgacttcaaggaggacggcaacatcctggggcacaagctggagtacaactacaacagccacaacgtctatatcatggccgacaagcagaagaacggcatcaaggtgaacttcaagatccgccacaacatcgaggacggcagcgtgcagctcgccgaccactaccagcagaacacccccatcggcgacggccccgtgctgctgcccgacaaccactacctgagcacccagtccgccctgagcaaagaccccaacgagaagcgcgatcacatggtcctgctggagttcgtgaccgccgccgggatcactctcggcatggacgagctgtacaagtactcagatctcgagctcaagtagggatcctctagagtcgacctgcagaagcttgcctcgagcagcgctgctcgagagatctacgggtggcatccctgtgacccctccccagtgcctctcctggccctggaagttgccactccagtgcccaccagccttgtcctaataaaattaagttgcatcattttgtctgactaggtgtccttctataatattatggggtggaggggggtggtatggagcaaggggcaagttgggaagacaacctgtagggcctgcggggtctattgggaaccaagctggagtgcagtggcacaatcttggctcactgcaatctccgcctcctgggttcaagcgattctcctgcctcagcctcccgagttgttgggattccaggcatgcatgaccaggctcagctaatttttgtttttttggtagagacggggtttcaccatattggccaggctggtctccaactcctaatctcaggtgatctacccaccttggcctcccaaattgctgggattacaggcgtgaaccactgctcccttccctgtccttctgattttgtaggtaaccacgtgcggaccgagcggccgcaggaacccctagtgatggagttggccactccctctctgcgcgctcgctcgctcactgaggccgggcgaccaaaggtcgcccgacgcccgggctttgcccgggcggcctcagtgagcgagcgagcgcgcagctgcctgcaggggcgcctgatgcggtattttctccttacgcatctgtgcggtatttcacaccgcatacgtcgtagctgatcaattggcgcgccgaattcgttaacaagctttaattaacgcgtacgataagcttgatatctataacaagaaaatatatatataataagttatcacgtaagtagaacatgaaataacaatataattatcgtatgagttaaatcttaaaagtcacgtaaaagataatcatgcgtcattttgactcacgcggtcgttatagttcaaaatcagtgacacttaccgcattgacaagcacgcctcacgggagctccaagcggcgactgagatgtcctaaatgcacagcgacggattcgcgctatttagaaagagagagcaatatttcaagaatgcatgcgtcaattttacgcagactatctttctagggttaatctagctgcatcaggatcatatcgtcgggtcttttttccggctcagtcatcgcccaagctggcgctatctgggcatcggggaggaagaagcccgtgccttttcccgcgaggttgaagcggcatggaaagagtttgccgaggatgactgctgctgcattgacgttgagcgaaaacgcacgtttaccatgatgattcgggaaggtgtggccatgcacgcctttaacggtgaactgttcgttcaggccacctgggataccagttcgtcgcggcttttccggacacagttccggatggtcagcccgaagcgcatcagcaacccgaacaataccggcgacagccggaactgccgtgccggtgtgcagattaatgacagcggtgcggcgctgggatattacgtcagcgaggacgggtatcctggctggatgccgcagaaatggacatggataccccgtgagttacccggcgggcgcgcttggcgtaatcatggtcatagctgtttcctgctcgtgtccgataactgtaattatcggacatgattgtgaaattgttatccgctcacaattccacacaacatacgagccggaagcataaagtgtaaagcctggggtgcctaatgagtgagctaactcacattaattgcgttgcgctcactgcccgctttccagtcgggaaacctgtcgtgccagctgcattaatgaatcggccaacgcgcggggagaggcggtttgcgtattgggcgctcttccgcttcctcgctcactgactcgctgcgctcggtcgttcggctgcggcgagcggtatcagctcactcaaaggcggtaatacggttatccacagaatcaggggataacgcaggaaagaacatgtgagcaaaaggccagcaaaaggccaggaaccgtaaaaaggccgcgttgctggcgtt

SEQ ID NO: 20 - DNA, 20257 bp, synthetic construct
  misc_feature 1..20257: note = plasmid
  source 1..20257: mol_type = other DNA
atgactctcttaaggtagccaaatttccataggctccgcccccctgacgagcatcacaaaaatcgacgctcaagtcagaggtggcgaaacccgacaggactataaagataccaggcgtttccccctggaagctccctcgtgcgctctcctgttccgaccctgccgcttaccggatacctgtccgcctttctcccttcgggaagcgtggcgctttctcatagctcacgctgtaggtatctcagttcggtgtaggtcgttcgctccaagctgggctgtgtgcacgaaccccccgttcagcccgaccgctgcgccttatccggtaactatcgtcttgagtccaacccggtaagacacgacttatcgccactggcagcagccactggtaacaggattagcagagcgaggtatgtaggcggtgctacagagttcttgaagtggtggcctaactacggctacactagaaggacagtatttggtatctgcgctctgctgaagccagttaccttcggaaaaagagttggtagctcttgatccggcaaacaaaccaccgctggtagcggtggtttttttgtttgcaagcagcagattacgcgcagaaaaaaaggatctcaagaagatcctttgatcttttctacggggtctgacgctcagtggaacgaaaactcacgttaagggattttggtcatgagattatcaaaaaggatcttcacctagatccttttaaattaaaaatgaagttttaaatcaatctaaagtatatatgagtaaacttggtctgacagttaccaatgcttaatcagtgaggcacctatctcagcgatctgtctatttcgttcatccatagttgcctgactccccgtcgtgtagataactacgatacgggagggcttaccatctggccccagtgctgcaatgataccgcgagacccacgctcaccggctccagatttatcagcaataaaccagccagccggaagggccgagcgcagaagtggtcctgcaactttatccgcctccatccagtctattaattgttgccgggaagctagagtaagtagttcgccagttaatagtttgcgcaacgttgttgccattgctacaggcatcgtggtgtcacgctcgtcgtttggtatggcttcattcagctccggttcccaacgatcaaggcgagttacatgatcccccatgttgtgcaaaaaagcggttagctccttcggtcctccgatcgttgtcagaagtaagttggccgcagtgttatcactcatggttatggcagcactgcataattctcttactgtcatgccatccgtaagatgcttttctgtgactggtgagtactcaaccaagtcattctgagaatagtgtatgcggcgaccgagttgctcttgcccggcgtcaatacgggataataccgcgccacatagcagaactttaaaagtgctcatcattggaaaacgttcttcggggcgaaaactctcaaggatcttaccgctgttgagatccagttcgatgtaacccactcgtgcacccaactgatcttcagcatcttttactttcaccagcgtttctgggtgagcaaaaacaggaaggcaaaatgccgcaaaaaagggaataagggcgacacggaaatgttgaatactcatactcttcctttttcaatattattgaagcatttatcagggttattgtctcatgagcggatacatatttgaatgtatttagaaaaataaacaaataggggttccgcgcacatttccccgaaaagtgccacctaaattgtaagcgttaatattttgttaaaattcgcgttaaatttttgttaaatcagctcattttttaaccaataggccgaaatcggcaaaatcccttataaatcaaaagaatagaccgagatagggttgagtgttgttccagtttggaacaagagtccactattaaagaacgtggactccaacgtcaaagggcgaaaaaccgtctatcagggcgatggcccactacgtgaaccatcaccctaatcaagttttttggggtcgaggtgccgtaaagcactaaatcggaaccctaaagggagcccccgatttagagcttgacggggaaagccggcgaacgtggcgagaaaggaagggaagaaagcgaaaggagcgggcgctagggcgctggcaagtgtagcggtcacgctgcgcgtaaccaccacacccgccgcgcttaatgcgccgctacagggcgcgtcccattcgccattcaggctgcgcaactgttgggaagggcgatcggtgcgggcctcttcgctattacgccagctggcgaaagggggatgtgctgcaaggcgattaagttgggtaacgccagggttttcccagtcacgacgttaccccacagtggggccactagggtcaatttctgagaactgtcattctcggaaattgagtaaaacgacggccagtgagcgcgcctcgttcattcacgtttttgaacccgtggaggacgggcagactcgcggtgcaaatgtgttttacagcgtgatggagcagatgaagatgctcgacacgctgcagaacacgcagctagattaaccctagaaagataatcatattgtgacgtacgttaaagataatcatgcgtaaaattgacgcatgtgttttatcggtctgtatatcgaggtttatttattaatttgaatagatattaagttttattatatttacacttacatactaataataaattcaacaaacaatttatttatgtttatttatttattaaaaaaaaacaaaaactcaaaatttcttctataaagtaacaaaacttttatcgaattcctgcagcccgggggatccactagttctagagggacagcccccccccaaagcccccagggatgtaattacgtccctcccccgctagggggcagcagcgagccgcccggggctccgctccggtccggcgctccccccgcatccccgagccggcagcgtgcggggacagcccgggcacggggaaggtggcacgggatcgctttcctctgaacgcttctcgctgctctttgagcctgcagacacctggggggatacggggaaaaggcctccaaggccagcttcccacaataagttgggtgaattttggctcattcctcctttctataggattgaggtcagagctttgtgatgggaattctgtggaatgtgtgtcagttagggtgtggaaagtccctttactccctatcagtgatagagaacgtatgaagagtttactccctatcagtgatagagaacgtatgcagactttactccctatcagtgatagagaacgtataaggagtttactccctatcagtgatagagaacgtatgaccagtttactccctatcagtgatagagaacgtatctacagtttactccctatcagtgatagagaacgtatatccagtttactccctatcagtgatagagaacgtatgtcgaggtaggcgtgtacggtgggcgcctataaaagcagagctcgtttagtgaaccgtcagatcgcctggagcaattccacaacacttttgtcttatacttggtttagtgaaccgtcagatcagatctttgtcgatcctaccatccactcgacacacccgccagcggccgcagttgcgcagccatcgacgtcagacgcggaagcttcgatcaactacgcagacaggtaccaaaacaaatgttctcgtcacgtgggcatgaatctgatgctgtttccctgcagacaatgcgagagaatgaatcagaattcaaatatctgcttcactcacggacagaaagactgtttagagtgctttcccgtgtcagaatctcaacccgtttctgtcgtcaaaaaggcgtatcagaaactgtgctacattcatcatatcatgggaaaggtgccagacgcttgcactgcctgcgatctggtcaatgtggatttggatgactgcatctttgaacaataaatgatttaaatcaggtatgtcttttgttgatcaccctccagattggttggaagaagttggtgaaggtcttcgcgagtttttgggccttgaagcgggcccaccgaaaccaaaacccaatcagcagcatcaagatcaagcccgtggtcttgtgctgcctggttataactatctcggacccggaaacggtctcgatcgaggagagcctgtcaacagggcagacgaggtcgcgcgagagcacgacatctcgtacaacgagcagcttgaggcgggagacaacccctacctcaagtacaaccacgcggacgccgagtttcaggagaagctcgccgacgacacatccttcgggggaaacctcggaaaggcagtctttcaggccaagaaaagggttctcgaaccttttggcctggttgaagagggtgctaagacggcccctaccggaaagcggatagacgaccactttccaaaaagaaagaaggctcggaccgaagaggactccaagccttccacctcgtcagacgccgaagctggacccagcggatcccagcagctgcaaatcccagcccaaccagcctcaagtttgggagctgatacaatgtctgcgggaggtggcggcccattgggcgacaataaccaaggtgccgatggagtgggcaatgcctcgggagattggcattgcgattccacgtggatgggggacagagtcgtcaccaagtccacccgaacctgggtgctgcccagctacaacaaccaccagtaccgagagatcaaaagcggctccgtcgacggaagcaacgccaacgcctactttggatacagcaccccctgggggtactttgactttaaccgcttccacagccactggagcccccgagactggcaaagactcatcaacaactactggggcttcagaccccggtccctcagagtcaaaatcttcaacattcaagtcaaagaggtcacggtgcaggactccaccaccaccatcgccaacaacctcacctccaccgtccaagtgtttacggacgacgactaccagctgccctacgtcgtcggcaacgggaccgagggatgcctgccggccttccctccgcaggtctttacgctgccgcagtacggttacgcgacgctgaaccgcgacaacacagaaaatcccaccgagaggagcagcttcttctgcctagagtactttcccagcaagatgctgagaacgggcaacaactttgagtttacctacaactttgaggaggtgcccttccactccagcttcgctcccagtcagaacctgttcaagctggccaacccgctggtggaccagtacttgtaccgcttcgtgagcacaaataacactggcggagtccagttcaacaagaacctggccgggagatacgccaacacctacaaaaactggttcccggggcccatgggccgaacccagggctggaacctgggctccggggtcaaccgcgccagtgtcagcgccttcgccacgaccaataggatggagctcgagggcgcgagttaccaggtgcccccgcagccgaacggcatgaccaacaacctccagggcagcaacacctatgccctggagaacactatgatcttcaacagccagccggcgaacccgggcaccaccgccacgtacctcgagggcaacatgctcatcaccagcgagagcgagacgcagccggtgaaccgcgtggcgtacaacgtcggcgggcagatggccaccaacaaccagagctccaccactgcccccgcgaccggcacgtacaacctccaggaaatcgtgcccggcagcgtgtggatggagagggacgtgtacctccaaggacccatctgggccaagatcccagagacgggggcgcactttcacccctctccggccatgggcggattcggactcaaacacccaccgcccatgatgctcatcaagaacacgcctgtgcccggaaatatcaccagcttctcggacgtgcccgtcagcagcttcatcacccagtacagcaccgggcaggtcaccgtggagatggagtgggagctcaagaaggaaaactccaagaggtggaacccagagatccagtacacaaacaactacaacgacccccagtttgtggactttgccccggacagcaccggggaatacagaaccaccagacctatcggaacccgataccttacccgacccctttaagcgcggcagaacccctttgatttttaacccgggagttctagggatctggcggccgctcgagtctagagggcccgtttaaacccgctgatcagcctcgactgtgccttctagttgccagccatctgttgtttgcccctcccccgtgccttccttgaccctggaaggtgccactcccactgtcctttcctaataaaatgaggaaattgcatcgcattgtctgagtaggtgtcattctattctggggggtggggtggggcaggacagcaagggggaggattgggaagacaatagcaggcatgctggggatgcggtgggctctatgggcgatcgctagcgtttaaacttaagcttggtaccgagctcggatccactagtccagtgtggtggaattcctgcttcgcgatgtacgggccagatatacgcgttgtttacgctccggtgcccgtcagtgggcagagcgcacatcgcccacagtccccgagaagttggggggaggggtcggcaattgaaccggtgcctagagaaggtggcgcggggtaaactgggaaagtgatgtcgtgtactggctccgcctttttcccgagggtgggggagaaccgtatataagtgcagtagtcgccgtgaacgttctttttcgcaacgggtttgccgccagaacacaggtaagtgccgtgtgtggttcccgcgggcctggcctctttacgggttatggcccttgcgtgccttgaattacttccacgcccctggctgcagtacgtgattcttgatcccgagcttcgggttggaagtgggtgggagagttcgaggccttgcgcttaaggagccccttcgcctcgtgcttgagttgaggcctggcttgggcgctggggccgccgcgtgcgaatctggtggcaccttcgcgcctgtctcgctgctttcgataagtctctagccatttaaaatttttgatgacctgctgcgacgctttttttctggcaagatagtcttgtaaatgcgggccaagatctgcacactggtatttcggtttttggggccgcgggcggcgacggggcccgtgcgtcccagcgcacatgttcggcgaggcggggcctgcgagcgcggccaccgagaatcggacgggggtagtctcaagctggccggcctgctctggtgcctggcctcgcgccgccgtgtatcgccccgccctgggcggcaaggctggcccggtcggcaccagttgcgtgagcggaaagatggccgcttcccggccctgctgcagggagctcaaaatggaggacgcggcgctcgggagagcgggcgggtgagtcacccacacaaaggaaaagggcctttccgtcctcagccgtcgcttcatgtgactccacggagtaccgggcgccgtccaggcacctcgattagttctcgagcttttggagtacgtcgtctttaggttggggggaggggttttatgcgatggagtttccccacactgagtgggtggagactgaagttaggccagcttggcacttgatgtaattctccttggaatttgccctttttgagtttggatcttggttcattctcaagcctcagacagtggttcaaagtttttttcttccatttcaggtgtcgtgaacctgcaggatttaaattctagttcaccatgtctagactggacaagagcaaagtcataaactctgctctggaattactcaatggagtcggtatcgaaggcctgacgacaaggaaactcgctcaaaagctgggagttgagcagcctaccctgtactggcacgtgaagaacaagcgggccctgctcgatgccctgccaatcgagatgctggacaggcatcatacccactcctgccccctggaaggcgagtcatggcaagactttctgcggaacaacgccaagtcataccgctgtgctctcctctcacatcgcgacggggctaaagtgcatctcggcacccgcccaacagagaaacagtacgaaaccctggaaaatcagctcgcgttcctgtgtcagcaaggcttctccctggagaacgcactgtacgctctgtccgccgtgggccactttacactgggctgcgtattggaggaacaggagcatcaagtagcaaaagaggaaagagagacacctaccaccgattctatgcccccacttctgaaacaagcaattgagctgttcgaccggcagggagccgaacctgccttccttttcggcctggaactaatcatatgtggcctggagaaacagctaaagtgcgaaagcggcgggccgaccgacgcccttgacgattttgacttagacatgctcccagccgatgcccttgacgactttgaccttgatatgctgcctgctgacgctcttgacgattttgaccttgacatgctccccgggtaagcgtacagcggctcccgggagttctagggatctgcccctctccctcccccccccctaacgttactggccgaagccgcttggaataaggccggtgtgcgtttgtctatatgttattttccaccatattgccgtcttttggcaatgtgagggcccggaaacctggccctgtcttcttgacgagcattcctaggggtctttcccctctcgccaaaggaatgcaaggtctgttgaatgtcgtgaaggaagcagttcctctggaagcttcttgaagacaaacaacgtctgtagcgaccctttgcaggcagcggaaccccccacctggcgacaggtgcctctgcggccaaaagccacgtgtataagatacacctgcaaaggcggcacaaccccagtgccacgttgtgagttggatagttgtggaaagagtcaaatggctctcctcaagcgtattcaacaaggggctgaaggatgcccagaaggtaccccattgtatgggatctgatctggggcctcggtgcacatgctttacatgtgtttagtcgaggttaaaaaaacgtctaggccccccgaaccacggggacgtggttttcctttgaaaaacacgatgataaggatccaccggaggccaccatgaccgagtacaagcccacggtgcgcctcgccacccgcgacgacgtccccagggccgtacgcaccctcgccgccgcgttcgccgactaccccgccacgcgccacaccgtcgatccggaccgccacatcgagcgggtcaccgagctgcaagaactcttcctcacgcgcgtcgggctcgacatcggcaaggtgtgggtcgcggacgacggcgccgcggtggcggtctggaccacgccggagagcgtcgaagcgggggcggtgttcgccgagatcggcccgcgcatggccgagttgagcggttcccggctggccgcgcagcaacagatggaaggcctcctggcgccgcaccggcccaaggagcccgcgtggttcctggccaccgtcggcgtctcgcccgaccaccagggcaagggtctgggcagcgccgtcgtgctccccggagtggaggcggccgagcgcgccggggtgcccgccttcctggagacctccgcgccccgcaacctccccttctacgagcggctcggcttcaccgtcaccgccgacgtcgaggtgcccgaaggaccgcgcacctggtgcatgacccgcaagcccggtgcctgaccgcgtctggaacaatcaacctctggattacaaaatttgtgaaagattgactggtattcttaactatgttgctccttttacgctatgtggatacgctgctttaatgcctttgtatcatgctattgcttcccgtatggctttcattttctcctccttgtataaatcctggttgctgtctctttatgaggagttgtggcccgttgtcaggcaacgtggcgtggtgtgcactgtgtttgctgacgcaacccccactggttggggcattgccaccacctgtcagctcctttccgggactttcgctttccccctccctattgccacggcggaactcatcgccgcctgccttgcccgctgctggacaggggctcggctgttgggcactgacaattccgtggtgttgtcggggaagctgacgtcctttccatggctgctcgcctgtgttgccacctggattctgcgcgggacgtccttctgctacgtcccttcggccctcaatccagcggaccttccttcccgcggcctgctgccggctctgcggcctcttccgcgtcttcgccttcgccctcagacgagtcggatctccctttgggccgcctccccgcaaaatgaccgaccaagcgacgcccaacctgccatcacgagatttcgattccaccgccgccttctatgatcatgtctgggggtgggcgaagaactccagcatgagatccccgcgctggaggatcatccagccggcgtcccggaaaacgattccgaagcccaacctttgcctgcaggtcgactctagaggatccgaaaaaacctcccacacctccccctgaacctgaaacataaaatgaatgcaattgttgttgttaacttgtttattgcagcttataatggttacaaataaagcaatagcatcacaaatttcacaaataaagcatttttttcactgcattctagttgtggtttgtccaaactcatcaatgtatcttatcatgtctggatccccgcggccgcggtacccacgtgggcgcgccatttaaatgataactcagagagagtgtcctcgagccaatctggaagataaccatcggcagccatacctgatttaaatcatttattgttcaaagatgcagtcatccaaatccacattgaccagatcgcaggcagtgcaagcgtctggcacctttcccatgatatgatgaatgtagcacagtttctgatacgcctttttgacgacagaaacgggttgagattctgacacgggaaagcactctaaacagtctttctgtccgtgagtgaagcagatatttgaattctgattcattctctcgcattgtctgcagggaaacagcatcagattcatgcccacgtgacgagaacatttgttttggtacctgtctgcgtagttgatcgaagcttccgcgtctgacgtcgatggctgcgcaactgactcgcgcacccgtttgggctcacttatatctgcgtcactgggggcgggtcttttcttggctccaccctttttgacgtagaattcatgctccacctcaaccacgtgatcctttgcccaccggaaaaagtctttgacttcctgcttggtgaccttcccaaagtcatgatccagacggcgggtgagttcaaatttgaacatccggtcttgcaacggctgctggtgttcgaaggtcgttgagttcccgtcaatcacggcgcacatgttggtgttggaggtgacgatcacgggagtcgggtctatctgggccgaggacttgcatttctggtccacgcgcaccttgcttcctccgagaatggctttggccgactccacgaccttggcggtcatcttcccctcctcccaccagatcaccatcttgtcgacacagtcgttgaagggaaagttctcattggtccagtttacgcacccgtagaagggcacagtgtgggctatggcctccgcgatgttggtcttcccggtagttgcaggcccaaacagccagatggtgttcctcttgccgaactttttcgtggcccatcccagaaagacggaagccgcatattggggatcgtacccgtttagttccaaaattttataaatccgattgctggaaatgtcctccacgggctgctggcccaccaggtagtcgggggcggttttagtcaggctcataatctttcccgcattgtccaaggcagccttgatttgggaccgcgagttggaggccgcattgaaggagatgtatgaggcctggtcctcctggatccactgcttctccgaggtaatccccttgtccacgagccacccgaccagctccatgtacctggctgaagtttttgatctgatcaccggcgcatcagaattgggattctgattctctttgttctgctcctgcgtctgcgacacgtgcgtcagatgctgcgccaccaaccgtttacgctccgtgagattcaaacaggcgcttaaatactgttccatattagtccacgcccactggagctcaggctgggttttggggagcaagtaattggggatgtagcactcatccaccaccttgttcccgcctccggcgccatttctggtctttgtgaccgcgaaccagtttggcaaagtcggctcgatcccgcggtaaattctctgaatcagtttttcgcgaatctgactcaggaaacgtcccaaaaccatggatttcaccccggtggtttccacgagcacgtgcatgtggaagtagctctctcccttctcaaattgcacaaagaaaagggcctccggggccttactcacacggcgccattccgtcagaaagtcgcgctgcagcttctcggccacggtcaggggtgcctgctcaatcagattcagatccatgtcagaatctggcggcaactcccattccttctcggccacccagttcacaaagctgtcagaaatgccgggcagatgctcgtcaaggtcgctggggaccttaatcacaatctcgtaaaaccccggcatggcggcgataactattatcatcgtgtttttcaaaggaaaaccacgtccccgtggttcggggggcctagacgtttttttaacctcgactaaacacatgtaaagcatgtgcaccgaggccccagatcagatcccatacaatggggtaccttctgggcatccttcagccccttgttgaatacgcttgaggagagccatttgactctttccacaactatccaactcacaacgtggcactggggttgtgccgcctttgcaggtgtatcttatacacgtggcttttggccgcagaggcacctgtcgccaggtggggggttccgctgcctgcaaagggtcgctacagacgttgtttgtcttcaagaagcttccagaggaactgcttccttcacgacattcaacagaccttgcattcctttggcgagaggggaaagacccctaggaatgctcgtcaagaagacagggccaggtttccgggccctcacattgccaaaagacggcaatatggtggaaaataacatatagacaaacgcacaccggccttattccaagcggcttcggccagtaacgttagggggggggggcggaattctatccctcagttatctcagagagagtgtcctcgagccaatctggaagataaccatcggcagccatacctgatttaaatcatttattgttcaaagatgcagtcatccaaatccacattgaccagatcgcaggcagtgcaagcgtctggcacctttcccatgatatgatgaatgtagcacagtttctgatacgcctttttgacgacagaaacgggttgagattctgacacgggaaagcactctaaacagtctttctgtccgtgagtgaagcagatatttgaattctgattcattctctcgcattgtctgcagggaaacagcatcagattcatgcccacgtgacgagaacatttgttttggtacctgtctgcgtagttgatcgaagcttccgcgtctgacgtcgatggctgcgcaactgactcgcgcacccgtttgggctcacttatatctgcgtcactgggggcgggtcttttcttggctccaccctttttgacgtagaattcatgctccacctcaaccacgtgatcctttgcccaccggaaaaagtctttgacttcctgcttggtgaccttcccaaagtcatgatccagacggcgggtgagttcaaatttgaacatccggtcttgcaacggctgctggtgttcgaaggtcgttgagttcccgtcaatcacggcgcacatgttggtgttggaggtgacgatcacgggagtcgggtctatctgggccgaggacttgcatttctggtccacgcgcaccttgcttcctccgagaatggctttggccgactccacgaccttggcggtcatcttcccctcctcccaccagatcaccatcttgtcgacacagtcgttgaagggaaagttctcattggtccagtttacgcacccgtagaagggcacagtgtgggctatggcctccgcgatgttggtcttcccggtagttgcaggcccaaacagccagatggtgttcctcttgccgaactttttcgtggcccatcccagaaagacggaagccgcatattggggatcgtacccgtttagttccaaaattttataaatccgattgctggaaatgtcctccacgggctgctggcccaccaggtagtcgggggcggttttagtcaggctcataatctttcccgcattgtccaaggcagccttgatttgggaccgcgagttggaggccgcattgaaggagatgtatgaggcctggtcctcctggatccactgcttctccgaggtaatccccttgtccacgagccacccgaccagctccatggtggcgttatccggccgatcgatagatctgggccccggtgtcgactttacgagggtaggaagtggtacggaaagttggtataagacaaaagtgttgtggaattgctggaggcgatctgacggttcactaaacgagctctgcttttataggcgcccaccgtacacgcctaaagcttatacgttctctatcactgatagggagtaaactggatatacgttctctatcactgatagggagtaaactgtagatacgttctctatcactgatagggagtaaactggtcatacgttctctatcactgatagggagtaaactccttatacgttctctatcactgatagggagtaaagtctgcatacgttctctatcactgatagggagtaaactcttcatacgttctctatcactgatagggagtaaacgaatggctaggatccggccggcctgcaggtgtcctcacaggaacgaagtccctaaagaaacagtggcagccaggtttagccccggaattgactggattccttttttagggcccattggtatggctttttccccgtatccccccaggtgtctgcaggctcaaagagcagcgagaagcgttcagaggaaagcgatcccgtgccaccttccccgtgcccgggctgtccccgcacgctgccggctcggggatgcggggggagcgccggaccggagcggagccccgggcggctcgctgctgccccctagcgggggagggacgtaattacatccctgggggctttgggggggggctgtccctctagagcggccgccaccgcggtggagctccagcttttgttccctttagtgagggttaattagatcttaatacgactcactatagggcgaattgggtaccgggccccccctcgaggtcgacggtatcgcctccaaggccagcttcccacaataagttgggtgaattttggctcattcctcctttctataggattgaggtcagagctttgtgatgggaattctgtggaatgtgtgtcagttagggtgtggaaagtcccgcgatcgctagcaaacgccagcaacgcggcctttttacggttcctggccttttgctggccttttgctcacatgtcctgcaggcagctgcgcgctcgctcgctcactgaggccgcccgggcaaagcccgggcgtcgggcgacctttggtcgcccggcctcagtgagcgagcgagcgcgcagagagggagtggccaactccatcactaggggttcctgcggccgcacgcgtggagctagttattaatagtaatcaattacggggtcattagttcatagcccatatatggagttccgcgttacataacttacggtaaatggcccgcctggctgaccgcccaacgacccccgcccattgacgtcaataatgacgtatgttcccatagtaacgtcaatagggactttccattgacgtcaatgggtggagtatttacggtaaactgcccacttggcagtacatcaagtgtatcatatgccaagtacgccccctattgacgtcaatgacggtaaatggcccgcctggcattatgcccagtacatgaccttatgggactttcctacttggcagtacatctacgtattagtcatcgctattaccatggtgatgcggttttggcagtacatcaatgggcgtggatagcggtttgactcacggggatttccaagtctccaccccattgacgtcaatgggagtttgttttgcaccaaaatcaacgggactttccaaaatgtcgtaacaactccgccccattgacgcaaatgggcggtaggcgtgtacggtgggaggtctatataagcagagctcgtttagtgaaccgtcagatcgcctggagacgccatccacgctgttttgacctccatagaagacaccgggaccgatccagcctccgcggattcgaatcccggccgggaacggtgcattggaacgcggattccccgtgccaagagtgacgtaagtaccgcctatagagtctataggcccacaaaaaatgctttcttcttttaatatacttttttgtttatcttatttctaatactttccctaatctctttctttcagggcaataatgatacaatgtatcatgcctctttgcaccattctaaagaataacagtgataatttctgggttaaggcaatagcaatatttctgcatataaatatttctgcatataaattgtaactgatgtaagaggtttcatattgctaatagcagctacaatccagctaccattctgcttttattttatggttgggataaggctggattattctgagtccaagctaggcccttttgctaatcatgttcatacctcttatcttcctcccacagctcctgggcaacgtgctggtctgtgtgctggcccatcactttggcaaagaattgggattcgaacatcgattgaattctgaatggtgagcaagggcgaggagctgttcaccggggtggtgcccatcctggtcgagctggacggcgacgtaaacggccacaagttcagcgtgtccggcgagggcgagggcgatgccacctacggcaagctgaccctgaagttcatctgcaccaccggcaagctgcccgtgccctggcccaccctcgtgaccaccctgacctacggcgtgcagtgcttcagccgctaccccgaccacatgaagcagcacgacttcttcaagtccgccatgcccgaaggctacgtccaggagcgcaccatcttcttcaaggacgacggcaactacaagacccgcgccgaggtgaagttcgagggcgacaccctggtgaaccgcatcgagctgaagggcatcgacttcaaggaggacggcaacatcctggggcacaagctggagtacaactacaacagccacaacgtctatatcatggccgacaagcagaagaacggcatcaaggtgaacttcaagatccgccacaacatcgaggacggcagcgtgcagctcgccgaccactaccagcagaacacccccatcggcgacggccccgtgctgctgcccgacaaccactacctgagcacccagtccgccctgagcaaagaccccaacgagaagcgcgatcacatggtcctgctggagttcgtgaccgccgccgggatcactctcggcatggacgagctgtacaagtactcagatctcgagctcaagtagggatcctctagagtcgacctgcagaagcttgcctcgagcagcgctgctcgagagatctacgggtggcatccctgtgacccctccccagtgcctctcctggccctggaagttgccactccagtgcccaccagccttgtcctaataaaattaagttgcatcattttgtctgactaggtgtccttctataatattatggggtggaggggggtggtatggagcaaggggcaagttgggaagacaacctgtagggcctgcggggtctattgggaaccaagctggagtgcagtggcacaatcttggctcactgcaatctccgcctcctgggttcaagcgattctcctgcctcagcctcccgagttgttgggattccaggcatgcatgaccaggctcagctaatttttgtttttttggtagagacggggtttcaccatattggccaggctggtctccaactcctaatctcaggtgatctacccaccttggcctcccaaattgctgggattacaggcgtgaaccactgctcccttccctgtccttctgattttgtaggtaaccacgtgcggaccgagcggccgcaggaacccctagtgatggagttggccactccctctctgcgcgctcgctcgctcactgaggccgggcgaccaaaggtcgcccgacgcccgggctttgcccgggcggcctcagtgagcgagcgagcgcgcagctgcctgcaggggcgcctgatgcggtattttctccttacgcatctgtgcggtatttcacaccgcatacgtcgtagctgatcaattggcgcgccgaattcgttaacaagctttaattaacgcgtacgataagcttgatatctataacaagaaaatatatatataataagttatcacgtaagtagaacatgaaataacaatataattatcgtatgagttaaatcttaaaagtcacgtaaaagataatcatgcgtcattttgactcacgcggtcgttatagttcaaaatcagtgacacttaccgcattgacaagcacgcctcacgggagctccaagcggcgactgagatgtcctaaatgcacagcgacggattcgcgctatttagaaagagagagcaatatttcaagaatgcatgcgtcaattttacgcagactatctttctagggttaatctagctgcatcaggatcatatcgtcgggtcttttttccggctcagtcatcgcccaagctggcgctatctgggcatcggggaggaagaagcccgtgccttttcccgcgaggttgaagcggcatggaaagagtttgccgaggatgactgctgctgcattgacgttgagcgaaaacgcacgtttaccatgatgattcgggaaggtgtggccatgcacgcctttaacggtgaactgttcgttcaggccacctgggataccagttcgtcgcggcttttccggacacagttccggatggtcagcccgaagcgcatcagcaacccgaacaataccggcgacagccggaactgccgtgccggtgtgcagattaatgacagcggtgcggcgctgggatattacgtcagcgaggacgggtatcctggctggatgccgcagaaatggacatggataccccgtgagttacccggcgggcgcgcttggcgtaatcatggtcatagctgtttcctgctcgtgtccgataactgtaattatcggacatgattgtgaaattgttatccgctcacaattccacacaacatacgagccggaagcataaagtgtaaagcctggggtgcctaatgagtgagctaactcacattaattgcgttgcgctcactgcccgctttccagtcgggaaacctgtcgtgccagctgcattaatgaatcggccaacgcgcggggagaggcggtttgcgtattgggcgctcttccgcttcctcgctcactgactcgctgcgctcggtcgttcggctgcggcgagcggtatcagctcactcaaaggcggtaatacggttatccacagaatcaggggataacgcaggaaagaacatgtgagcaaaaggccagcaaaaggccaggaaccgtaaaaaggccgcgttgctggcgttatgactctcttaaggtagccaaaatggtgcactctcagtacaatctgctctgatgccgcatagtatgttgtaactaaagatctactgtggataactctgtcaggaagcttggatcaaccggtagttatccaaagaacaactgttgttcagtttttgagttgtgtataacccctcattctgatcccagcttatacggtccaggatcaccgatcattcacagttaatgatcctttccaggttgttgatcttaaaagccggatccttgttatccacagggcagtgcgatcctaataagagatcacaatagaacagatctctaaataaatagatcttctttttaatactttagttacaacatactgttaagccagccccgacacccgccaacacccgctgacgcg

SEQ ID NO: 21 - DNA, 8681 bp, synthetic construct
  misc_feature 1..8681: note = plasmid
  source 1..8681: mol_type = other DNA
taagcggccgctacgtcgacgtttaaaccatacaatcagcattggtagctgctgtattgctacttgtgattgctccatgtttttctaggtctcgactgcagaattaattccaggcggggaggcggcccaaagggagatccgactcgtctgagggcgaaggcgaagacgcggaagaggccgcagagccggcagcaggccgcgggaaggaaggtccgctggattgagggccgaagggacgtagcagaaggacgtcccgcgcagaatccaggtggcaacacaggcgagcagccatggaaaggacgtcagcttccccgacaacaccacggaattgtcagtgcccaacagccgagcccctgtccagcagcgggcaaggcaggcggcgatgagttccgccgtggcaatagggagggggaaagcgaaagtcccggaaaggagctgacaggtggtggcaatgccccaaccagtgggggttgcgtcagcaaacacagtgcacaccacgccacgttgcctgacaacgggccacaactcctcataaagagacagcaaccaggatttatacaaggaggagaaaatgaaagccatacgggaagcaatagcatgatacaaaggcattaaagcagcgtatccacatagcgtaaaaggagcaacatagttaagaataccagtcaatctttcacaaattttgtaatccagaggttgattgttccagacgcgttcagaagaactcgtcaagaaggcgatagaaggcgatgcgctgcgaatcgggagcggcgataccgtaaagcacgaggaagcggtcagcccattcgccgccaagctcttcagcaatatcacgggtagccaacgctatgtcctgatagcggtccgccacacccagccggccacagtcgatgaatccagaaaagcggccattttccaccatgatattcggcaagcaggcatcgccatgggtcacgacgagatcctcgccgtcgggcatgcgcgccttgagcctggcgaacagttcggctggcgcgagcccctgatgctcttcgtccagatcatcctgatcgacaagaccggcttccatccgagtacgtgctcgctcgatgcgatgtttcgcttggtggtcgaatgggcaggtagccggatcaagcgtatgcagccgccgcattgcatcagccatgatggatactttctcggcaggagcaaggtgagatgacaggagatcctgccccggcacttcgcccaatagcagccagtcccttcccgcttcagtgacaacgtcgagcacagctgcgcaaggaacgcccgtcgtggccagccacgatagccgcgctgcctcgtcctgcagttcattcagggcaccggacaggtcggtcttgacaaaaagaaccgggcgcccctgcgctgacagccggaacacggcggcatcagagcagccgattgtctgttgtgcccagtcatagccgaatagcctctccacccaagcggccggagaacctgcgtgcaatccatcttgttcagccatggcggcgttaactgcaggtcgaaaggcccggagatgaggaagaggagaacagcgcggcagacgtgcgcttttgaagcgtgcagaatgccgggcctccggaggaccttcgggcgcccgccccgcccctgagcccgcccctgagcccgcccccggacccaccccttcccagcctctgagcccagaaagcgaaggagcaaagctgctattggccgctgccccaaaggcctacccgcttccattgctcagcggtgctgtccatctgcacgagactagtgagacgtgctacttccatttgtcacgtcctgcacgacgcgagctgcggggcgggggggaacttcctgactaggggaggagtagaaggtggcgcgaaggggccaccaaagaacggagccggttggcgcctaccggtggatgtggaatgtgtgcgaggccagaggccacttgtgtagcgccaagtgcccagcggggctgctaaagcgcatgctccagactgccttgggaaaagcgcctcccctacccggtagaattggatctagttacccggggagcatgtcaaggtcaaaatcgtcaagagcgtcagcaggcagcatatcaaggtcaaagtcgtcaagggcatcggctgggagcatgtctaagtcaaaatcgtcaagggcgtcggtcggcccgccgctttcgcactttagctgtttctccaggccacatatgattagttccaggccgaaaaggaaggcaggttcggctccctgccggtcgaacagctcaattgcttgtttcagaagtgggggcatagaatcggtggtaggtgtctctctttcctcttttgctacttgatgctcctgttcctccaatacgcagcccagtgtaaagtggcccacggcggacagagcgtacagtgcgttctccagggagaagccttgctgacacaggaacgcgagctgattttccagggtttcgtactgtttctctgttgggcgggtgccgagatgcactttagccccgtcgcgatgtgagaggagagcacagcggtatgacttggcgttgttccgcagaaagtcttgccatgactcgccttccagggggcaggagtgggtatgatgcctgtccagcatctcgattggcagggcatcgagcagggcccgcttgttcttcacgtgccagtacagggtaggctgctcaactcccagcttttgagcgagtttccttgtcgtcaggccttcgataccgactccattgagtaattccagagcagagtttatgactttgctcttgtccagtctagacatggtgaactagaatttaaatcctgcaggttcacgacacctgaaatggaagaaaaaaactttgaaccactgtctgaggcttgagaatgaaccaagatccaaactcaaaaagggcaaattccaaggagaattacatcaagtgccaagctggcctaacttcagtctccacccactcagtgtggggaaactccatcgcataaaacccctccccccaacctaaagacgacgtactccaaaagctcgagaactaatcgaggtgcctggacggcgcccggtactccgtggagtcacatgaagcgacggctgaggacggaaaggcccttttcctttgtgtgggtgactcacccgcccgctctcccgagcgccgcgtcctccattttgagctccctgcagcagggccgggaagcggccatctttccgctcacgcaactggtgccgaccgggccagccttgccgcccagggcggggcgatacacggcggcgcgaggccaggcaccagagcaggccggccagcttgagactacccccgtccgattctcggtggccgcgctcgcaggccccgcctcgccgaacatgtgcgctgggacgcacgggccccgtcgccgcccgcggccccaaaaaccgaaataccagtgtgcagatcttggcccgcatttacaagactatcttgccagaaaaaaagcgtcgcagcaggtcatcaaaaattttaaatggctagagacttatcgaaagcagcgagacaggcgcgaaggtgccaccagattcgcacgcggcggccccagcgcccaagccaggcctcaactcaagcacgaggcgaaggggctccttaagcgcaaggcctcgaactctcccacccacttccaacccgaagctcgggatcaagaatcacgtactgcagccaggggcgtggaagtaattcaaggcacgcaagggccataacccgtaaagaggccaggcccgcgggaaccacacacggcacttacctgtgttctggcggcaaacccgttgcgaaaaagaacgttcacggcgactactgcacttatatacggttctcccccaccctcgggaaaaaggcggagccagtacacgacatcactttcccagtttaccccgcgccaccttctctaggcaccggttcaattgccgacccctccccccaacttctcggggactgtgggcgatgtgcgctctgcccactgacgggcaccggagcctcacgaattcgatatcgataaactggatctctgctgtccctgtaataaacccgaatatgatcagctcactcaaaggcggtaatacggttatccacagaatcaggggataacgcaggaaagaacatgtgagcaaaaggccagcaaaaggccaggaaccgtaaaaaggccgcgttgctggcgtttttccataggctccgcccccctgacgagcatcacaaaaatcgacgctcaagtcagaggtggcgaaacccgacaggactataaagataccaggcgtttccccctggaagctccctcgtgcgctctcctgttccgaccctgccgcttaccggatacctgtccgcctttctcccttcgggaagcgtggcgctttctcatagctcacgctgtaggtatctcagttcggtgtaggtcgttcgctccaagctgggctgtgtgcacgaaccccccgttcagcccgaccgctgcgccttatccggtaactatcgtcttgagtccaacccggtaagacacgacttatcgccactggcagcagccactggtaacaggattagcagagcgaggtatgtaggcggtgctacagagttcttgaagtggtggcctaactacggctacactagaagaacagtatttggtatctgcgctctgctgaagccagttaccttcggaaaaagagttggtagctcttgatccggcaaacaaaccaccgctggtagcggtggtttttttgtttgcaagcagcagattacgcgcagaaaaaaaggatctcaagaagatcctttgatcttttctacggggtctgacgctcagtggaacgaaaactcacgttaagggattttggtcatgagattatcaaaaaggatcttcacctagatccttttaaattaaaaatgaagttttaaatcaatctaaagtatatatgagtaaacttggtctgacagttaccaatgcttaatcagtgaggcacctatctcagcgatctgtctatttcgttcatccatagttgcctgactccccgtcgtgtagataactacgatacgggagggcttaccatctggccccagtgctgcaatgataccgcgagacccacgctcaccggctccagatttatcagcaataaaccagccagccggaagggccgagcgcagaagtggtcctgcaactttatccgcctccatccagtctattaattgttgccgggaagctagagtaagtagttcgccagttaatagtttgcgcaacgttgttgccattgctacaggcatcgtggtgtcacgctcgtcgtttggtatggcttcattcagctccggttcccaacgatcaaggcgagttacatgatcccccatgttgtgcaaaaaagcggttagctccttcggtcctccgatcgttgtcagaagtaagttggccgcagtgttatcactcatggttatggcagcactgcataattctcttactgtcatgccatccgtaagatgcttttctgtgactggtgagtactcaaccaagtcattctgagaatagtgtatgcggcgaccgagttgctcttgcccggcgtcaatacgggataataccgcgccacatagcagaactttaaaagtgctcatcattggaaaacgttcttcggggcgaaaactctcaaggatcttaccgctgttgagatccagttcgatgtaacccactcgtgcacccaactgatcttcagcatcttttactttcaccagcgtttctgggtgagcaaaaacaggaaggcaaaatgccgcaaaaaagggaataagggcgacacggaaatgttgaatactcatactcttcctttttcaatattattgaagcatttatcagggttattgtctcatgagcggatacatatttgaatgtatttagaaaaataaacaaataggggttccgcgcacatttccccgaaaagtgccacctaaattgtaagcgttaatattttgttaaaattcgcgttaaatttttgttaaatcagctcattttttaaccaataggccgaaatcggcaaaatcccttataaatcaaaagaatagaccgagatagggttgagtgttgttccagtttggaacaagagtccactattaaagaacgtggactccaacgtcaaagggcgaaaaaccgtctatcagggcgatggcccactacgtgaaccatcaccctaatcaagttttttggggtcgaggtgccgtaaagcactaaatcggaaccctaaagggagcccccgatttagagcttgacggggaaagccggcgaacgtggcgagaaaggaagggaagaaagcgaaaggagcgggcgctagggcgctggcaagtgtagcggtcacgctgcgcgtaaccaccacacccgccgcgcttaatgcgccgctacagggcgcgatggatccgcggccgcttaagccataccaatggtttactccctatcagtgatagagaacgtatgaagagtttactccctatcagtgatagagaacgtatgcagactttactccctatcagtgatagagaacgtataaggagtttactccctatcagtgatagagaacgtatgaccagtttactccctatcagtgatagagaacgtatctacagtttactccctatcagtgatagagaacgtatatccagtttactccctatcagtgatagagaacgtatgtcgaggtaggcgtgtacggtgggcgcctataaaagcagagctcgtttagtgaaccgtcagatcgcctggagcaattccacaacacttttgtcttatacttggtttagtgaaccgtcagatcagatctttgtcgatcctaccatccactcgacacacccgccagcggccggccaccatggccagtcgggaagaggagcagcgcgaaaccacccccgagcgcggacgcggtgcggcgcgacgtcccccaaccatggaggacgtgtcgtccccgtccccgtcgccgccgcctccccgggcgcccccaaaaaagcggatgaggcggcgtatcgagtccgaggacgaggaagactcatcacaagacgcgctggtgccgcgcacacccagcccgcggccatcgacctcggcggcggatttggccattgcgcccaagaagaaaaagaagcgcccttctcccaagcccgagcgcccgccatcaccagaggtaatcgtggacagcgaggaagaaagagaagatgtggcgctacaaatggtgggtttcagcaacccaccggtgctaatcaagcatggcaaaggaggtaagcgcacagtgcggcggctgaatgaagacgacccagtggcgcgtggtatgcggacgcaagaggaagaggaagagcccagcgaagcggaaagtgaaattacggtgatgaacccgctgagtgtgccgatcgtgtctgcgtgggagaagggcatggaggctgcgcgcgcgctgatggacaagtaccacgtggataacgatctaaaggcgaacttcaaactactgcctgaccaagtggaagctctggcggccgtatgcaagacctggctgaacgaggagcaccgcgggttgcagctgaccttcaccagcaacaagacctttgtgacgatgatggggcgattcctgcaggcgtacctgcagtcgtttgcagaggtgacctacaagcatcacgagcccacgggctgcgcgttgtggctgcaccgctgcgctgagatcgaaggcgagcttaagtgtctacacggaagcattatgataaataaggagcacgtgattgaaatggatgtgacgagcgaaaacgggcagcgcgcgctgaaggagcagtctagcaaggccaagatcgtgaagaaccggtggggccgaaatgtggtgcagatctccaacaccgacgcaaggtgctgcgtgcacgacgcggcctgtccggccaatcagttttccggcaagtcttgcggcatgttcttctctgaaggcgcaaaggctcaggtggcttttaagcagatcaaggcttttatgcaggcgctgtatcctaacgcccagaccgggcacggtcaccttttgatgccactacggtgcgagtgcaactcaaagcctgggcacgcgccctttttgggaaggcagctaccaaagttgactccgttcgccctgagcaacgcggaggacctggacgcggatctgatctccgacaagagcgtgctggccagcgtgcaccacccggcgctgatagtgttccagtgctgcaaccctgtgtatcgcaactcgcgcgcgcagggcggaggccccaactgcgacttcaagatatcggcgcccgacctgctaaacgcgttggtgatggtgcgcagcctgtggagtgaaaacttcaccgagctgccgcggatggttgtgcctgagtttaagtggagcactaaacaccagtatcgcaacgtgtccctgccagtggcgcatagcgatgcgcggcagaacccctttgattttgattacaaggacgacgatgacaagtaaggatccaattctaccatcgatttctggatccgcaggcctctgctagcttgactgactgagatacagcgtaccttcagctcacagacatgataagatacattgatgagtttggacaaaccacaactagaatgcagtgaaaaaaatgctttatttgtgaaatttgtgatgctattgctttatttgtaaccattataagctgcaataaacaagtttcatgtctg

SEQ ID NO: 22 - DNA, 22033 bp, synthetic construct; identical to SEQ ID NO: 19
  misc_feature 1..22033: note = plasmid
  source 1..22033: mol_type = other DNA

SEQ ID NO: 23 - DNA, 7601 bp, synthetic construct
  misc_feature 1..7601: note = plasmid
  source 1..7601: mol_type = other DNA
tcgcgcgtttcggtgatgacggtgaaaacctctgacacatgcagctcccggagactgtcacagcttgtctgtaagcggatgccgggagcagacaagcccgtcagggcgcgtcagcgggtgttggcgggtgtcggggctggcttaactatgcggcatcagagcagattgtactgagagtgcaccatatgcggtgtgaaataccgcacagatgcgtaaggagaaaataccgcatcaggcgccattcgccattcaggctgcgcaactgttgggaagggcgatcggtgcgggcctcttcgctattacgccagctggcgaaagggggatgtgctgcaaggcgattaagttgggtaacgccagggttttcccagtcacgacgttgtaaaacgacggccagtgaattgacgcgtattgggatggatccgcggccgcttaagccataccaatggtttactccctatcagtgatagagaacgtatgaagagtttactccctatcagtgatagagaacgtatgcagactttactccctatcagtgatagagaacgtataaggagtttactccctatcagtgatagagaacgtatgaccagtttactccctatcagtgatagagaacgtatctacagtttactccctatcagtgatagagaacgtatatccagtttactccctatcagtgatagagaacgtatgtcgaggtaggcgtgtacggtgggcgcctataaaagcagagctcgtttagtgaaccgtcagatcgcctggagcaattccacaacacttttgtcttatacttggtttagtgaaccgtcagatcagatctttgtcgatcctaccatccactcgacacacccgccagcggccggccaccatggcccttagtaagcacggcctgactaaggacatgaccatgaagtaccatatggagggctcggtggacgggcacaagttcgtgattacgggccacgggaacggcaacccattcgaggggaaacagacaatgaacctgtgtgtggtggaaggcggacccctgcccttctcggaggacatcctgtccgcaacctttgactacggcaatcgcgtgttcacagagtatccacagggtatggtggatttctttaagaacagctgtcccgcaggatacacctggcaccgcagcctgctcttcgaggacggggcggtgtgtaccacctccgctgatatcaccgtgtccgtcgaggagaactgcttctaccacaacagcaaattccacggcgtgaactttcctgccgacgggcctgtgatgaagaaaatgactacgaattgggagcccagctgcgagaaaatcatcccggtccctcgtcagggaatcttgaagggcgacatcgcaatgtacctcctgctcaaggacgggggaagataccgatgccagttcgataccatctacaaggcaaagtccgatcccaaggagatgccagagtggcacttcatccagcacaaactcacccgcgaggaccgctcagatgccaagaaccagaagtggcaactggtcgagcacgccgtggcatcccgtagcgccctgccagggtaatcgttactggccgaagccgcttggaataaggccggtgtgcgtttgtctatatgttattttccaccatattgccgtcttttggcaatgtgagggcccggaaacctggccctgtcttcttgacgagcattcctaggggtctttcccctctcgccaaaggaatgcaaggtctgttgaatgtcgtgaaggaagcagttcctctggaagcttcttgaagacaaacaacgtctgtagcgaccctttgcaggcagcggaaccccccacctggcgacaggtgcctctgcggccaaaagccacgtgtataagatacacctgcaaaggcggcacaaccccagtgccacgttgtgagttggatagttgtggaaagagtcaaatggctcccctcaagcgtattcaacaaggggctgaaggatgcccagaaggtaccccattgtatgggatctgatctggggcctcggtgcacatgctttacatgtgtttagtcgaggttaaaaaacgtctaggccccccgaaccacggggacgtggttttctttgaaaaacacgatgataatacggaaatatgactacgtccggcgttccatttggcatgacactacgaccaacacgatctcggttgtctcggcgcactccgtacagtagggatcgcctacctccttttgagacagagacccgcgctaccatactggaggatcatccgctgctgcccgaatgtaacactttgacaatgcacaacgtgagttacgtgcgaggtcttccctgcagtgtgggatttacgctgattcaggaatgggttgttccctgggatatggttctgacgcgggaggagcttgtaatcctgaggaagtgtatgcacgtgtgcctgtgttgtgccaacattgatatcatgacgagcatgatgatccatggttacgagtcctgggctctccactgtcattgttccagtcccggttccctgcagtgcatagccggcgggcaggttttggccagctggtttaggatggtggtggatggcgccatgtttaatcagaggtttatatggtaccgggaggtggtgaattacaacatgccaaaagaggtaatgtttatgtccagcgtgtttatgaggggtcgccacttaatctacctgcgcttgtggtatgatggccacgtgggttctgtggtccccgccatgagctttggatacagcgccttgcactgtgggattttgaacaatattgtggtgctgtgctgcagttactgtgctgatttaagtgagatcagggtgcgctgctgtgcccggaggacaaggcgtctcatgctgcgggcggtgcgaatcatcgctgaggagaccactgccatgttgtattcctgcaggacggagcggcggcggcagcagtttattcgcgcgctgctgcagcaccaccgccctatcctgatgcacgattatgactctacccccatgtaggcggccgctcgagtctagagggcccgtttaaacccgctgatcagcctcgactgtgccttctagttgccagccatctgttgtttgcccctcccccgtgccttccttgaccctggaaggtgccactcccactgtcctttcctaataaaatgaggaaattgcatcgcattgtctgagtaggtgtcattctattctggggggtggggtggggcaggacagcaagggggaggattgggaagacaatagcaggcatgctggggatgcggtgggctctatggtcatgttctagactgtaagcggccgctacgtcgacgtttaaaccatacaatcagcattggtagctgctgtattgctacttgtgattgctccatgtttttctaggtctcgactgcagaattaattccagagatctatcgataaggacagggaagggagcagtggttcacgcctgtaatcccagcaatttgggaggccaaggtgggtagatcacctgagattaggagttggagaccagcctggccaatatggtgaaaccccgtctctaccaaaaaaacaaaaattagctgagcctggtcatgcatgcctggaatcccaacaactcgggaggctgaggcaggagaatcgcttgaacccaggaggcggagattgcagtgagccaagattgtgccactgcactccagcttggttcccaatagaccccgcaggccctacaggttgtcttcccaacttgccccttgctccataccacccccctccaccccataatattatagaaggacacctagtcagacaaaatgatgcaacttaattttattaggacaaggctggtgggcactggagtggcaacttccagggccaggagaggcactggggaggggtcacagggatgccacccgtggatcaactgatacaaaggcattaaagcagcgtatccacatagcgtaaaaggagcaacatagttaagaataccagtcaatctttcacaaattttgtaatccagaggttgatttcagaagaactcgtcaagaaggcgatagaaggcgatgcgctgcgaatcgggagcggcgataccgtaaagcacgaggaagcggtcagcccattcgccgccaagctcttcagcaatatcacgggtagccaacgctatgtcctgatagcggtccgccacacccagccggccacagtcgatgaatccagaaaagcggccattttccaccatgatattcggcaagcaggcatcgccatgggtcacgacgagatcctcgccgtcgggcatgcgcgccttgagcctggcgaacagttcggctggcgcgagcccctgatgctcttcgtccagatcatcctgatcgacaagaccggcttccatccgagtacgtgctcgctcgatgcgatgtttcgcttggtggtcgaatgggcaggtagccggatcaagcgtatgcagccgccgcattgcatcagccatgatggatactttctcggcaggagcaaggtgagatgacaggagatcctgccccggcacttcgcccaatagcagccagtcccttcccgcttcagtgacaacgtcgagcacagctgcgcaaggaacgcccgtcgtggccagccacgatagccgcgctgcctcgtcctgcagttcattcagggcaccggacaggtcggtcttgacaaaaagaaccgggcgcccctgcgctgacagccggaacacggcggcatcagagcagccgattgtctgttgtgcccagtcatagccgaatagcctctccacccaagcggccggagaacctgcgtgcaatccatcttgttcagccatggcggcgttaactgcaggtcgaaaggcccggagatgaggaagaggagaacagcgcggcagacgtgcgcttttgaagcgtgcagaatgccgggcctccggaggaccttcgggcgcccgccccgcccctgagcccgcccctgagcccgcccccggacccaccccttcccagcctctgagcccagaaagcgaaggagcaaagctgctattggccgctgccccaaaggcctacccgcttccattgctcagcggtgctgtccatctgcacgagactagtgagacgtgctacttccatttgtcacgtcctgcacgacgcgagctgcggggcgggggggaacttcctgactaggggaggagtagaaggtggcgcgaaggggccaccaaagaacggagccggttggcgcctaccggtggatgtggaatgtgtgcgaggccagaggccacttgtgtagcgccaagtgcccagcggggctgctaaagcgcatgctccagactgccttgggaaaagcgcctcccctacccggtagaattggatctatcccaatggcgcgccgagcttggcgtaatcatggtcatagctgtttcctgtgtgaaattgttatccgctcacaattccacacaacatacgagccggaagcataaagtgtaaagcctggggtgcctaatgagtgagctaactcacattaattgcgttgcgctcactgcccgctttccagtcgggaaacctgtcgtgccagctgcattaatgaatcggccaacgcgcggggagaggcggtttgcgtattgggcgctgttccgcttcctcgctcactgactcgctgcgctcggtcgttcggctgcggcgagcggtatcagctcactcaaaggcggtaatacggttatccacagaatcaggggataacgcaggaaagaacatgtgagcaaaaggccagcaaaaggccaggaaccgtaaaaaggccgcgttgctggcgtttttccataggctccgcccccctgacgagcatcacaaaaatcgacgctcaagtcagaggtggcgaaacccgacaggactataaagataccaggcgtttccccctggaagctccctcgtgcgctctcctgttccgaccctgccgcttaccggatacctgtccgcctttctcccttcgggaagcgtggcgctttctcatagctcacgctgtaggtatctcagttcggtgtaggtcgttcgctccaagctgggctgtgtgcacgaaccccccgttcagcccgaccgctgcgccttatccggtaactatcgtcttgagtccaacccggtaagacacgacttatcgccactggcagcagccactggtaacaggattagcagagcgaggtatgtaggcggtgctacagagttcttgaagtggtggcctaactacggctacactagaagaacagtatttggtatctgcgctctgctgaagccagttaccttcggaaaaagagttggtagctcttgatccggcaaacaaaccaccgctggtagcggtggtttttttgtttgcaagcagcagattacgcgcagaaaaaaaggatctcaagaagatcctttgatcttttctacggggtctgacgctcagtggaacgaaaactcacgttaagggattttggtcatgagattatcaaaaaggatcttcacctagatccttttaaattaaaaatgaagttttaaatcaatctaaagtatatatgagtaaacttggtctgacagttaccaatgcttaatcagtgaggcacctatctcagcgatctgtctatttcgttcatccatagttgcctgactccccgtcgtgtagataactacgatacgggagggcttaccatctggccccagtgctgcaatgataccgcgagaaccacgctcaccggctccagatttatcagcaataaaccagccagccggaagggccgagcgcagaagtggtcctgcaactttatccgcctccatccagtctattaattgttgccgggaagctagagtaagtagttcgccagttaatagtttgcgcaacgttgttgccattgctacaggcatcgtggtgtcacgctcgtcgtttggtatggcttcattcagctccggttcccaacgatcaaggcgagttacatgatcccccatgttgtgcaaaaaagcggttagctccttcggtcctccgatcgttgtcagaagtaagttggccgcagtgttatcactcatggttatggcagcactgcataattctcttactgtcatgccatccgtaagatgcttttctgtgactggtgagtactcaaccaagtcattctgagaatagtgtatgcggcgaccgagttgctcttgcccggcgtcaatacgggataataccgcgccacatagcagaactttaaaagtgctcatcattggaaaacgttcttcggggcgaaaactctcaaggatcttaccgctgttgagatccagttcgatgtaacccactcgtgcacccaactgatcttcagcatcttttactttcaccagcgtttctgggtgagcaaaaacaggaaggcaaaatgccgcaaaaaagggaataagggcgacacggaaatgttgaatactcatactcttcctttttcaatattattgaagcatttatcagggttattgtctcatgagcggatacatatttgaatgtatttagaaaaataaacaaataggggttccgcgcacatttccccgaaaagtgccacctgacgtctaagaaaccattattatcatgacattaacctataaaaataggcgtatcacgaggcccttttgtc

SEQ ID NO: 24 - DNA, 23857 bp, synthetic construct
  misc_feature 1..23857: note = plasmid
  source 1..23857: mol_type = other DNA
atgactctcttaaggtagccaaatttccataggctccgcccccctgacgagcatcacaaaaatcgacgctcaagtcagaggtggcgaaacccgacaggactataaagataccaggcgtttccccctggaagctccctcgtgcgctctcctgttccgaccctgccgcttaccggatacctgtccgcctttctcccttcgggaagcgtggcgctttctcatagctcacgctgtaggtatctcagttcggtgtaggtcgttcgctccaagctgggctgtgtgcacgaaccccccgttcagcccgaccgctgcgccttatccggtaactatcgtcttgagtccaacccggtaagacacgacttatcgccactggcagcagccactggtaacaggattagcagagcgaggtatgtaggcggtgctacagagttcttgaagtggtggcctaactacggctacactagaaggacagtatttggtatctgcgctctgctgaagccagttaccttcggaaaaagagttggtagctcttgatccggcaaacaaaccaccgctggtagcggtggtttttttgtttgcaagcagcagattacgcgcagaaaaaaaggatctcaagaagatcctttgatcttttctacggggtctgacgctcagtggaacgaaaactcacgttaagggattttggtcatgagattatcaaaaaggatcttcacctagatccttttaaattaaaaatgaagttttaaatcaatctaaagtatatatgagtaaacttggtctgacagttaccaatgcttaatcagtgaggcacctatctcagcgatctgtctatttcgttcatccatagttgcctgactccccgtcgtgtagataactacgatacgggagggcttaccatctggccccagtgctgcaatgataccgcgagacccacgctcaccggctccagatttatcagcaataaaccagccagccggaagggccgagcgcagaagtggtcctgcaactttatccgcctccatccagtctattaattgttgccgggaagctagagtaagtagttcgccagttaatagtttgcgcaacgttgttgccattgctacaggcatcgtggtgtcacgctcgtcgtttggtatggcttcattcagctccggttcccaacgatcaaggcgagttacatgatcccccatgttgtgcaaaaaagcggttagctccttcggtcctccgatcgttgtcagaagtaagttggccgcagtgttatcactcatggttatggcagcactgcataattctcttactgtcatgccatccgtaagatgcttttctgtgactggtgagtactcaaccaagtcattctgagaatagtgtatgcggcgaccgagttgctcttgcccggcgtcaatacgggataataccgcgccacatagcagaactttaaaagtgctcatcattggaaaacgttcttcggggcgaaaactctcaaggatcttaccgctgttgagatccagttcgatgtaacccactcgtgcacccaactgatcttcagcatcttttactttcaccagcgtttctgggtgagcaaaaacaggaaggcaaaatgccgcaaaaaagggaataagggcgacacggaaatgttgaatactcatactcttcctttttcaatattattgaagcatttatcagggttattgtctcatgagcggatacatatttgaatgtatttagaaaaataaacaaataggggttccgcgcacatttccccgaaaagtgccacctaaattgtaagcgttaatattttgttaaaattcgcgttaaatttttgttaaatcagctcattttttaaccaataggccgaaatcggcaaaatcccttataaatcaaaagaatagaccgagatagggttgagtgttgttccagtttggaacaagagtccactattaaagaacgtggactccaacgtcaaagggcgaaaaaccgtctatcagggcgatggcccactacgtgaaccatcaccctaatcaagttttttggggtcgaggtgccgtaaagcactaaatcggaaccctaaagggagcccccgatttagagcttgacggggaaagccggcgaacgtggcgagaaaggaagggaagaaagcgaaaggagcgggcgctagggcgctggcaagtgtagcggtcacgctgcgcgtaaccaccacacccgccgcgcttaatgcgccgctacagggcgcgtcccattcgccattcaggctgcgcaactgttgggaagggcgatcggtgcgggcctcttcgctattacgccagctggcgaaagggggatgtgctgcaaggcgattaagttgggtaacgccagggttttcccagtcacgacgttaccccacagtggggccactagggtcaatttctgagaactgtcattctcggaaattgagtaaaacgacggccagtgagcgcgcctcgttcattcacgtttttgaacccgtggaggacgggcagactcgcggtgcaaatgtgttttacagcgtgatggagcagatgaagatgctcgacacgctgcagaacacgcagctagattaaccctagaaagataatcatattgtgacgtacgttaaagataatcatgcgtaaaattgacgcatgtgttttatcggtctgtatatcgaggtttatttattaatttgaatagatattaagttttattatatttacacttacatactaataataaattcaacaaacaatttatttatgtttatttatttattaaaaaaaaacaaaaactcaaaatttcttctataaagtaacaaaacttttatcgaattcctgcagcccgggggatccactagttctagagggacagcccccccccaaagcccccagggatgtaattacgtccctcccccgctagggggcagcagcgagccgcccggggctccgctccggtccggcgctccccccgcatccccgagccggcagcgtgcggggacagcccgggcacggggaaggtggcacgggatcgctttcctctgaacgcttctcgctgctctttgagcctgcagacacctggggggatacggggaaaaggcctccaaggccagcttcccacaataagttgggtgaattttggctcattcctcctttctataggattgaggtcagagctttgtgatgggaattctgtggaatgtgtgtcagttagggtgtggaaagtccctttactccctatcagtgatagagaacgtatgaagagtttactccctatcagtgatagagaacgtatgcagactttactccctatcagtgatagagaacgtataaggagtttactccctatcagtgatagagaacgtatgaccagtttactccctatcagtgatagagaacgtatctacagtttactccctatcagtgatagagaacgtatatccagtttactccctatcagtgatagagaacgtatgtcgaggtaggcgtgtacggtgggcgcctataaaagcagagctcgtttagtgaaccgtcagatcgcctggagcaattccacaacacttttgtcttatacttggtttagtgaaccgtcagatcagatctttgtcgatcctaccatccactcgacacacccgccagcggccgcagttgcgcagccatcgacgtcagacgcggaagcttcgatcaactacgcagacaggtaccaaaacaaatgttctcgtcacgtgggcatgaatctgatgctgtttccctgcagacaatgcgagagaatgaatcagaattcaaatatctgcttcactcacggacagaaagactgtttagagtgctttcccgtgtcagaatctcaacccgtttctgtcgtcaaaaaggcgtatcagaaactgtgctacattcatcatatcatgggaaaggtgccagacgcttgcactgcctgcgatctggtcaatgtggatttggatgactgcatctttgaacaataaatgatttaaatcaggtatgtcttttgttgatcaccctccagattggttggaagaagttggtgaaggtcttcgcgagtttttgggccttgaagcgggcccaccgaaaccaaaacccaatcagcagcatcaagatcaagcccgtggtcttgtgctgcctggttataactatctcggacccggaaacggtctcgatcgaggagagcctgtcaacagggcagacgaggtcgcgcgagagcacgacatctcgtacaacgagcagcttgaggcgggagacaacccctacctcaagtacaaccacgcggacgccgagtttcaggagaagctcgccgacgacacatccttcgggggaaacctcggaaaggcagtctttcaggccaagaaaagggttctcgaaccttttggcctggttgaagagggtgctaagacggcccctaccggaaagcggatagacgaccactttccaaaaagaaagaaggctcggaccgaagaggactccaagccttccacctcgtcagacgccgaagctggacccagcggatcccagcagctgcaaatcccagcccaaccagcctcaagtttgggagctgatacaatgtctgcgggaggtggcggcccattgggcgacaataaccaaggtgccgatggagtgggcaatgcctcgggagattggcattgcgattccacgtggatgggggacagagtcgtcaccaagtccacccgaacctgggtgctgcccagctacaacaaccaccagtaccgagagatcaaaagcggctccgtcgacggaagcaacgccaacgcctactttggatacagcaccccctgggggtactttgactttaaccgcttccacagccactggagcccccgagactggcaaagactcatcaacaactactggggcttcagaccccggtccctcagagtcaaaatcttcaacattcaagtcaaagaggtcacggtgcaggactccaccaccaccatcgccaacaacctcacctccaccgtccaagtgtttacggacgacgactaccagctgccctacgtcgtcggcaacgggaccgagggatgcctgccggccttccctccgcaggtctttacgctgccgcagtacggttacgcgacgctgaaccgcgacaacacagaaaatcccaccgagaggagcagcttcttctgcctagagtactttcccagcaagatgctgagaacgggcaacaactttgagtttacctacaactttgaggaggtgcccttccactccagcttcgctcccagtcagaacctgttcaagctggccaacccgctggtggaccagtacttgtaccgcttcgtgagcacaaataacactggcggagtccagttcaacaagaacctggccgggagatacgccaacacctacaaaaactggttcccggggcccatgggccgaacccagggctggaacctgggctccggggtcaaccgcgccagtgtcagcgccttcgccacgaccaataggatggagctcgagggcgcgagttaccaggtgcccccgcagccgaacggcatgaccaacaacctccagggcagcaacacctatgccctggagaacactatgatcttcaacagccagccggcgaacccgggcaccaccgccacgtacctcgagggcaacatgctcatcaccagcgagagcgagacgcagccggtgaaccgcgtggcgtacaacgtcggcgggcagatggccaccaacaaccagagctccaccactgcccccgcgaccggcacgtacaacctccaggaaatcgtgcccggcagcgtgtggatggagagggacgtgtacctccaaggacccatctgggccaagatcccagagacgggggcgcactttcacccctctccggccatgggcggattcggactcaaacacccaccgcccatgatgctcatcaagaacacgcctgtgcccggaaatatcaccagcttctcggacgtgcccgtcagcagcttcatcacccagtacagcaccgggcaggtcaccgtggagatggagtgggagctcaagaaggaaaactccaagaggtggaacccagagatccagtacacaaacaactacaacgacccccagtttgtggactttgccccggacagcaccggggaatacagaaccaccagacctatcggaacccgataccttacccgacccctttaacccgggagttctagggatctgcccctctccctcccccccccctaacgttactggccgaagccgcttggaataaggccggtgtgcgtttgtctatatgttattttccaccatattgccgtcttttggcaatgtgagggcccggaaacctggccctgtcttcttgacgagcattcctaggggtctttcccctctcgccaaaggaatgcaaggtctgttgaatgtcgtgaaggaagcagttcctctggaagcttcttgaagacaaacaacgtctgtagcgaccctttgcaggcagcggaaccccccacctggcgacaggtgcctctgcggccaaaagccacgtgtataagatacacctgcaaaggcggcacaaccccagtgccacgttgtgagttggatagttgtggaaagagtcaaatggctctcctcaagcgtattcaacaaggggctgaaggatgcccagaaggtaccccattgtatgggatctgatctggggcctcggtgcacatgctttacatgtgtttagtcgaggttaaaaaaacgtctaggccccccgaaccacggggacgtggttttcctttgaaaaacacgatgataaggatccaccggaggccaccatggccagtcgggaagaggagcagcgcgaaaccacccccgagcgcggacgcggtgcggcgcgacgtcccccaaccatggaggacgtgtcgtccccgtccccgtcgccgccgcctccccgggcgcccccaaaaaagcggatgaggcggcgtatcgagtccgaggacgaggaagactcatcacaagacgcgctggtgccgcgcacacccagcccgcggccatcgacctcggcggcggatttggccattgcgcccaagaagaaaaagaagcgcccttctcccaagcccgagcgcccgccatcaccagaggtaatcgtggacagcgaggaagaaagagaagatgtggcgctacaaatggtgggtttcagcaacccaccggtgctaatcaagcatggcaaaggaggtaagcgcacagtgcggcggctgaatgaagacgacccagtggcgcgtggtatgcggacgcaagaggaagaggaagagcccagcgaagcggaaagtgaaattacggtgatgaacccgctgagtgtgccgatcgtgtctgcgtgggagaagggcatggaggctgcgcgcgcgctgatggacaagtaccacgtggataacgatctaaaggcgaacttcaaactactgcctgaccaagtggaagctctggcggccgtatgcaagacctggctgaacgaggagcaccgcgggttgcagctgaccttcaccagcaacaagacctttgtgacgatgatggggcgattcctgcaggcgtacctgcagtcgtttgcagaggtgacctacaagcatcacgagcccacgggctgcgcgttgtggctgcaccgctgcgctgagatcgaaggcgagcttaagtgtctacacggaagcattatgataaataaggagcacgtgattgaaatggatgtgacgagcgaaaacgggcagcgcgcgctgaaggagcagtctagcaaggccaagatcgtgaagaaccggtggggccgaaatgtggtgcagatctccaacaccgacgcaaggtgctgcgtgcacgacgcggcctgtccggccaatcagttttccggcaagtcttgcggcatgttcttctctgaaggcgcaaaggctcaggtggcttttaagcagatcaaggcttttatgcaggcgctgtatcctaacgcccagaccgggcacggtcaccttttgatgccactacggtgcgagtgcaactcaaagcctgggcacgcgccctttttgggaaggcagctaccaaagttgactccgttcgccctgagcaacgcggaggacctggacgcggatctgatctccgacaagagcgtgctggccagcgtgcaccacccggcgctgatagtgttccagtgctgcaaccctgtgtatcgcaactcgcgcgcgcagggcggaggccccaactgcgacttcaagatatcggcgcccgacctgctaaacgcgttggtgatggtgcgcagcctgtggagtgaaaacttcaccgagctgccgcggatggttgtgcctgagtttaagtggagcactaaacaccagtatcgcaacgtgtccctgccagtggcgcatagcgatgcgcggcagaacccctttgatttttaacccgggagttctagggatctggcggccgctcgagtctagagggcccgtttccaccatattgccgtcttttggcaatgtgagggcccggaaacctggccctgtcttcttgacgagcattcctaggggtctttcccctctcgccaaaggaatgcaaggtctgttgaatgtcgtgaaggaagcagttcctctggaagcttcttgaagacaaacaacgtctgtagcgaccctttgcaggcagcggaaccccccacctggcgacaggtgcctctgcggccaaaagccacgtgtataagatacacctgcaaaggcggcacaaccccagtgccacgttgtgagttggatagttgtggaaagagtcaaatggctcccctcaagcgtattcaacaaggggctgaaggatgcccagaaggtaccccattgtatgggatctgatctggggcctcggtgcacatgctttacatgtgtttagtcgaggttaaaaaacgtctaggccccccgaaccacggggacgtggttttctttgaaaaacacgatgataatacatgactacgtccggcgttccatttggcatgacactacgaccaacacgatctcggttgtctcggcgcactccgtacagtagggatcgcctacctccttttgagacagagacccgcgctaccatactggaggatcatccgctgctgcccgaatgtaacactttgacaatgcacaacgtgagttacgtgcgaggtcttccctgcagtgtgggatttacgctgattcaggaatgggttgttccctgggatatggttctgacgcgggaggagcttgtaatcctgaggaagtgtatgcacgtgtgcctgtgttgtgccaacattgatatcatgacgagcatgatgatccatggttacgagtcctgggctctccactgtcattgttccagtcccggttccctgcagtgcatagccggcgggcaggttttggccagctggtttaggatggtggtggatggcgccatgtttaatcagaggtttatatggtaccgggaggtggtgaattacaacatgccaaaagaggtaatgtttatgtccagcgtgtttatgaggggtcgccacttaatctacctgcgcttgtggtatgatggccacgtgggttctgtggtccccgccatgagctttggatacagcgccttgcactgtgggattttgaacaatattgtggtgctgtgctgcagttactgtgctgatttaagtgagatcagggtgcgctgctgtgcccggaggacaaggcgtctcatgctgcgggcggtgcgaatcatcgctgaggagaccactgccatgttgtattcctgcaggacggagcggcggcggcagcagtttattcgcgcgctgctgcagcaccaccgccctatcctgatgcacgattatgactctacccccatgtaggcggccgctcgagtctagagggcccgtttaaacccgctgatcagcctcgactgtgccttctagttgccagccatctgttgtttgcccctcccccgtgccttccttgaccctggaaggtgccactcccactgtcctttcctaataaaatgaggaaattgcatcgcattgtctgagtaggtgtcattctattctggggggtggggtggggcaggacagcaagggggaggattgggaagacaatagcaggcatgctggggatgcggtgggctctatggtcatgtctgtaagcggccgctacgtcgacgtttaaacttaagcttggtaccgagctcggatccactagtccagtgtggtggaattcctgcttcgcgatgtacgggccagatatacgcgttgtttacgctccggtgcccgtcagtgggcagagcgcacatcgcccacagtccccgagaagttggggggaggggtcggcaattgaaccggtgcctagagaaggtggcgcggggtaaactgggaaagtgatgtcgtgtactggctccgcctttttcccgagggtgggggagaaccgtatataagtgcagtagtcgccgtgaacgttctttttcgcaacgggtttgccgccagaacacaggtaagtgccgtgtgtggttcccgcgggcctggcctctttacgggttatggcccttgcgtgccttgaattacttccacgcccctggctgcagtacgtgattcttgatcccgagcttcgggttggaagtgggtgggagagttcgaggccttgcgcttaaggagccccttcgcctcgtgcttgagttgaggcctggcttgggcgctggggccgccgcgtgcgaatctggtggcaccttcgcgcctgtctcgctgctttcgataagtctctagccatttaaaatttttgatgacctgctgcgacgctttttttctggcaagatagtcttgtaaatgcgggccaagatctgcacactggtatttcggtttttggggccgcgggcggcgacggggcccgtgcgtcccagcgcacatgttcggcgaggcggggcctgcgagcgcggccaccgagaatcggacgggggtagtctcaagctggccggcctgctctggtgcctggcctcgcgccgccgtgtatcgccccgccctgggcggcaaggctggcccggtcggcaccagttgcgtgagcggaaagatggccgcttcccggccctgctgcagggagctcaaaatggaggacgcggcgctcgggagagcgggcgggtgagtcacccacacaaaggaaaagggcctttccgtcctcagccgtcgcttcatgtgactccacggagtaccgggcgccgtccaggcacctcgattagttctcgagcttttggagtacgtcgtctttaggttggggggaggggttttatgcgatggagtttccccacactgagtgggtggagactgaagttaggccagcttggcacttgatgtaattctccttggaatttgccctttttgagtttggatcttggttcattctcaagcctcagacagtggttcaaagtttttttcttccatttcaggtgtcgtgaacctgcaggatttaaattctagttcaccatgtctagactggacaagagcaaagtcataaactctgctctggaattactcaatggagtcggtatcgaaggcctgacgacaaggaaactcgctcaaaagctgggagttgagcagcctaccctgtactggcacgtgaagaacaagcgggccctgctcgatgccctgccaatcgagatgctggacaggcatcatacccactcctgccccctggaaggcgagtcatggcaagactttctgcggaacaacgccaagtcataccgctgtgctctcctctcacatcgcgacggggctaaagtgcatctcggcacccgcccaacagagaaacagtacgaaaccctggaaaatcagctcgcgttcctgtgtcagcaaggcttctccctggagaacgcactgtacgctctgtccgccgtgggccactttacactgggctgcgtattggaggaacaggagcatcaagtagcaaaagaggaaagagagacacctaccaccgattctatgcccccacttctgaaacaagcaattgagctgttcgaccggcagggagccgaacctgccttccttttcggcctggaactaatcatatgtggcctggagaaacagctaaagtgcgaaagcggcgggccgaccgacgcccttgacgattttgacttagacatgctcccagccgatgcccttgacgactttgaccttgatatgctgcctgctgacgctcttgacgattttgaccttgacatgctccccgggtaagcgtacagcggctcccgggagttctagggatctgcccctctccctcccccccccctaacgttactggccgaagccgcttggaataaggccggtgtgcgtttgtctatatgttattttccaccatattgccgtcttttggcaatgtgagggcccggaaacctggccctgtcttcttgacgagcattcctaggggtctttcccctctcgccaaaggaatgcaaggtctgttgaatgtcgtgaaggaagcagttcctctggaagcttcttgaagacaaacaacgtctgtagcgaccctttgcaggcagcggaaccccccacctggcgacaggtgcctctgcggccaaaagccacgtgtataagatacacctgcaaaggcggcacaaccccagtgccacgttgtgagttggatagttgtggaaagagtcaaatggctctcctcaagcgtattcaacaaggggctgaaggatgcccagaaggtaccccattgtatgggatctgatctggggcctcggtgcacatgctttacatgtgtttagtcgaggttaaaaaaacgtctaggccccccgaaccacggggacgtggttttcctttgaaaaacacgatgataaggatccaccggaggccaccatgaccgagtacaagcccacggtgcgcctcgccacccgcgacgacgtccccagggccgtacgcaccctcgccgccgcgttcgccgactaccccgccacgcgccacaccgtcgatccggaccgccacatcgagcgggtcaccgagctgcaagaactcttcctcacgcgcgtcgggctcgacatcggcaaggtgtgggtcgcggacgacggcgccgcggtggcggtctggaccacgccggagagcgtcgaagcgggggcggtgttcgccgagatcggcccgcgcatggccgagttgagcggttcccggctggccgcgcagcaacagatggaaggcctcctggcgccgcaccggcccaaggagcccgcgtggttcctggccaccgtcggcgtctcgcccgaccaccagggcaagggtctgggcagcgccgtcgtgctccccggagtggaggcggccgagcgcgccggggtgcccgccttcctggagacctccgcgccccgcaacctccccttctacgagcggctcggcttcaccgtcaccgccgacgtcgaggtgcccgaaggaccgcgcacctggtgcatgacccgcaagcccggtgcctgaccgcgtctggaacaatcaacctctggattacaaaatttgtgaaagattgactggtattcttaactatgttgctccttttacgctatgtggatacgctgctttaatgcctttgtatcatgctattgcttcccgtatggctttcattttctcctccttgtataaatcctggttgctgtctctttatgaggagttgtggcccgttgtcaggcaacgtggcgtggtgtgcactgtgtttgctgacgcaacccccactggttggggcattgccaccacctgtcagctcctttccgggactttcgctttccccctccctattgccacggcggaactcatcgccgcctgccttgcccgctgctggacaggggctcggctgttgggcactgacaattccgtggtgttgtcggggaagctgacgtcctttccatggctgctcgcctgtgttgccacctggattctgcgcgggacgtccttctgctacgtcccttcggccctcaatccagcggaccttccttcccgcggcctgctgccggctctgcggcctcttccgcgtcttcgccttcgccctcagacgagtcggatctccctttgggccgcctccccgcaaaatgaccgaccaagcgacgcccaacctgccatcacgagatttcgattccaccgccgccttctatgatcatgtctgggggtgggcgaagaactccagcatgagatccccgcgctggaggatcatccagccggcgtcccggaaaacgattccgaagcccaacctttgcctgcaggtcgactctagaggatccgaaaaaacctcccacacctccccctgaacctgaaacataaaatgaatgcaattgttgttgttaacttgtttattgcagcttataatggttacaaataaagcaatagcatcacaaatttcacaaataaagcatttttttcactgcattctagttgtggtttgtccaaactcatcaatgtatcttatcatgtctggatccccgcggccgcggtacccacgtgggcgcgccatttaaatgataactcagagagagtgtcctcgagccaatctggaagataaccatcggcagccatacctgatttaaatcatttattgttcaaagatgcagtcatccaaatccacattgaccagatcgcaggcagtgcaagcgtctggcacctttcccatgatatgatgaatgtagcacagtttctgatacgcctttttgacgacagaaacgggttgagattctgacacgggaaagcactctaaacagtctttctgtccgtgagtgaagcagatatttgaattctgattcattctctcgcattgtctgcagggaaacagcatcagattcatgcccacgtgacgagaacatttgttttggtacctgtctgcgtagttgatcgaagcttccgcgtctgacgtcgatggctgcgcaactgactcgcgcacccgtttgggctcacttatatctgcgtcactgggggcgggtcttttcttggctccaccctttttgacgtagaattcatgctccacctcaaccacgtgatcctttgcccaccggaaaaagtctttgacttcctgcttggtgaccttcccaaagtcatgatccagacggcgggtgagttcaaatttgaacatccggtcttgcaacggctgctggtgttcgaaggtcgttgagttcccgtcaatcacggcgcacatgttggtgttggaggtgacgatcacgggagtcgggtctatctgggccgaggacttgcatttctggtccacgcgcaccttgcttcctccgagaatggctttggccgactccacgaccttggcggtcatcttcccctcctcccaccagatcaccatcttgtcgacacagtcgttgaagggaaagttctcattggtccagtttacgcacccgtagaagggcacagtgtgggctatggcctccgcgatgttggtcttcccggtagttgcaggcccaaacagccagatggtgttcctcttgccgaactttttcgtggcccatcccagaaagacggaagccgcatattggggatcgtacccgtttagttccaaaattttataaatccgattgctggaaatgtcctccacgggctgctggcccaccaggtagtcgggggcggttttagtcaggctcataatctttcccgcattgtccaaggcagccttgatttgggaccgcgagttggaggccgcattgaaggagatgtatgaggcctggtcctcctggatccactgcttctccgaggtaatccccttgtccacgagccacccgaccagctccatgtacctggctgaagtttttgatctgatcaccggcgcatcagaattgggattctgattctctttgttctgctcctgcgtctgcgacacgtgcgtcagatgctgcgccaccaaccgtttacgctccgtgagattcaaacaggcgcttaaatactgttccatattagtccacgcccactggagctcaggctgggttttggggagcaagtaattggggatgtagcactcatccaccaccttgttcccgcctccggcgccatttctggtctttgtgaccgcgaaccagtttggcaaagtcggctcgatcccgcggtaaattctctgaatcagtttttcgcgaatctgactcaggaaacgtcccaaaaccatggatttcaccccggtggtttccacgagcacgtgcatgtggaagtagctctctcccttctcaaattgcacaaagaaaagggcctccggggccttactcacacggcgccattccgtcagaaagtcgcgctgcagcttctcggccacggtcaggggtgcctgctcaatcagattcagatccatgtcagaatctggcggcaactcccattccttctcggccacccagttcacaaagctgtcagaaatgccgggcagatgctcgtcaaggtcgctggggaccttaatcacaatctcgtaaaaccccggcatggcggcgataactattatcatcgtgtttttcaaaggaaaaccacgtccccgtggttcggggggcctagacgtttttttaacctcgactaaacacatgtaaagcatgtgcaccgaggccccagatcagatcccatacaatggggtaccttctgggcatccttcagccccttgttgaatacgcttgaggagagccatttgactctttccacaactatccaactcacaacgtggcactggggttgtgccgcctttgcaggtgtatcttatacacgtggcttttggccgcagaggcacctgtcgccaggtggggggttccgctgcctgcaaagggtcgctacagacgttgtttgtcttcaagaagcttccagaggaactgcttccttcacgacattcaacagaccttgcattcctttggcgagaggggaaagacccctaggaatgctcgtcaagaagacagggccaggtttccgggccctcacattgccaaaagacggcaatatggtggaaaataacatatagacaaacgcacaccggccttattccaagcggcttcggccagtaacgttagggggggggggcggaattctatccctcagttatctcagagagagtgtcctcgagccaatctggaagataaccatcggcagccatacctgatttaaatcatttattgttcaaagatgcagtcatccaaatccacattgaccagatcgcaggcagtgcaagcgtctggcacctttcccatgatatgatgaatgtagcacagtttctgatacgcctttttgacgacagaaacgggttgagattctgacacgggaaagcactctaaacagtctttctgtccgtgagtgaagcagatatttgaattctgattcattctctcgcattgtctgcagggaaacagcatcagattcatgcccacgtgacgagaacatttgttttggtacctgtctgcgtagttgatcgaagcttccgcgtctgacgtcgatggctgcgcaactgactcgcgcacccgtttgggctcacttatatctgcgtcactgggggcgggtcttttcttggctccaccctttttgacgtagaattcatgctccacctcaaccacgtgatcctttgcccaccggaaaaagtctttgacttcctgcttggtgaccttcccaaagtcatgatccagacggcgggtgagttcaaatttgaacatccggtcttgcaacggctgctggtgttcgaaggtcgttgagttcccgtcaatcacggcgcacatgttggtgttggaggtgacgatcacgggagtcgggtctatctgggccgaggacttgcatttctggtccacgcgcaccttgcttcctccgagaatggctttggccgactccacgaccttggcggtcatcttcccctcctcccaccagatcaccatcttgtcgacacagtcgttgaagggaaagttctcattggtccagtttacgcacccgtagaagggcacagtgtgggctatggcctccgcgatgttggtcttcccggtagttgcaggcccaaacagccagatggtgttcctcttgccgaactttttcgtggcccatcccagaaagacggaagccgcatattggggatcgtacccgtttagttccaaaattttataaatccgattgctggaaatgtcctccacgggctgctggcccaccaggtagtcgggggcggttttagtcaggctcataatctttcccgcattgtccaaggcagccttgatttgggaccgcgagttggaggccgcattgaaggagatgtatgaggcctggtcctcctggatccactgcttctccgaggtaatccccttgtccacgagccacccgaccagctccatggtggcgttatccggccgatcgatagatctgggccccggtgtcgactttacgagggtaggaagtggtacggaaagttggtataagacaaaagtgttgtggaattgctggaggcgatctgacggttcactaaacgagctctgcttttataggcgcccaccgtacacgcctaaagcttatacgttctctatcactgatagggagtaaactggatatacgttctctatcactgatagggagtaaactgtagatacgttctctatcactgatagggagtaaactggtcatacgttctctatcactgatagggagtaaactccttatacgttctctatcactgatagggagtaaagtctgcatacgttctctatcactgatagggagtaaactcttcatacgttctctatcactgatagggagtaaacgaatggctaggatccggccggcctgcaggtgtcctcacaggaacgaagtccctaaagaaacagtggcagccaggtttagccccggaattgactggattccttttttagggcccattggtatggctttttccccgtatccccccaggtgtctgcaggctcaaagagcagcgagaagcgttcagaggaaagcgatcccgtgccaccttccccgtgcccgggctgtccccgcacgctgccggctcggggatgcggggggagcgccggaccggagcggagccccgggcggctcgctgctgccccctagcgggggagggacgtaattacatccctgggggctttgggggggggctgtccctctagagcggccgccaccgcggtggagctccagcttttgttccctttagtgagggttaattagatcttaatacgactcactatagggcgaattgggtaccgggccccccctcgaggtcgacggtatcgcctccaaggccagcttcccacaataagttgggtgaattttggctcattcctcctttctataggattgaggtcagagctttgtgatgggaattctgtggaatgtgtgtcagttagggtgtggaaagtcccgcgatcgctagcaaacgccagcaacgcggcctttttacggttcctggccttttgctggccttttgctcacatgtcctgcaggcagctgcgcgctcgctcgctcactgaggccgcccgggcaaagcccgggcgtcgggcgacctttggtcgcccggcctcagtgagcgagcgagcgcgcagagagggagtggccaactccatcactaggggttcctgcggccgcacgcgtggagctagttattaatagtaatcaattacggggtcattagttcatagcccatatatggagttccgcgttacataacttacggtaaatggcccgcctggctgaccgcccaacgacccccgcccattgacgtcaataatgacgtatgttcccatagtaacgtcaatagggactttccattgacgtcaatgggtggagtatttacggtaaactgcccacttggcagtacatcaagtgtatcatatgccaagtacgccccctattgacgtcaatgacggtaaatggcccgcctggcattatgcccagtacatgaccttatgggactttcctacttggcagtacatctacgtattagtcatcgctattaccatggtgatgcggttttggcagtacatcaatgggcgtggatagcggtttgactcacggggatttccaagtctccaccccattgacgtcaatgggagtttgttttgcaccaaaatcaacgggactttccaaaatgtcgtaacaactccgccccattgacgcaaatgggcggtaggcgtgtacggtgggaggtctatataagcagagctcgtttagtgaaccgtcagatcgcctggagacgccatccacgctgttttgacctccatagaagacaccgggaccgatccagcctccgcggattcgaatcccggccgggaacggtgcattggaacgcggattccccgtgccaagagtgacgtaagtaccgcctatagagtctataggcccacaaaaaatgctttcttcttttaatatacttttttgtttatcttatttctaatactttccctaatctctttctttcagggcaataatgatacaatgtatcatgcctctttgcaccattctaaagaataacagtgataatttctgggttaaggcaatagcaatatttctgcatataaatatttctgcatataaattgtaactgatgtaagaggtttcatattgctaatagcagctacaatccagctaccattctgcttttattttatggttgggataaggctggattattctgagtccaagctaggcccttttgctaatcatgttcatacctcttatcttcctcccacagctcctgggcaacgtgctggtctgtgtgctggcccatcactttggcaaagaattgggattcgaacatcgattgaattctgaatggtgagcaagggcgaggagctgttcaccggggtggtgcccatcctggtcgagctggacggcgacgtaaacggccacaagttcagcgtgtccggcgagggcgagggcgatgccacctacggcaagctgaccctgaagttcatctgcaccaccggcaagctgcccgtgccctggcccaccctcgtgaccaccctgacctacggcgtgcagtgcttcagccgctaccccgaccacatgaagcagcacgacttcttcaagtccgccatgcccgaaggctacgtccaggagcgcaccatcttcttcaaggacgacggcaactacaagacccgcgccgaggtgaagttcgagggcgacaccctggtgaaccgcatcgagctgaagggcatcgacttcaaggaggacggcaacatcctggggcacaagctggagtacaactacaacagccacaacgtctatatcatggccgacaagcagaagaacggcatcaaggtgaacttcaagatccgccacaacatcgaggacggcagcgtgcagctcgccgaccactaccagcagaacacccccatcggcgacggccccgtgctgctgcccgacaaccactacctgagcacccagtccgccctgagcaaagaccccaacgagaagcgcgatcacatggtcctgctggagttcgtgaccgccgccgggatcactctcggcatggacgagctgtacaagtactcagatctcgagctcaagtagggatcctctagagtcgacctgcagaagcttgcctcgagcagcgctgctcgagagatctacgggtggcatccctgtgacccctccccagtgcctctcctggccctggaagttgccactccagtgcccaccagccttgtcctaataaaattaagttgcatcattttgtctgactaggtgtccttctataatattatggggtggaggggggtggtatggagcaaggggcaagttgggaagacaacctgtagggcctgcggggtctattgggaaccaagctggagtgcagtggcacaatcttggctcactgcaatctccgcctcctgggttcaagcgattctcctgcctcagcctcccgagttgttgggattccaggcatgcatgaccaggctcagctaatttttgtttttttggtagagacggggtttcaccatattggccaggctggtctccaactcctaatctcaggtgatctacccaccttggcctcccaaattgctgggattacaggcgtgaaccactgctcccttccctgtccttctgattttgtaggtaaccacgtgcggaccgagcggccgcaggaacccctagtgatggagttggccactccctctctgcgcgctcgctcgctcactgaggccgggcgaccaaaggtcgcccgacgcccgggctttgcccgggcggcctcagtgagcgagcgagcgcgcagctgcctgcaggggcgcctgatgcggtattttctccttacgcatctgtgcggtatttcacaccgcatacgtcgtagctgatcaattggcgcgccgaattcgttaacaagctttaattaacgcgtacgataagcttgatatctataacaagaaaatatatatataataagttatcacgtaagtagaacatgaaataacaatataattatcgtatgagttaaatcttaaaagtcacgtaaaagataatcatgcgtcattttgactcacgcggtcgttatagttcaaaatcagtgacacttaccgcattgacaagcacgcctcacgggagctccaagcggcgactgagatgtcctaaatgcacagcgacggattcgcgctatttagaaagagagagcaatatttcaagaatgcatgcgtcaattttacgcagactatctttctagggttaatctagctgcatcaggatcatatcgtcgggtcttttttccggctcagtcatcgcccaagctggcgctatctgggcatcggggaggaagaagcccgtgccttttcccgcgaggttgaagcggcatggaaagagtttgccgaggatgactgctgctgcattgacgttgagcgaaaacgcacgtttaccatgatgattcgggaaggtgtggccatgcacgcctttaacggtgaactgttcgttcaggccacctgggataccagttcgtcgcggcttttccggacacagttccggatggtcagcccgaagcgcatcagcaacccgaacaataccggcgacagccggaactgccgtgccggtgtgcagattaatgacagcggtgcggcgctgggatattacgtcagcgaggacgggtatcctggctggatgccgcagaaatggacatggataccccgtgagttacccggcgggcgcgcttggcgtaatcatggtcatagctgtttcctgctcgtgtccgataactgtaattatcggacatgattgtgaaattgttatccgctcacaattccacacaacatacgagccggaagcataaagtgtaaagcctggggtgcctaatgagtgagctaactcacattaattgcgttgcgctcactgcccgctttccagtcgggaaacctgtcgtgccagctgcattaatgaatcggccaacgcgcggggagaggcggtttgcgtattgggcgctcttccgcttcctcgctcactgactcgctgcgctcggtcgttcggctgcggcgagcggtatcagctcactcaaaggcggtaatacggttatccacagaatcaggggataacgcaggaaagaacatgtgagcaaaaggccagcaaaaggccaggaaccgtaaaaaggccgcgttgctggcgttatgactctcttaaggtagccaaaatggtgcactctcagtacaatctgctctgatgccgcatagtatgttgtaactaaagatctactgtggataactctgtcaggaagcttggatcaaccggtagttatccaaagaacaactgttgttcagtttttgagttgtgtataacccctcattctgatcccagcttatacggtccaggatcaccgatcattcacagttaatgatcctttccaggttgttgatcttaaaagccggatccttgttatccacagggcagtgcgatcctaataagagatcacaatagaacagatctctaaataaatagatcttctttttaatactttagttacaacatactgttaagccagccccgacacccgccaacacccgctgacgcg

SEQ ID NO: 25 - DNA, 20257 bp, synthetic construct; identical to SEQ ID NO: 20
  misc_feature 1..20257: note = plasmid
  source 1..20257: mol_type = other DNA

SEQ ID NO: 26 - DNA, 9873 bp, synthetic construct
  misc_feature 1..9873: note = plasmid
  source 1..9873: mol_type = other DNA
taagcggccgctacgtcgacgtttaaaccatacaatcagcattggtagctgctgtattgctacttgtgattgctccatgtttttctaggtctcgactgcagaattaattccaggcggggaggcggcccaaagggagatccgactcgtctgagggcgaaggcgaagacgcggaagaggccgcagagccggcagcaggccgcgggaaggaaggtccgctggattgagggccgaagggacgtagcagaaggacgtcccgcgcagaatccaggtggcaacacaggcgagcagccatggaaaggacgtcagcttccccgacaacaccacggaattgtcagtgcccaacagccgagcccctgtccagcagcgggcaaggcaggcggcgatgagttccgccgtggcaatagggagggggaaagcgaaagtcccggaaaggagctgacaggtggtggcaatgccccaaccagtgggggttgcgtcagcaaacacagtgcacaccacgccacgttgcctgacaacgggccacaactcctcataaagagacagcaaccaggatttatacaaggaggagaaaatgaaagccatacgggaagcaatagcatgatacaaaggcattaaagcagcgtatccacatagcgtaaaaggagcaacatagttaagaataccagtcaatctttcacaaattttgtaatccagaggttgattgttccagacgcgttcagaagaactcgtcaagaaggcgatagaaggcgatgcgctgcgaatcgggagcggcgataccgtaaagcacgaggaagcggtcagcccattcgccgccaagctcttcagcaatatcacgggtagccaacgctatgtcctgatagcggtccgccacacccagccggccacagtcgatgaatccagaaaagcggccattttccaccatgatattcggcaagcaggcatcgccatgggtcacgacgagatcctcgccgtcgggcatgcgcgccttgagcctggcgaacagttcggctggcgcgagcccctgatgctcttcgtccagatcatcctgatcgacaagaccggcttccatccgagtacgtgctcgctcgatgcgatgtttcgcttggtggtcgaatgggcaggtagccggatcaagcgtatgcagccgccgcattgcatcagccatgatggatactttctcggcaggagcaaggtgagatgacaggagatcctgccccggcacttcgcccaatagcagccagtcccttcccgcttcagtgacaacgtcgagcacagctgcgcaaggaacgcccgtcgtggccagccacgatagccgcgctgcctcgtcctgcagttcattcagggcaccggacaggtcggtcttgacaaaaagaaccgggcgcccctgcgctgacagccggaacacggcggcatcagagcagccgattgtctgttgtgcccagtcatagccgaatagcctctccacccaagcggccggagaacctgcgtgcaatccatcttgttcagccatggcggcgttaactgcaggtcgaaaggcccggagatgaggaagaggagaacagcgcggcagacgtgcgcttttgaagcgtgcagaatgccgggcctccggaggaccttcgggcgcccgccccgcccctgagcccgcccctgagcccgcccccggacccaccccttcccagcctctgagcccagaaagcgaaggagcaaagctgctattggccgctgccccaaaggcctacccgcttccattgctcagcggtgctgtccatctgcacgagactagtgagacgtgctacttccatttgtcacgtcctgcacgacgcgagctgcggggcgggggggaacttcctgactaggggaggagtagaaggtggcgcgaaggggccaccaaagaacggagccggttggcgcctaccggtggatgtggaatgtgtgcgaggccagaggccacttgtgtagcgccaagtgcccagcggggctgctaaagcgcatgctccagactgccttgggaaaagcgcctcccctacccggtagaattggatctagttacccggggagcatgtcaaggtcaaaatcgtcaagagcgtcagcaggcagcatatcaaggtcaaagtcgtcaagggcatcggctgggagcatgtctaagtcaaaatcgtcaagggcgtcggtcggcccgccgctttcgcactttagctgtttctccaggccacatatgattagttccaggccgaaaaggaaggcaggttcggctccctgccggtcgaacagctcaattgcttgtttcagaagtgggggcatagaatcggtggtaggtgtctctctttcctcttttgctacttgatgctcctgttcctccaatacgcagcccagtgtaaagtggcccacggcggacagagcgtacagtgcgttctccagggagaagccttgctgacacaggaacgcgagctgattttccagggtttcgtactgtttctctgttgggcgggtgccgagatgcactttagccccgtcgcgatgtgagaggagagcacagcggtatgacttggcgttgttccgcagaaagtcttgccatgactcgccttccagggggcaggagtgggtatgatgcctgtccagcatctcgattggcagggcatcgagcagggcccgcttgttcttcacgtgccagtacagggtaggctgctcaactcccagcttttgagcgagtttccttgtcgtcaggccttcgataccgactccattgagtaattccagagcagagtttatgactttgctcttgtccagtctagacatggtgaactagaatttaaatcctgcaggttcacgacacctgaaatggaagaaaaaaactttgaaccactgtctgaggcttgagaatgaaccaagatccaaactcaaaaagggcaaattccaaggagaattacatcaagtgccaagctggcctaacttcagtctccacccactcagtgtggggaaactccatcgcataaaacccctccccccaacctaaagacgacgtactccaaaagctcgagaactaatcgaggtgcctggacggcgcccggtactccgtggagtcacatgaagcgacggctgaggacggaaaggcccttttcctttgtgtgggtgactcacccgcccgctctcccgagcgccgcgtcctccattttgagctccctgcagcagggccgggaagcggccatctttccgctcacgcaactggtgccgaccgggccagccttgccgcccagggcggggcgatacacggcggcgcgaggccaggcaccagagcaggccggccagcttgagactacccccgtccgattctcggtggccgcgctcgcaggccccgcctcgccgaacatgtgcgctgggacgcacgggccccgtcgccgcccgcggccccaaaaaccgaaataccagtgtgcagatcttggcccgcatttacaagactatcttgccagaaaaaaagcgtcgcagcaggtcatcaaaaattttaaatggctagagacttatcgaaagcagcgagacaggcgcgaaggtgccaccagattcgcacgcggcggccccagcgcccaagccaggcctcaactcaagcacgaggcgaaggggctccttaagcgcaaggcctcgaactctcccacccacttccaacccgaagctcgggatcaagaatcacgtactgcagccaggggcgtggaagtaattcaaggcacgcaagggccataacccgtaaagaggccaggcccgcgggaaccacacacggcacttacctgtgttctggcggcaaacccgttgcgaaaaagaacgttcacggcgactactgcacttatatacggttctcccccaccctcgggaaaaaggcggagccagtacacgacatcactttcccagtttaccccgcgccaccttctctaggcaccggttcaattgccgacccctccccccaacttctcggggactgtgggcgatgtgcgctctgcccactgacgggcaccggagcctcacgaattcgatatcgataaactggatctctgctgtccctgtaataaacccgaatatgatcagctcactcaaaggcggtaatacggttatccacagaatcaggggataacgcaggaaagaacatgtgagcaaaaggccagcaaaaggccaggaaccgtaaaaaggccgcgttgctggcgtttttccataggctccgcccccctgacgagcatcacaaaaatcgacgctcaagtcagaggtggcgaaacccgacaggactataaagataccaggcgtttccccctggaagctccctcgtgcgctctcctgttccgaccctgccgcttaccggatacctgtccgcctttctcccttcgggaagcgtggcgctttctcatagctcacgctgtaggtatctcagttcggtgtaggtcgttcgctccaagctgggctgtgtgcacgaaccccccgttcagcccgaccgctgcgccttatccggtaactatcgtcttgagtccaacccggtaagacacgacttatcgccactggcagcagccactggtaacaggattagcagagcgaggtatgtaggcggtgctacagagttcttgaagtggtggcctaactacggctacactagaagaacagtatttggtatctgcgctctgctgaagccagttaccttcggaaaaagagttggtagctcttgatccggcaaacaaaccaccgctggtagcggtggtttttttgtttgcaagcagcagattacgcgcagaaaaaaaggatctcaagaagatcctttgatcttttctacggggtctgacgctcagtggaacgaaaactcacgttaagggattttggtcatgagattatcaaaaaggatcttcacctagatccttttaaattaaaaatgaagttttaaatcaatctaaagtatatatgagtaaacttggtctgacagttaccaatgcttaatcagtgaggcacctatctcagcgatctgtctatttcgttcatccatagttgcctgactccccgtcgtgtagataactacgatacgggagggcttaccatctggccccagtgctgcaatgataccgcgagacccacgctcaccggctccagatttatcagcaataaaccagccagccggaagggccgagcgcagaagtggtcctgcaactttatccgcctccatccagtctattaattgttgccgggaagctagagtaagtagttcgccagttaatagtttgcgcaacgttgttgccattgctacaggcatcgtggtgtcacgctcgtcgtttggtatggcttcattcagctccggttcccaacgatcaaggcgagttacatgatcccccatgttgtgcaaaaaagcggttagctccttcggtcctccgatcgttgtcagaagtaagttggccgcagtgttatcactcatggttatggcagcactgcataattctcttactgtcatgccatccgtaagatgcttttctgtgactggtgagtactcaaccaagtcattctgagaatagtgtatgcggcgaccgagttgctcttgcccggcgtcaatacgggataataccgcgccacatagcagaactttaaaagtgctcatcattggaaaacgttcttcggggcgaaaactctcaaggatcttaccgctgttgagatccagttcgatgtaacccactcgtgcacccaactgatcttcagcatcttttactttcaccagcgtttctgggtgagcaaaaacaggaaggcaaaatgccgcaaaaaagggaataagggcgacacggaaatgttgaatactcatactcttcctttttcaatattattgaagcatttatcagggttattgtctcatgagcggatacatatttgaatgtatttagaaaaataaacaaataggggttccgcgcacatttccccgaaaagtgccacctaaattgtaagcgttaatattttgttaaaattcgcgttaaatttttgttaaatcagctcattttttaaccaataggccgaaatcggcaaaatcccttataaatcaaaagaatagaccgagatagggttgagtgttgttccagtttggaacaagagtccactattaaagaacgtggactccaacgtcaaagggcgaaaaaccgtctatcagggcgatggcccactacgtgaaccatcaccctaatcaagttttttggggtcgaggtgccgtaaagcactaaatcggaaccctaaagggagcccccgatttagagcttgacggggaaagccggcgaacgtggcgagaaaggaagggaagaaagcgaaaggagcgggcgctagggcgctggcaagtgtagcggtcacgctgcgcgtaaccaccacacccgccgcgcttaatgcgccgctacagggcgcgatggatccgcggccgcttaagccataccaatggtttactccctatcagtgatagagaacgtatgaagagtttactccctatcagtgatagagaacgtatgcagactttactccctatcagtgatagagaacgtataaggagtttactccctatcagtgatagagaacgtatgaccagtttactccctatcagtgatagagaacgtatctacagtttactccctatcagtgatagagaacgtatatccagtttactccctatcagtgatagagaacgtatgtcgaggtaggcgtgtacggtgggcgcctataaaagcagagctcgtttagtgaaccgtcagatcgcctggagcaattccacaacacttttgtcttatacttggtttagtgaaccgtcagatcagatctttgtcgatcctaccatccactcgacacacccgccagcggccgatggccagtcgggaagaggagcagcgcgaaaccacccccgagcgcggacgcggtgcggcgcgacgtcccccaaccatggaggacgtgtcgtccccgtccccgtcgccgccgcctccccgggcgcccccaaaaaagcggatgaggcggcgtatcgagtccgaggacgaggaagactcatcacaagacgcgctggtgccgcgcacacccagcccgcggccatcgacctcggcggcggatttggccattgcgcccaagaagaaaaagaagcgcccttctcccaagcccgagcgcccgccatcaccagaggtaatcgtggacagcgaggaagaaagagaagatgtggcgctacaaatggtgggtttcagcaacccaccggtgctaatcaagcatggcaaaggaggtaagcgcacagtgcggcggctgaatgaagacgacccagtggcgcgtggtatgcggacgcaagaggaagaggaagagcccagcgaagcggaaagtgaaattacggtgatgaacccgctgagtgtgccgatcgtgtctgcgtgggagaagggcatggaggctgcgcgcgcgctgatggacaagtaccacgtggataacgatctaaaggcgaacttcaaactactgcctgaccaagtggaagctctggcggccgtatgcaagacctggctgaacgaggagcaccgcgggttgcagctgaccttcaccagcaacaagacctttgtgacgatgatggggcgattcctgcaggcgtacctgcagtcgtttgcagaggtgacctacaagcatcacgagcccacgggctgcgcgttgtggctgcaccgctgcgctgagatcgaaggcgagcttaagtgtctacacggaagcattatgataaataaggagcacgtgattgaaatggatgtgacgagcgaaaacgggcagcgcgcgctgaaggagcagtctagcaaggccaagatcgtgaagaaccggtggggccgaaatgtggtgcagatctccaacaccgacgcaaggtgctgcgtgcacgacgcggcctgtccggccaatcagttttccggcaagtcttgcggcatgttcttctctgaaggcgcaaaggctcaggtggcttttaagcagatcaaggcttttatgcaggcgctgtatcctaacgcccagaccgggcacggtcaccttttgatgccactacggtgcgagtgcaactcaaagcctgggcacgcgccctttttgggaaggcagctaccaaagttgactccgttcgccctgagcaacgcggaggacctggacgcggatctgatctccgacaagagcgtgctggccagcgtgcaccacccggcgctgatagtgttccagtgctgcaaccctgtgtatcgcaactcgcgcgcgcagggcggaggccccaactgcgacttcaagatatcggcgcccgacctgctaaacgcgttggtgatggtgcgcagcctgtggagtgaaaacttcaccgagctgccgcggatggttgtgcctgagtttaagtggagcactaaacaccagtatcgcaacgtgtccctgccagtggcgcatagcgatgcgcggcagaacccctttgatttttcgttactggccgaagccgcttggaataaggccggtgtgcgtttgtctatatgttattttccaccatattgccgtcttttggcaatgtgagggcccggaaacctggccctgtcttcttgacgagcattcctaggggtctttcccctctcgccaaaggaatgcaaggtctgttgaatgtcgtgaaggaagcagttcctctggaagcttcttgaagacaaacaacgtctgtagcgaccctttgcaggcagcggaaccccccacctggcgacaggtgcctctgcggccaaaagccacgtgtataagatacacctgcaaaggcggcacaaccccagtgccacgttgtgagttggatagttgtggaaagagtcaaatggctcccctcaagcgtattcaacaaggggctgaaggatgcccagaaggtaccccattgtatgggatctgatctggggcctcggtgcacatgctttacatgtgtttagtcgaggttaaaaaacgtctaggccccccgaaccacggggacgtggttttctttgaaaaacacgatgataatacatgactacgtccggcgttccatttggcatgacactacgaccaacacgatctcggttgtctcggcgcactccgtacagtagggatcgcctacctccttttgagacagagacccgcgctaccatactggaggatcatccgctgctgcccgaatgtaacactttgacaatgcacaacgtgagttacgtgcgaggtcttccctgcagtgtgggatttacgctgattcaggaatgggttgttccctgggatatggttctgacgcgggaggagcttgtaatcctgaggaagtgtatgcacgtgtgcctgtgttgtgccaacattgatatcatgacgagcatgatgatccatggttacgagtcctgggctctccactgtcattgttccagtcccggttccctgcagtgcatagccggcgggcaggttttggccagctggtttaggatggtggtggatggcgccatgtttaatcagaggtttatatggtaccgggaggtggtgaattacaacatgccaaaagaggtaatgtttatgtccagcgtgtttatgaggggtcgccacttaatctacctgcgcttgtggtatgatggccacgtgggttctgtggtccccgccatgagctttggatacagcgccttgcactgtgggattttgaacaatattgtggtgctgtgctgcagttactgtgctgatttaagtgagatcagggtgcgctgctgtgcccggaggacaaggcgtctcatgctgcgggcggtgcgaatcatcgctgaggagaccactgccatgttgtattcctgcaggacggagcggcggcggcagcagtttattcgcgcgctgctgcagcaccaccgccctatcctgatgcacgattatgactctacccccatgtagtcatgtctg

SEQ ID NO: 27 - DNA, 5494 bp, synthetic construct
  misc_feature 1..5494: note = plasmid
  source 1..5494: mol_type = other DNA
tcgcgcgtttcggtgatgacggtgaaaacctctgacacatgcagctcccggagactgtcacagcttgtctgtaagcggatgccgggagcagacaagcccgtcagggcgcgtcagcgggtgttggcgggtgtcggggctggcttaactatgcggcatcagagcagattgtactgagagtgcaccatatgcggtgtgaaataccgcacagatgcgtaaggagaaaataccgcatcaggcgccattcgccattcaggctgcgcaactgttgggaagggcgatcggtgcgggcctcttcgctattacgccagctggcgaaagggggatgtgctgcaaggcgattaagttgggtaacgccagggttttcccagtcacgacgttgtaaaacgacggccagtgaattgacgcgtattgggatcctgcaggtcgttacataacttacggtaaatggcccgcctggctgaccgcccaacgacccccgcccattgacgtcaataatgacgtatgttcccatagtaacgccaatagggactttccattgacgtcaatgggtggagtatttacggtaaactgcccacttggcagtacatcaagtgtatcatatgccaagtacgccccctattgacgtcaatgacggtaaatggcccgcctggcattatgcccagtacatgaccttatgggactttcctacttggcagtacatctacgtattagtcatcgctattaccatggtgatgcggttttggcagtacatcaatgggcgtggatagcggtttgactcacggggatttccaagtctccaccccattgacgtcaatgggagtttgttttggcaccaaaatcaacgggactttccaaaatgtcgtaacaactccgccccattgacgcaaatgggcggtaggcgtgtacggtgggaggtctatataagcagagctcgtttagtgaaccgtcagatcgcctggagacgccatccacgctgttttgacctccatagaagacaccgggaccgatccagcctccggactctagaggatccggtactagaggaactgaaaaaccagaaagttaactggtaagtttagtctttttgtcttttatttcaggtcccggatccggtggtggtgcaaatcaaagaactgctcctcagtggatgttgcctttacttctaggcctgtacggaagtgttacttctgctctaaaagctgcggaattgtacccgcgggcccaccatgtacccatacgatgttccagattacgctcttatggccatggaggcccgaattcggtcgaccatgggtagttctttagacgatgagcatatcctctctgctcttctgcaaagcgatgacgagcttgttggtgaggattctgacagtgaaatatcagatcacgtaagtgaagatgacgtccagagcgatacagaagaagcgtttatagatgaggtacatgaagtgcagccaacgtcaagcggtagtgaaatattagacgaacaaaatgttattgaacaaccaggttcttcattggcttctaacagaatcttgaccttgccacagaggactattagaggtaagaataaacattgttggtcaacttcaaagtccacgaggcgtagccgagtctctgcactgaacattgtcagatctcaaagaggtccgacgcgtatgtgccgcaatatatatgacccacttttatgcttcaaactattttttactgatgagataatttcggaaattgtaaaatggacaaatgctgagatatcattgaaacgtcgggaatctatgacaggtgctacatttcgtgacacgaatgaagatgaaatctatgctttctttggtattctggtaatgacagcagtgagaaaagataaccacatgtccacagatgacctctttgatcgatctttgtcaatggtgtacgtctctgtaatgagtcgtgatcgttttgattttttgatacgatgtcttagaatggatgacaaaagtatacggcccacacttcgagaaaacgatgtatttactcctgttagaaaaatatgggatctctttatccatcagtgcatacaaaattacactccaggggctcatttgaccatagatgaacagttacttggttttagaggacggtgtccgtttaggatgtatatcccaaacaagccaagtaagtatggaataaaaatcctcatgatgtgtgacagtggtacgaagtatatgataaatggaatgccttatttgggaagaggaacacagaccaacggagtaccactcggtgaatactacgtgaaggagttatcaaagcctgtgcacggtagttgtcgtaatattacgtgtgacaattggttcacctcaatccctttggcaaaaaacttactacaagaaccgtataagttaaccattgtgggaaccgtgcgatcaaacaaacgcgagataccggaagtactgaaaaacagtcgctccaggccagtgggaacatcgatgttttgttttgacggaccccttactctcgtctcatataaaccgaagccagctaagatggtatacttattatcatcttgtgatgaggatgcttctatcaacgaaagtaccggtaaaccgcaaatggttatgtattataatcaaactaaaggcggagtggacacgctagaccaaatgtgttctgtgatgacctgcagtaggaagacgaataggtggcctatggcattattgtacggaatgataaacattgcctgcataaattcttttattatatacagccataatgtcagtagcaagggagaaaaggttcaaagtcgcaaaaaatttatgagaaacctttacatgagcctgacgtcatcgtttatgcgtaagcgtttagaagctcctactttgaagagatatttgcgcgataatatctctaatattttgccaaatgaagtgcctggtacatcagatgacagtactgaagagccagtaatgaaaaaacgtacttactgtacttactgcccctctaaaataaggcgaaaggcaaatgcatcgtgcaaaaaatgcaaaaaagttatttgtcgagagcataatattgatatgtgccaaagttgtttctgagagatctctcgaggtaccgcggccgcggggatccagacatgataagatacattgatgagtttggacaaaccacaactagaatgcagtgaaaaaaatgctttatttgtgaaatttgtgatgctattgctttatttgtaaccattataagctgcaataaacaagttatcccaatggcgcgccgagcttggcgtaatcatggtcatagctgtttcctgtgtgaaattgttatccgctcacaattccacacaacatacgagccggaagcataaagtgtaaagcctggggtgcctaatgagtgagctaactcacattaattgcgttgcgctcactgcccgctttccagtcgggaaacctgtcgtgccagctgcattaatgaatcggccaacgcgcggggagaggcggtttgcgtattgggcgctgttccgcttcctcgctcactgactcgctgcgctcggtcgttcggctgcggcgagcggtatcagctcactcaaaggcggtaatacggttatccacagaatcaggggataacgcaggaaagaacatgtgagcaaaaggccagcaaaaggccaggaaccgtaaaaaggccgcgttgctggcgtttttccataggctccgcccccctgacgagcatcacaaaaatcgacgctcaagtcagaggtggcgaaacccgacaggactataaagataccaggcgtttccccctggaagctccctcgtgcgctctcctgttccgaccctgccgcttaccggatacctgtccgcctttctcccttcgggaagcgtggcgctttctcatagctcacgctgtaggtatctcagttcggtgtaggtcgttcgctccaagctgggctgtgtgcacgaaccccccgttcagcccgaccgctgcgccttatccggtaactatcgtcttgagtccaacccggtaagacacgacttatcgccactggcagcagccactggtaacaggattagcagagcgaggtatgtaggcggtgctacagagttcttgaagtggtggcctaactacggctacactagaagaacagtatttggtatctgcgctctgctgaagccagttaccttcggaaaaagagttggtagctcttgatccggcaaacaaaccaccgctggtagcggtggtttttttgtttgcaagcagcagattacgcgcagaaaaaaaggatctcaagaagatcctttgatcttttctacggggtctgacgctcagtggaacgaaaactcacgttaagggattttggtcatgagattatcaaaaaggatcttcacctagatccttttaaattaaaaatgaagttttaaatcaatctaaagtatatatgagtaaacttggtctgacagttaccaatgcttaatcagtgaggcacctatctcagcgatctgtctatttcgttcatccatagttgcctgactccccgtcgtgtagataactacgatacgggagggcttaccatctggccccagtgctgcaatgataccgcgagaaccacgctcaccggctccagatttatcagcaataaaccagccagccggaagggccgagcgcagaagtggtcctgcaactttatccgcctccatccagtctattaattgttgccgggaagctagagtaagtagttcgccagttaatagtttgcgcaacgttgttgccattgctacaggcatcgtggtgtcacgctcgtcgtttggtatggcttcattcagctccggttcccaacgatcaaggcgagttacatgatcccccatgttgtgcaaaaaagcggttagctccttcggtcctccgatcgttgtcagaagtaagttggccgcagtgttatcactcatggttatggcagcactgcataattctcttactgtcatgccatccgtaagatgcttttctgtgactggtgagtactcaaccaagtcattctgagaatagtgtatgcggcgaccgagttgctcttgcccggcgtcaatacgggataataccgcgccacatagcagaactttaaaagtgctcatcattggaaaacgttcttcggggcgaaaactctcaaggatcttaccgctgttgagatccagttcgatgtaacccactcgtgcacccaactgatcttcagcatcttttactttcaccagcgtttctgggtgagcaaaaacaggaaggcaaaatgccgcaaaaaagggaataagggcgacacggaaatgttgaatactcatactcttcctttttcaatattattgaagcatttatcagggttattgtctcatgagcggatacatatttgaatgtatttagaaaaataaacaaataggggttccgcgcacatttccccgaaaagtgccacctgacgtctaagaaaccattattatcatgacattaacctataaaaataggcgtatcacgaggcccttttgtc

SEQ ID NO: 28 - DNA, 17 bp, synthetic construct
  misc_feature 1..17: note = primer
  source 1..17: mol_type = other DNA
tcagcatggcggtgttt

SEQ ID NO: 29 - DNA, 16 bp, synthetic construct
  misc_feature 1..16: note = primer
  source 1..16: mol_type = other DNA
gctgtctccacaagtc

SEQ ID NO: 30 - DNA, 22 bp, synthetic construct
  misc_feature 1..22: note = probe
  source 1..22: mol_type = other DNA
ttctgacctgaaggctctgcgc

SEQ ID NO: 31 - DNA, 18 bp, synthetic construct
  misc_feature 1..18: note = primer
  source 1..18: mol_type = other DNA
ggcagccttgatttggga

SEQ ID NO: 32 - DNA, 23 bp, synthetic construct
  misc_feature 1..23: note = primer
  source 1..23: mol_type = other DNA
gaccaggcctcatacatctcctt

SEQ ID NO: 33 - DNA, 20 bp, synthetic construct
  misc_feature 1..20: note = probe
  source 1..20: mol_type = other DNA
aatgcggcctccaactcgcg

SEQ ID NO: 34 - DNA, 23 bp, synthetic construct
  misc_feature 1..23: note = primer
  source 1..23: mol_type = other DNA
actttgactttaaccgcttccac

SEQ ID NO: 35 - DNA, 19 bp, synthetic construct
  misc_feature 1..19: note = primer
  source 1..19: mol_type = other DNA
cctgcaccgtgacctcttt

SEQ ID NO: 36 - DNA, 19 bp, synthetic construct
  misc_feature 1..19: note = probe
  source 1..19: mol_type = other DNA
agactcatcaacaactact

SEQ ID NO: 37 - DNA, 20 bp, synthetic construct
  misc_feature 1..20: note = primer
  source 1..20: mol_type = other DNA
caccgtgctttcactttccg

SEQ ID NO: 38 - DNA, 20 bp, synthetic construct
  misc_feature 1..20: note = primer
  source 1..20: mol_type = other DNA
acccaccggtgctaatcaag

SEQ ID NO: 39 - DNA, 29 bp, synthetic construct
  misc_feature 1..29: note = probe
  source 1..29: mol_type = other DNA
ccgcataccccgcgccactgggtcgtctt

SEQ ID NO: 40 - DNA, 22 bp, synthetic construct
  misc_feature 1..22: note = primer
  source 1..22: mol_type = other DNA
tggtttaggatggtggtggatg

SEQ ID NO: 41 - DNA, 21 bp, synthetic construct
  misc_feature 1..21: note = primer
  source 1..21: mol_type = other DNA
cgcaggtagattaagtggcga

SEQ ID NO: 42 - DNA, 24 bp, synthetic construct
  misc_feature 1..24: note = probe
  source 1..24: mol_type = other DNA
gaggtaatgtttatgtccagcgtg